European Patent Application EP 4 682 252 A1, published January 21, 2026. Title: Recombinant phage and methods of preparation thereof. Applicant: 国立感染症研究所長. Application JP. The sequence listing filed with the application follows.

SEQUENCE LISTING (118 sequences)

SEQ ID NO: 1 - DNA, 32767 bp, T5n phage
  source 1..32767: mol_type = genomic DNA
gaaccacagaaattttcacttgtcaagctattttgccccctttagctaataaaattttactttttctgcacctatctcaaatcttcccaaattatctcaactcttccccaaaatccccgcaaatcaggtgctccgcaccaatcctgcgcccatatccttctagcctcccaaatttctctcgctctctcatcttcccctcaaacccatacaatcacacaccctcccatcgaagtcacaaaaatcttgtcggattcgcacatctcaacacatgtcggatttgcacatactctagctaattccacaggattcgaacgcagttcgtgattgctggagtttttgggaaaattcattgtcggatttgcacactataaaaatttttcgggtcggattcgcacactaccaaaaattgtcggatttgcacatacacgcccacgcgtaatccatgggggcaaatgtcggatttgcacaaaagcgcagggcaattgccctgctcgcctgaatgcgaatgataatgagaatcaatctcatttaaaaagtgaaatgcaaatgataatgattctcatttaagaaagggaatgagaactattcaggaagtgaaatgattctcatttaaaaagcggaatgattctcatttaaaaagcggaatacgaatgataatgattcgtatttaaaaacggaagtgagaaacactgttatttaagttatccacagacttatcaacagcacgattcgccttgacaaaatcctagccattttgaagcgttatcaacagacttatccccaggttatcctactgtatatttatacagtattcctacgcagtgaataattctaatatatgcctaaaacgtcctagatcgcattctaacgcgtttaattttgatggggatactaaaacaaagggggatttaactggaggcgtgaaaaacggggagctgatccccgtcggttatcagagaagtgggcaattgttacgctttgccatttcccgccaatcatcttgctgtctagacttgcgatgccgtactaaaaaccgtttataccagtgattaaaccatcgtttcataaatccccctcgggtaatcgatgcgtgatcttctcctcttccccgtaggaatcgaccaaatgctgataataaccatcggcatcataaataacgctatcatactcgccccgctcgaccgctccccgattctccggcgtatcgggcacataaaaaacgtctaccattgtggtagttttggtcacaataattttattgctcataataacgccccgttattagttgactatctcaaagatagcgttctcaagtgtcgcccttagaatcccatcgcgtcctactacggaatacttgagatcgggtattttgtaacgctcaattgttttgagtaattgatctttttgggctttatatttttgcccttctcgcgctatcgtgtcgccttcggctttaacgcaaatcagtgtaatcataataaccctagtaaatatatttttgccaatagtggcgaacgttatcgccaccagcggaatcattcgcagcctcaacattaccaacgaaaatatatagcttcattgcgccacctttctgaaagctgtttcaatactttccgcagttgactgaatatatgcgcctttcattatcaggcgctcggtgtataccttgcggaagatattaataaaatcatcttcattttctgcaattaacgcttcacccatgacctgaatatcacaagatgcgaaagtcaaaaattgaaatgctaattcacgggcaacgaccgcattaatcttataatgcgccttgccctcataaatattaatgacgcctttatattcaggtgacacctgatttaagtagtttgctaataatcccggtcggcaaatagcaacaaagcgattgccttcataaattaccattttataacactccacgaaaagccgcgtaaaaggtggcaaaatgtttaaccgtttcagctatcacgttgccgcgcttatcaaatttcttttctgtaacacgaaaggcgtttttattacgtgctacatattcgattttacaatcttcccgctcgaatgtgttaacatccaccagcttaaaaccctttgaacgagcaagagaaacgttgcggatcatttttattctcctttattcatgcagcccagcagataagaaaatacagcgatacccgcgccaataataaccataggtttagtatttactaaaccacaataagaatcttgaataccgtaagcggtagcaaaaagggtcagaatagcgcccaagatacctgccagaatagctcgaaaaataaccatttgtaatactcccctagttagtggggcgaaagtaacgccccgttattaattacattaaaacaattttggcggcttgttttttagtacagtgttccgctttcagggtatccagcaaaaagcccgccgtttgctgatcgatttgatcattatcataaagcgcctgaatggtagtgtaagttttagcaatgccgaactcctgcaccatttcttgaatgatccagcgatttgatacccagccttttccagtgaaaagagcgtcagaagaagaataagcaaccattttaagcctccaaaattttgggaaaattttcaaccgtcctcaaacggtgtaaaggcattataacaaaaaaggccgccgattatggcgacctttacaaaactttacattaggttaattattactcgctttcggtgttaacggtaaaagtagaaatatcaatacctttcaccatttcatcaatcatttcagcgatgttaaaactttgcaccatttctagcatagccgcttccatagctgcacccgctaccgctttcgccttttggttgctaggggcgtactggtcaaccgctacgctcagcaggttagcaataactacccgaccaataggcgtatcaatataacctttaatcataaatggtgcttttttagccgctactttcgtgatttgagttaatgcaattttgcccgcttccagttttgcagcatttacaacggcggatttattagcggcaacgatattagcgatcttggtcatggcattttttcctttgttttcagtgatttgagtgttaacgctttgagtgttagaatttacagcatgtttttccgtgttgtcaatgatctgattctcatctttccagaaaataaaacccgcttcttgtactagctcattatatacatacggatataattccgatggtaataaaaaattaccgtcgccatcaaaagccattacagccgtatattgagatccatcactatcaggtctatgccatccagcagataaatacttccagataacatctaaaaatccctcaaggctagaaagtccgtttattaattcaagcccaacaagctcaaaattatttatattaaatgattgacggcctgaattgctatgatacgcaacgatattattaccctgcgcaacaataaaatcagtatccggccccgctcccctgcccgtaaagatatggcaatcacgattatataagataatcgttgccccctgcttatataggggtagaaaactatccatatcataggcatcataatcattaaaaaagttttggtgaatagtttcagccttgttaataaaatgtttaatgctggttgtcctgctaccatccagcaggttgcgcaaggcgccctttaagacggttgcgttatctggtttatatagccgcatttgttggcctccctcgttaatcggtgagtgaatgataaaggtaattttctagcataggcaaatattattttacctttttattttccttgcctagcgcctagttttatgctaaccgcgcagcggtatagtaaagagcaaaacacggcgaagccaccagggcgacgcgttgaggctttactttaatattaccctatagcgttttgctcgttagaaagcgttttaggccgcttattttgggcatcattataatatgttttccatttaccctgtatatttatacagtggaataacctgtggataagtctgtgtaaaagtgctataaagccttcctattgtgtcaagttaatttacaaaatgtataaggctgtggataacttaaatgatagtgtttctcactaactaatttatgcagttattatataacaaaatatagttagttggctaataggattttaaagtgattatgagtctgctaattaaacctgaaaaactcattaggtagtttgctaatggttttgatataatataatagagattaaattaataacataaggaaactataacaatgggtctatttaaagatatagattattcgcttgctaatgataacttttattatgatgaaacatccccatcatttctaagatggaaagtacagaaaggtaatagtaaggtgggtgatattgcagggcattatagtaacacaggttactatcgagtaaagttagcaggcgaacaatacgcagtgcatagaataatatgggtattatttaatggtgagattgatagcaatctaacaatcgatcataatgatcgtaaccgtgctaataataacattaataatcttcgcttagtagaccataagcagaatatgaataacaagaaagattataagcgtgctaataagttgcctaagcatatctattataatggttctagagttgataataacggaagaaactatttgcgcgctatagttaaagatcctactagtaacaaaagtgttagtaaatcaggttatgatttacaagagttattattatgggtagaaactaaaaaagctgaatttggaattgtcaattaattaattttataaaataactcgtttagtcttgatttttaaaagtcaatatcttttccaactatttttcaattttgcttttgttaaatatttgttaaatcgaaaataagccgcctaaaacgctttctgacgcggtaaatttttcaggcatcccatcataaggggataacccgtttatcgtcaccacgagctttctaagatttgtcaactagggcaaggcaaatataaaggaaaaaattacttgccaacctgctaggttttatggtattcgcgcgcccgtttcctttaaacttaggtgagcgccggacgtgttgccttctttacgtttctttacaaaaataaggttgcgccatttttgggtatcccctattatttatctcgtagggcggcaatgacgaactacacggcgggaagtttaccgccacgctctttaaaaattgggtacatcttaaagtctatcggcggtaaacttatatattataaggaatcgacgatatgaaacaaactttattgatcactggtaaaccagctaaaaaattagatggtactactaaaaaattgttgacaatagcccagcaatcggtaaaatatcgatttaggcagtacaagaaaggccgccagcaaggtctggaaatgatctggcgaaacattatgattgacttgaaagaaaatcataaaaaactgcaaaaaatagtttgacaccctagccgataggctttaagatgtacccagttcgatgagagcgataacttgataaaatatgacggtcggcacttaccataatgtgtcccgccccctaactgggatatagcggcctgagtggagttctttaaattgattatattggcgagcggattgttgcttattacctgccactacttttacagcaggtaatgcggaacaatcccccttaataaactggagtttatattatgcaaaacgttactactgcgccaaaaattggtcaatccgtttttatccctttcgttactaaaacggatgaggtaaccggaaaaaccgaacgcattaaaggcgcggcgcttatgccgtttgatgtaattgatgcggtatacgctgaaacggaacggagtaacaacggaaaaactgtttacaacgttcgggttaaatccggcgacgttgtaaaggttgcccagcgtaacgaaaaatgggaagccgtagcgtaatagtgttacttttatatcccccagtagttcgggggatataacgattaacattatgttaatcttatcccttaaattaaataaacaggagttacatcatgactaacgctaaaaccgcaaaattcgcttggaatgaagaaaacactcagaaagctgtttccatgtaccagcagttaattaatgaaaacggtttagatttcgcaaatagcgacggtttaaaagagattgcaaaagcagttggcgcggcttctcccgtgtctgttcgctcaaaattgaccagcgcgaaagcgtatcagaaaagcgataaacctcgcaaggttggcggcggcagttctatccgcaaagcgcactacgtgcgtgtgattgcaaaacatgccatcgattccggtattatcaaagacgctgacgatctggcatcactggaaagtgcaaaattggaaacgctggacgccgtggcgcaactgttaggcgttgccgatgaagtaaaacaagccgcaggcgaataaatttaattagtggggaatattccccactataatttccctttgactggagttttaaaatgatcttttaccctactgaatccctcattctaggcttgtttattatggcggcctcgttattgttcgcttattttcaaaatgatttagattcgtattattttaaacgtaaatctaagttagcaaagcgtttaggtctgatttgttttattgccgccgttgcttgtggtgttagttctagccttatgcctttaaattaatgttgcaaattataacgcctattattcaaggcgttatatttggcaatattgccaataacaaacgttttttaatccctttaatggagttttattattatggttatttccgcagaaaaacaaaccgttatcctgaaaatggccgctgactttaatttctacggtaaacgtctgcgcgctactaaattggaagtttgcgacgatatttcaaaaatggtttacgatacaacaaaacactctaccgcaatttgtgactggctggaagcaaataaaccagcgaaaccgaaagcggcgaaagtagcaaaagccattaaaaacgatgagcgcccagaagcggcggggattgtttctagcacggttgagcaatgggaagtaaaacaaggtaaacgctttattattacatcgattcagaataatacgttcccgcataaaaactttttagcctcacttgaacaatacgcccaatttatcggcgctgatttgctggttagcaagtttatctataacaaaaacggttttcaaaatggcgagggcgccgacggtatcagatacgattccgcatttgacaaatatatctgcaataaaaacgtgtttttaaataatcgccgatttgctttcatggctgaaattaacgttttacccaccgcagattatccgctttctggattcgctgaaactgcaaccgcgctgaatcttgaaggtctagcaattggagcggctaaaatcaccgccgaaagcgtgccagctttaaaaggtgaaattgtgcgccgtatgtattcaaccggaacggcaacgctaaaaaattacatccagcagaaagcaggacaaaaggccgaggcgctgcataacttcggtgcgcttattgttgagtttgacgaggacggtgagttttttgtgcgccagcttgaaacgatggacgagagcggcgtgttttatgatttgaatacttgcgccactcctgccggatgttatgaaacaacggggcacgttttaggtttacaatatggcgacattcacgctgaaaaattagatgaggagtgcgccgctgcgtcttgggggcatggtgacacctacgggcttgttgatattcttaaaccaaaatatcagtttgtacacgacgtgcatgattttacatcacgcaaccatcacaaccgcgcatctggcgtattcctagcgaaacaatatgccgccggacgtgataaggtattagatgatcttatcgatacggggcgcgtactggaatcaatggagcgtgatttttctcaaacaatcattgttgaatctaatcatgatctggcgctatcccgctggttagatgatcgtaatgctaacattaaagacgacccagcaaacgcggaactatatcaccgcctgaatgctgcgatttatggagctattgcagaaaaagacgatacttttaacgtgcttgattatgcgctgcgcaaggttgcaggctgtgaatttaacgccattttcctgaccactgaccaatctttcaagattgcaggcattgaatgcggcgtacacggtcacaacggcattaacgggagccgtggcaacccgaaacagtttaagaaattgggcaaattaaacaccggacacacccacaccgccagcatttacggcggcgtttataccgctggcgtgactggtagtctggacatgggttacaacgttggcgcgtctagctggactcaaacgcatattattacctatgcaaacggtcaacgcactttgattgactttaagaatggtaaattctttgcgtaattaaattattcccctagcggcttgagatatagccgctattacaggagctaaattaaatggctattaaaattaatcttcccagcatgaaaaacaccgctgatacatggtcgcttgatgttttacggcatggtactgtataccgcaatttaaaagataataattgttatatttatcaaaatgaactaaacgggcatatttatataattgagtccggcgatttttattcttttgaaaatgagtatgaagcgaaagaccatttacaggaaaatgatattcctgacgtatggaaagaaacaaatctcgcttttgttgtaagtcttgaagctagcaaataaattaaatcccttattaaactaattggagttataaacatggctaaatctaaccgtatcccattcgatcgcgctcagtcttctattgttctggtttattctaatggtcagcgttatcacgtcgaggccggtcacgttattgatgagctattagatttcaatgacgcgatgcaagttacaacgtttgcatatatgcagggcaaactaacaagccatattaaagcaaaaggtgtttatgttgacactatgaaacaggaaacaatcattattgacgcggtaaaatccggtttagctttcgcagtagtcgcaccttgccccgcttgccttgatgatcagctaatgagcgcaaaggtgtatacatgcgctggcattcgttccagcgtatcgggcgaggatgttagttttatcgctgatgcgctagcgtatggcctttaatagttaatttattattacccgctatttaatagcgggtaatgctgaattaatctaatccctcaaatggagaacgtaacaaaatgaatcaagttaaaacgaatattacccgtaatttcccgcatatttcccgcgtcatgatttgggatctggacggcactatcattaattcgtttcatcgtgtagcgccttgctttgatagcgagggcaatttagatttaaataagtataaaaatgaagcctgcaaacatgatttaataatgcaagatacactattgccccttgttacatatatgcgccagtgcatgaatgacgcaaatactttaaacattatttgcaccgctcgactaatgagcaagtcggactattattatttgcgtaaacaagggttgcgcggtcgtggtgatagtaatatccgtgtattttcccgcgatacactacacaaatattttgaggctgataaagttagcgagatataccacagcaaagacgcagtttataaaagttactattttgggctattcaaacaattatatccgaacgctgattttacaatgattgatgatcataaaggcgtgctatcagcggcagcgtcatacggatttaaaacgctggacgcacaagccgttaatgatattctatcaatcggcgtgacattgataggtgaaacctttattgatgaatctcttgaggatgataatgattatcagttcctagccgaccgcctgcaattatgttgggaaggtatgaccgaagaagaacgcgcagaatatagttgcagcccgcaacaatatattgagaaattaaaagttgcgtaataattaaagttgaaattgtttcaccctgcaattaaaatggttgcagggtgaaacagttagcatggtaatagtaacgggggtggcggttagcagactaagtattttcgccggaggcagtggacacaccttcatgtgtaatcttatgaaatttcgagatttcccaattagcgcatagaatggtcatcaactccgtattttggtctgaactcacggaatctcttccgcgacgcccgagaaccgtccgaccactcccgctcaaactccgcacgtttttcgtcaaacttccgctccctttccgcaatctcccgcgatacttccgcaatgtatttacgatgcttgttaatagccgcagtcattccgaaaactcccgcgattattccgataataaaagcaactataatgctaaacatctaattccctctcaatttgcagaatacgaatgctatcacaacgttggagttctactaatttttctatagcaaattgttgttgttttacttgagcttctagagtttttaggcgaacgtacacggtgcaagaagcaatgaaaattgcccagactagtattactgttattatagctactacttccatcatttacgcttctccgttaataaagtttcaattctagctaagtgattatctaaaatacattgtccaataatcacaacccctagcaacgcaataattacccattccattaaatccaccccgccatagctgctaaccaaaaacctacgaaaataaagaataaaatagttcctaatccaaagctattaatccagctatcgtacacttctccacgtctgctctttcttttgtttgacatatctttcatgctcctataagtgtggtatttaaaatactctagcaattgcagtgattagtgtaaatattcccatcacaccttccatagtgtcttgtgtggtatcctgaactaattctgcactaggttcatcttaagtggtgatggttactaaggtggtttttacttagaaaactccctcgcatgtatttccttcggtaaagtagcttacgggggcccagaaagatccataggccataattggtgacaccaaaaacatatcccctttcctatcaaaaacattagccttatatttcacatgatcctgcatatagtatgcctcacatttaatatctttaggtccaaaagtagagcaagccgaaagaagtaccactgccatagctaaaaataattttttcatttacattctcccctatttaatttataatactattatacagaattatggcagtataagcaactaaatttttggagaacttatgagttttttcgctggcaagctaaataacaaatctatactctcactgcgaaggggtagtggtggagatactaaccaacatatcaaccctgattcccaaaccatctttcattcagatatgtcgcacgtaattataacggaaactcattctactggattaagattggatcagggggctggtgactattactggtctgaaatgcctagtagagttacacagctacataataatgaccctaatagagttgtattaacagagattgagttttctgatggctctagacatatgctatctggcatgtctatgggagtaggtgcaaaagcctatggtattataaatcctcagattatgtctcagggtggattaaaaacacaaataacagctagtgccgatctttcacttgatgtaggttattttaatacgggtactagtggcactataccacaaaagttaagagatggcacaggatgtcaacatatgttcggtgcttttagtgggagaagggggtttgcatcaagtgcaatgtacttaggtggtgctgctctttacaaatctgcgtggagtggttccggttatgtggtggctgatgcaggaaccttaactatccctagtgattatgttagacacccaggagctaggaactttggttttaatgctatatacgttcgtggtaggtcttgtaatagggttctttatggtatggaaggaccaaactatactaccggtggggctgtgcagggagcttcgagctctggagcccttaactttacgtataaccccagtaatccagaatcaccaaagtattccgtaggtttcgcacgtgctgatcctactaactatgcttactgggaaagtatgggagatcctaatgattctgccaatggacctataggtatctacagcgaacatttaggcatttatccatctaaaattacatggtatgttactaacctagtatacaatggttctgggtataatatagacggtgggttatttaacggtaatgacattaagctcagcccaagagaatttattattaaaggggttaatgttaataatacatcttggaaatttattaattttatagagaaaaatttcaacgttggtaacagagctgattttcgtgatgttggttgtaatctaagtaaagattctccctcaacaggaatatcaggtatagcaacatttgggctaccaaccacagagagcaataatgctcctagtattaaaggtggtaatgttggtggcttacatgctaatgttgttagtatttataattttttaccttcagcatcttggtatgtatctagtaatccaccaaaaataggtaataactatggcgacgtttggagtgagaatttattaccattaagactcctgggaggtagtggtagcactatattatctggaaacatagtattccagggtaatggatctgtacatgttggtactgtggggttagatcttaatagcagtagaaatggtgctattgtatgtactatggagtttatagatgatacatggctatccgcaggcggtattggttgcttcaatcctacagaaatgttatcccaaggggcagaatacggtgatagtagatttaggataggggggaataccataaataaaaaactgcatcaaatactatctctaccagccggagaatacgttccattctttactataaaaggtacagttgtaaacgcttgtaaattgcaggctgctgcgtataatccaacaccatattgggtatctgggttgcctggatctgttgggcaaacaggatactatactctaacttactatatgagaaatgatggaaataataatatctctatttggttagattcttccatgagtaatataattggcatgaaagcatgcttacctaatattaaacttataattcaacgccttacctaaaggaggaaatatggcaaatgatgtattagtaccagatcttatgtcccctgaagggatggatgtgattgaagcttatttacagtgtggcagcgacgtgccttctgccgcacgtagtcttggaatgtccgaaattgcttttcgagatattatgaatcgtagtgaagttaagaactacttaaatgatatttttatggagagtggtttccgtaacagagatcgtttatttggtgttctggatgaagttatcaagcgtaaactagaggaactggaagaaactggcatgggttctgaccaagatattatggatattctctggaaagcacataaaatgaaaatggaagaaatgaaaatgatggtagaactggagaaagtgaaggcagcagcccgtactccagctaaccagaccaacatccagaataatattattgctggagctggggatcaaaactacatggacttaattacttccctagctactggaggtaagaagtaatggaagtatcaagaccctacgttaatacagtagatgttatcgatttcgggatagataaacgtttctttcgtctacctgtttcaggaatactagcacaagaaggtattacacctaatggtcctcaaatagcgattattaatgccctagaggaccctagacatcgttttgtaacagcgtgtgtgtcacgtcgtgtaggcaaatccttcatcgcatacacacttgggttcctaaaattgctggaacctaatgtgaaggtactagtagttgcccctaactactcactggctaacattggttggtcacagattcgtggtcttatcaagaagtatggcctacaaaccgaacgtgaaaacgccaaagataaagagattgagctggcaaacggctcgctcttcaaactagcttctgcggcgcaggctgactccgcagttggacgttcatatgattttatcatctttgacgaagcggcaatttccgatgtgggtggtgatgctttcagggttcagctgcgtcctactctggataaacctaattctaaggctctatttatttccacccctcgtggaggtaactggtttaaagagttttacgcctacggatttgatgatacgttgcctaactgggtatctattcatggtacatatcgtgataacccacgtgctgacttgaatgatattgaggaagcacgccgtacagttagtaaaaactacttccgccaagaatacgaggctgacttctctgtattcgagggccagatctttgatacctttaatgctatcgatcatgttaaagacctcaaaggtatgcgtcacttctttaaagatgatgaagcattcgaaacgttgcttggtattgacgttggttatcgtgatcctacagcagttcttactattaaatatcattacgatacggatacttactatgtattagaagagtaccagcaggcggagaaaactacagctcagcatgctgcttatattcagcactgtatagatcgttataaagttgatcgtatttttgttgactctgcagcagctcagttccgccaggatttagcatatgagcatgaaattgcatctgctccagctaaaaagtctgtcctagatggtctagcatgcctgcaagcgctattccagcagggcaagattattgtagatgcttcatgttcctccttaattcatgcattgcagaactataagtgggacttccaagaaggcgaagagaaattatcacgtgaaaaaccacgtcatgatgctaactctcacctttgtgatgcgctccgctatggaatttactctatttcccgtggtaaataaataagtataggatgggatactactcagttggtatcccattcctgtattttaaaatcccctttacaaattcgatacgattatgtatactatattcattgatcgggagaacttctcccataatagaacgtaaacaagaaaaattaatgctctacatgggtgtaggagattctatgggtcgacaaaagctaacaataaaagatataaatattagattagctgatcgtggaatccaaattgtcggtgaatatgtaaaccaacgtacaaaaacagtatttaaatgccagagagcacacgtttgggaagcaacaccacattctatactccatatgaggagaggttgtccacactgctccaataatacaatatcgttagatgaagttagtaacagaatatctaatatagggtatactctgttaagcagctatactaatgctaaaacaaaactacatctacgctgcaataatgggcatgactgtttcattaccttagatggattgactcaaggtaagagatgtccttattgttctcttaagtgggagaatggtggattcctctatatcatgtccttctctagcggtactaaagtaggcataagcttatatcccgagaaacggttgaatgaagttaaaagagaatctggattttctgacctgtacttgttcaccatgtatcatctgccagatagagagactgctttagatttagaaaaggaagttcacagagaatattataataaaaactgtgggttttctaattttacaggaagcacggaattttttaatgttgctcctgaggatatagtaatctttctaaatagctttggattggaggagtatggccactaatactaagtacaaacgtgatgccatttccataatgagggatggtataaaatctaggtatagtaaggatggttgctgtgctatatgtggtagtagtgaagacctagaacttcatcactatcatactatatctcagctaataaaaaaatttgctaaagaactccagctggatttcactgatgagaatatcgtcctttcaaatagggaagcattctacaagaaatatgagcatgagttagttagggacgtggtaacattgtgccagcaccatcaccaattattacataaggtttacacgaaagaacctccattattttctgctaataaacagaaagcatgggttcaaaagcagaaagacaaaatacagaatcctcaagaaaagacacaagtcaagactgaaacaaaatcaggattcgcaaggttcttataatgggttttaaaagctggattactgaaaagctaaatccgggtcaacgtattataagagacatggaaccagttagtcatcgcactaaccgtaagccttttaccactggacaagcctacagtaaaattgagattctcaatagaactgctaatatggttatagatagtgcggcggagtgttcttatactgtcggagataaatataatattgttacgtacgctaatggcgtcaaaacaaagactctagacactctcttaaatgtacgacctaatccattcatggatataagcacattccgtagacttgtagtcactgacctactttttgaaggttgtgcatacatctattgggatggcacatcgctttaccatgtcccggccgctcttatgcaggtcgaggcagatgccaataagtttatcaaaaaatttatatttaataatcagataaactatcgcgtagatgagattatctttataaaggataacagttacgtgtgtggcacaaactctcaaatttctggccaatctcgtgttgctactgttattgattctcttgagaagcgttctaagatgcttaactttaaagagaaattcctcgataacggaaccgtgattggtcttattcttgagacggatgaaatcctgaacaagaaattgcgtgagcgtaaacaagaagaattacaactcgattataatcctagtacgggtcagtcctctgtcctgattctagatggtggtatgaaagctaaaccgtactcccaaatatcctcttttaaagatctagactttaaggaagacatagaagggtttaataaatctatttgtctagcctttggagttccgcaagtactgcttgatggtggtaataatgcgaatattcgaccaaacatcgaattgttctattatatgactatcattcctatgctgaacaaactgactagttctcttactttcttttttggttataagatcactcctaatactaaggaagtcgcagcattaacaccagataaagaagcagaggctaaacatttaacctcattggttaataatggtattataaccggtaacgaagctcgttcagagctgaacctggagcctttagatgatgagcagatgaataagatccgtattcctgctaacgtcgctggttctgcaacaggtgtatctggtcaagaaggtggtagacctaaaggttccaccgagggagattaagaatgattgattatagtggtctaaggaccatttttggtgaaaaactaccagaatctcatatcttctttgctacggttgctgcgcataaatatgttcctagctatgcttttctgcgtagagaactagggctttcatctgcgcatactaaccgtaaagtatggaagaaatttgtagaggcttatggtaaagcaattcctccggccccaccggctccaccattaactctttctaaagatttaactgctagcatgtcagttgaagagggagcagcattaacactttctgttactgcaactggtggtactggtccatatacttatgcatggactaaagatggttctcctattccggatgcttcaggagctacctatactaagcctacagcagcagctgaggatgccggctcttataaagtaactgtaacagatagtaagcaagtaagtaaggattctactacatgtgctgtgacagttaatcctactgttcctggaggctaataaatgacacaagctgctattgactataacaagttaaaatcagcacccgttcatttagatgcttatattaaatctattgatagcgaatccaaagaaggtgttgtaaaaatccgtggattcgctaacacaattagtaaagatcgcgctggtgatgtaattcctgcttctgcgtggaaaacgtctaatgcacttactaactacatgaaaaacccgattattcttttcggacacgatcatcgtcgtccaatcggtaagtgtattgatcttaaccctactgaaatgggtctcgaaatcgaatgtgagatctatgaaagttctgacccggctatcttttcactaattaaaaacggtgtactgaaaacttttagtatcggattccgctgcctagatgcagagtgggatgaagctactgatatatttattattaaagatttagaactatacgaagtttcggtagtttctgtaccttgtaatcaggactcaacattcaatctcgctaagagcatgaatggtcatgattatactgaatggcgtaaatcttttactgcaataagttctaaagctgtcccagctcaagaacgtaatctttctgaactagaaaaacttgcgatagctttaggctacgttaaagaataacggagaattatttaaaaatgactattgatattaataagctgaaagaagaacttggtctgggtgatctggctaaatctctggaaggtctgaccgctgctcagaaagctcaggaagctgaacgtatgcgtaaagagcaggaagaaaaagaactggctcgtatgaatgacctggtttctaaagcagttggcgaagaccgtaagcgtctggaagaggctctggaactggttaagtcgctggatgagaaatctaagaagagtaatgaactgtttgcgcagacagtagaaaaacagcaggaaactattgttggtcttcaggatgaaatcaaatctctgctgacagctcgtgaaggtcgttccttcgtcggtgatagcgtagctaaagcactgtatggtactcaggaaaactttgaagacgaagtagaaaaactggttctgttatcttatgtaatggaaaaaggcgtattcgagaccgagcatggtcagagacacctgaaagcagtgaatcagtcttcttccgtagaagtttctagtgaaagctatgaaactattttctctcagcgtattatccgcgacctgcagaaagagctggtagttggcgcactgttcgaagaactgccgatgtccagtaagattcttactatgctggttgaaccggatgctggtaaagctacttgggttgctgcttctacttatggtaccgatacaactactggtgaggaagttaaaggagctcttaaagaaatccacttcagtacttacaaactggctgccaagtcctttattactgatgaaactgaagaagatgcaatcttctccctgctgccgctgttgcgtaagcgtctgattgaagcacacgctgtttctatcgaagaagctttcatgactggtgatggttctggtaagccgaaaggtctgctgacccttgctagtgaagatagtgctaaggttgttactgaggctaaagctgatggttctgttctagtaactgctaaaactatctccaaactgcgtcgtaaactgggtcgtcatggtctgaaactgagcaaactggtactgatcgtatctatggatgcttactacgatctgctggaagatgaagaatggcaggatgttgcccaggttggtaacgattctgttaaactgcaaggtcaggttggtcgtatttatggtctgccggttgtagtttccgagtatttcccagctaaagctaactcagcagagttcgcagttattgtttataaagataacttcgtaatgccacgtcagcgcgctgttactgttgaacgtgagcgccaagctggtaaacagcgtgatgcgtactacgttactcagcgtgttaacctgcaacgttactttgcaaatggcgttgtatctggtacttacgctgcgtcttaatacaggcttttcagccgataaggagagcttcggctctccttttttattgggaaaaataaatgcaaataatcacagctgaagactatagattatatggtggtttaaaacgaccggaactagaatctggagtagaggtgatgattactgctgccaatgcgctgattactagccttttaggtatggatgatgctgacgcagtagaccagttaatcactacaaaacctactcgtaaaaaatactttttaagttctccctcagctacttcagtaaccaaaatgactattaatgataaggagatagatcctgaacagtataagttgtattctgatggggttatacttcttaaatttaatcctccagaaggttatatggacgtagaatatacacagggtgggtttaacccaatgcctgaggatctcaaacttgcagcatgtatgctagtagatcattggcacaaacaagattatcgccaagctagaacaattggtggtgaaacagtaaccttcaataacactaaatctggtattccagagcatattcgtactattattgaagtgtataggagagtataatgtctctttctgatctagctagacaaattattaaagagcagctagatactgcaagccgatctgaaaacaataagaatactgttgtatactctgttgaaacagggttaaaagatcctaccagagatggtactgttgctcaagtatcctttaagttttcaaaacctgtatcacaagatctccttaacattaggacagcttctatactaaaagctgtatcctctagtttagatctttctggagatttaggtgctctggagaatctaatacaagcaaccgccggtaaaaaatcctcagtaggtaaaaaacgttctactggtagggtacaggtaaactttggtgatcctagtgatgttgaagatggatattctggtgcagtaacaggtgcttctggacgttttgtgtctaacagcaatatgaagattatactagaaatagttgctaaagaatacttaataaaggatatgaaaaaagctggagcaccattaaagtttagaactggtcgctttgcaaactctttaaaaattaaagatgttatgcttcgtgattctgaaactagtaaaggctctcctgaattaaacgtaacatataactatatgactcgtccatattctgtgttcaatccggcagtatctacatatagaagattatccctacgaccttatcctggcgctagaaacccacaaaaacttattggtgaggctatagcaaaagctgcaagagacctgattcactccagatataaaattaaggttaatcaaggaacctaataaatggatcatagaacaagtattgcacaagctatggttgaccgaatctctaaacaaatggatggttctcaacctgacgaatattttaataacctatatggaaacgtttctcgtcaaacttataaatttgaggaaatacgagagtttccttatgtagcagttcatatcggaactgaaactgggcagtatcttccttcaggccaacagtggatgtttttagaacttccaatcctggtgtacgataaagagaaaacagacattcaagagcaacttgaaaaactcgtagcggatataaaaaccgttattgacacaggtggaaatttagaatatactgttagtaaacctaatggatcgaccttcccatgtgaggcaactgatatgatcattacatcagttagtacagatgagggtctactggccccatatggtttagcagaaataaatgtaacagtgaggtatcagcctccacgtaggtcacttcgcagataagttacagattaggagaaaataattaaatgtctttacaactattacgtaatactcgaatcttcgtgtctacggttaagactggtcataataagaccaacacgcaagagattctagttcaggatgatatttcttggggtcaggacagtaactcaacagatattactgttaatgaagctggtccgcgtccaactcgtggttctaaacgttttaacgactctttaaacgcagctgagtggagtttctctacttatatcctgccgtataaagataaaaatactagcaaacaaattgttcctgactatatgttatggcatgcactttctagtggtagagctattaatcttgaaggaactactggagcacataataatgctactaacttcatggttaactttaaagataattcctatcatgagttagcaatgctacatatttacattctgactgataaaacgtggagttatatcgattcctgtcagattaatcaggcagaagttaacgttgatattgaagatattggtcgtgtaacttggtctggtaatggtaaccagctaatcccactggatgagcaaccatttgatccagatcaaataggtattgatgatgaaacttatatgactatccagggttcttacattaagaacaaactaacgatcttgaagatcaaggacatggataccaataagtcttatgatataccaattaccggtggtacttttactattaacaacaacattacttacctaacacctaatgtaatgtcccgtgttactattccaattggttcctttactggtgcttttgaattaactggttcattaactgcttacctgaatgataaatctcttggttctatggaactgtataaagatcttatcaaaactctgaaggtagttaaccgctttgaaatcgccctagtacttggtggcgagtatgatgatgaacgtcctgcagctattctagtagctaaacaggcgcacgttaatattcctactattgagactgatgatgtacttggtacttcagtagaatttaaggctattccgtcagatctggatgctggtgacgaaggttacttaggcttctctagtaagtatactagaacaactattaataatctaattgttaatggtgacggtgctactgatgctgtaaccgcaattactgttaagtctgctggaaatgttactacattaaatcgatcagctactcttcagatgagtgttgaagttactccttcttccgcaaggaataaggaagttacttgggctatcactgccggtgatgcagctactatcaatgcaacagggttactaagagcagatgctagtaaaaccggtgcggtaactgttgaagccacggctaaagacggctctggtgttaaaggcactaaagttattactgtaacagcaggtggttaattaaatgttttattctctcatgcgagagtctaaaatagttattgagtatgacggtagagggtatcatttcgatgccctctctaactatgacgctagtacgtcttttcaagagtttaaaactcttagacgtactattcataatcgtacaaactatgcagactctattattaatgctcaagatccttcatctatttcattggcaataaatttcagtactacgcttattgaatctaacttctttgattggatgggattcacgcgtgagggaaattctttatttttgccaagaaatactcccaatattgaacctattatgttcaatatgtatattattaatcataataatagctgtatttatttcgaaaactgttatgtatcaacagttgatttttctctagataagagtataccgatcctaaatgttggtattgagtctggaaaattctctgaagtatctactttccgagatggatatacaattacacagggtgaagttcttccatatagcgctcctgctgtgtacactaatagctctccgttgccagcgctaatttcagcatctatgtctttccagcaacaatgttcttggagagaagatagaaatatatttgatataaataaaatttatactaataaacgagcttatgtcaatgagatgaatgcttccgcaacgctagctttctattatgttaagagattggtaggagataagttcttgaatctagatcctgaaacaagaactccactaattattaaaaataaatatgtttctataacattccctttagcacgtatttcaaaacgcctaaacttctcagatttgtatcaggtagagtatgacgtaatccctactgctgattcagaccctgtagaaataaacttctttggagaaagaaaataatgattaacttaaaagatattactttagaaactcgtactgtcactctttcatacccaggtatgccaaactttaagctagagcttaattatatgtctcgtgctacttctaaacgagttatcacctctgctaagcgtgacgagtgggttaatggtactttgattcaggtacaggatgatgataagtttattgaagctttcgttgatgctgcgattaaaggttggactggtttgactgtaggtgacgttgaaaaactgatgctgattgaaacagatgctgatcctgctactgaagttccatttagtcgtgataatgctgtaatgcttatgcagaactctgctgcgtttgattcttggatcaaccagacagtgttccacctagatacttttcgtagctcaaaagcgtaaagaattactagatgctgttgctgattttgcagataagtgtattaaaagctcagcatctaaaatgactaaacaacaatatttaatactttgtgaatcaatgggtatagagcctgatcctaaggccatgcctgttgaacttgaagactttccacctattgtagctattagtatgaatatttataatagtctagttgactgtttcatacctggtgacttccctatctttataggtaaagacaaggctgctttaggtgttttatttgatatttatgggattacagatcctatagagaaagaatttgttctacacattatcaatatatttgatgctaaagctgtagacgctgcacgtaaacgtgctgagaagcataagccgcaaaacggtagaatacctaacgttaagccacatgccaaatctcgagcacggtaaaagtttcctccaatggggcgttccacgatgaggcttggctctgggtgatatgcccagagccttttttatttataaacatataggttggtatagtatgggaaagaagattactaaacaggatagagagtctcagataagcaacatttgcaatgataaaaatttatcctttgttggctggataggtgagtacactaatattaaaagcacccttacacttaagtgtaataaatgttattacacctggtctcctaggttggataactttttacggattactgcccaaaaatgccctgcatgcgcaggcaaagctagatggacgaaggaagaaagagaagaacaaataaaaagtaagtgtgccgagaaaggatataactttctatcttggtcttccacctatattaataaagattctaagattatacttaagtgtttaaaagatggttgtatctgggatgtgtctatacaccattttattaatcacgatacagggtgtcctgattgtgcttcaggaggatttaatcctaatataccagctactttttatatacagaaattaacgtatcaagggactcactttctaaaatttgggatcactggtaaggatgtactagagagaatgaggcagcagagcaataaatcactatgcgagcactcggtaattttttctcatactttttcttatggttctatggctagggggctagaaaaagtagtaaaggactcagtaaacacaggagtattagataaacgtatccttccagatgggtacaccgaaacttgtcactactctgagctagaaactatactatctttaactaatagttttatacaggaaaacattagatgactgataagctaatacgagaattactaatagacgttaaacagaagggggcaacccgtactgcaaagtctattgaaaacgtatctgatgcattagaaaatgctgctgctgcttccgaactgacaaatgaacagttaggtaaaatgcccagaactctatactccattgagagggcagcagatagagcagcaaaaagtcttactaaaatgcaggctagtaggggtatggctggtatcactaaatccattgatggtattggtgataagctagattacctggctatccaacttattgaagtaacagataaactagaaattggattcgatggggtttctagatctgttaaagcaatgggtaatgatgttgcagctgcaacagagaaagttcaagatagattgtatgacaccaatagagctttaggtggtacatctaagggttttaatgacactgctggtgctgctggtagggcttctagagctttaggtaatacttccggttccgcacgcggagctactcgtgactttgcagcaatggctaagatcggcggtaggttacctattatgtacgcagctcttgcttctaacgtattcgtcctacagactgcttttgagagcctaaaagtaggtgaccagctaaataggctggaacagttcggtactattgtcggcaccatgacaggtacaccggtacagacactagctttatcactacaaaacgctactaatggtgctatatcctttgaagaggctatgcgtcaagcatcctctgcttccgcttatggatttgacagcgaacaactagagcagttcggtttagtagcacgtcgtgcggctgctgttcttggtgttgatatgactgatgcacttaaccgtgtaattaagggtgtatcaaaacaagaaatcgaacttctggatgaacttggtgttactattcgtcttaacgatgcgtatgaaaattacgttaaacaattaaatgctaccagtacaggtattaaatatactgtagatagtttaactacataccagaaacaacaagcgtatgcaaatgaagttattgcagagtctactcgtagatttggatacctagatgatgctcttaaggcaacctcttgggaacaatttgctgccaatgctaactcagctctaagaagtttacaacaaagtgctgctacatacttaaatcctgttatggatacccttaatactttcttataccaaactaaatcttcccagatgagagtttccgcaatggcacgtagtgcatccgctaaaactactccagctgaaaacgttacagctttaatagagaatgctgtaggggcgcgagaagatctagatacatatcttaaagaaagcgaagaacgtgttaagaaagctcaagagcttaagcagcaattggatgatcttaaggcaaaacaggcggctactgctcctatcgccaatgcccttactgctggcggtattggtggtgatgagagtaataagttagtagtacaactcactaatgaattggctcgtcaaaacaaagagatagaagaacgcactaaaactgagaaggttctaagacaagcggtacaggatactggagaagctctgttacgtaatggcaaactagctgagcagttaggcgctaagatgaagtatgctgatactgctgttccaggagacaaaggagtattcgaagttgatcctaataacctcaaagctgtatcagagatacagaagaactttgatttcctgaagaaaagctctagtgatactgcaaataacataagaatggcggcaagtagtattactaacgctaaaaaagcctctagtgacctaaatagtgttgtaaaagcagtagaagatacttctaaagtaaccgggcaaagtgcggatactctagttaagaacctaaatctaggtttctcaagcctagaccaaatgaaggctgcacagaaaggtctatcagaatatgtaactgctatggataagagtgagcaaaatgcactggaagtagctaagcgtaaagatgaggtttacaaccagactaaggataaggccaaggcagaagcagcagctagagaggtgttactacgacaacagcaggaacagcttacggcggcaaaagcgttgctagctattaaccctaatgatcccgaagcattaaaacaagtagctaagatagagacagaaattcttaatactaaagcccagggattcgaaaatgctaagaagactaaagactatactgataagattcttggtgttgatagagaaatagctcttctgaatgaccgcactatgacgagtactcagtatcgtttggcgcagttaagactagagctgcagttagagcaggaaaaaacggaattatactctaaacaagcggatggtcaagctaaagtagagcagtctagacgtgctcaagcacaaataagtagagaaatatgggaagcggagaaacagggaacagcctcacatgtatcagccctcatggatgcactagaggtcagtcaaacgcagagaaatgttactggtcaatctcaaattcttacggagagattatccattctccagcaacagctggaactatctaagggtaatacggaagaggagcttaagtatcgtaatgagatttataaaacttcagcagctttagagcagcttaaaaagcagcgagaaagtcaaatgcagcaacaggtaggatcttctgttggggctacttatactcctactactgggttaatcggagaagataaagattttgctgatatgcaaaatagaatggcttcttatgaccaggcgatctctaagttgtctgaattaaattccgaagcaaccgctgtggctcaaagcatgggtaatttaactaatgctatgattcagttctctcagggatctttagatactacgtctatgattgcttccggtatgcagactgtagcttctatgattcaatacagtactagtcagcaggttagtgcaattgatcaggctattgcagcagaacagaagcgtgatggcaaatctgaggcatctaaagctaagctgaaaaaattagaagctgaaaagctgaagattcagcaagatgcagctaagaaacagatcatcattcagacagcagtagcagtaatgcaagcagcaacagctgtaccatacccgttctctattcctttgatggtggcggcaggtttagcaggtgcgttagctcttgctcaagcatcttctgcatctggcatgtcttctattgcggattctggggcagatactactcagtacttaactctaggtgagcgacagaaaaatgttgatgtatctatgcaagctagttcaggagaactatcctacctacgcggtgataaaggtattggtaatgccaactcatttgttccgcgtgctgagggcggtatgatgtaccctggagttagttatcaaatgggtgagcatggtaccgaagtagtaactcctatggttcctatgaaagctacacctaatgatcagctttccgatggatcaaagactacctctggaagacctattatcctgaatatcagcactatggatgcggcaagcttcagagattttgcatcgaataacagtactgctttcagagatgccgtggaactggctcttaatgagaatggaaccaccctgaaatctcttggtaattcttaatattggaggaggactttatgtcctccttttctttatggaaaaataaaaatttcttgataaaattttccaatactattataatattgttattaaagaggagaaattaactatgagactaccagatccatacacgaacccagagtacccagggttaggttttgaaagcgtcaatttagtagataacgaccctatgattcgtgatgaattacctaatggtaaagtcaaagaggttaaaatatctgctcaatactggggaattaatatctcatacccggaacttttcccggatgaatatgcatttctagactctaggcttttagagtataaaagaactggagattatttagatgtactcctgcctcagtatgaagcatttagagtacgtggtgataccaagagtgttaccatacccgccggtcaaaaaggttctcaaattatactaaatactaatggaaccctaactgggcagccaaaagctggggatttatttaaattatctactcatcctaaagtttataaaataacaaattttagtagttcaggaaacgtatggaatatttccctgtatcctgatctatttattactactacgggtagtgaaaaaccagtttttaatggtatcttatttagaactaagctaatgaacggagattccttcggttctaccctaaataacaatggtacttactctggtatttcactttccttgagggaaagtctatgaagaaaatactcgatagtgctaaaaattacctgaatacccatgataaattaaagacagcatgtcttatagctcttgaattgccaagttcatctggttccgcagctacttatatctacttaacagattattttagagatgttacatataatggtattttgtacagatcaggtaaagtaaaaagtataagctcccataaacagaaccgtcaattatctattggtagtctatccttcacaataactggtactgccgaagatgaggtactaaagctagttcaaaatggagtatctttcctagataggggtataactatccatcaggcaataatcaatgaagaaggaaatattcttcctgtagatcctgatacagatggccctttattattcttccgcggtagaattaccggaggcggaataaaagataacgttaatacttccggaataggtacatcagttattacttggaactgttctaatcaattttatgattttgatagagtaaacggcaggtatacagatgatgcatctcatagaggtcttgaagttgttaatggaactcttcagccatcaaatggggctaaacgtcctgagtaccaagaagactatggattcttccactctaataaaagtacaactattctagctaaataccaagttaaagaagaacgatataaattacagtctaagaaaaagttatttggtctgtctagaagctacagccttaaaaaatactatgagactgtaactaaagaagttgacctagactttaacttagcagctaaatttatacctgtagtatatggtgttcagaaaattcctggtatacctatttttgcagatacggaactaaataaccctaatatagtatacgtagtatatgcttttgcagaaggtgagatagatggatttctagatttctatatcggagatagccctatgatatgttttgatgaaacagactccgatactagaacttgttttggacgtaaaaagatagtcggtgatacaatgcaccgtctagctgctggtacaagtacatctcaaccttctgttcatggacaagaatataagtataacgatggtaatggggatataagaatctggacctttcatggaaaaccagaccagactgctgcacaagtacttgtagacattgctaagaaaaaaggattttatctacagaatcagaacggcaacggaccggaatactgggattctcgttataagttattggatacagcttatgctatagttagatttactattaatgagaatagaactgaaattcctgaaattagcgcagaagtgcagggtaagaaagttaaagtatacaactctgatggtactataaaagcagataagactagcttaaatggtatctggcaacttatggattacctgacttcagatcgttatggtgctgatattactttagatcagttcccgctacaaaaagtaatatcagaggcaaaaatacttgatataattgacgagtcctaccagactagttggcagccctactggcgttacgttgggtggaatgaccccctatctgagaatcgtcaaatagttcaactaaatactatactggatacttctgaatcagtttttaaaaacgttcaaggtatattagaatcctttggtggagctataaataacctatcaggtgagtatagaataacagtagaaaaatattctacgaatcctctgagaataaattttctagatacttatggagatttagacttatctgatactactggtagaaataagtttaactcagtacaggcatccttagtagaccctgcactaagctggaaaacaaactctattacgttctataactcgaagtttaaagagcaggataaaggtcttgacaagaaacttcagttatcttttgctaatattactaattactacactgctaggagttacgcagatagggaacttaagaaatctagatactcccgtactttaagtttttccgtaccctataaatttataggtatagagcctaacgatcctattgctttcacatatgaacgttacggctggaaggacaaattcttcctggttgacgaagtagaaaatactcgtgatggtaaaattaatctagtcctccaagagtatggagaagatgtatttattaattccgaacaggtagataatagtggtaatgatattcctgatattagtaataacgttctaccgcctagagactttaagtacacccctactccaggtggcgtagttggtgctataggtaagaatggtgagctatcctggcttcctagtcttacaaataacgtagtatactattctattgcacattctggacatgttaatccctacatagttcaacaactggaaaataatcctaatgagagaatgattcaggagattataggggagcc

SEQ ID NO: 2 - DNA, 32767 bp, T5j phage
  source 1..32767: mol_type = genomic DNA
gagccacagaaattttcacttgtcaagctattttgccccctttagctaataaaattttactttttctgcacctatctcaaatcttcccaaattatctcaactcttccccaaaatccccgcaaatcaggtgctccgcaccaatcctgcgcccatatccttctagcctcccaaatttctctcgctctctcatcttcccctcaaacccatacaatcacacaccctcccatcgaagtcacaaaaatcttgtcggattcgcacatctcaacacatgtcggatttgcacatactctagctaattccacaggattcgaacgcagttcgtgattgctggagtttttgggaaaattcattgtcggatttgcacactataaaaatttttcgggtcggattcgcacactaccaaaaattgtcggatttgcacatacacgcccacgcgtaatccatgggggcaaatgtcggatttgcacaaaagcgcagggcaattgccctgctcgcctgaatgcgaatgataatgagaatcaatctcatttaaaaagtgaaatgcaaatgataatgattctcatttaagaaagggaatgagaactattcaggaagtgaaatgattctcatttaaaaagcggaatgattctcatttaaaaagcggaatacgaatgataatgattcgtatttaaaaacggaagtgagaaacactgttatttaagttatccacagacttatcaacagcacgattcgccttgacaaaatcctagccattttgaagcgttatcaacagacttatccccaggttatcctactgtatatttatacagtattcctacgcagtgaataattctaatatatgcctaaaacgtcctagatcgcattctaacgcgtttaattttgatggggatactaaaacaaagggggatttaactggaggcgtgaaaaacggggagctgatccccgtcggttatcagagaagtgggcaattgttacgctttgccatttcccgccaatcatcttgctgtctagacttgcgatgccgtactaaaaaccgtttataccagtgattaaaccatcgtttcataaatccccctcgggtaatcgatgcgtgatcttctcctcttccccgtaggaatcgaccaaatgctgataataaccatcggcatcataaataacgctatcatactcgccccgctcgaccgctccccgattctccggcgtatcgggcacataaaaaacgtctaccattgtggtagttttggtcacaataattttattgctcataataacgccccgttattagttgactatctcaaagatagcgttctcaagtgtcgcccttagaatcccatcgcgtcctactacggaatacttgagatcgggtattttgtaacgctcaattgttttgagtaattgatctttttgggctttatatttttgcccttctcgcgctatcgtgtcgccttcggctttaacgcaaatcagtgtaatcataataaccctagtaaatatatttttgccaatagtggcgaacgttatcgccaccagcggaatcattcgcagcctcaacattaccaacgaaaatatatagcttcattgcgccacctttctgaaagctgtttcaatactttccgcagttgactgaatatatgcgcctttcattatcaggcgctcggtgtataccttgcggaagatattaataaaatcatcttcattttctgcaattaacgcttcacccatgacctgaatatcacaagatgcgaaagtcaaaaattgaaatgctaattcacgggcaacgaccgcattaatcttataatgcgccttgccctcataaatattaatgacgcctttatattcaggtgacacctgatttaagtagtttgctaataatcccggtcggcaaatagcaacaaagcgattgccttcataaattaccattttataacactccacgaaaagccgcgtaaaaggtggcaaaatgtttaaccgtttcagctatcacgttgccgcgcttatcaaatttcttttctgtaacacgaaaggcgtttttattacgtgctacatattcgattttacaatcttcccgctcgaatgtgttaacatccaccagcttaaaaccctttgaacgagcaagagaaacgttgcggatcatttttattctcctttattcatgcagcccagcagataagaaaatacagcgatacccgcgccaataataaccataggtttagtatttactaaaccacaataagaatcttgaataccgtaagcggtagcaaaaagggtcagaatagcgcccaagatacctgccagaatagctcgaaaaataaccatttgtaatactcccctagttagtggggcgaaagtaacgccccgttattaattacattaaaacaattttggcggcttgttttttagtacagtgttccgctttcagggtatccagcaaaaagcccgccgtttgctgatcgatttgatcattatcataaagcgcctgaatggtagtgtaagttttagcaatgccgaactcctgcaccatttcttgaatgatccagcgatttgatacccagccttttccagtgaaaagagcgtcagaagaagaataagcaaccattttaagcctccaaaattttgggaaaattttcaaccgtcctcaaacggtgtaaaggcattataacaaaaaaggccgccgattatggcgacctttacaaaactttacattaggttaattattactcgctttcggtgttaacggtaaaagtagaaatatcaatacctttcaccatttcatcaatcatttcagcgatgttaaaactttgcaccatttctagcatagccgcttccatagctgcacccgctaccgctttcgccttttggttgctaggggcgtactggtcaaccgctacgctcagcaggttagcaataactacccgaccaataggcgtatcaatataacctttaatcataaatggtgcttttttagccgctactttcgtgatttgagttaatgcaattttgcccgcttccagttttgcagcatttacaacggcggatttattagcggcaacgatattagcgatcttggtcatggcattttttcctttgttttcagtgatttgagtgttaacgctttgagtgttagaatttacagcatgtttttccgtgttgtcaatgatctgattctcatctttccagaaaataaaacccgcttcttgtactagctcattatatacatacggatataattccgatggtaataaaaaattaccgtcgccatcaaaagccattacagccgtatattgagatccatcactatcaggtctatgccatccagcagataaatacttccagataacatctaaaaatccctcaaggctagaaagtccgtttattaattcaagcccaacaagctcaaaattatttatattaaatgattgacggcctgaattgctatgatacgcaacgatattattaccctgcgcaacaataaaatcagtatccggccccgctcccctgcccgtaaagatatggcaatcacgattatataagataatcgttgccccctgcttatataggggtagaaaactatccatatcataggcatcataatcattaaaaaagttttggtgaatagtttcagccttgttaataaaatgtttaatgctggttgtcctgctaccatccagcaggttgcgcaaggcgccctttaagacggttgcgttatctggtttatatagccgcatttgttggcctccctcgttaatcggtgagtgaatgataaaggtaattttctagcataggcaaatattattttacctttttattttccttgcctagcgcctagttttatgctaaccgcgcagcggtatagtaaagagcaaaacacggcgaagccaccagggcgacgcgttgaggctttactttaatattaccctatagcgttttgctcgttagaaagcgttttaggccgcttattttgggcatcattataatatgttttccatttaccctgtatatttatacagtggaataacctgtggataagtctgtgtaaaagtgctataaagccttcctattgtgtcaagttaatttacaaaatgtataaggctgtggataacttaaatgatagtgtttctcactaactaatttatgcagttattatataacaaaatatagttagttggctaataggattttaaagtgattatgagtctgctaattaaacctgaaaaactcattaggtagtttgctaatggttttgatataatataatagagattaaattaataacataaggaaactataacaatgggtctatttaaagatatagattattcgcttgctaatgataacttttattatgatgaaacatccccatcatttctaagatggaaagtacagaaaggtaatagtaaggtgggtgatattgcagggcattatagtaacacaggttactatcgagtaaagttagcaggcgaacaatacgcagtgcatagaataatatgggtattatttaatggtgagattgatagcaatctaacaatcgatcataatgatcgtaaccgtgctaataataacattaataatcttcgcttagtagaccataagcagaatatgaataacaagaaagattataagcgtgctaataagttgcctaagcatatctattataatggttctagagttgataataacggaagaaactatttgcgcgctatagttaaagatcctactagtaacaaaagtgttagtaaatcaggttatgatttacaagagttattattatgggtagaaactaaaaaagctgaatttggaattgtcaattaattaattttataaaataactcgtttagtcttgatttttaaaagtcaatatcttttccaactatttttcaattttgcttttgttaaatatttgttaaatcgaaaataagccgcctaaaacgctttctgacgcggtaaatttttcaggcatcccatcataaggggataacccgtttatcgtcaccacgagctttctaagatttgtcaactagggcaaggcaaatataaaggaaaaaattacttgccaacctgctaggttttatggtattcgcgcgcccgtttcctttaaacttaggtgagcgccggacgtgttgccttctttacgtttctttacaaaaataaggttgcgccatttttgggtatcccctattatttatctcgtagggcggcaatgacgaactacacggcgggaagtttaccgccacgctctttaaaaattgggtacatcttaaagtctatcggcggtaaacttatatattataaggaatcgacgatatgaaacaaactttattgatcactggtaaaccagctaaaaaattagatggtactactaaaaaattgttgacaatagcccagcaatcggtaaaatatcgatttaggcagtacaagaaaggccgccagcaaggtctggaaatgatctggcgaaacattatgattgacttgaaagaaaatcataaaaaactgcaaaaaatagtttgacaccctagccgataggctttaagatgtacccagttcgatgagagcgataacttgataaaatatgacggtcggcacttaccataatgtgtcccgccccctaactgggatatagcggcctgagtggagttctttaaattgattatattggcgagcggattgttgcttattacctgccactacttttacagcaggtaatgcggaacaatcccccttaataaactggagtttatattatgcaaaacgttactactgcgccaaaaattggtcaatccgtttttatccctttcgttactaaaacggatgaggtaaccggaaaaaccgaacgcattaaaggcgcggcgcttatgccgtttgatgtaattgatgcggtatacgctgaaacggaacggagtaacaacggaaaaactgtttacaacgttcgggttaaatccggcgacgttgtaaaggttgcccagcgtaacgaaaaatgggaagccgtagcgtaatagtgttacttttatatcccccagtagttcgggggatataacgattaacattatgttaatcttatcccttaaattaaataaacaggagttacatcatgactaacgctaaaaccgcaaaattcgcttggaatgaagaaaacactcagaaagctgtttccatgtaccagcagttaattaatgaaaacggtttagatttcgcaaatagcgacggtttaaaagagattgcaaaagcagttggcgcggcttctcccgtgtctgttcgctcaaaattgaccagcgcgaaagcgtatcagaaaagcgataaacctcgcaaggttggcggcggcagttctatccgcaaagcgcactacgtgcgtgtgattgcaaaacatgccatcgattccggtattatcaaagacgctgacgatctggcatcactggaaagtgcaaaattggaaacgctggacgccgtggcgcaactgttaggcgttgccgatgaagtaaaacaagccgcaggcgaataaatttaattagtggggaatattccccactataatttccctttgactggagttttaaaatgatcttttaccctactgaatccctcattctaggcttgtttattatggcggcctcgttattgttcgcttattttcaaaatgatttagattcgtattattttaaacgtaaatctaagttagcaaagcgtttaggtctgatttgttttattgccgccgttgcttgtggtgttagttctagccttatgcctttaaattaatgttgcaaattataacgcctattattcaaggcgttatatttggcaatattgccaataacaaacgttttttaatccctttaatggagttttattattatggttatttccgcagaaaaacaaaccgttatcctgaaaatggccgctgactttaatttctacggtaaacgtctgcgcgctactaaattggaagtttgcgacgatatttcaaaaatggtttacgatacaacaaaacactctaccgcaatttgtgactggctggaagcaaataaaccagcgaaaccgaaagcggcgaaagtagcaaaagccattaaaaacgatgagcgcccagaagcggcggggattgtttctagcacggttgagcaatgggaagtaaaacaaggtaaacgctttattattacatcgattcagaataatacgttcccgcataaaaactttttagcctcacttgaacaatacgcccaatttatcggcgctgatttgctggttagcaagtttatctataacaaaaacggttttcaaaatggcgagggcgccgacggtatcagatacgattccgcatttgacaaatatatctgcaataaaaacgtgtttttaaataatcgccgatttgctttcatggctgaaattaacgttttacccaccgcagattatccgctttctggattcgctgaaactgcaaccgcgctgaatcttgaaggtctagcaattggagcggctaaaatcaccgccgaaagcgtgccagctttaaaaggtgaaattgtgcgccgtatgtattcaaccggaacggcaacgctaaaaaattacatccagcagaaagcaggacaaaaggccgaggcgctgcataacttcggtgcgcttattgttgagtttgacgaggacggtgagttttttgtgcgccagcttgaaacgatggacgagagcggcgtgttttatgatttgaatacttgcgccactcctgccggatgttatgaaacaacggggcacgttttaggtttacaatatggcgacattcacgctgaaaaattagatgaggagtgcgccgctgcgtcttgggggcatggtgacacctacgggcttgttgatattcttaaaccaaaatatcagtttgtacacgacgtgcatgattttacatcacgcaaccatcacaaccgcgcatctggcgtattcctagcgaaacaatatgccgccggacgtgataaggtattagatgatcttatcgatacggggcgcgtactggaatcaatggagcgtgatttttctcaaacaatcattgttgaatctaatcatgatctggcgctatcccgctggttagatgatcgtaatgctaacattaaagacgacccagcaaacgcggaactatatcaccgcctgaatgctgcgatttatggagctattgcagaaaaagacgatacttttaacgtgcttgattatgcgctgcgcaaggttgcaggctgtgaatttaacgccattttcctgaccactgaccaatctttcaagattgcaggcattgaatgcggcgtacacggtcacaacggcattaacgggagccgtggcaacccgaaacagtttaagaaattgggcaaattaaacaccggacacacccacaccgccagcatttacggcggcgtttataccgctggcgtgactggtagtctggacatgggttacaacgttggcgcgtctagctggactcaaacgcatattattacctatgcaaacggtcaacgcactttgattgactttaagaatggtaaattctttgcgtaattaaattattcccctagcggcttgagatatagccgctattacaggagctaaattaaatggctattaaaattaatcttcccagcatgaaaaacaccgctgatacatggtcgcttgatgttttacggcatggtactgtataccgcaatttaaaagataataattgttatatttatcaaaatgaactaaacgggcatatttatataattgagtccggcgatttttattcttttgaaaatgagtatgaagcgaaagaccatttacaggaaaatgatattcctgacgtatggaaagaaacaaatctcgcttttgttgtaagtcttgaagctagcaaataaattaaatcccttattaaactaattggagttataaacatggctaaatctaaccgtatcccattcgatcgcgctcagtcttctattgttctggtttattctaatggtcagcgttatcacgtcgaggccggtcacgttattgatgagctattagatttcaatgacgcgatgcaagttacaacgtttgcatatatgcagggcaaactaacaagccatattaaagcaaaaggtgtttatgttgacactatgaaacaggaaacaatcattattgacgcggtaaaatccggtttagctttcgcagtagtcgcaccttgccccgcttgccttgatgatcagctaatgagcgcaaaggtgtatacatgcgctggcattcgttccagcgtatcgggcgaggatgttagttttatcgctgatgcgctagcgtatggcctttaatagttaatttattattacccgctatttaatagcgggtaatgctgaattaatctaatccctcaaatggagaacgtaacaaaatgaatcaagttaaaacgaatattacccgtaatttcccgcatatttcccgcgtcatgatttgggatctggacggcactatcattaattcgtttcatcgtgtagcgccttgctttgatagcgagggcaatttagatttaaataagtataaaaatgaagcctgcaaacatgatttaataatgcaagatacactattgccccttgttacatatatgcgccagtgcatgaatgacgcaaatactttaaacattatttgcaccgctcgactaatgagcaagtcggactattattatttgcgtaaacaagggttgcgcggtcgtggtgatagtaatatccgtgtattttcccgcgatacactacacaaatattttgaggctgataaagttagcgagatataccacagcaaagacgcagtttataaaagttactattttgggctattcaaacaattatatccgaacgctgattttacaatgattgatgatcataaaggcgtgctatcagcggcagcgtcatacggatttaaaacgctggacgcacaagccgttaatgatattctatcaatcggcgtgacattgataggtgaaacctttattgatgaatctcttgaggatgataatgattatcagttcctagccgaccgcctgcaattatgttgggaaggtatgaccgaagaagaacgcgcagaatatagttgcagcccgcaacaatatattgagaaattaaaagttgcgtaataattaaagttgaaattgtttcaccctgcaattaaaatggttgcagggtgaaacagttagcatggtaatagtaacgggggtggcggttagcagactaagtattttcgccggaggcagtggacacaccttcatgtgtaatcttatgaaatttcgagatttcccaattagcgcatagaatggtcatcaactccgtattttggtctgaactcacggaatctcttccgcgacgcccgagaaccgtccgaccactcccgctcaaactccgcacgtttttcgtcaaacttccgctccctttccgcaatctcccgcgatacttccgcaatgtatttacgatgcttgttaatagccgcagtcattccgaaaactcccgcgattattccgataataaaagcaactataatgctaaacatctaattccctctcaatttgcagaatacgaatgctatcacaacgttggagttctactaatttttctatagcaaattgttgttgttttacttgagcttctagagtttttaggcgaacgtacacggtgcaagaagcaatgaaaattgcccagactagtattactgttattatagctactacttccatcatttacgcttctccgttaataaagtttcaattctagctaagtgattatctaaaatacattgtccaataatcacaacccctagcaacgcaataattacccattccattaaatccaccccgccatagctgctaaccaaaaacctacgaaaataaagaataaaatagttcctaatccaaagctattaatccagctatcgtacacttctccacgtctgctctttcttttgtttgacatatctttcatgctcctataagtgtggtatttaaaatactctagcaattgcagtgattagtgtaaatattcccatcacaccttccatagtgtcttgtgtggtatcctgaactaattctgcactaggttcatcttaagtggtgatggttactaaggtggtttttacttagaaaactccctcgcatgtatttccttcggtaaagtagcttacgggggcccagaaagatccataggccataattggtgacaccaaaaacatatcccctttcctatcaaaaacattagccttatatttcacatgatcctgcatatagtatgcctcacatttaatatctttaggtccaaaagtagagcaagccgaaagaagtaccactgccatagctaaaaataattttttcatttacattctcccctatttaatttataatactattatacagaattatggcagtataagcaactaaatttttggagaacttatgagttttttcgctggcaagctaaataacaaatctatactctcactgcgaaggggtagtggtggagatactaaccaacatatcaaccctgattcccaaaccatctttcattcagatatgtcgcacgtaattataacggaaactcattctactggattaagattggatcagggggctggtgactattactggtctgaaatgcctagtagagttacacagctacataataatgaccctaatagagttgtattaacagagattgagttttctgatggctctagacatatgctatctggcatgtctatgggagtaggtgcaaaagcctatggtattataaatcctcagattatgtctcagggtggattaaaaacacaaataacagctagtgccgatctttcacttgatgtaggttattttaatacgggtactagtggcactataccacaaaagttaagagatggcacaggatgtcaacatatgttcggtgcttttagtgggagaagggggtttgcatcaagtgcaatgtacttaggtggtgctgctctttacaaatctgcgtggagtggttccggttatgtggtggctgatgcaggaaccttaactatccctagtgattatgttagacacccaggagctaggaactttggttttaatgctatatacgttcgtggtaggtcttgtaatagggttctttatggtatggaaggaccaaactatactaccggtggggctgtgcagggagcttcgagctctggagcccttaactttacgtataaccccagtaatccagaatcaccaaagtattccgtaggtttcgcacgtgctgatcctactaactatgcttactgggaaagtatgggagatcctaatgattctgccaatggacctataggtatctacagcgaacatttaggcatttatccatctaaaattacatggtatgttactaacctagtatacaatggttctgggtataatatagacggtgggttatttaacggtaatgacattaagctcagcccaagagaatttattattaaaggggttaatgttaataatacatcttggaaatttattaattttatagagaaaaatttcaacgttggtaacagagctgattttcgtgatgttggttgtaatctaagtaaagattctccctcaacaggaatatcaggtatagcaacatttgggctaccaaccacagagagcaataatgctcctagtattaaaggtggtaatgttggtggcttacatgctaatgttgttagtatttataattttttaccttcagcatcttggtatgtatctagtaatccaccaaaaataggtaataactatggcgacgtttggagtgagaatttattaccattaagactcctgggaggtagtggtagcactatattatctggaaacatagtattccagggtaatggatctgtacatgttggtactgtggggttagatcttaatagcagtagaaatggtgctattgtatgtactatggagtttatagatgatacatggctatccgcaggcggtattggttgcttcaatcctacagaaatgttatcccaaggggcagaatacggtgatagtagatttaggataggggggaataccataaataaaaaactgcatcaaatactatctctaccagccggagaatacgttccattctttactataaaaggtacagttgtaaacgcttgtaaattgcaggctgctgcgtataatccaacaccatattgggtatctgggttgcctggatctgttgggcaaacaggatactatactctaacttactatatgagaaatgatggaaataataatatctctatttggttagattcttccatgagtaatataattggcatgaaagcatgcttacctaatattaaacttataattcaacgccttacctaaaggaggaaatatggcaaatgatgtattagtaccagatcttatgtcccctgaagggatggatgtgattgaagcttatttacagtgtggcagcgacgtgccttctgccgcacgtagtcttggaatgtccgaaattgcttttcgagatattatgaatcgtagtgaagttaagaactacttaaatgatatttttatggagagtggtttccgtaacagagatcgtttatttggtgttctggatgaagttatcaagcgtaaactagaggaactggaagaaactggcatgggttctgaccaagatattatggatattctctggaaagcacataaaatgaaaatggaagaaatgaaaatgatggtagaactggagaaagtgaaggcagcagcccgtactccagctaaccagaccaacatccagaataatattattgctggagctggggatcaaaactacatggacttaattacttccctagctactggaggtaagaagtaatggaagtatcaagaccctacgttaatacagtagatgttatcgatttcgggatagataaacgtttctttcgtctacctgtttcaggaatactagcacaagaaggtattacacctaatggtcctcaaatagcgattattaatgccctagaggaccctagacatcgttttgtaacagcgtgtgtgtcacgtcgtgtaggcaaatccttcatcgcatacacacttgggttcctaaaattgctggaacctaatgtgaaggtactagtagttgcccctaactactcactggctaacattggttggtcacagattcgtggtcttatcaagaagtatggcctacaaaccgaacgtgaaaacgccaaagataaagagattgagctggcaaacggctcgctcttcaaactagcttctgcggcgcaggctgactccgcagttggacgttcatatgattttatcatctttgacgaagcggcaatttccgatgtgggtggtgatgctttcagggttcagctgcgtcctactctggataaacctaattctaaggctctatttatttccacccctcgtggaggtaactggtttaaagagttttacgcctacggatttgatgatacgttgcctaactgggtatctattcatggtacatatcgtgataacccacgtgctgacttgaatgatattgaggaagcacgccgtacagttagtaaaaactacttccgccaagaatacgaggctgacttctctgtattcgagggccagatctttgatacctttaatgctatcgatcatgttaaagacctcaaaggtatgcgtcacttctttaaagatgatgaagcattcgaaacgttgcttggtattgacgttggttatcgtgatcctacagcagttcttactattaaatatcattacgatacggatacttactatgtattagaagagtaccagcaggcggagaaaactacagctcagcatgctgcttatattcagcactgtatagatcgttataaagttgatcgtatttttgttgactctgcagcagctcagttccgccaggatttagcatatgagcatgaaattgcatctgctccagctaaaaagtctgtcctagatggtctagcatgcctgcaagcgctattccagcagggcaagattattgtagatgcttcatgttcctccttaattcatgcattgcagaactataagtgggacttccaagaaggcgaagagaaattatcacgtgaaaaaccacgtcatgatgctaactctcacctttgtgatgcgctccgctatggaatttactctatttcccgtggtaaataaataagtataggatgggatactactcagttggtatcccattcctgtattttaaaatcccctttacaaattcgatacgattatgtatactatattcattgatcgggagaacttctcccataatagaacgtaaacaagaaaaattaatgctctacatgggtgtaggagattctatgggtcgacaaaagctaacaataaaagatataaatattagattagctgatcgtggaatccaaattgtcggtgaatatgtaaaccaacgtacaaaaacagtatttaaatgccagagagcacacgtttgggaagcaacaccacattctatactccatatgaggagaggttgtccacactgctccaataatacaatatcgttagatgaagttagtaacagaatatctaatatagggtatactctgttaagcagctatactaatgctaaaacaaaactacatctacgctgcaataatgggcatgactgtttcattaccttagatggattgactcaaggtaagagatgtccttattgttctcttaagtgggagaatggtggattcctctatatcatgtccttctctagcggtactaaagtaggcataagcttatatcccgagaaacggttgaatgaagttaaaagagaatctggattttctgacctgtacttgttcaccatgtatcatctgccagatagagagactgctttagatttagaaaaggaagttcacagagaatattataataaaaactgtgggttttctaattttacaggaagcacggaattttttaatgttgctcctgaggatatagtaatctttctaaatagctttggattggaggagtatggccactaatactaagtacaaacgtgatgccatttccataatgagggatggtataaaatctaggtatagtaaggatggttgctgtgctatatgtggtagtagtgaagacctagaacttcatcactatcatactatatctcagctaataaaaaaatttgctaaagaactccagctggatttcactgatgagaatatcgtcctttcaaatagggaagcattctacaagaaatatgagcatgagttagttagggacgtggtaacattgtgccagcaccatcaccaattattacataaggtttacacgaaagaacctccattattttctgctaataaacagaaagcatgggttcaaaagcagaaagacaaaatacagaatcctcaagaaaagacacaagtcaagactgaaacaaaatcaggattcgcaaggttcttataatgggttttaaaagctggattactgaaaagctaaatccgggtcaacgtattataagagacatggaaccagttagtcatcgcactaaccgtaagccttttaccactggacaagcctacagtaaaattgagattctcaatagaactgctaatatggttatagatagtgcggcggagtgttcttatactgtcggagataaatataatattgttacgtacgctaatggcgtcaaaacaaagactctagacactctcttaaatgtacgacctaatccattcatggatataagcacattccgtagacttgtagtcactgacctactttttgaaggttgtgcatacatctattgggatggcacatcgctttaccatgtcccggccgctcttatgcaggtcgaggcagatgccaataagtttatcaaaaaatttatatttaataatcagataaactatcgcgtagatgagattatctttataaaggataacagttacgtgtgtggcacaaactctcaaatttctggccaatctcgtgttgctactgttattgattctcttgagaagcgttctaagatgcttaactttaaagagaaattcctcgataacggaaccgtgattggtcttattcttgagacggatgaaatcctgaacaagaaattgcgtgagcgtaaacaagaagaattacaactcgattataatcctagtacgggtcagtcctctgtcctgattctagatggtggtatgaaagctaaaccgtactcccaaatatcctcttttaaagatctagactttaaggaagacatagaagggtttaataaatctatttgtctagcctttggagttccgcaagtactgcttgatggtggtaataatgcgaatattcgaccaaacatcgaattgttctattatatgactatcattcctatgctgaacaaactgactagttctcttactttcttttttggttataagatcactcctaatactaaggaagtcgcagcattaacaccagataaagaagcagaggctaaacatttaacctcattggttaataatggtattataaccggtaacgaagctcgttcagagctgaacctggagcctttagatgatgagcagatgaataagatccgtattcctgctaacgtcgctggttctgcaacaggtgtatctggtcaagaaggtggtagacctaaaggttccaccgagggagattaagaatgattgattatagtggtctaaggaccatttttggtgaaaaactaccagaatctcatatcttctttgctacggttgctgcgcataaatatgttcctagctatgcttttctgcgtagagaactagggctttcatctgcgcatactaaccgtaaagtatggaagaaatttgtagaggcttatggtaaagcaattcctccggccccaccggctccaccattaactctttctaaagatttaactgctagcatgtcagttgaagagggagcagcattaacactttctgttactgcaactggtggtactggtccatatacttatgcatggactaaagatggttctcctattccggatgcttcaggagctacctatactaagcctacagcagcagctgaggatgccggctcttataaagtaactgtaacagatagtaagcaagtaagtaaggattctactacatgtgctgtgacagttaatcctactgttcctggaggctaataaatgacacaagctgctattgactataacaagttaaaatcagcacccgttcatttagatgcttatattaaatctattgatagcgaatccaaagaaggtgttgtaaaaatccgtggattcgctaacacaattagtaaagatcgcgctggtgatgtaattcctgcttctgcgtggaaaacgtctaatgcacttactaactacatgaaaaacccgattattcttttcggacacgatcatcgtcgtccaatcggtaagtgtattgatcttaaccctactgaaatgggtctcgaaatcgaatgtgagatctatgaaagttctgacccggctatcttttcactaattaaaaacggtgtactgaaaacttttagtatcggattccgctgcctagatgcagagtgggatgaagctactgatatatttattattaaagatttagaactatacgaagtttcggtagtttctgtaccttgtaatcaggactcaacattcaatctcgctaagagcatgaatggtcatgattatactgaatggcgtaaatcttttactgcaataagttctaaagctgtcccagctcaagaacgtaatctttctgaactagaaaaacttgcgatagctttaggctacgttaaagaataacggagaattatttaaaaatgactattgatattaataagctgaaagaagaacttggtctgggtgatctggctaaatctctggaaggtctgaccgctgctcagaaagctcaggaagctgaacgtatgcgtaaagagcaggaagaaaaagaactggctcgtatgaatgacctggtttctaaagcagttggcgaagaccgtaagcgtctggaagaggctctggaactggttaagtcgctggatgagaaatctaagaagagtaatgaactgtttgcgcagacagtagaaaaacagcaggaaactattgttggtcttcaggatgaaatcaaatctctgctgacagctcgtgaaggtcgttccttcgtcggtgatagcgtagctaaagcactgtatggtactcaggaaaactttgaagacgaagtagaaaaactggttctgttatcttatgtaatggaaaaaggcgtattcgagaccgagcatggtcagagacacctgaaagcagtgaatcagtcttcttccgtagaagtttctagtgaaagctatgaaactattttctctcagcgtattatccgcgacctgcagaaagagctggtagttggcgcactgttcgaagaactgccgatgtccagtaagattcttactatgctggttgaaccggatgctggtaaagctacttgggttgctgcttctacttatggtaccgatacaactactggtgaggaagttaaaggagctcttaaagaaatccacttcagtacttacaaactggctgccaagtcctttattactgatgaaactgaagaagatgcaatcttctccctgctgccgctgttgcgtaagcgtctgattgaagcacacgctgtttctatcgaagaagctttcatgactggtgatggttctggtaagccgaaaggtctgctgacccttgctagtgaagatagtgctaaggttgttactgaggctaaagctgatggttctgttctagtaactgctaaaactatctccaaactgcgtcgtaaactgggtcgtcatggtctgaaactgagcaaactggtactgatcgtatctatggatgcttactacgatctgctggaagatgaagaatggcaggatgttgcccaggttggtaacgattctgttaaactgcaaggtcaggttggtcgtatttatggtctgccggttgtagtttccgagtatttcccagctaaagctaactcagcagagttcgcagttattgtttataaagataacttcgtaatgccacgtcagcgcgctgttactgttgaacgtgagcgccaagctggtaaacagcgtgatgcgtactacgttactcagcgtgttaacctgcaacgttactttgcaaatggcgttgtatctggtacttacgctgcgtcttaatacaggcttttcagccgataaggagagcttcggctctccttttttattgggaaaaataaatgcaaataatcacagctgaagactatagattatatggtggtttaaaacgaccggaactagaatctggagtagaggtgatgattactgctgccaatgcgctgattactagccttttaggtatggatgatgctgacgcagtagaccagttaatcactacaaaacctactcgtaaaaaatactttttaagttctccctcagctacttcagtaaccaaaatgactattaatgataaggagatagatcctgaacagtataagttgtattctgatggggttatacttcttaaatttaatcctccagaaggttatatggacgtagaatatacacagggtgggtttaacccaatgcctgaggatctcaaacttgcagcatgtatgctagtagatcattggcacaaacaagattatcgccaagctagaacaattggtggtgaaacagtaaccttcaataacactaaatctggtattccagagcatattcgtactattattgaagtgtataggagagtataatgtctctttctgatctagctagacaaattattaaagagcagctagatactgcaagccgatctgaaaacaataagaatactgttgtatactctgttgaaacagggttaaaagatcctaccagagatggtactgttgctcaagtatcctttaagttttcaaaacctgtatcacaagatctccttaacattaggacagcttctatactaaaagctgtatcctctagtttagatctttctggagatttaggtgctctggagaatctaatacaagcaaccgccggtaaaaaatcctcagtaggtaaaaaacgttctactggtagggtacaggtaaactttggtgatcctagtgatgttgaagatggatattctggtgcagtaacaggtgcttctggacgttttgtgtctaacagcaatatgaagattatactagaaatagttgctaaagaatacttaataaaggatatgaaaaaagctggagcaccattaaagtttagaactggtcgctttgcaaactctttaaaaattaaagatgttatgcttcgtgattctgaaactagtaaaggctctcctgaattaaacgtaacatataactatatgactcgtccatattctgtgttcaatccggcagtatctacatatagaagattatccctacgaccttatcctggcgctagaaacccacaaaaacttattggtgaggctatagcaaaagctgcaagagacctgattcactccagatataaaattaaggttaatcaaggaacctaataaatggatcatagaacaagtattgcacaagctatggttgaccgaatctctaaacaaatggatggttctcaacctgacgaatattttaataacctatatggaaacgtttctcgtcaaacttataaatttgaggaaatacgagagtttccttatgtagcagttcatatcggaactgaaactgggcagtatcttccttcaggccaacagtggatgtttttagaacttccaatcctggtgtacgataaagagaaaacagacattcaagagcaacttgaaaaactcgtagcggatataaaaaccgttattgacacaggtggaaatttagaatatactgttagtaaacctaatggatcgaccttcccatgtgaggcaactgatatgatcattacatcagttagtacagatgagggtctactggccccatatggtttagcagaaataaatgtaacagtgaggtatcagcctccacgtaggtcacttcgcagataagttacagattaggagaaaataattaaatgtctttacaactattacgtaatactcgaatcttcgtgtctacggttaagactggtcataataagaccaacacgcaagagattctagttcaggatgatatttcttggggtcaggacagtaactcaacagatattactgttaatgaagctggtccgcgtccaactcgtggttctaaacgttttaacgactctttaaacgcagctgagtggagtttctctacttatatcctgccgtataaagataaaaatactagcaaacaaattgttcctgactatatgttatggcatgcactttctagtggtagagctattaatcttgaaggaactactggagcacataataatgctactaacttcatggttaactttaaagataattcctatcatgagttagcaatgctacatatttacattctgactgataaaacgtggagttatatcgattcctgtcagattaatcaggcagaagttaacgttgatattgaagatattggtcgtgtaacttggtctggtaatggtaaccagctaatcccactggatgagcaaccatttgatccagatcaaataggtattgatgatgaaacttatatgactatccagggttcttacattaagaacaaactaacgatcttgaagatcaaggacatggataccaataagtcttatgatataccaattaccggtggtacttttactattaacaacaacattacttacctaacacctaatgtaatgtcccgtgttactattccaattggttcctttactggtgcttttgaattaactggttcattaactgcttacctgaatgataaatctcttggttctatggaactgtataaagatcttatcaaaactctgaaggtagttaaccgctttgaaatcgccctagtacttggtggcgagtatgatgatgaacgtcctgcagctattctagtagctaaacaggcgcacgttaatattcctactattgagactgatgatgtacttggtacttcagtagaatttaaggctattccgtcagatctggatgctggtgacgaaggttacttaggcttctctagtaagtatactagaacaactattaataatctaattgttaatggtgacggtgctactgatgctgtaaccgcaattactgttaagtctgctggaaatgttactacattaaatcgatcagctactcttcagatgagtgttgaagttactccttcttccgcaaggaataaggaagttacttgggctatcactgccggtgatgcagctactatcaatgcaacagggttactaagagcagatgctagtaaaaccggtgcggtaactgttgaagccacggctaaagacggctctggtgttaaaggcactaaagttattactgtaacagcaggtggttaattaaatgttttattctctcatgcgagagtctaaaatagttattgagtatgacggtagagggtatcatttcgatgccctctctaactatgacgctagtacgtcttttcaagagtttaaaactcttagacgtactattcataatcgtacaaactatgcagactctattattaatgctcaagatccttcatctatttcattggcaataaatttcagtactacgcttattgaatctaacttctttgattggatgggattcacgcgtgagggaaattctttatttttgccaagaaatactcccaatattgaacctattatgttcaatatgtatattattaatcataataatagctgtatttatttcgaaaactgttatgtatcaacagttgatttttctctagataagagtataccgatcctaaatgttggtattgagtctggaaaattctctgaagtatctactttccgagatggatatacaattacacagggtgaagttcttccatatagcgctcctgctgtgtacactaatagctctccgttgccagcgctaatttcagcatctatgtctttccagcaacaatgttcttggagagaagatagaaatatatttgatataaataaaatttatactaataaacgagcttatgtcaatgagatgaatgcttccgcaacgctagctttctattatgttaagagattggtaggagataagttcttgaatctagatcctgaaacaagaactccactaattattaaaaataaatatgtttctataacattccctttagcacgtatttcaaaacgcctaaacttctcagatttgtatcaggtagagtatgacgtaatccctactgctgattcagaccctgtagaaataaacttctttggagaaagaaaataatgattaacttaaaagatattactttagaaactcgtactgtcactctttcatacccaggtatgccaaactttaagctagagcttaattatatgtctcgtgctacttctaaacgagttatcacctctgctaagcgtgacgagtgggttaatggtactttgattcaggtacaggatgatgataagtttattgaagctttcgttgatgctgcgattaaaggttggactggtttgactgtaggtgacgttgaaaaactgatgctgattgaaacagatgctgatcctgctactgaagttccatttagtcgtgataatgctgtaatgcttatgcagaactctgctgcgtttgattcttggatcaaccagacagtgttccacctagatacttttcgtagctcaaaagcgtaaagaattactagatgctgttgctgattttgcagataagtgtattaaaagctcagcatctaaaatgactaaacaacaatatttaatactttgtgaatcaatgggtatagagcctgatcctaaggccatgcctgttgaacttgaagactttccacctattgtagctattagtatgaatatttataatagtctagttgactgtttcatacctggtgacttccctatctttataggtaaagacaaggctgctttaggtgttttatttgatatttatgggattacagatcctatagagaaagaatttgttctacacattatcaatatatttgatgctaaagctgtagacgctgcacgtaaacgtgctgagaagcataagccgcaaaacggtagaatacctaacgttaagccacatgccaaatctcgagcacggtaaaagtttcctccaatggggcgttccacgatgaggcttggctctgggtgatatgcccagagccttttttatttataaacatataggttggtatagtatgggaaagaagattactaaacaggatagagagtctcagataagcaacatttgcaatgataaaaatttatcctttgttggctggataggtgagtacactaatattaaaagcacccttacacttaagtgtaataaatgttattacacctggtctcctaggttggataactttttacggattactgcccaaaaatgccctgcatgcgcaggcaaagctagatggacgaaggaagaaagagaagaacaaataaaaagtaagtgtgccgagaaaggatataactttctatcttggtcttccacctatattaataaagattctaagattatacttaagtgtttaaaagatggttgtatctgggatgtgtctatacaccattttattaatcacgatacagggtgtcctgattgtgcttcaggaggatttaatcctaatataccagctactttttatatacagaaattaacgtatcaagggactcactttctaaaatttgggatcactggtaaggatgtactagagagaatgaggcagcagagcaataaatcactatgcgagcactcggtaattttttctcatactttttcttatggttctatggctagggggctagaaaaagtagtaaaggactcagtaaacacaggagtattagataaacgtatccttccagatgggtacaccgaaacttgtcactactctgagctagaaactatactatctttaactaatagttttatacaggaaaacattagatgactgataagctaatacgagaattactaatagacgttaaacagaagggggcaacccgtactgcaaagtctattgaaaacgtatctgatgcattagaaaatgctgctgctgcttccgaactgacaaatgaacagttaggtaaaatgcccagaactctatactccattgagagggcagcagatagagcagcaaaaagtcttactaaaatgcaggctagtaggggtatggctggtatcactaaatccattgatggtattggtgataagctagattacctggctatccaacttattgaagtaacagataaactagaaattggattcgatggggtttctagatctgttaaagcaatgggtaatgatgttgcagctgcaacagagaaagttcaagatagattgtatgacaccaatagagctttaggtggtacatctaagggttttaatgacactgctggtgctgctggtagggcttctagagctttaggtaatacttccggttccgcacgcggagctactcgtgactttgcagcaatggctaagatcggcggtaggttacctattatgtacgcagctcttgcttctaacgtattcgtcctacagactgcttttgagagcctaaaagtaggtgaccagctaaataggctggaacagttcggtactattgtcggcaccatgacaggtacaccggtacagacactagctttatcactacaaaacgctactaatggtgctatatcctttgaagaggctatgcgtcaagcatcctctgcttccgcttatggatttgacagcgaacaactagagcagttcggtttagtagcacgtcgtgcggctgctgttcttggtgttgatatgactgatgcacttaaccgtgtaattaagggtgtatcaaaacaagaaatcgaacttctggatgaacttggtgttactattcgtcttaacgatgcgtatgaaaattacgttaaacaattaaatgctaccagtacaggtattaaatatactgtagatagtttaactacataccagaaacaacaagcgtatgcaaatgaagttattgcagagtctactcgtagatttggatacctagatgatgctcttaaggcaacctcttgggaacaatttgctgccaatgctaactcagctctaagaagtttacaacaaagtgctgctacatacttaaatcctgttatggatacccttaatactttcttataccaaactaaatcttcccagatgagagtttccgcaatggcacgtagtgcatccgctaaaactactccagctgaaaacgttacagctttaatagagaatgctgtaggggcgcgagaagatctagatacatatcttaaagaaagcgaagaacgtgttaagaaagctcaagagcttaagcagcaattggatgatcttaaggcaaaacaggcggctactgctcctatcgccaatgcccttactgctggcggtattggtggtgatgagagtaataagttagtagtacaactcactaatgaattggctcgtcaaaacaaagagatagaagaacgcactaaaactgagaaggttctaagacaagcggtacaggatactggagaagctctgttacgtaatggcaaactagctgagcagttaggcgctaagatgaagtatgctgatactgctgttccaggagacaaaggagtattcgaagttgatcctaataacctcaaagctgtatcagagatacagaagaactttgatttcctgaagaaaagctctagtgatactgcaaataacataagaatggcggcaagtagtattactaacgctaaaaaagcctctagtgacctaaatagtgttgtaaaagcagtagaagatacttctaaagtaaccgggcaaagtgcggatactctagttaagaacctaaatctaggtttctcaagcctagaccaaatgaaggctgcacagaaaggtctatcagaatatgtaactgctatggataagagtgagcaaaatgcactggaagtagctaagcgtaaagatgaggtttacaaccagactaaggataaggccaaggcagaagcagcagctagagaggtgttactacgacaacagcaggaacagcttacggcggcaaaagcgttgctagctattaaccctaatgatcccgaagcattaaaacaagtagctaagatagagacagaaattcttaatactaaagcccagggattcgaaaatgctaagaagactaaagactatactgataagattcttggtgttgatagagaaatagctcttctgaatgaccgcactatgacgagtactcagtatcgtttggcgcagttaagactagagctgcagttagagcaggaaaaaacggaattatactctaaacaagcggatggtcaagctaaagtagagcagtctagacgtgctcaagcacaaataagtagagaaatatgggaagcggagaaacagggaacagcctcacatgtatcagccctcatggatgcactagaggtcagtcaaacgcagagaaatgttactggtcaatctcaaattcttacggagagattatccattctccagcaacagctggaactatctaagggtaatacggaagaggagcttaagtatcgtaatgagatttataaaacttcagcagctttagagcagcttaaaaagcagcgagaaagtcaaatgcagcaacaggtaggatcttctgttggggctacttatactcctactactgggttaatcggagaagataaagattttgctgatatgcaaaatagaatggcttcttatgaccaggcgatctctaagttgtctgaattaaattccgaagcaaccgctgtggctcaaagcatgggtaatttaactaatgctatgattcagttctctcagggatctttagatactacgtctatgattgcttccggtatgcagactgtagcttctatgattcaatacagtactagtcagcaggttagtgcaattgatcaggctattgcagcagaacagaagcgtgatggcaaatctgaggcatctaaagctaagctgaaaaaattagaagctgaaaagctgaagattcagcaagatgcagctaagaaacagatcatcattcagacagcagtagcagtaatgcaagcagcaacagctgtaccatacccgttctctattcctttgatggtggcggcaggtttagcaggtgcgttagctcttgctcaagcatcttctgcatctggcatgtcttctattgcggattctggggcagatactactcagtacttaactctaggtgagcgacagaaaaatgttgatgtatctatgcaagctagttcaggagaactatcctacctacgcggtgataaaggtattggtaatgccaactcatttgttccgcgtgctgagggcggtatgatgtaccctggagttagttatcaaatgggtgagcatggtaccgaagtagtaactcctatggttcctatgaaagctacacctaatgatcagctttccgatggatcaaagactacctctggaagacctattatcctgaatatcagcactatggatgcggcaagcttcagagattttgcatcgaataacagtactgctttcagagatgccgtggaactggctcttaatgagaatggaaccaccctgaaatctcttggtaattcttaatattggaggaggactttatgtcctccttttctttatggaaaaataaaaatttcttgataaaattttccaatactattataatattgttattaaagaggagaaattaactatgagactaccagatccatacacgaacccagagtacccagggttaggttttgaaagcgtcaatttagtagataacgaccctatgattcgtgatgaattacctaatggtaaagtcaaagaggttaaaatatctgctcaatactggggaattaatatctcatacccggaacttttcccggatgaatatgcatttctagactctaggcttttagagtataaaagaactggagattatttagatgtactcctgcctcagtatgaagcatttagagtacgtggtgataccaagagtgttaccatacccgccggtcaaaaaggttctcaaattatactaaatactaatggaaccctaactgggcagccaaaagctggggatttatttaaattatctactcatcctaaagtttataaaataacaaattttagtagttcaggaaacgtatggaatatttccctgtatcctgatctatttattactactacgggtagtgaaaaaccagtttttaatggtatcttatttagaactaagctaatgaacggagattccttcggttctaccctaaataacaatggtacttactctggtatttcactttccttgagggaaagtctatgaagaaaatactcgatagtgctaaaaattacctgaatacccatgataaattaaagacagcatgtcttatagctcttgaattgccaagttcatctggttccgcagctacttatatctacttaacagattattttagagatgttacatataatggtattttgtacagatcaggtaaagtaaaaagtataagctcccataaacagaaccgtcaattatctattggtagtctatccttcacaataactggtactgccgaagatgaggtactaaagctagttcaaaatggagtatctttcctagataggggtataactatccatcaggcaataatcaatgaagaaggaaatattcttcctgtagatcctgatacagatggccctttattattcttccgcggtagaattaccggaggcggaataaaagataacgttaatacttccggaataggtacatcagttattacttggaactgttctaatcaattttatgattttgatagagtaaacggcaggtatacagatgatgcatctcatagaggtcttgaagttgttaatggaactcttcagccatcaaatggggctaaacgtcctgagtaccaagaagactatggattcttccactctaataaaagtacaactattctagctaaataccaagttaaagaagaacgatataaattacagtctaagaaaaagttatttggtctgtctagaagctacagccttaaaaaatactatgagactgtaactaaagaagttgacctagactttaacttagcagctaaatttatacctgtagtatatggtgttcagaaaattcctggtatacctatttttgcagatacggaactaaataaccctaatatagtatacgtagtatatgcttttgcagaaggtgagatagatggatttctagatttctatatcggagatagccctatgatatgttttgatgaaacagactccgatactagaacttgttttggacgtaaaaagatagtcggtgatacaatgcaccgtctagctgctggtacaagtacatctcaaccttctgttcatggacaagaatataagtataacgatggtaatggggatataagaatctggacctttcatggaaaaccagaccagactgctgcacaagtacttgtagacattgctaagaaaaaaggattttatctacagaatcagaacggcaacggaccggaatactgggattctcgttataagttattggatacagcttatgctatagttagatttactattaatgagaatagaactgaaattcctgaaattagcgcagaagtgcagggtaagaaagttaaagtatacaactctgatggtactataaaagcagataagactagcttaaatggtatctggcaacttatggattacctgacttcagatcgttatggtgctgatattactttagatcagttcccgctacaaaaagtaatatcagaggcaaaaatacttgatataattgacgagtcctaccagactagttggcagccctactggcgttacgttgggtggaatgaccccctatctgagaatcgtcaaatagttcaactaaatactatactggatacttctgaatcagtttttaaaaacgttcaaggtatattagaatcctttggtggagctataaataacctatcaggtgagtatagaataacagtagaaaaatattctacgaatcctctgagaataaattttctagatacttatggagatttagacttatctgatactactggtagaaataagtttaactcagtacaggcatccttagtagaccctgcactaagctggaaaacaaactctattacgttctataactcgaagtttaaagagcaggataaaggtcttgacaagaaacttcagttatcttttgctaatattactaattactacactgctaggagttacgcagatagggaacttaagaaatctagatactcccgtactttaagtttttccgtaccctataaatttataggtatagagcctaacgatcctattgctttcacatatgaacgttacggctggaaggacaaattcttcctggttgacgaagtagaaaatactcgtgatggtaaaattaatctagtcctccaagagtatggagaagatgtatttattaattccgaacaggtagataatagtggtaatgatattcctgatattagtaataacgttctaccgcctagagactttaagtacacccctactccaggtggcgtagttggtgctataggtaagaatggtgagctatcctggcttcctagtcttacaaataacgtagtatactattctattgcacattctggacatgttaatccctacatagttcaacaactggaaaataatcctaatgagagaatgattcaggagattataggggagcc

SEQ ID NO: 3 - DNA, 32767 bp, SP15m phage
  source 1..32767: mol_type = genomic DNA
ggtgcagtgggtcgggcgaaaatacttagtctgctaaccgccacccccgttacaattaccatgctaattgtttcaccctgcaaccattttaattgcagggtgaaacaatttcaactttaattattacgcaacttttaatttctcaatatattgttgcgggctgcaactatattctgcgcgttcttcttcggtcatactttcccaacataattgcaggcggtcggctaggaattgataatcattatcatcgtcgagcgattcatcaataaaggtttcacctatcaatgtaacaccgattgatagaatatcgttaatagcttgcgcgtccagcgttttaaatccgtatgatgccgccgctgatagcacgcctttatgatcatcaatcatcgtaaaatcagcgttcggatataactgtttaaataactcaaaataataagatttataaactgcgtctttgctgtggtatatttcgctaactttatcagcttcaaaatatttgtgcagcgtgtcacgggagaacacgcggatattgctgttcccacgccctcgcaatccttgcttgcgtaggaagtaataatctgacttgctcattagtcgagcggtgcaaataatgtttaaagtatttgcgtcattcatgcactggcgcatatatgtaacaaggggcaataaggaatcttgcattattaaatcatgtttgcaggcttcatttttatacttatttaaatctaaattgccctcgctatcaaagcaaggcgctacacgatgaaacgaattaatgatagtgccgtctaaatcccaaatcataacgcgggaaatatgcgggaaattacgggtaatattcattttaacttgattcattttgttacgttctccatttaagggattagattaattcaatctagcccactaattatattttgttagtgggctatgtttaattaactattagaatgctagaccgaaagcgagagcgtcggcaataaagctaacatcttcacctgatacataggaacgaatccccgcacaagtatatacttttgcgctgatcaattgatcatcgaggcaagcggggcaaggcgcgacaactgcaaaggctaggccggattttacagcgtcgatgataatcgtttcttgtttcaccgtatcaatataaacgcctgcggccttaatgtaactacttgcgcagccttgcgtataggcaaaggtagtaacctgcaaggcgtcgttaaattcgattaaatcatcgacaacgtgccccgcctcgacgtgataacgctcaccattagaataaaccagaacaattgaggattgagcgcgatcgaatggaatattttgctttttcatatttatataactccaattagtttaataaggggtttaatttatttgataataatctgcatttgatacggcgttaattcaccgtttacgggtaaattattatcgcttagccactcataaaaagcaccatcatcatcaaaagggacaatatcgttatcacgggaatcgacggaaataataccatccgtattagttttggcggctaggataggcccgaagctgtaaactttatcagattccatttcatccggtgaaatgaatactttttcgtccaatgttttgggtaatgtaactttcattctaatttagctcctgtaatagcggctatatttcaagccgctagggtaataatttaattatgcaaagaatttaccgttcttaaagtcgatcaaagtacgctgaccgtttgcataggtaattaaatgcgtttgtgtccagcttgacgcgccaacgttgtaacccatatccagactaccagctacgccagcggtatataccccgccgtaaatgctggcggtatgagtgtgccccgtgttcagtttacccaatttcttaaactgtttcggattgccacggctgccgtttatgccattgtgaccgtgtacgccgcattcaatgcctgcaattttaaatgattggtcagtcgttaggaaaatggcgttaaactcgcaacctgcaaccttacgcagcgcataatctagcacgttgaaagtatcgtctttttctgcaatagctccataaatcgcggcattaaggcggtgatatagttccgcgtttgctgggtcgtctttaatgttagcattacgatcatcaagccaacgggataacgccagatcatggttagattcaacaatgattgtttgcgagaaatcgcgctccattgattccagtacgcgccccgtatcgatgagatcatccagaactttatcacgtccggaggcatactgttttgctaggaatacacccgaagcgcggttgtgatggttgcgtgatgtaaagtcgtgaacgtcatggataaactgatattttggtttaagaatatcaagcaagctattttcgccagcccatgacgcagcggcgcattcttcatctaatttttcagcgtggatgtcgccatattgtaaacctaaaacgtgccccgttgtttcatagcatccggcaggagtagcgcaaacattcagatcataaaacacgccgctttcgtccattgtttcaagctggcgaacaaaaaattccccgtcctcatcgaactcaacaatcagcgcaccgaaattatgcagcgcctcggccttttgtcctgctttctgctgaatgtaatttttgagcgttgccgttccggttgaatacatgcggcgcacaatttcaccttttaaagctggcacgctttcggcggtgattttagccgctccaattgccagaccttccagattaagcgcggttgcagtttcagcgaatccagaaagcggataatctgcggttggcaaaacattaatttcagccatgaaagcaaaacggcggttatttaaaaacacgtttttattgcagatatatttatcaaaagcggaatcatatttgattccgtctgcgccctcgccattttgaaaaccgtttttgttatagatatattttgaaacgagcaaatcagcgccgatatatttagcaaattgctccagtgaggctaaaaagtttttatgcgggaaagtattattctgaatcgatgtaataataaagcgtttgccttgttttacttcccagctttccaccgtgctagaaacaatccccgccgcttctgggcgctcatcgtttttaatggcttttgctactttcgccgctttcggtttagctggtttatttgcttccaaccagtcgcagatagcggtcgagtgttttgttgtatcgtagaccgcttttgatatatcgtcgcagacctccagtttagtagcgcgcagacgtttaccatagaaattaaagtcagcggccattttcaggataacggtttgtttttctgcggaaataatcatagtataaaactccattaaagggactaggttaataacggcaatattgccaaatataacgccgcaaatgagtggcgttataatttgcaacattaatttaaaggtataaggctagaactaacaccacaagcaacggcggcaataaaacaaatcagacctaaacgctttgccaatttagacttacgtttaaaataatatgaatctaaatcattttgaaaataagcgaatagtaacgaggccgccataataaataagcctagaatgagggattcagtagggtaaaagatcattttaataactccagtcaaagggaaattatagtggggaatattccccactaattaaatttattcgcctgcggcttgtttcacttcatcggcaacgcctaacagttgcgccacggcgtccagcgtttccagttttgcgctttccagtgatgccagatcgtcggcgtctttgataatgccggaatcgatggcgtgttttgcaattacgcgcacataatgcgctttgcggattgagctaccgccgccaactttgcgcggcttatcgcttttctgatacgctttcgcgctggtcaattttgagcgaacggacacgggagaagccgcgcccactgctttcgcgatctctttcaggccgtcgctatttgcgaaatctaaaccgttttcattaattaactgctggtacatggtaacagctttttgggtgttttcttcattccatgcaaattttgcggatttttcggttttaacgttagccatgattgtagctcctattagtttaatttaagggataagattaacataatgttaatcgttatataccccgaactactggggtatataaagttaacactaaattataaaacagcttcccatttttcgttacgctggacaacctttacaacgtcgccggatttaacgcgaacgctaaaaacggttttgccgttgttactacgttccgtttcagcgtataccgcgtcgattgtatcaaatggcataagcgccgcgcctttaatgcgttcggcctttccggttaattcatccgttttagtaacgaaaggaataaaaacggattgaccaattttaggcgtggtaataatgttttgcatagtataaactccaagttatttaggggattgttccgcattacctgctagaaagtagcaggtaataagcaacaatccgctcgccaatataatcaatttaaagaactccacgcaggccgctatatcccagttagggggcggggcacattatggtaagtgccgaccgtcaaattttatcaaattatcgctcttatcgaactgggtacatcttaaagcctatcggctagggtgtcaaactattttttgcagttttttatggttttccttcaggtcgatcataatattacgccagatcatttccagaccttgctggcggcctttcttgtactgcgtgaatcggtattttaccgatctttgcgctactgtcaacaaattttttgttttgctatctagtgccttgctaggcttgccagtgatcaataaagtttgtttcatatcgtcgattccttataatgtataagtttaccgccgataggctttaagatgtacccaatttttaaagagcgcggcggtaacttcccgccgtgtagttcgtcattgccgtcctacgtgataaataataggggattcccgaaaatggcgcaaccttatttttgtaaagaaacgtaaagacacgattcaccgcacgccgtccggcggcatgggcgcggcgcactaaaattaaaagaaacgggcgcgcgagtaccacaaaacagagcaaataggcaagtaattttttcatttatatttgctttgccctacttgacaaaacttaaaaagctcgtggtagcgataaacgagggtaggcaatgcaatggcacggctaaaactttcatcgcgttctagggcgttttaggcgcattctagccttgttgataacttatccccaaaagcaaaaatgaaattttcctagttatccacttgacttttattttccagtggataactacttattttatgaaataaattaattgacttttatttgttagtatgcatcggaagaatagcagactaataattactagaataataatcatgctggtggattgtaacggcctaaactatcagcagactattaatcacgaaaaatctcgttagctaactaactatttcatgatgtataatatacatataaattaatgagaaataataattataataaataataactacagtaaataataactataagaaactatcggcctaagtgagaaccactatcatttaagttatccacaacgttatccacagcacaaaataatttgacacgataggcggcgatataagggcttatccacagacttatccacaggttatcctactgtataaatatacagggtagaaaggtagtgttaacaactgcaatcaattttaagcggcctaaaacgctttctaacgagctaaatgcggtggggtaatattaaagtaaagccttcacccgtcgccctggtggcttcgccgtgttttgctctttattgcaccgctgcgcggttagcataaaactaggcgctaggcaaggaaaataaaaaggtaaaataatatttgcctatgttagaaaattacctttatcattcactcaccgattaacgagggaggccgaacaaatgaggctatataaaccagataacgcaaccgtcttaaaaggtgcgctgcgtaacctgctggacggtagcagaacaaccagcatcaaacattttgttttcaatattgaaactattcatcaaaacttttttggtgattatgatgcttataatatggatagttttctaccgttatataaacaaggggcaacgcttgttttatataatcaggaatctcacttgcttactagtcgagggccagatactgattttattttagtaaaaggcaacacagtaaaagcctatgatgcgggggcgggcttagaagttttcacaatagaaaactatgaggctaatgataatgatctttatgatgtagaaaattttctcgattcattttggcgttatttatcagttggatggaatcgatcagattatgacgggtatcgttttgcggctgtaatggcttttgatgataacggtaattttttattaccatcggaattatacccgtatgtgcataatgagctagtacaagaagcgggttttattttctggaaagatgaagatcagattattgacagcgtagaaaaccatgctgtaaattctaacactcaaagcgttaaaactcaaactactgaaaacaaaggaaaaaacaccatgaccaagatcgctaatattgttgccgctaataaatccgctgttgtaaacgctgcaaaactggaagcgggtaaaattgcactgactcaaattacgaaagtagcggctaaaaaagcaccgtttatgattaaaggttatattgatacacctatcggtcgagtagtgattgccaacctgctgagcgtagcggttgaccagtacgccccaagtaaccaaaaggcgaaagcggtggcaggtgcagctatggaagcggctatgttagaaatggtgcaaagttttaacatcgctgagatgattgatgaaatggtaaaaggtattgatatttctacttttaccactagcaccgaaagcgagtaataatattaagcggggattgttaccccgctttactattcccttgttaactaataggaggctaataaatggcggatgaaaaatatggcttctcactgggagaagtgagcacggcaaaacatgatatgatcattttggtcgattgtcatactggctattgcggggaagggaacaccgaggaatattttgttcctactggtacggatctggacgctttcgctcaggaaatggctattgataatgcctctcgttttggtagcgatggttacgaagacgaagaaactggcgaatggtatgataatgaaaacgtatatgcaagcctttatcattatcaattaagtaaatccggcacatatgtaaacggcggcgatcctattaattccgtcatgagattaattattaaatatggcggcgtcgagataattgacaacaaagcggtaatatatgcaaaccgattaaaacagcttgtttatattcctgatagtacccgatgggatgaatatgctgttttgcatgacgaattgaaacgatgtttcaatattgaatccttacaagtagtctaatgtaaagttttgtaaaggtcgccttttatggtggccttttttgttataatgcctttacaccgtttgaggacggttgaaaattttcccaaaaattggaggcttaaaatggttgcttactcttctgctagtcatctgttcaccgctcaaggctgggtatctaaccgcgttattattcacgaaatggtgcaagaatatggcattgctaaaacttacactaccattcaggcgctttatgataatgatcaaatcgatcagcaaacggctggctttttgctggataccctgaaagcagaacattgcaccaaaaaacaagcggctaaaattgttttaatgtaattaataacgggggatattatatcccccgctaactaggaggatgaaaatggttatttttcgagctattctggcgggtatcttgggcgctattttatctttatttgcaatagctttcgacgttcacgcggttattatcggcgcgggtatcgctgtattttcttatctgctgggctgcatgactagtaaaggagaataaaaatgatccgcaacgtttcccttgcacgttcgaaaggctttaagctggtggacgttaacacgttcgagcgtgaagattgtaaaatcgaatatgtagcacgtaataagaatgcctttcgtgttaccgagaaaaaattcgataagcgcggcaacgtgatcgctgaaacggttaaacactttgccaccttttacgctgcgtttcggggagtgttataaaatggtaatttatgaaggtaatcgttttgttgctaattgccgtccggcattattagcaaactatttaaaccagctttcaccagcttataagggcgttattaatatttatgagggcacggcgcattataaaatcaatgcggtcgttgcccgtgaactagcgtttcaatttttgacctttgcatcttgtgacgttcaggttatgggtgaagcgttaattgcagaaaatgaagatgattttattaatattttccgcaagatatgcaccgagcgcctgataatgaaaggcgcgtatattcaatccactgcggatagtattgaaacagcgtttcgaaaggtggcgcaatgagattatatattttcgcgggtaatgttgaggctgcaaatgattccgctggtggcgataacgttcgtcactactggcaaaaatatatttactaggggttattatgagcaataaaattattgtgaccaaaactaccacaacggttgacgttttttatgtgcctgatacgccggaaaaccggcaagcggtcgagcggggcgaatatgatagcgttatttatgatcacgatggttactaccaacatttggtggattcctacggggaggaggaaaaaatcacgcatcaattaccggactgacaacaagcggggatctgctccccgtttttcacgcctccagttaaatacctctttgttttagtatccccaccaaaattaaacgcgtcagaatgcgatctaggacgttttagcggtatattagaattattcactacataggaatactgtatatttatacagtaggataagctgtggataagtctgttaataacgcttcaaaatggctaggattctgtcaagtcaaatcgtgctgttaataagtctgtggataacttaaataacagtgtttctcacttccattcttaaatgagaatcattatcattcgcattccactgtctaaccgataatcatttcactttttgaatagttctcatttcacttcttaaatgagaatcattatcattcgcattccacttcttaaatgataatgattctcattcaaagtcgcagggcaattgccctgcgcttttgtgcaaatccgacatttgcccccatggattacgcgtgggcatgtatgtgcaaatccgacaatttttggtagtgtgcaaatccgacccgaaaaatttttatagtgtgcaaatccgacaatgaattttcccaaaaactccagcaatcacgaactgcgttcgaatcctgtggaattagctagaatatgtgcaaatccgacatgtgttgaggtgtgcgaatccgacaagatttttatgacttcgatgagaaggtgtgtgattgtataggtttgaggaaaagatgagagagcgagagaaattttggggctagaaggatgtgggcgcaggattggtgcggagcacctgatttgcaggtattttgggggagagttgagataatttgggaagatttgagataggtgcagaaaaagtaaaattttattagctaaatggggcaaaatagcttgacaagtgaaaattcttgtggctctaaaaactcaggcaatcacgggccttcggcccgaaataatgctgctattttcaggagagtaagagttcctaaaaacttaggcgtttgtgcaaatccgaccataaatttctagaaacacaatgtgcaaatccgacagtaaaatccagaaatgtgttttcaaaaaatgtctcctagaaataaccgccctccctataaccgccctatattaaccgcctattgctagagtttctaggaacaatgaaaaccgcctgagttgactagagttttcctagaaacttaggagtctagaagaaagtgttgtgccatcctagtagatgagcggcaacaggtgtatcatcttgaacacagatattgcctttaaaaatatttaaataatataaagaaaaagagacccccaatttcatgagaatctctcctgggggcgcgtgattaattacgtgagtactcatgccgtcataccgctgttgctaggccgcaagctatacgagacattcgtgtaataatcatcgcccctagagttaatcaactagagtagttgttaatctatgagattattataacatgtttgggtatgagaatgcaagaactttttgttaacttttattcctccttcttggatttgagtttgatgcctaaggatgcgaagtagatataagttgctaaataggaagcagtggatcctgtatcatcgtaatccatagttccacgagctgctctagtatattcaggagcatagtttaatatcgtgtaacttggcattcctagcgacttacatagttctttaaatgtatcttcgtatttatggcacatgaaatgcacagcattttctaatggcgttaactctagatctttatggagagctacagtcaaactcgctagcattgtgccaatcccacgataaacttcatctttaactagagttggtttctctttttctagtggaggaaggtgggcatatttcccatgtttgaaagggataagatcttcgctagctaatgcttctttaaatgatgcttccttaaatcttgggagatcttcatcgattaggatatgaatagcattagaggagaaaccttttgcttcaggatctaaagctttcaacgctttattcacttctacatatgagcctgaccaaactacttgttttgcatctcgatcatacttgatcttacctttatcccacctagcaggataatgatctcctaaaaacattactgcatatttttcttcctcagttagctgggaaagactcttttgtgtagcaccacgcgctaactgaatgagacgttttaatttttcagcttctttaatcatatatcagacgcttgctcccctgtttctttcttttctgtcttaggttttcttgcaacttctccaaaggttcctttggttctttctttagctggaagatctactttataccataggattcctaattgttgcgctaaatgggctatattctttggtgttatacttggaacatcttccctatcagaaactttagaaattatatcaagtaactctcctatttttggcttactagtagttattagaatatattctaatgtttctatttctacattttcatctttatagtaaagactaagagtaattaaatcgtcaccagcagaagttatttttgttttaccaaatatcattaactacctctcttatcttcattaagagcagctcccaacgcttcaaggatagtatcatttatactcccaggcctaagattattaaagtgagtaacatagatgggacttctaaaaccctcagcatccgcaggtgctacgcttcgcatatcagattcaaaagcttcttgagtatgttgcaactgtacagaagggccgtaatcttcaccaactcgatatgaggaattattttctataacgccaccacatggaacattgtgcaaatccgacgttattttaggattaaatgcgataccacttttggtccaggaacctccaacagtcacaggagtactagggcggttcacctcagtctttacgagtttataaccagcatctattaatgcgttaataaggttatcagctggaatccgagccttgccaaagatcttacgagcttcttttaatttatgctcaagatctttacaggctttaatatcagtgtgcgcaaaggttaatttcatagatttgaactgtacagtggcagttaagtctttaaaatcataatcccatgtatttaattcatggtctggtactacttgaacaggttgttgtgcatataaagtcattacttattctccaatttgtctagtagcttgtgcgctgctatgttatattgtttaagttcacgattaaggatttggttttcacactttagctctagattcttattattaagaatattgcagatcagtagaagtgctaatataactagcaaggaacctacgagcattaaaagaaaaagagtttccattatttaactcccatgtaacgtttgagatatatgatgaagtcttctgctgtatgctctacgctaccttgagctacaaatagtttgagggcttcacgttgtagtttaagagcagccaactcaccacgtaattttattagatcttctgctagttctttagctctgcgcataatagcaaatgatacaaatgttacaataaataacataactgctaaaataattactatgatctccatattaacatccagctcttatcatatatttgggcatgttctactaattcatttatcgatgtagaattatcgtagataccctctagtaaacgttttctgtcaaatttatcaaccaaatactctgtgccatttatcactaccctatacagctctggaactaaggggtgtttgtttggtattgggcgactacctaagtctatttcattatatccccacgttgttttaaatagtttgttgctaagtgctgctagtgggtttgaccatacaatatagctactcactacttatctccattcttagctttgaaaacttattataccaaattatatgattatcgtcaattacaaatttatggtaacatgctggtacggtataagttccataatccgtgacacgctgcacaaccttgtgtgcacacagtcgacaaccatgcccttctaaatgagatctagcagtttgccagtaataaccatcgtgatctggacaatagatctcgacttgctgttgcattgtcttataatttacacgctcatatccgaagaaagccccgtgagctgcaacggctttcttgataaatataaggtttagtgcttcttgctggaagtcgggatgtagctgcttaatcttagttctattaatagatccatccgatttaatgaacctatttattggaaagttgttagcttcctcgattaataattcatttactttctctctcatattaaatagtctcacagttaaggtagaaacattcgtaagcatctccagtaaactctttatcttgtagtaaacacttagcttggtcttccggtactccagcatctaataattgttgtttacttggcttttcagcgaatacttttacaaaatactcaccatcctgattatactcatttatatctctggtaaggacatatacttgcatttgaagttccttgaaaacataaaaggccagaacaattaagtcctggcctctagaattaatgaagttgtttaccacttcgtaacatagtggctgtttccataagacctagcgtagcatcacgcttattgatctgtttaccaagttcatcggtacgtttaccaatgtaagcgttaatagccatattcatagctgtagcgagatcttctttggttatctcttcatcgtctaaggctaatttagccaaagaatcaaatgtgctagagagtcctataagatctgaggtttctccagccagaataggattaatattatctactgttacttctagcatggagttaacaatatcttcaccatctattagaccagattcaatattactctcccactccttcatctgctccaataatggatttttcttttctgtcatggtagaggtttcctgtgtcagtcggtaagaaggatgattgagctttaggcggatgttgtttagcaatccagctaagaatcagtacacgactaggaacaatatcagtgttgtaccagaaatcatgaacccattgacgagcattctcaaacttaccaaatttatatgctttcttaaacaattcaaacccaaaacaatctggtgtaaagtctacttcacgatattgaactactttagaaccagttaggtcttggatcgctgcattaatttctgtatgcgagaattttgtttcgtgaaacttattaaagaatcggtagttgaagcgtccgttcgtttcgacaaacaactggatgaaaagatcgttaaattggttatcaaaccagtaattctgtagttgttgtagtgctgtcatttacgaactccgttaattgccacgatgatgccttcatacataaaaggaagtagttcagaagtgtagaagatattttccgttattcctagatgtcgaaaaagtatattaaataatgctgttagaaatacaatctggggcagtaatacaaaatactcagttacaatctttggtgcccgataaacaagacgttttatcattgtttttaagtctccttattactttggcctgctccacaataatgaaaactgcgagcactaatagtgctattagccccgcagtaattggtactaaatcaatcatgggagacgccatacgtaattagctgtctgtagaaccttaggtgtgtcatcatgatacattactacagactttggtgaatagctatcagctagctctttacgaatcatcttacattcttcaccagtatcgatatttttaactatcactttcatattaagaggtgttaatacagaaagcggtttccagaagtcctcaatctcaattcctacctttttctcgattaccatgaggacttctagtgtatcatctggaatactaatattattattcacaaactgtaatatctcatgtaaggtatttaattcattaaaattaagcttcatctttaagaatatcctcaaccatatcacaggactgttgcaattcgtcagcaatgcgcttaatatcggtcttcgtcactctaccgattaacatcaccagtaacatagaaagtataataagtgggactggaataacaaataaagctaccttaacaacattctttggcgtccatgtgtggtacttggtaaccagtacaccaaccacaattagataaaacgctagaataaacatcatcattttttaatctccgtaattatctgtgcacgcattactttattaggtaattttgtattcccagctattgcttcaatattatttagtttttcttttagaatatctgagcgtctctgtgctagttcaatatcttgttcttgttctattaagcggcagtgaagtccactattagtagtaagcatactctctatattttttcgcatgcttacaataccaataatcccgccaatcgctactagtgtagtaagaactagtaacccaataagaatttcaatcaacattaattatatactcccttagtccttatttcttacctttcagttgcttaacttcacgctcaaaagatgctgcacgacgttcggcagtcgcttgatgctctttagcaaaacgagcttcctgttttgcaaggttgaacgccatagcattcttattcagagaatcatacatctttttcatcgccggaatagacatcttcatgagctgaccctcaaaaccctgcatgtcgaggagaattgccagaacgttagccatttcgtttttagtcatgttttccattagaatttcctctctcattaacttatgaacttattatacagaattttaaggcttaaagcaactgaattttttaattacttaccaatcgttaacaacgccggagaactcagaagcaaaaactttttcaaatttctctgcaatttcaggatgatctttgcagatcagctcaatacatgcttctggagtcattccttcatcttcaggatcaccatagtatttatcccaaagatcatcgggaatgatatgctccgccaaatcttggaaagagactaactgataacgttctgcctcctcagcgataagaatttcgcatagatctttatctatatcgctacgataatccgcaattaataaggcattgcaagcatgacactcccaaaccatcaagcgttcagaaataggattagacttatcctgtacgtaagactgaaacagggttcggaaagttgccttaacttgttcaaacttatctgctgctgcgaaaactagagctttatcaactttgttcattttgattccttctcatcaatttatacagtaattatacagaaacttaagcattttagcaaataaaacttttaattaaaatgcctaatcctgtgccaatagcaatacaaatgattataagtattgctatcgcctgtatgattcgtttaataataacctcagctatatacttagacatttatatcgccacgcaatacagcagctacgtcttctcctatttgtaatacctcgccggtagtacaattaaccactctatcgtaactagtaaacttaccagacacaatatcctctagtggaattggagttctactcatttcaaatgagacattaatataacgtgggtcacgtaaagaagtagtatgtacatgtccgtgaatatttagtttgccacgaagttcattgggatgcaaagggcagtgagatagccaaaactttttgccacctccagtctgtttgcctagagcttgaatatcgtcataaacttccgctaagtccctaatactcagtccttgacgctccgcatcatgattacccataatgagttgattagggacattgtggataaccgactttaatttggccagaccttcacgacctactgcaatatctcctagcaaaataagttttgttcgtttaccaatatgcttggacaaagtatctagaatatactcgtcgtgctctttcatgttcttaaaccacggacggaaacgtaacgctccagggtggtctagatgcaagtctgaccagaatttaactttcattactcttttccttattctgtattaaactatcaacccaagaggttaacactttggttttaaactcctcgggagtctctccttccttaaggtctacctcattaaggtaggtagtaagccttgtttctatatctatttcagtaggagaattaaaacaaaaattgactgctattccagaatatattactccggtatctcctttgacgaaagcattaactaatgccctccaacgaagggcatcaatacgcattgctcgtaattcttctcgtacttctttcattctatcattcattaaagagtcctctgtacaccgcagctattatttttgtctgtggtaaatgtggtgattttgccagtttcatcattaacttgcgcaaccgtcaactgcccgttgaagacaccgccagtatctaggtaaacacggtttttatagagaagcgggtaaggtactccagtatgcccatggaacacaaagtctactccactaactggaggtacttctaccatgtatttttctttaaatcctgcataacgctggaaatacgagtgttcctcgccatttttagacaaatggaagcctatttcttggattacatctcgatcccataagtatggttcaacatggtatccaggatggtcatgcgggtcttccttagctgcttctacttgtgcaataaggttatcccatactggggtttctacttcgttaccacattctttgtacgtaaaaggtacaccaccatgaacaacaccatacttcttaccacgatgtctaacagttaggaatactggcattttttcagccatgtcttcggcaatatttttaatggtatctgcatctagctcattcatagcccacataccaccgttatacatccaattagcccaatctcccacaatcataaactggtcgtggtttccacgaacgctacaaaaacgtggattatataagaatttagctaaaacttgtaggttctgcgtgcctcgatcaattaaatcccccacgcatataacgcaatctttcttgccgttatagccagctaattgtagggcatcttctagcaaatcattgcatccatgaatatcgccaacaaagaataagttaacatcatcaggtactactagtgttttatgcacattaaattcttttttcataattattcccaaataacatttaaaatagttgtgccatattcattagatagttggagagtataaccctctttattgagggcttttatagcttcataactaatttcgtcacggttaaactgcacataagaacctccaatctctacagaagatactatcctccgcttaacccatctatatgttttctttcggctcttaagggacgcggctctatttatcctagctaaacgttttgcttgctctgctaacatttaatcctcctatcaatctatacaaatattataccaaaatttttagcaaaaagcaagtaaaataaaagcctgatccgctaagatcaggcttggtttattaatcctctggattatcatccaggaaatttttaatagcttcgtgcatagtttctttacgaagctgacgtccaatcaaaatatgattagcttctattcgaccattaggtaagcgatctgccagaactactacaggtacttgacgtacaccaaatttctgcattaattctgtattatcagtctctttatggatttccaaattatagtcattgactactttatcaaatactggttcgaaaagtttacatgggttacaggtggaaccttttaatagatagactaatttagacatttttatttcctttgctggcaaactcaccgtggagttcttctagtttttcatctctccatgcaattgcttcttccaaagaactgcacgttttcatataattgattcctgctctagagatttttactctaaaagacttccctctttgagatatattttttaatcccaataggttatttttattagccgatttcctattaaaagcattttgagcttttgtagcttctcttaagttaccaatacgattgtttagcgtattggtatcatcatgatctactatatcaggtaaatagcctttgtgcataaagaagattgctctatgcgcaagtattcgttctccatcaatagagagcattagatagccatcagcattaatagacccagcaggcatattgttaaggctagtattccaacctcttgtaccttccggtctaggtttccaggttagagtaccatcttcgtggtactctaatacctctaataatctctccctagtaatcacaatttattaatggcctctaagaagtttttcatagtttttacggttgcggtgctcagatcaagatttacacccaaacactcggttaatgcttcctgataaggagcctttaatctgccttctgggacttctaccttcttatactctttatttttgacctttttaatcatagtctctagtacaagaagcggtaatttagcaccttcaatatcagtacccaaaagttcagttaaaattttattaagatcaagacgagttaactttttgcccttagacatagatgcacctacctttgtatcaatagatttttccgctttcttttcgagctttttgtactcaggagagtcatgatcacggagtgcaatgtttagctcgtaatgtggtatacgaaaatgttccgccatttgagtgtagaaacgatcagacataatatatacctctcttaactaatttatgtatatattatataataactagggctaaaagtcaactacttttttatcttaatctactgcatgtataaatcttttcctaactagatacatagttattgggtaaattgagtacataagtatcggggagaaaagggtgaaatacgctgtaactcccccagctaacatcaaaggtattaatgctagagtaagggccataagaatcataccgaatgaaacagccagagctatggatataggattctctagttccatccataaccaacaatatttcgtatctctatggcaattgcatttacaaacgccgaatgaacccataattatatactctagtccgtgaataacctttattaataagctatttcgggtagttaatgcaatgatagtaaagactatcattaaaacgaatactactagacttattttccagatacctagcagcatcatagtgaatagttctgcaaacatggctttctcctatcttcaaaaattattaaagccccctttgcctaaaaaggcgggaatattcccgcctaagttattaattaaactagttcgacatgaccgccatcataggtaccacgttttatttcatcgtgatagtctcccgaagcattccaatcagcaccaaaacgaagtttaatgcctagctctttaccagcttgttcaaaagcctttttaactgcccaaaatgcttctaagtcattccaatcaattttgccattaatatatggagcaaaatcaatagcatccccagtaatatgtttgcttttactaggatcttttagaaatgaagtaccattagcaatgttctgggcactttgtgctactgtacgaataccttgcacgattgtgaaatcatacggagatagttctaaagccctacgagctactttttgtagctcgggcttaacggtagctaattgtttttcactatttttaccaaatttaaaactcatattgatctacctaaagatctctgttgtggggaacagagctttgctaaatattccttgaactgttcagaatcagctgtatctaccggattatctttccaagcaataccaatgtacccagcatagatattttttagattgaagtatggacaagtgtatatgtaattaaaagtaacgtttttaaacgcaggtatatttaaccccatatatttatttactcttacacttaaatccgatgcgtagttaaagccctctaaatgacgtctgtataattcagacgttttatttaccgctttatcggccaagtcagccctatctaattgcgcattactttcccatgcaataatattggaataatcattgatagcatctggtttatacttgactacaaaaacagcatctgcacccgtttgagagaagagaaccatgctcttttccctcgccacattagggaagttatctatcctctgggtttgtaaatcttgtaaaactgcagacgtggaaaaagtctttaagaatgacatcacttcactagtattactaacaaataagaaaataatgacagcaactaagatagttagcagacgtttaagaagcgatgctggatctttcgcttcttggagcagtaccgttaataattgtaagaacttttccaattgtaacctcctctaaccagtaccattatactaattttggaggaaaattacaatgtgtttttaaagatcacttctggagcataaaattttgtcgttgtcaagaagaattttagataaaagaaaagccagggtcgttaaaccctggcttaaaattacttactcttcgttatgctcctcggattgaggtaactgggctttattatattgctcagatcgatattttgccaagatttcaatacgcttatggatttctttgctatctagatagatatttttgttgtcttttaccatctcgtcgatttcgtctatagagaagaacggatagtagacatctagcatcatatcttctacgaacttgttgtaagattcataggctttcttgatttcttgacccttctcacagaatccgccagagaacgtgtgtcccattagcgtagcatgtggatgtactacccatccatgacaggataggaaaattgtgcagtaagcagaagcactaggaccaatcaggtgtcctataactgttccacggcaattagcaattaagttagataactgtgcagcagtatcaacataaccaccagggccattaatcatcagattaatttcgtcgtcctcatttgcttgcataagtaccattgataaatcacggtattcatccggcgggcctaattcttcatcaaagaaaaaggtatactcattagactggcgaatggagtgaaacaggttagtcttttcttcttttttattagtcatagcgatccttgattatccaactagtggttctagctctaagtcacagaagttataaacttctagtttaaggttattgataccatcgaatttattaactaattcgtgagtaatatattttgcaggaataccactttcagatggatgatctgatttaatagtgaacttctgctcagcgggtactacatttactatcaaagaatccatatctaaatggtttgtttctctgagtaactctccttcattggggaatctaacatctgttattacggcgacatctgggtcgtctttagcgatggattgctccagaattatgagccaaatgcgttcatgtaccagctgccttcctagctctgttcctacgagctgtaacatttttctcggagaaataaataaactataaagtccgtcttctttattctctgagataagttgttgaggattaagatatttttcctcaaaaatcggccaaacgtacgagaagtcttcaaacttattgataccgtatttaaaccatacgtctctagctcgctccaattgagattgtgtgaccgtaaaccattggtcaatctctttccccctgcgctctcctagaaactctggagttacaccgaggattacggatgcaagttcataaacgggcttagcaaaactataacgacggggtaaacacgttggatacgtgtcattacaccaatcgataattaattttgcaacggtatcttttcccgaaccagcttcaccatgtaaaccgactaatactgacattaatctttcctattgttaattggtggataatatactaaacaacgtttttcttgcaaatcttggcggtagaagcaaaccatactagtcagtcgtgagatatatgaatattctgcctcacggcattttgccaacatattccaatctttgtatggtacaacaactactacgccatcttccccatttgtagctaatttcttttcaaacttaaagtcaaagctacaaggctgaagtcctttaggccaatccacatgggcttgctttaactcatgtgacggctctggtactaccgtttctgcacagcctgtgattgtgattgcggctgcgagcagtattccaagtttccagttaaacatgctaatctttcctcgaactccttactctgctttttagcaattaatgtaaccaatccaggctttgcagctataatatcttggcgactaagagctttgtctaactgcttaatctttttgtctagatctgcttgcgaaatattattcattgtgaaatactgattcattctagtctcacgaagttcgctttcagctttcaccttattgagggaagtctctagagaagaaatctttttagtagccaccgcaagatctcctgctaaagtctccactttatctactaagtgataagcaccgaacccgatgcctatcgctagacctgctcccaggatatacatcttgttattccaaactaagtctacaaaccatttccgcattagcctgtactcgcaaactcaccgtggagttctttgagtttggtatcccgccattttatagcctcttccaaactcttaagtgttttcgaaacttgcttaccatgtttggtaattcttacttggtaagtcccatttgtttttctatggatatttttaacgcctaaatggttatcgcttcttactttttggttacaagcattatcagatcttgtagcaggccttagattctcaaatctatcattagttgagtctttgtccttgtgatcaactatttcaggccattctccagtatgccatgcatagattaatctatgtgcccctatagctatggaaccattatatagttcaactactctatgccctgtactttgtctagatcctgctactgttccggcgaatatcttattaaaatgttcgtccccttccctgggtttccagataagattaccatcttcttggtaatcgaacattcttcttagctcttccttactgatcatcttttcatattcctaaaagaagtaacagtatcaaatccatgtgcagctaagcgatccttatcggaaatcgtaatagtatttggttcgccggttcctaacacgccccagatatattgctcgatcatctggtgcaaacggtataagttactttcaatttcctgccacggaatacctgactgatggaaacgaatgttagtctgaatcacgaagttacgaacatcatcgttatcgttcttcttgatacctttcacatatgcaatcggtacacgcagttcggacaagatacgttctgctttaggttttgcttcaacgagcaaatcacgcattgtttcacgaacatctccgcgactcttatccattaagtaagagcgagcatgcaatcccatctcttccattttatcgaacatagtgtcgaggttgaacgttttgaagctaaatgctggatgccagcagtacagctcgtgtaaccagtaaacttcacctgcaacaaatagtgggtttacaaaatattcgaaatcaccacggaaagatagcgaaccatcacgaaatacctgacgactatgcacgatgttcttttctgcatcatcagttactttaaccagtagctcttcagttttacgctcccaaacacgatctgcatcaaataaactgttctgcaaatcatatacatcggcgaatttagaaatgatcctcatatttaatcctcttgcctcaatctataaacatattatacaaaagttgggcatctaagcaactaaaattttattataaaaatagcccagtcgcaaaagtgcaggctgggctttgtcattatttgcttttgctagtaagctgacttagtgtcaatcttatgtaatattagtttctctagctttgcgtagtacccctgcatttctccacaatttgatgtcagcaactgtttctttataaggagctatggtaaaacctagtgggccagcactaaataatcctaagaaccctacaatacgcatgtagaacaagcattctttggctgtcatattatttactgcttttttctgcttttcatctttaaacttctgttcttgatcaccaatacgtagatatttaacaaaccattcagcagaatgttcgtccaaatgtctaataatagctatcgcatatccagcaccgattaaaaaccaagttgcaacaagaattagtaatatagtcatattatctccagttagggctagcagccacctcaccacttaccgcactaaggggcacgactcccttatccgtaacagttgcaggtgacgcaactcggtcctacgcgagttctttaagtattctgcatttcagctttaaattttttcatattacgagtttttctataaaagaaaaacacagatgttgggcctagaagaatatccacaataaatatcacagatctagcacatctgagtaatgttttatcatcaagaggtggcagatctaacggtcgagttttatgtataacgtataatattacatctttattcttagaaatataaagatcatcaaccaagctgtaaatagcaaccacagatccaatgacaaaccaaagagcaaatggagagataatcatttcagatccttttcattaattagaatattagtaaacagtggagtaactcctagactcatagtaggtccaaacgtattcatggctacccatagctgcatagtgatcatcccatctttaatctctggatctttatattcttcgatacgtttcttggtaaaagcaactatatctggattatttttattttcctgaatatagtcatgccaaaactgagtattctcactacgtaggaatgttaaaacatccttagttgctggaatctgcactgtgctgttgatgtttagtcttttcacgttcttctctccgacgtttgcgttcttttatcatatgagctgctacaacttcatggtagtagtcattaatgttatcttctggcaagaaatgcttaatagtctctagctgacaaataactcgatgaagatggttatttggtagacacaattttatacctgcaacaaatccagagaagcctggaacactgaacatgggttgggcttctactctaccttcagagttgatattaagctcaattgagatacccattttcacgctataaagctggcaatattctccgttaccagaccttgaccaaacagtgaagtcctcatcaatttgatcttgaatttctgtaatagcaaatttaattctaggatctaaattattcatcttcaccttcaaagtcgcaatcataacgacaagtaaaagaatcagaactattagtacgttgagtggttatttcaccgcgtttgctaatagtaacggctggagtagagaagtttttattagtatatatttctactttaccattacgttccttaacatcacgcactttaccatactcggtaataatgccgttctgttggactttaacattaccatttttcatagaaactttggtagatgccagagaaccgaaactaactgtggagatcatcagtgcaataataaacttattcatcttcatcctccccactacaatcacgacatacatcataatcgttgaaagaacgttcgtgagcttcacaccaccaagaacaagaatcgcagagaaacatttcggttttctctagtgcttgacctaaaagatcatcagcttcctcagcagtaatcttcaatccgcacacatctgccacacgttctttaattaaacgacctgcttcgtgataagacatacaggttcccacaacatcatgttcaagaacatgaacagcacagtctagacgagttttcatttcaaacctctctcatcaatttataaatatattatagcaagaaaagagaggtttagcaaatgaattatttcagaatttagtcatagcaccaccataatccacgcttacgcatgtcatgatcgcgattataatcataattttctggatctttcatcacgcggtggagttcttgacgattcccttgacgaaccattttattagaatgccacttaacattcttactaatagaattccagttataaccatcctttttctcattacgaatggttgcttccttcatttcctgttctacatcatcccaggatttagcataaataacacgaatccagtagccattttctttgatgaaagaatattcttgagagaattgttctttagacttccaccactgatcaccagattgtttacgataagtacggctcatattacctccattaagtcttttaaattaacctaatgtggatgaattttgttatacatatattatgtacctttatacagaaaaaccccagactacttattcaatagctggggtttgttattaattacagatcggggcgttcatcttcgaaacagcctgagctaattccttctccgaatcctacaaagccatcaaattcatcatttgagatgcccataatcattgcttccattttcctaatctccgaaattttcatgcctgctttactattcttataatatttgcgagggttcccgcacatccaacaagaacagatgcaaggagtagtagtgataatacctaaccgcttagggctttcttcatgtgggaagactgtccaatacttcttgcggttgttcttcacacgttgccggtgatggcgtcttaatgctcgatccacacatttctcctaaaacttgggagataaacggagtttgctcgactaccttgcgtagctgggagaaatcatatccaaaccccattacatcgcctgagtaaatgtacgactaataacgtcgttctgttgttcacgagtcagtgcattaaatcgaacagcgtagccagagacacggatggtcaactgaggatatttttcaggatgtttctgcgcatccaaaagctgatcacggcttaacacattgacatttaggtgctgaccaccttcgatttgaggggcgacttccaccttaacttcacggaaggcttcgggatcgaattgtggtgtgataccttctagatcttcaactagaactttctgtttaagttcaccattgtcggagtatagctgaataatctgattttcatgaacaaggttaattacgccagacttaagattttgatatgctttcattagatctccctgatgttagaatttggctcagctctttattgtctatagtttaccacgatatacagaaactgtcttaccagtttggttcataacgtatgctacttcatcttcttttaagaagattgcttgatctattccagaaatagctatgcttttatttctgggattaaaccctacgcttttaccaacatgaatctgctcaccaccatcagtggacattattttaactgttaacataattgctcctatatttagctatctctagctcttttaatggtagttagtagtggatttgaaccactgtagtcgctccgtatgaaggaggtgcataaccactctgccaactaactgttatgttttactagactaagtaagtattctttatactctttagaccaattagcttttttaaactttcctggacgcatagtcttaattcctagatttggtactccgggagggatttaaacccccgatctctcggttatcagccgagtgctttagatcgctaagctaccgaagtattagaatatttacatcatacactgtctaagtaagaagtataatggaatttagcttctccagtcttatctacttctacctcagttcgtggtacttgacgaaccacaccatgaatcatcttatagcgaatgcctttagctggttcatgatcttttgggaatacttgtttaaccgttactactttatatccttcacgcggtgttaacactactacttgatcaccttctttgattttccaagaagatggaaattcataggtatatctttgaccaccagtttggaatactacagaaagataacgtttcatttggtttccctctcattaatttatatagatattataacaagaaataagagagaaggcaaatgaatttttaaatttggtgctcccaccaggaatcgaacccggttcagatgcttacaaggcaactgcatcgccagcaatgctttaggagcgatgatcccgttatttcaacgggatttctttttcaataacaggagacttatcagtcataactgtcattgccatttgttgtagaaattcaaaggtgaaggctacacgttcttcaccaatctctacttctacacgtttcttttgtttatcaatctttacttttaggttgtcagccatcttcgggttctcgttgctgtactacttctagccagtctggtagaagaaactttgtacgaaattcttcgtaagtttctttgggataaaagctaaaacctcctttctcatcattcaggataacagaaccgtcagtttgttcatatgctcgatatgtttctccaataatgataactcgcttatcagtacttttattatgaaactcaaaaacgtgcataatgtttccttaaagttggagcggctagagggaatcgaaccctactcagcgaggcttggaaggcctgcgacacaacccgtgtgcttaaccgcttattatttggctggagaaggaggaatcgaacctaccattaacggagtcaaaggccgttgtgctaaccgttacactactctccaagtatttggctgggatgccacggattgaacgtggaaccttcggagtcagaggccgacgatctgccaattgatctacatcccaataattctttactttatgtaaatagggtaactgtgctaacggtcaggtaattaatcaaatcgctgtaagtcttggtgctatcactcagactctggctggtctgcaggctaaactgccggcttaatattaaggggaggagcccattatgagtaaatatggttttgtaaataacggacttaatcaaagtatgggctcccagcagcccattccgggtctggataacccctacttacaacaattgcaacagcgtttagcagaagcgcaacagatgcaacaacaactccagcaaaaccctggaagtgtgagtcctatgcaaatgatgcagcaaatgagcgggcagtcgcaaatgcctcaacaaatgcagcaacagatgccgcagcagcaagttcagcagcaaacccaacaaccgcaggtttctgcggaaggacaggcagtactagcccttttcgaagacttcacaaagacagaggatgggaagcagcttgtatcacttatgggtaagtttaatagcttctgccaaagccaagttgcaaaagctcaaaatggtggtaataactcctaaggagaaattatgtgttgcagaaaacctgtttcgtgctgcccaatgcctgtagcacgttgttgctctccagcaatgtttacacaaataccggcgttcaatccctttgcctttaagcctactcttatcctgccccctagagtagattttcagtcaagattggcctcccgtatgggtggttgctgtacaccgagagtgtggttctgaagaaccaaacaataaagcccctagtcgaaagacttaggggcttttctgtatttaagataaaagaaaagccctgcgctctccagggaacgcagggcttacttcagatgttacatgcggatattatttattacgcatatccatgatcatttgaccatcgtagccagtacctaccacagtctgtggtacaccaccttgatatttctgagcacgaatcatttcgacttccagttgtttccaacgaatcatctcaggagtaatggtacgttgcagtgcggcgttagcttcagcttctttcttagctgcgtacagtttagcatctgcgtcacgttcattagcgatagcttggttgttgcgagcttcacgatctgcttctgcttgtttaactttttgctgtgcttcctgttcaacacgagctaattcagctttagcagcattaacctgttcttcacgaactttggtattctgtacctgttccatgattaccggtggcaaagtaatatcctgaaggaatacctgcttaactgtgtaaccatatgggcgtgcatactcttcaacttcctgttgaattgcagtttgcaattgagcctgaattttagcatcaaacaaatcttgtgctttaggtacagacttaccaaactcacgaatagtagacagtaatttttcagttacatatttgtctaacgcttgatcctgagtacctgcgttaatacggttaattggtgccttagaaccatcaaactgcaacataacagtcaggtcaacagtggatttaaacttatcctggctaggaacctgaagtttatctaattttacagcaatatcttttgtactaaaagtgtcgaaagatgcaaatgggtttacaagatggaaacctggtaatactgggttaggatctactttacccagaaatgtttgggttttaaccgtaccatcagaaacaatagtatatgaattaaaggctagaatcaagcctgctaaaccaactacagcaccaataccccaacgtttaatagtacgaattactttctgctcagaagtcagttctttcatatttttagtattaaacatatatttcctttgttttagttacagttaataaaattggccgaggtgacaggattcgaacctgcataaaggaatttagaagactcctgcctctcccttagactacaccccgtttaaatatttttaagaactctcgtaaaaactcttaaaaatacagacgataccgggagagtcataagtctcactcattaagtatttcaagacaaaatacagtaacgtctattattttccagtttaagtcagggtgacttagtggttaggtcctgcggtatattgaggactcggttaggcttggggtcatgacttcccgccttttgctgctactcaacaggagttatcgcgaattacctgtgctattgtgcaccattagtgacatctctcatgtcagcatttcccactttgtggatagcttgaaaaactactccgatatggagaaaaaacttcactatcctagaataccttctaaagttcttctttagcctggacatagttaaatcgtaataaaactattcagcagactggttggttagcctggaaccaactaccgcgtggtttaggcagtgcgcaactaacctcggaagcttttacgttaaaagcatcagttatccagttcttaccgaccgtaggattcgaacctatatcttccaccagttacggcttgataataccaattatactaggacggcagtgttactacataagtgatttccacaccccactatttataaattagagaagagtttaggggagaggtttcagacgcctcattttacacgttctagccactaaccgggattgccgccccctgtgtactagttttacaactaacctaccgactctattcaacgaatcttagtgctcgacgcatcttacattaagacaagttcagcgtaatcggctcgctgttctctaatttatgaatatattatacagaatttataagcatttagcaaataaatttttaattaaattcaccagcaatctgagcagcagtaccaccatcataacgcccaggaaattcttccttaatcgctttcatcagcataccttttgtaattcca

SEQ ID NO: 4 - DNA, 32767 bp, SP15 phage
  source 1..32767: mol_type = genomic DNA
ggtgcagtgggtcgggcgaaaatacttagtctgctaaccgccacccccgttacaattaccatgctaattgtttcaccctgcaaccattttaattgcagggtgaaacaatttcaactttaattattacgcaacttttaatttctcaatatattgttgcgggctgcaactatattctgcgcgttcttcttcggtcatactttcccaacataattgcaggcggtcggctaggaattgataatcattatcatcgtcgagcgattcatcaataaaggtttcacctatcaatgtaacaccgattgatagaatatcgttaatagcttgcgcgtccagcgttttaaatccgtatgatgccgccgctgatagcacgcctttatgatcatcaatcatcgtaaaatcagcgttcggatataactgtttaaataactcaaaataataagatttataaactgcgtctttgctgtggtatatttcgctaactttatcagcttcaaaatatttgtgcagcgtgtcacgggagaacacgcggatattgctgttcccacgccctcgcaatccttgcttgcgtaggaagtaataatctgacttgctcattagtcgagcggtgcaaataatgtttaaagtatttgcgtcattcatgcactggcgcatatatgtaacaaggggcaataaggaatcttgcattattaaatcatgtttgcaggcttcatttttatacttatttaaatctaaattgccctcgctatcaaagcaaggcgctacacgatgaaacgaattaatgatagtgccgtctaaatcccaaatcataacgcgggaaatatgcgggaaattacgggtaatattcattttaacttgattcattttgttacgttctccatttaagggattagattaattcaatctagcccactaattatattttgttagtgggctatgtttaattaactattagaatgctagaccgaaagcgagagcgtcggcaataaagctaacatcttcacctgatacataggaacgaatccccgcacaagtatatacttttgcgctgatcaattgatcatcgaggcaagcggggcaaggcgcgacaactgcaaaggctaggccggattttacagcgtcgatgataatcgtttcttgtttcaccgtatcaatataaacgcctgcggccttaatgtaactacttgcgcagccttgcgtataggcaaaggtagtaacctgcaaggcgtcgttaaattcgattaaatcatcgacaacgtgccccgcctcgacgtgataacgctcaccattagaataaaccagaacaattgaggattgagcgcgatcgaatggaatattttgctttttcatatttatataactccaattagtttaataaggggtttaatttatttgataataatctgcatttgatacggcgttaattcaccgtttacgggtaaattattatcgcttagccactcataaaaagcaccatcatcatcaaaagggacaatatcgttatcacgggaatcgacggaaataataccatccgtattagttttggcggctaggataggcccgaagctgtaaactttatcagattccatttcatccggtgaaatgaatactttttcgtccaatgttttgggtaatgtaactttcattctaatttagctcctgtaatagcggctatatttcaagccgctagggtaataatttaattatgcaaagaatttaccgttcttaaagtcgatcaaagtacgctgaccgtttgcataggtaattaaatgcgtttgtgtccagcttgacgcgccaacgttgtaacccatatccagactaccagctacgccagcggtatataccccgccgtaaatgctggcggtatgagtgtgccccgtgttcagtttacccaatttcttaaactgtttcggattgccacggctgccgtttatgccattgtgaccgtgtacgccgcattcaatgcctgcaattttaaatgattggtcagtcgttaggaaaatggcgttaaactcgcaacctgcaaccttacgcagcgcataatctagcacgttgaaagtatcgtctttttctgcaatagctccataaatcgcggcattaaggcggtgatatagttccgcgtttgctgggtcgtctttaatgttagcattacgatcatcaagccaacgggataacgccagatcatggttagattcaacaatgattgtttgcgagaaatcgcgctccattgattccagtacgcgccccgtatcgatgagatcatccagaactttatcacgtccggaggcatactgttttgctaggaatacacccgaagcgcggttgtgatggttgcgtgatgtaaagtcgtgaacgtcatggataaactgatattttggtttaagaatatcaagcaagctattttcgccagcccatgacgcagcggcgcattcttcatctaatttttcagcgtggatgtcgccatattgtaaacctaaaacgtgccccgttgtttcatagcatccggcaggagtagcgcaaacattcagatcataaaacacgccgctttcgtccattgtttcaagctggcgaacaaaaaattccccgtcctcatcgaactcaacaatcagcgcaccgaaattatgcagcgcctcggccttttgtcctgctttctgctgaatgtaatttttgagcgttgccgttccggttgaatacatgcggcgcacaatttcaccttttaaagctggcacgctttcggcggtgattttagccgctccaattgccagaccttccagattaagcgcggttgcagtttcagcgaatccagaaagcggataatctgcggttggcaaaacattaatttcagccatgaaagcaaaacggcggttatttaaaaacacgtttttattgcagatatatttatcaaaagcggaatcatatttgattccgtctgcgccctcgccattttgaaaaccgtttttgttatagatatattttgaaacgagcaaatcagcgccgatatatttagcaaattgctccagtgaggctaaaaagtttttatgcgggaaagtattattctgaatcgatgtaataataaagcgtttgccttgttttacttcccagctttccaccgtgctagaaacaatccccgccgcttctgggcgctcatcgtttttaatggcttttgctactttcgccgctttcggtttagctggtttatttgcttccaaccagtcgcagatagcggtcgagtgttttgttgtatcgtagaccgcttttgatatatcgtcgcagacctccagtttagtagcgcgcagacgtttaccatagaaattaaagtcagcggccattttcaggataacggtttgtttttctgcggaaataatcatagtataaaactccattaaagggactaggttaataacggcaatattgccaaatataacgccgcaaatgagtggcgttataatttgcaacattaatttaaaggtataaggctagaactaacaccacaagcaacggcggcaataaaacaaatcagacctaaacgctttgccaatttagacttacgtttaaaataatatgaatctaaatcattttgaaaataagcgaatagtaacgaggccgccataataaataagcctagaatgagggattcagtagggtaaaagatcattttaataactccagtcaaagggaaattatagtggggaatattccccactaattaaatttattcgcctgcggcttgtttcacttcatcggcaacgcctaacagttgcgccacggcgtccagcgtttccagttttgcgctttccagtgatgccagatcgtcggcgtctttgataatgccggaatcgatggcgtgttttgcaattacgcgcacataatgcgctttgcggattgagctaccgccgccaactttgcgcggcttatcgcttttctgatacgctttcgcgctggtcaattttgagcgaacggacacgggagaagccgcgcccactgctttcgcgatctctttcaggccgtcgctatttgcgaaatctaaaccgttttcattaattaactgctggtacatggtaacagctttttgggtgttttcttcattccatgcaaattttgcggatttttcggttttaacgttagccatgattgtagctcctattagtttaatttaagggataagattaacataatgttaatcgttatataccccgaactactggggtatataaagttaacactaaattataaaacagcttcccatttttcgttacgctggacaacctttacaacgtcgccggatttaacgcgaacgctaaaaacggttttgccgttgttactacgttccgtttcagcgtataccgcgtcgattgtatcaaatggcataagcgccgcgcctttaatgcgttcggcctttccggttaattcatccgttttagtaacgaaaggaataaaaacggattgaccaattttaggcgtggtaataatgttttgcatagtataaactccaagttatttaggggattgttccgcattacctgctagaaagtagcaggtaataagcaacaatccgctcgccaatataatcaatttaaagaactccacgcaggccgctatatcccagttagggggcggggcacattatggtaagtgccgaccgtcaaattttatcaaattatcgctcttatcgaactgggtacatcttaaagcctatcggctagggtgtcaaactattttttgcagttttttatggttttccttcaggtcgatcataatattacgccagatcatttccagaccttgctggcggcctttcttgtactgcgtgaatcggtattttaccgatctttgcgctactgtcaacaaattttttgttttgctatctagtgccttgctaggcttgccagtgatcaataaagtttgtttcatatcgtcgattccttataatgtataagtttaccgccgataggctttaagatgtacccaatttttaaagagcgcggcggtaacttcccgccgtgtagttcgtcattgccgtcctacgtgataaataataggggattcccgaaaatggcgcaaccttatttttgtaaagaaacgtaaagacacgattcaccgcacgccgtccggcggcatgggcgcggcgcactaaaattaaaagaaacgggcgcgcgagtaccacaaaacagagcaaataggcaagtaattttttcatttatatttgctttgccctacttgacaaaacttaaaaagctcgtggtagcgataaacgagggtaggcaatgcaatggcacggctaaaactttcatcgcgttctagggcgttttaggcgcattctagccttgttgataacttatccccaaaagcaaaaatgaaattttcctagttatccacttgacttttattttccagtggataactacttattttatgaaataaattaattgacttttatttgttagtatgcatcggaagaatagcagactaataattactagaataataatcatgctggtggattgtaacggcctaaactatcagcagactattaatcacgaaaaatctcgttagctaactaactatttcatgatgtataatatacatataaattaatgagaaataataattataataaataataactacagtaaataataactataagaaactatcggcctaagtgagaaccactatcatttaagttatccacaacgttatccacagcacaaaataatttgacacgataggcggcgatataagggcttatccacagacttatccacaggttatcctactgtataaatatacagggtagaaaggtagtgttaacaactgcaatcaattttaagcggcctaaaacgctttctaacgagctaaatgcggtggggtaatattaaagtaaagccttcacccgtcgccctggtggcttcgccgtgttttgctctttattgcaccgctgcgcggttagcataaaactaggcgctaggcaaggaaaataaaaaggtaaaataatatttgcctatgttagaaaattacctttatcattcactcaccgattaacgagggaggccgaacaaatgaggctatataaaccagataacgcaaccgtcttaaaaggtgcgctgcgtaacctgctggacggtagcagaacaaccagcatcaaacattttgttttcaatattgaaactattcatcaaaacttttttggtgattatgatgcttataatatggatagttttctaccgttatataaacaaggggcaacgcttgttttatataatcaggaatctcacttgcttactagtcgagggccagatactgattttattttagtaaaaggcaacacagtaaaagcctatgatgcgggggcgggcttagaagttttcacaatagaaaactatgaggctaatgataatgatctttatgatgtagaaaattttctcgattcattttggcgttatttatcagttggatggaatcgatcagattatgacgggtatcgttttgcggctgtaatggcttttgatgataacggtaattttttattaccatcggaattatacccgtatgtgcataatgagctagtacaagaagcgggttttattttctggaaagatgaagatcagattattgacagcgtagaaaaccatgctgtaaattctaacactcaaagcgttaaaactcaaactactgaaaacaaaggaaaaaacaccatgaccaagatcgctaatattgttgccgctaataaatccgctgttgtaaacgctgcaaaactggaagcgggtaaaattgcactgactcaaattacgaaagtagcggctaaaaaagcaccgtttatgattaaaggttatattgatacacctatcggtcgagtagtgattgccaacctgctgagcgtagcggttgaccagtacgccccaagtaaccaaaaggcgaaagcggtggcaggtgcagctatggaagcggctatgttagaaatggtgcaaagttttaacatcgctgagatgattgatgaaatggtaaaaggtattgatatttctacttttaccactagcaccgaaagcgagtaataatattaagcggggattgttaccccgctttactattcccttgttaactaataggaggctaataaatggcggatgaaaaatatggcttctcactgggagaagtgagcacggcaaaacatgatatgatcattttggtcgattgtcatactggctattgcggggaagggaacaccgaggaatattttgttcctactggtacggatctggacgctttcgctcaggaaatggctattgataatgcctctcgttttggtagcgatggttacgaagacgaagaaactggcgaatggtatgataatgaaaacgtatatgcaagcctttatcattatcaattaagtaaatccggcacatatgtaaacggcggcgatcctattaattccgtcatgagattaattattaaatatggcggcgtcgagataattgacaacaaagcggtaatatatgcaaaccgattaaaacagcttgtttatattcctgatagtacccgatgggatgaatatgctgttttgcatgacgaattgaaacgatgtttcaatattgaatccttacaagtagtctaatgtaaagttttgtaaaggtcgccttttatggtggccttttttgttataatgcctttacaccgtttgaggacggttgaaaattttcccaaaaattggaggcttaaaatggttgcttactcttctgctagtcatctgttcaccgctcaaggctgggtatctaaccgcgttattattcacgaaatggtgcaagaatatggcattgctaaaacttacactaccattcaggcgctttatgataatgatcaaatcgatcagcaaacggctggctttttgctggataccctgaaagcagaacattgcaccaaaaaacaagcggctaaaattgttttaatgtaattaataacgggggatattatatcccccgctaactaggaggatgaaaatggttatttttcgagctattctggcgggtatcttgggcgctattttatctttatttgcaatagctttcgacgttcacgcggttattatcggcgcgggtatcgctgtattttcttatctgctgggctgcatgactagtaaaggagaataaaaatgatccgcaacgtttcccttgcacgttcgaaaggctttaagctggtggacgttaacacgttcgagcgtgaagattgtaaaatcgaatatgtagcacgtaataagaatgcctttcgtgttaccgagaaaaaattcgataagcgcggcaacgtgatcgctgaaacggttaaacactttgccaccttttacgctgcgtttcggggagtgttataaaatggtaatttatgaaggtaatcgttttgttgctaattgccgtccggcattattagcaaactatttaaaccagctttcaccagcttataagggcgttattaatatttatgagggcacggcgcattataaaatcaatgcggtcgttgcccgtgaactagcgtttcaatttttgacctttgcatcttgtgacgttcaggttatgggtgaagcgttaattgcagaaaatgaagatgattttattaatattttccgcaagatatgcaccgagcgcctgataatgaaaggcgcgtatattcaatccactgcggatagtattgaaacagcgtttcgaaaggtggcgcaatgagattatatattttcgcgggtaatgttgaggctgcaaatgattccgctggtggcgataacgttcgtcactactggcaaaaatatatttactaggggttattatgagcaataaaattattgtgaccaaaactaccacaacggttgacgttttttatgtgcctgatacgccggaaaaccggcaagcggtcgagcggggcgaatatgatagcgttatttatgatcacgatggttactaccaacatttggtggattcctacggggaggaggaaaaaatcacgcatcaattaccggactgacaacaagcggggatctgctccccgtttttcacgcctccagttaaatacctctttgttttagtatccccaccaaaattaaacgcgtcagaatgcgatctaggacgttttagcggtatattagaattattcactacataggaatactgtatatttatacagtaggataagctgtggataagtctgttaataacgcttcaaaatggctaggattctgtcaagtcaaatcgtgctgttaataagtctgtggataacttaaataacagtgtttctcacttccattcttaaatgagaatcattatcattcgcattccactgtctaaccgataatcatttcactttttgaatagttctcatttcacttcttaaatgagaatcattatcattcgcattccacttcttaaatgataatgattctcattcaaagtcgcagggcaattgccctgcgcttttgtgcaaatccgacatttgcccccatggattacgcgtgggcatgtatgtgcaaatccgacaatttttggtagtgtgcaaatccgacccgaaaaatttttatagtgtgcaaatccgacaatgaattttcccaaaaactccagcaatcacgaactgcgttcgaatcctgtggaattagctagaatatgtgcaaatccgacatgtgttgaggtgtgcgaatccgacaagatttttatgacttcgatgagaaggtgtgtgattgtataggtttgaggaaaagatgagagagcgagagaaattttggggctagaaggatgtgggcgcaggattggtgcggagcacctgatttgcaggtattttgggggagagttgagataatttgggaagatttgagataggtgcagaaaaagtaaaattttattagctaaatggggcaaaatagcttgacaagtgaaaattcttgtggctctaaaaactcaggcaatcacgggccttcggcccgaaataatgctgctattttcaggagagtaagagttcctaaaaacttaggcgtttgtgcaaatccgaccataaatttctagaaacacaatgtgcaaatccgacagtaaaatccagaaatgtgttttcaaaaaatgtctcctagaaataaccgccctccctataaccgccctatattaaccgcctattgctagagtttctaggaacaatgaaaaccgcctgagttgactagagttttcctagaaacttaggagtctagaagaaagtgttgtgccatcctagtagatgagcggcaacaggtgtatcatcttgaacacagatattgcctttaaaaatatttaaataatataaagaaaaagagacccccaatttcatgagaatctctcctgggggcgcgtgattaattacgtgagtactcatgccgtcataccgctgttgctaggccgcaagctatacgagacattcgtgtaataatcatcgcccctagagttaatcaactagagtagttgttaatctatgagattattataacatgtttgggtatgagaatgcaagaactttttgttaacttttattcctccttcttggatttgagtttgatgcctaaggatgcgaagtagatataagttgctaaataggaagcagtggatcctgtatcatcgtaatccatagttccacgagctgctctagtatattcaggagcatagtttaatatcgtgtaacttggcattcctagcgacttacatagttctttaaatgtatcttcgtatttatggcacatgaaatgcacagcattttctaatggcgttaactctagatctttatggagagctacagtcaaactcgctagcattgtgccaatcccacgataaacttcatctttaactagagttggtttctctttttctagtggaggaaggtgggcatatttcccatgtttgaaagggataagatcttcgctagctaatgcttctttaaatgatgcttccttaaatcttgggagatcttcatcgattaggatatgaatagcattagaggagaaaccttttgcttcaggatctaaagctttcaacgctttattcacttctacatatgagcctgaccaaactacttgttttgcatctcgatcatacttgatcttacctttatcccacctagcaggataatgatctcctaaaaacattactgcatatttttcttcctcagttagctgggaaagactcttttgtgtagcaccacgcgctaactgaatgagacgttttaatttttcagcttctttaatcatatatcagacgcttgctcccctgtttctttcttttctgtcttaggttttcttgcaacttctccaaaggttcctttggttctttctttagctggaagatctactttataccataggattcctaattgttgcgctaaatgggctatattctttggtgttatacttggaacatcttccctatcagaaactttagaaattatatcaagtaactctcctatttttggcttactagtagttattagaatatattctaatgtttctatttctacattttcatctttatagtaaagactaagagtaattaaatcgtcaccagcagaagttatttttgttttaccaaatatcattaactacctctcttatcttcattaagagcagctcccaacgcttcaaggatagtatcatttatactcccaggcctaagattattaaagtgagtaacatagatgggacttctaaaaccctcagcatccgcaggtgctacgcttcgcatatcagattcaaaagcttcttgagtatgttgcaactgtacagaagggccgtaatcttcaccaactcgatatgaggaattattttctataacgccaccacatggaacattgtgcaaatccgacgttattttaggattaaatgcgataccacttttggtccaggaacctccaacagtcacaggagtactagggcggttcacctcagtctttacgagtttataaccagcatctattaatgcgttaataaggttatcagctggaatccgagccttgccaaagatcttacgagcttcttttaatttatgctcaagatctttacaggctttaatatcagtgtgcgcaaaggttaatttcatagatttgaactgtacagtggcagttaagtctttaaaatcataatcccatgtatttaattcatggtctggtactacttgaacaggttgttgtgcatataaagtcattacttattctccaatttgtctagtagcttgtgcgctgctatgttatattgtttaagttcacgattaaggatttggttttcacactttagctctagattcttattattaagaatattgcagatcagtagaagtgctaatataactagcaaggaacctacgagcattaaaagaaaaagagtttccattatttaactcccatgtaacgtttgagatatatgatgaagtcttctgctgtatgctctacgctaccttgagctacaaatagtttgagggcttcacgttgtagtttaagagcagccaactcaccacgtaattttattagatcttctgctagttctttagctctgcgcataatagcaaatgatacaaatgttacaataaataacataactgctaaaataattactatgatctccatattaacatccagctcttatcatatatttgggcatgttctactaattcatttatcgatgtagaattatcgtagataccctctagtaaacgttttctgtcaaatttatcaaccaaatactctgtgccatttatcactaccctatacagctctggaactaaggggtgtttgtttggtattgggcgactacctaagtctatttcattatatccccacgttgttttaaatagtttgttgctaagtgctgctagtgggtttgaccatacaatatagctactcactacttatctccattcttagctttgaaaacttattataccaaattatatgattatcgtcaattacaaatttatggtaacatgctggtacggtataagttccataatccgtgacacgctgcacaaccttgtgtgcacacagtcgacaaccatgcccttctaaatgagatctagcagtttgccagtaataaccatcgtgatctggacaatagatctcgacttgctgttgcattgtcttataatttacacgctcatatccgaagaaagccccgtgagctgcaacggctttcttgataaatataaggtttagtgcttcttgctggaagtcgggatgtagctgcttaatcttagttctattaatagatccatccgatttaatgaacctatttattggaaagttgttagcttcctcgattaataattcatttactttctctctcatattaaatagtctcacagttaaggtagaaacattcgtaagcatctccagtaaactctttatcttgtagtaaacacttagcttggtcttccggtactccagcatctaataattgttgtttacttggcttttcagcgaatacttttacaaaatactcaccatcctgattatactcatttatatctctggtaaggacatatacttgcatttgaagttccttgaaaacataaaaggccagaacaattaagtcctggcctctagaattaatgaagttgtttaccacttcgtaacatagtggctgtttccataagacctagcgtagcatcacgcttattgatctgtttaccaagttcatcggtacgtttaccaatgtaagcgttaatagccatattcatagctgtagcgagatcttctttggttatctcttcatcgtctaaggctaatttagccaaagaatcaaatgtgctagagagtcctataagatctgaggtttctccagccagaataggattaatattatctactgttacttctagcatggagttaacaatatcttcaccatctattagaccagattcaatattactctcccactccttcatctgctccaataatggatttttcttttctgtcatggtagaggtttcctgtgtcagtcggtaagaaggatgattgagctttaggcggatgttgtttagcaatccagctaagaatcagtacacgactaggaacaatatcagtgttgtaccagaaatcatgaacccattgacgagcattctcaaacttaccaaatttatatgctttcttaaacaattcaaacccaaaacaatctggtgtaaagtctacttcacgatattgaactactttagaaccagttaggtcttggatcgctgcattaatttctgtatgcgagaattttgtttcgtgaaacttattaaagaatcggtagttgaagcgtccgttcgtttcgacaaacaactggatgaaaagatcgttaaattggttatcaaaccagtaattctgtagttgttgtagtgctgtcatttacgaactccgttaattgccacgatgatgccttcatacataaaaggaagtagttcagaagtgtagaagatattttccgttattcctagatgtcgaaaaagtatattaaataatgctgttagaaatacaatctggggcagtaatacaaaatactcagttacaatctttggtgcccgataaacaagacgttttatcattgtttttaagtctccttattactttggcctgctccacaataatgaaaactgcgagcactaatagtgctattagccccgcagtaattggtactaaatcaatcatgggagacgccatacgtaattagctgtctgtagaaccttaggtgtgtcatcatgatacattactacagactttggtgaatagctatcagctagctctttacgaatcatcttacattcttcaccagtatcgatatttttaactatcactttcatattaagaggtgttaatacagaaagcggtttccagaagtcctcaatctcaattcctacctttttctcgattaccatgaggacttctagtgtatcatctggaatactaatattattattcacaaactgtaatatctcatgtaaggtatttaattcattaaaattaagcttcatctttaagaatatcctcaaccatatcacaggactgttgcaattcgtcagcaatgcgcttaatatcggtcttcgtcactctaccgattaacatcaccagtaacatagaaagtataataagtgggactggaataacaaataaagctaccttaacaacattctttggcgtccatgtgtggtacttggtaaccagtacaccaaccacaattagataaaacgctagaataaacatcatcattttttaatctccgtaattatctgtgcacgcattactttattaggtaattttgtattcccagctattgcttcaatattatttagtttttcttttagaatatctgagcgtctctgtgctagttcaatatcttgttcttgttctattaagcggcagtgaagtccactattagtagtaagcatactctctatattttttcgcatgcttacaataccaataatcccgccaatcgctactagtgtagtaagaactagtaacccaataagaatttcaatcaacattaattatatactcccttagtccttatttcttacctttcagttgcttaacttcacgctcaaaagatgctgcacgacgttcggcagtcgcttgatgctctttagcaaaacgagcttcctgttttgcaaggttgaacgccatagcattcttattcagagaatcatacatctttttcatcgccggaatagacatcttcatgagctgaccctcaaaaccctgcatgtcgaggagaattgccagaacgttagccatttcgtttttagtcatgttttccattagaatttcctctctcattaacttatgaacttattatacagaattttaaggcttaaagcaactgaattttttaattacttaccaatcgttaacaacgccggagaactcagaagcaaaaactttttcaaatttctctgcaatttcaggatgatctttgcagatcagctcaatacatgcttctggagtcattccttcatcttcaggatcaccatagtatttatcccaaagatcatcgggaatgatatgctccgccaaatcttggaaagagactaactgataacgttctgcctcctcagcgataagaatttcgcatagatctttatctatatcgctacgataatccgcaattaataaggcattgcaagcatgacactcccaaaccatcaagcgttcagaaataggattagacttatcctgtacgtaagactgaaacagggttcggaaagttgccttaacttgttcaaacttatctgctgctgcgaaaactagagctttatcaactttgttcattttgattccttctcatcaatttatacagtaattatacagaaacttaagcattttagcaaataaaacttttaattaaaatgcctaatcctgtgccaatagcaatacaaatgattataagtattgctatcgcctgtatgattcgtttaataataacctcagctatatacttagacatttatatcgccacgcaatacagcagctacgtcttctcctatttgtaatacctcgccggtagtacaattaaccactctatcgtaactagtaaacttaccagacacaatatcctctagtggaattggagttctactcatttcaaatgagacattaatataacgtgggtcacgtaaagaagtagtatgtacatgtccgtgaatatttagtttgccacgaagttcattgggatgcaaagggcagtgagatagccaaaactttttgccacctccagtctgtttgcctagagcttgaatatcgtcataaacttccgctaagtccctaatactcagtccttgacgctccgcatcatgattacccataatgagttgattagggacattgtggataaccgactttaatttggccagaccttcacgacctactgcaatatctcctagcaaaataagttttgttcgtttaccaatatgcttggacaaagtatctagaatatactcgtcgtgctctttcatgttcttaaaccacggacggaaacgtaacgctccagggtggtctagatgcaagtctgaccagaatttaactttcattactcttttccttattctgtattaaactatcaacccaagaggttaacactttggttttaaactcctcgggagtctctccttccttaaggtctacctcattaaggtaggtagtaagccttgtttctatatctatttcagtaggagaattaaaacaaaaattgactgctattccagaatatattactccggtatctcctttgacgaaagcattaactaatgccctccaacgaagggcatcaatacgcattgctcgtaattcttctcgtacttctttcattctatcattcattaaagagtcctctgtacaccgcagctattatttttgtctgtggtaaatgtggtgattttgccagtttcatcattaacttgcgcaaccgtcaactgcccgttgaagacaccgccagtatctaggtaaacacggtttttatagagaagcgggtaaggtactccagtatgcccatggaacacaaagtctactccactaactggaggtacttctaccatgtatttttctttaaatcctgcataacgctggaaatacgagtgttcctcgccatttttagacaaatggaagcctatttcttggattacatctcgatcccataagtatggttcaacatggtatccaggatggtcatgcgggtcttccttagctgcttctacttgtgcaataaggttatcccatactggggtttctacttcgttaccacattctttgtacgtaaaaggtacaccaccatgaacaacaccatacttcttaccacgatgtctaacagttaggaatactggcattttttcagccatgtcttcggcaatatttttaatggtatctgcatctagctcattcatagcccacataccaccgttatacatccaattagcccaatctcccacaatcataaactggtcgtggtttccacgaacgctacaaaaacgtggattatataagaatttagctaaaacttgtaggttctgcgtgcctcgatcaattaaatcccccacgcatataacgcaatctttcttgccgttatagccagctaattgtagggcatcttctagcaaatcattgcatccatgaatatcgccaacaaagaataagttaacatcatcaggtactactagtgttttatgcacattaaattcttttttcataattattcccaaataacatttaaaatagttgtgccatattcattagatagttggagagtataaccctctttattgagggcttttatagcttcataactaatttcgtcacggttaaactgcacataagaacctccaatctctacagaagatactatcctccgcttaacccatctatatgttttctttcggctcttaagggacgcggctctatttatcctagctaaacgttttgcttgctctgctaacatttaatcctcctatcaatctatacaaatattataccaaaatttttagcaaaaagcaagtaaaataaaagcctgatccgctaagatcaggcttggtttattaatcctctggattatcatccaggaaatttttaatagcttcgtgcatagtttctttacgaagctgacgtccaatcaaaatatgattagcttctattcgaccattaggtaagcgatctgccagaactactacaggtacttgacgtacaccaaatttctgcattaattctgtattatcagtctctttatggatttccaaattatagtcattgactactttatcaaatactggttcgaaaagtttacatgggttacaggtggaaccttttaatagatagactaatttagacatttttatttcctttgctggcaaactcaccgtggagttcttctagtttttcatctctccatgcaattgcttcttccaaagaactgcacgttttcatataattgattcctgctctagagatttttactctaaaagacttccctctttgagatatattttttaatcccaataggttatttttattagccgatttcctattaaaagcattttgagcttttgtagcttctcttaagttaccaatacgattgtttagcgtattggtatcatcatgatctactatatcaggtaaatagcctttgtgcataaagaagattgctctatgcgcaagtattcgttctccatcaatagagagcattagatagccatcagcattaatagacccagcaggcatattgttaaggctagtattccaacctcttgtaccttccggtctaggtttccaggttagagtaccatcttcgtggtactctaatacctctaataatctctccctagtaatcacaatttattaatggcctctaagaagtttttcatagtttttacggttgcggtgctcagatcaagatttacacccaaacactcggttaatgcttcctgataaggagcctttaatctgccttctgggacttctaccttcttatactctttatttttgacctttttaatcatagtctctagtacaagaagcggtaatttagcaccttcaatatcagtacccaaaagttcagttaaaattttattaagatcaagacgagttaactttttgcccttagacatagatgcacctacctttgtatcaatagatttttccgctttcttttcgagctttttgtactcaggagagtcatgatcacggagtgcaatgtttagctcgtaatgtggtatacgaaaatgttccgccatttgagtgtagaaacgatcagacataatatatacctctcttaactaatttatgtatatattatataataactagggctaaaagtcaactacttttttatcttaatctactgcatgtataaatcttttcctaactagatacatagttattgggtaaattgagtacataagtatcggggagaaaagggtgaaatacgctgtaactcccccagctaacatcaaaggtattaatgctagagtaagggccataagaatcataccgaatgaaacagccagagctatggatataggattctctagttccatccataaccaacaatatttcgtatctctatggcaattgcatttacaaacgccgaatgaacccataattatatactctagtccgtgaataacctttattaataagctatttcgggtagttaatgcaatgatagtaaagactatcattaaaacgaatactactagacttattttccagatacctagcagcatcatagtgaatagttctgcaaacatggctttctcctatcttcaaaaattattaaagccccctttgcctaaaaaggcgggaatattcccgcctaagttattaattaaactagttcgacatgaccgccatcataggtaccacgttttatttcatcgtgatagtctcccgaagcattccaatcagcaccaaaacgaagtttaatgcctagctctttaccagcttgttcaaaagcctttttaactgcccaaaatgcttctaagtcattccaatcaattttgccattaatatatggagcaaaatcaatagcatccccagtaatatgtttgcttttactaggatcttttagaaatgaagtaccattagcaatgttctgggcactttgtgctactgtacgaataccttgcacgattgtgaaatcatacggagatagttctaaagccctacgagctactttttgtagctcgggcttaacggtagctaattgtttttcactatttttaccaaatttaaaactcatattgatctacctaaagatctctgttgtggggaacagagctttgctaaatattccttgaactgttcagaatcagctgtatctaccggattatctttccaagcaataccaatgtacccagcatagatattttttagattgaagtatggacaagtgtatatgtaattaaaagtaacgtttttaaacgcaggtatatttaaccccatatatttatttactcttacacttaaatccgatgcgtagttaaagccctctaaatgacgtctgtataattcagacgttttatttaccgctttatcggccaagtcagccctatctaattgcgcattactttcccatgcaataatattggaataatcattgatagcatctggtttatacttgactacaaaaacagcatctgcacccgtttgagagaagagaaccatgctcttttccctcgccacattagggaagttatctatcctctgggtttgtaaatcttgtaaaactgcagacgtggaaaaagtctttaagaatgacatcacttcactagtattactaacaaataagaaaataatgacagcaactaagatagttagcagacgtttaagaagcgatgctggatctttcgcttcttggagcagtaccgttaataattgtaagaacttttccaattgtaacctcctctaaccagtaccattatactaattttggaggaaaattacaatgtgtttttaaagatcacttctggagcataaaattttgtcgttgtcaagaagaattttagataaaagaaaagccagggtcgttaaaccctggcttaaaattacttactcttcgttatgctcctcggattgaggtaactgggctttattatattgctcagatcgatattttgccaagatttcaatacgcttatggatttctttgctatctagatagatatttttgttgtcttttaccatctcgtcgatttcgtctatagagaagaacggatagtagacatctagcatcatatcttctacgaacttgttgtaagattcataggctttcttgatttcttgacccttctcacagaatccgccagagaacgtgtgtcccattagcgtagcatgtggatgtactacccatccatgacaggataggaaaattgtgcagtaagcagaagcactaggaccaatcaggtgtcctataactgttccacggcaattagcaattaagttagataactgtgcagcagtatcaacataaccaccagggccattaatcatcagattaatttcgtcgtcctcatttgcttgcataagtaccattgataaatcacggtattcatccggcgggcctaattcttcatcaaagaaaaaggtatactcattagactggcgaatggagtgaaacaggttagtcttttcttcttttttattagtcatagcgatccttgattatccaactagtggttctagctctaagtcacagaagttataaacttctagtttaaggttattgataccatcgaatttattaactaattcgtgagtaatatattttgcaggaataccactttcagatggatgatctgatttaatagtgaacttctgctcagcgggtactacatttactatcaaagaatccatatctaaatggtttgtttctctgagtaactctccttcattggggaatctaacatctgttattacggcgacatctgggtcgtctttagcgatggattgctccagaattatgagccaaatgcgttcatgtaccagctgccttcctagctctgttcctacgagctgtaacatttttctcggagaaataaataaactataaagtccgtcttctttattctctgagataagttgttgaggattaagatatttttcctcaaaaatcggccaaacgtacgagaagtcttcaaacttattgataccgtatttaaaccatacgtctctagctcgctccaattgagattgtgtgaccgtaaaccattggtcaatctctttccccctgcgctctcctagaaactctggagttacaccgaggattacggatgcaagttcataaacgggcttagcaaaactataacgacggggtaaacacgttggatacgtgtcattacaccaatcgataattaattttgcaacggtatcttttcccgaaccagcttcaccatgtaaaccgactaatactgacattaatctttcctattgttaattggtggataatatactaaacaacgtttttcttgcaaatcttggcggtagaagcaaaccatactagtcagtcgtgagatatatgaatattctgcctcacggcattttgccaacatattccaatctttgtatggtacaacaactactacgccatcttccccatttgtagctaatttcttttcaaacttaaagtcaaagctacaaggctgaagtcctttaggccaatccacatgggcttgctttaactcatgtgacggctctggtactaccgtttctgcacagcctgtgattgtgattgcggctgcgagcagtattccaagtttccagttaaacatgctaatctttcctcgaactccttactctgctttttagcaattaatgtaaccaatccaggctttgcagctataatatcttggcgactaagagctttgtctaactgcttaatctttttgtctagatctgcttgcgaaatattattcattgtgaaatactgattcattctagtctcacgaagttcgctttcagctttcaccttattgagggaagtctctagagaagaaatctttttagtagccaccgcaagatctcctgctaaagtctccactttatctactaagtgataagcaccgaacccgatgcctatcgctagacctgctcccaggatatacatcttgttattccaaactaagtctacaaaccatttccgcattagcctgtactcgcaaactcaccgtggagttctttgagtttggtatcccgccattttatagcctcttccaaactcttaagtgttttcgaaacttgcttaccatgtttggtaattcttacttggtaagtcccatttgtttttctatggatatttttaacgcctaaatggttatcgcttcttactttttggttacaagcattatcagatcttgtagcaggccttagattctcaaatctatcattagttgagtctttgtccttgtgatcaactatttcaggccattctccagtatgccatgcatagattaatctatgtgcccctatagctatggaaccattatatagttcaactactctatgccctgtactttgtctagatcctgctactgttccggcgaatatcttattaaaatgttcgtccccttccctgggtttccagataagattaccatcttcttggtaatcgaacattcttcttagctcttccttactgatcatcttttcatattcctaaaagaagtaacagtatcaaatccatgtgcagctaagcgatccttatcggaaatcgtaatagtatttggttcgccggttcctaacacgccccagatatattgctcgatcatctggtgcaaacggtataagttactttcaatttcctgccacggaatacctgactgatggaaacgaatgttagtctgaatcacgaagttacgaacatcatcgttatcgttcttcttgatacctttcacatatgcaatcggtacacgcagttcggacaagatacgttctgctttaggttttgcttcaacgagcaaatcacgcattgtttcacgaacatctccgcgactcttatccattaagtaagagcgagcatgcaatcccatctcttccattttatcgaacatagtgtcgaggttgaacgttttgaagctaaatgctggatgccagcagtacagctcgtgtaaccagtaaacttcacctgcaacaaatagtgggtttacaaaatattcgaaatcaccacggaaagatagcgaaccatcacgaaatacctgacgactatgcacgatgttcttttctgcatcatcagttactttaaccagtagctcttcagttttacgctcccaaacacgatctgcatcaaataaactgttctgcaaatcatatacatcggcgaatttagaaatgatcctcatatttaatcctcttgcctcaatctataaacatattatacaaaagttgggcatctaagcaactaaaattttattataaaaatagcccagtcgcaaaagtgcaggctgggctttgtcattatttgcttttgctagtaagctgacttagtgtcaatcttatgtaatattagtttctctagctttgcgtagtacccctgcatttctccacaatttgatgtcagcaactgtttctttataaggagctatggtaaaacctagtgggccagcactaaataatcctaagaaccctacaatacgcatgtagaacaagcattctttggctgtcatattatttactgcttttttctgcttttcatctttaaacttctgttcttgatcaccaatacgtagatatttaacaaaccattcagcagaatgttcgtccaaatgtctaataatagctatcgcatatccagcaccgattaaaaaccaagttgcaacaagaattagtaatatagtcatattatctccagttagggctagcagccacctcaccacttaccgcactaaggggcacgactcccttatccgtaacagttgcaggtgacgcaactcggtcctacgcgagttctttaagtattctgcatttcagctttaaattttttcatattacgagtttttctataaaagaaaaacacagatgttgggcctagaagaatatccacaataaatatcacagatctagcacatctgagtaatgttttatcatcaagaggtggcagatctaacggtcgagttttatgtataacgtataatattacatctttattcttagaaatataaagatcatcaaccaagctgtaaatagcaaccacagatccaatgacaaaccaaagagcaaatggagagataatcatttcagatccttttcattaattagaatattagtaaacagtggagtaactcctagactcatagtaggtccaaacgtattcatggctacccatagctgcatagtgatcatcccatctttaatctctggatctttatattcttcgatacgtttcttggtaaaagcaactatatctggattatttttattttcctgaatatagtcatgccaaaactgagtattctcactacgtaggaatgttaaaacatccttagttgctggaatctgcactgtgctgttgatgtttagtcttttcacgttcttctctccgacgtttgcgttcttttatcatatgagctgctacaacttcatggtagtagtcattaatgttatcttctggcaagaaatgcttaatagtctctagctgacaaataactcgatgaagatggttatttggtagacacaattttatacctgcaacaaatccagagaagcctggaacactgaacatgggttgggcttctactctaccttcagagttgatattaagctcaattgagatacccattttcacgctataaagctggcaatattctccgttaccagaccttgaccaaacagtgaagtcctcatcaatttgatcttgaatttctgtaatagcaaatttaattctaggatctaaattattcatcttcaccttcaaagtcgcaatcataacgacaagtaaaagaatcagaactattagtacgttgagtggttatttcaccgcgtttgctaatagtaacggctggagtagagaagtttttattagtatatatttctactttaccattacgttccttaacatcacgcactttaccatactcggtaataatgccgttctgttggactttaacattaccatttttcatagaaactttggtagatgccagagaaccgaaactaactgtggagatcatcagtgcaataataaacttattcatcttcatcctccccactacaatcacgacatacatcataatcgttgaaagaacgttcgtgagcttcacaccaccaagaacaagaatcgcagagaaacatttcggttttctctagtgcttgacctaaaagatcatcagcttcctcagcagtaatcttcaatccgcacacatctgccacacgttctttaattaaacgacctgcttcgtgataagacatacaggttcccacaacatcatgttcaagaacatgaacagcacagtctagacgagttttcatttcaaacctctctcatcaatttataaatatattatagcaagaaaagagaggtttagcaaatgaattatttcagaatttagtcatagcaccaccataatccacgcttacgcatgtcatgatcgcgattataatcataattttctggatctttcatcacgcggtggagttcttgacgattcccttgacgaaccattttattagaatgccacttaacattcttactaatagaattccagttataaccatcctttttctcattacgaatggttgcttccttcatttcctgttctacatcatcccaggatttagcataaataacacgaatccagtagccattttctttgatgaaagaatattcttgagagaattgttctttagacttccaccactgatcaccagattgtttacgataagtacggctcatattacctccattaagtcttttaaattaacctaatgtggatgaattttgttatacatatattatgtacctttatacagaaaaaccccagactacttattcaatagctggggtttgttattaattacagatcggggcgttcatcttcgaaacagcctgagctaattccttctccgaatcctacaaagccatcaaattcatcatttgagatgcccataatcattgcttccattttcctaatctccgaaattttcatgcctgctttactattcttataatatttgcgagggttcccgcacatccaacaagaacagatgcaaggagtagtagtgataatacctaaccgcttagggctttcttcatgtgggaagactgtccaatacttcttgcggttgttcttcacacgttgccggtgatggcgtcttaatgctcgatccacacatttctcctaaaacttgggagataaacggagtttgctcgactaccttgcgtagctgggagaaatcatatccaaaccccattacatcgcctgagtaaatgtacgactaataacgtcgttctgttgttcacgagtcagtgcattaaatcgaacagcgtagccagagacacggatggtcaactgaggatatttttcaggatgtttctgcgcatccaaaagctgatcacggcttaacacattgacatttaggtgctgaccaccttcgatttgaggggcgacttccaccttaacttcacggaaggcttcgggatcgaattgtggtgtgataccttctagatcttcaactagaactttctgtttaagttcaccattgtcggagtatagctgaataatctgattttcatgaacaaggttaattacgccagacttaagattttgatatgctttcattagatctccctgatgttagaatttggctcagctctttattgtctatagtttaccacgatatacagaaactgtcttaccagtttggttcataacgtatgctacttcatcttcttttaagaagattgcttgatctattccagaaatagctatgcttttatttctgggattaaaccctacgcttttaccaacatgaatctgctcaccaccatcagtggacattattttaactgttaacataattgctcctatatttagctatctctagctcttttaatggtagttagtagtggatttgaaccactgtagtcgctccgtatgaaggaggtgcataaccactctgccaactaactgttatgttttactagactaagtaagtattctttatactctttagaccaattagcttttttaaactttcctggacgcatagtcttaattcctagatttggtactccgggagggatttaaacccccgatctctcggttatcagccgagtgctttagatcgctaagctaccgaagtattagaatatttacatcatacactgtctaagtaagaagtataatggaatttagcttctccagtcttatctacttctacctcagttcgtggtacttgacgaaccacaccatgaatcatcttatagcgaatgcctttagctggttcatgatcttttgggaatacttgtttaaccgttactactttatatccttcacgcggtgttaacactactacttgatcaccttctttgattttccaagaagatggaaattcataggtatatctttgaccaccagtttggaatactacagaaagataacgtttcatttggtttccctctcattaatttatatagatattataacaagaaataagagagaaggcaaatgaatttttaaatttggtgctcccaccaggaatcgaacccggttcagatgcttacaaggcaactgcatcgccagcaatgctttaggagcgatgatcccgttatttcaacgggatttctttttcaataacaggagacttatcagtcataactgtcattgccatttgttgtagaaattcaaaggtgaaggctacacgttcttcaccaatctctacttctacacgtttcttttgtttatcaatctttacttttaggttgtcagccatcttcgggttctcgttgctgtactacttctagccagtctggtagaagaaactttgtacgaaattcttcgtaagtttctttgggataaaagctaaaacctcctttctcatcattcaggataacagaaccgtcagtttgttcatatgctcgatatgtttctccaataatgataactcgcttatcagtacttttattatgaaactcaaaaacgtgcataatgtttccttaaagttggagcggctagagggaatcgaaccctactcagcgaggcttggaaggcctgcgacacaacccgtgtgcttaaccgcttattatttggctggagaaggaggaatcgaacctaccattaacggagtcaaaggccgttgtgctaaccgttacactactctccaagtatttggctgggatgccacggattgaacgtggaaccttcggagtcagaggccgacgatctgccaattgatctacatcccaataattctttactttatgtaaatagggtaactggctcaggttcttcaaggcgcttaccttcatgatctactcgaatgactccgcatccttcgcaaaccacaactgcaccataaccttctttgacttcggcttctgtaatcagaccagataagtcaccagtatctctgccccacatattaatggagcattgtttgcagaaatcagccatattttatttcctatttaagttaatttggggtggctagtggaattcgaatccacataggcctgattcacaatcaggatcattaaccaattatgatatagccacaattgaaaactcgcagggttagcgaaaccttcctcaattagcatgttctagaatactaatcaagttatctcctattgcacgcagctcaagacgagtacgaattttcaattgtggcagctctcagaaactcttctattctagccccagaagcttacccccgaacgcatgtcgggaaagtctttccaagcgcatcaaatagcaccgttacactttgagccattgatgtatcaaggaacagaaggatttgaaccttcacgagatagaccatttatctcaaccgcttttaaggtatatttctaggagtggatgttcctagtaaacctattcggcagtcccgtctaccaattccggcatattccaagaatttttataaaccagcagaagcctcatttaaagcatcaacaatagcttcacgttgggtcattccatacccagtggaatctaggtgtggcaaataagccatccatcccttatctgtttcatgaaggcatgctttaaattttttaccgtccttcattgttacagtaactgttttgctcataatgattccttatagttaattggaggaaggtaatggagtcgaaccatcaccgtatcactacagcgggctagttttcaagactagttgcgtaccactacgccctaccttccatttgtttggcggaagaggagagatttgaactctcaagccgttttaccagtcagccactttccaagcggttttcgtcgccaattcgatttgctcttccaaaaataagatgatgcctctatcacaccaggcagttacgccccgctgggattcgaacccattaaaacagctcaaccgagatagtaggtttaatttactctgaccatcaaatttggtgcgtgacaagggattcgaaccctcaaaacccgacttctaaggacggtatgtatgccaattccatcaatcacgcgtatttggtggaggataacgaattcgaatcgttctgatgtcctcggtgcaagcgaggtgtccactcccagcagacccatcccccaaaatctttagtttactaaggctattagctcggcgtaactacagcaccttcgcttcgagcggaaggaactacgtcatctcgcaaacccgatacactattcagttgccgctgaatctagtggactaatctagaacctctcccgagtcatagggatcgtgctttttggcagccagtcctaggtcgagctaataccttagtgaactatgatgaggatttctcctcatcaatttatataaacattatatcaagaaattaagcattaagcaactgaatttcttatttaattggtactcagtagtggaatcgaaccactgcaaccaccgtgtaaagatggagttctaccattaaactaaccgagcaaaagacgttctataatataggcttcagttataagctcataaaaccctgcgaatatcattgcaatagtaaaattatctatgattactattggctctttaattttttgaatgattaaataaaaccagatagtcatatctgacttcctcgtaatttggtagatcgcctgggactcgaacccagaaccttccgattaaaagtcggatgctactaaacctattgagctagcgacctattagtagccattatatacttctttaatagaatggacttttaagtaaggatgattaatcccaaactccgccattacttctttttcatcttttccataatgtgcaagtaaggatcttgaggtattattacctaaacgtttgtcatttactactaatcgaaatactttcatttcgaaatcctctattaaaatggaagcgggtgcaggaatcgaacctacctctttctagcttatgagactagcgatctctaccagagatctaacccgcaattgtttggtcagtgcggcaggactcgaacctgcgacccgaagcatccaaggctcccacgctaccaactgcgctacgcactgttaattcttttattgtggggggatattaataattcgtccatctacacaataaacggtactagggattgtactgtatatgtagaaattctttatattactctctccgccacagaaatttttagcaaattcatactctttattaatggttgagtcaagtttaaaacaaccagtaagtaggaatacagatagcaataaaactttcttcattttgctttccttctcttcactttataaaatatattatacagagaattaagtaaaatagcaaatgaatttttaataaatttacttattgtgtaggccacctggaggctatgaaccccacggctgacaaagaagtttgcgagacttctcttaaaagccagaatagacccgccgatctatcggaacctacataataagtaaactttatagtgtcattctagacaggactcgaacctgttatcacttgtgcggacttacgagaaccattctttcactcgaatcgaacgagcttctgccctagccaagctggtttccccatcaaccacgctagaatgtttgattgttttcagtgcaagagtccgagtcttggacacgaccgcttcgcaagtacataggcagcttatcatgagtcagca

SEQ ID NO: 5 - DNA, 519 bp, SP15 phage
  source 1..519: mol_type = genomic DNA
atgaatgttgatgagctaacacagcacctcttatctagaggatttgatacagataaatatcattgctggttaagtccggaaggatggctaacagtcccgttgtatgacttctctgggatgttgaggggctatcaaacttataatccttctgctccaaaaggtcatggtaagtgcccctttgaagctaaatactttacttattctactacccagtgtgtatggggactagaaactctcaatggagatgaaaaagtagtattgattgctgaatctgtatttaaggcagttgcgttacataatgctggttatccagccctagcaatgttgggttcttctccaggaaaagcgttattaaagcaactgaaattactaccttttaaattggtagctgtcggagataatgatcctgcgggtgaaaaatttgctagaaaattaaacggctttgtttctcccgtagatgtggatgagatgtctaccgaaaacttgaaaaattttcttgctatgaagctaaatttctaa

SEQ ID NO: 6 - DNA, 519 bp, T5j phage
  source 1..519: mol_type = genomic DNA
atgactgttgatgaactaacagaacatctcttatctagagggtttgatacagataaatatcattgctggttaagcccggaaggatggctaacagtccccttgtatgacttctctgggatgttgagaggctatcagacttataatccttctgctccaaaaggtcatggtaagtgcccccttgaagctagatattttacttattctactacacagtgtgtatggggactagaaactctcaatggagatgaaaaagtagtattgattgctgaatctgtatttaaggcagttgcgttacataacgctggttatccagccctggcaatgttgggttcttctccaggaaaagcgctattaaagcaattgaaattactaccttttaaattggtagctgttggggataatgatcctgctggcgaaaagtttgctagacagttaaatgggtttgtttcccctgtagatgtggatgagatgtctaccgaaaacttgaaaaattttcttgctatgaagctaaatttctaa

SEQ ID NO: 7 - DNA, 570 bp, Salmonella vB Sen_I1 phage
  source 1..570: mol_type = genomic DNA
atgcttaattctttgtataacatcttcataaacttacgcgaagagtccaatatgaccgttgacgaacttactgagcatcttctttcgcgcggcttcgacacagacaagtaccattgttggttatccccggaaggatggttaacagtcccgttatacgatttctccggaatgcttcgggggtatcagacttataatccctccgcaccgaaaggtcacggcaagtgcccctttgaagcacgctactttacctacagcactactcagtgcgtgtggggtcttgagactctgaatggggatgagaaggtggtgcttattgccgaaagcgtcttcaaggcagtcgcactgcataacgcgggttacccggcgcttgcgatgttgggttcctcaccagggaaagctctgttgaaacaacttaagcttttaccattcaagttggtcgccgtcggcgataatgatccagccggggaaaagttcgcacgtcagcttaacgggttcgtttctcctgtggatgttgatgagatgtcaacagagaacttgaagaacttcttagctatgaaattgaacttttaa

SEQ ID NO: 8 - DNA, 498 bp, Proteus phage Privateer phage
  source 1..498: mol_type = genomic DNA
atgttcaaggaacaccttatcagccgtggattcaacccggacgagtaccactgctggatgagtgatgacacgttgacggttcccctgtattgtcctaacaccgggcgctttttgggcgagcagagttataagccaacgagtaagcgtaagtacattacccactcgaccagctacgctttctgggggtgggaaacagttccagtggggtataacggcatctgtttcatcgctgaatctgtgttcaaggcggttgctctgcataatatcggatttgtcgctatcgcagcattaggcgtaaacttgccaaagcatgttaaggacttgttgcctaacaaagacaatgtcaaatacttcttaatcggcgacaacgatgtgcaaggcaaaaaggaaagtaagaaatttaatggttttgagcttgttagtcctgtggacttggatgagatgagccgcaaagacttgctggaatttattcgcggtaactcaggttacttcaagtaa

SEQ ID NO: 9 - DNA, 519 bp, Shigella Sonnei phage phage
  source 1..519: mol_type = genomic DNA
atgaatgtcgatgagcttactcagcatctgctgagtcgcgggtttgatacagacaagtatcactgttggctttcccccgaagggtggttaactgttccattatacgatttttctggcatgctgcgcgggtatcaaacctacaacccctccgcccctaaaggccacggcaagtgtccgtccgaggcaaagtattttacttatagtaacacgcaatgcgtctggggccttgagacgctgaatggtgatgagaaggtggttttaatcgctgagagcgtattcaaagccgttgcccttcataacgcgggctaccctgcgctggctatgcttggaagtagtccaggtaaggccttgctgaagcagttaaaattgttaccgttcaaattagttgcagttggagataatgacccggcgggagaaaagtttgcgcgtaaactgaatggttttgttagcccagttgatgtggacgagatgagtaccgaaaatttaaagaactttcttgcaatgaagttgaacttttaa

SEQ ID NO: 10 - protein, 172 aa, SP15 phage
MNVDELTQHLLSRGFDTDKYHCWLSPEGWLTVPLYDFSGMLRGYQTYNPSAPKGHGKCPFEAKYFTYSTTQCVWGLETLNGDEKVVLIAESVFKAVALHNAGYPALAMLGSSPGKALLKQLKLLPFKLVAVGDNDPAGEKFARKLNGFVSPVDVDEMSTENLKNFLAMKLNF

SEQ ID NO: 11 - protein, 172 aa, T5j phage
MTVDELTEHLLSRGFDTDKYHCWLSPEGWLTVPLYDFSGMLRGYQTYNPSAPKGHGKCPLEARYFTYSTTQCVWGLETLNGDEKVVLIAESVFKAVALHNAGYPALAMLGSSPGKALLKQLKLLPFKLVAVGDNDPAGEKFARQLNGFVSPVDVDEMSTENLKNFLAMKLNF

SEQ ID NO: 12 - protein, 189 aa, Salmonella vB Sen_I1 phage
MLNSLYNIFINLREESNMTVDELTEHLLSRGFDTDKYHCWLSPEGWLTVPLYDFSGMLRGYQTYNPSAPKGHGKCPFEARYFTYSTTQCVWGLETLNGDEKVVLIAESVFKAVALHNAGYPALAMLGSSPGKALLKQLKLLPFKLVAVGDNDPAGEKFARQLNGFVSPVDVDEMSTENLKNFLAMKLNF

SEQ ID NO: 13 - protein, 165 aa, Proteus phage Privateer phage
MFKEHLISRGFNPDEYHCWMSDDTLTVPLYCPNTGRFLGEQSYKPTSKRKYITHSTSYAFWGWETVPVGYNGICFIAESVFKAVALHNIGFVAIAALGVNLPKHVKDLLPNKDNVKYFLIGDNDVQGKKESKKFNGFELVSPVDLDEMSRKDLLEFIRGNSGYFK

SEQ ID NO: 14 - protein, 172 aa, Shigella Sonnei phage phage
MNVDELTQHLLSRGFDTDKYHCWLSPEGWLTVPLYDFSGMLRGYQTYNPSAPKGHGKCPSEAKYFTYSNTQCVWGLETLNGDEKVVLIAESVFKAVALHNAGYPALAMLGSSPGKALLKQLKLLPFKLVAVGDNDPAGEKFARKLNGFVSPVDVDEMSTENLKNFLAMKLNF

SEQ ID NO: 15 - RNA, 88 nt, T5 phage
  source 1..88: mol_type = tRNA
gggggagtattctgtaagtggtagcagagctgactgtaaattagttgtcattgcgactcgggtggttcgactccatcctcccctacca

SEQ ID NO: 16 - RNA, 91 nt, SP15 phage
  source 1..91: mol_type = tRNA
gttggattagtatcgtagaggtagcgaagcagactgtaaatctgccgactcggaagggtctcgggtggttcgactccatcatccaacacca

SEQ ID NO: 17 - RNA, 85 nt, Ec phage
  source 1..85: mol_type = tRNA
ggtggggttcccgagcggccaaagggagcagactgtaaatctgccgtcacagacttcgaaggttcgaatccttcccccaccacca

SEQ ID NO: 18 - RNA, 85 nt, Ec phage
  source 1..85: mol_type = tRNA
ggtggggttcccgagcggccaaagggagcagactgtaaatctgccgtcatcgacttcgaaggttcgaatccttcccccaccacca

SEQ ID NO: 19 - RNA, 87 nt, Klebsiella phage VB_KpP_HS106
  source 1..87: mol_type = tRNA
gggggaatagaccgtagaggtagcgggacagactgtaaatctgttgcctaagaagctcgggtggttcaactccatcttcccccacca

SEQ ID NO: 20 - DNA, 1653 bp, Escherichia coli ECONIH5
  source 1..1653: mol_type = genomic DNA
atgaccaagcaatatgaaagaaaagcaaagggtggaaatttactgtcagcattcgaactttaccaacgtaatagtgataaagcgcctggtctgggtgaaatgttagtgggtgagtggttcgaaatgtgcagggattacattcaggatggacatgttgatgagtcaggaatatttcgtccagataatgcgttctatcttcgccgcctgacgttaaaggattttcgccgtttctctcttctggaaattaaactcgaagaagatctgacagtcattattggcaacaatggtaaagggaagacaagtatcttatatgcgattgcaaaaacgctgagttggttcgtcgcgaacatcctgaaggaaggtggtagtggacaaaggttaagcgaaatgactgacataaaaaatgacgctgaagacaggtattcagatgtcagtagcactttcttctttggcaaaggacttaagagtgtgccgatcagattgtcacgctcagcccttggtacagccgaaaggcgggacagcgaggttaagcctgccaaggatttagctgatatatggcgagtcatcaatgaggtgaatacgatcaacttgccgacgttcgctctttacaacgttgagcgatcgcaaccgtttaaccgcaacataaaagataataccggacgcagagaagagcgctttgatgcctatagtcaaacgctcggtggcgcaggacgtttcgatcatttcgttgagtggtacatttacctccataagcgtactgtatcagatatctcaagttctattaaagaacttgaacaacaggttaatgacttacagcgtaccgttgatggcggtatggtttcggtaaaatcacttctggaacagatgaagtttaagcttagtgaagctatagaaagaaatgatgctgcggtttcctcgagagtgttaactgagtctgttcaaaaaagtattgttgagaaagcaatctgctcggttgtccctagtatcagcaatatatgggttgaaatgataacgggttctgatttagtcaaagttacaaatgatgggcatgatgttactattgaccaattatctgacgggcagcgtgtatttctgtcgttggtggccgatcttgcgcgaagaatggttatgctgaatcccctgctggaaaatccattagagggacgtggcattgttttaattgatgaaatagaacttcaccttcatcctaagtggcagcaggaagttatcctgaacctgcgcagtgcattccctaacattcaatttattattacaacacacagtcccattgttctttctacaattgagaaacgctgtattcgtgagtttgagcccaacgatgatggcgaccaatcattccttgattctcccgatatgcaaacaaagggaagtgagaatgctcaaattcttgagcaggtaatgaacgtacattctacaccgcctggtattgctgaatctcattggttaggtaattttgaactattgcttttagataattctggagaacttgataaccactctcaagtgctttacgaccaaatcaaggcgcactttggcatcgatagtattgagttgaagaaagcagatagccttattcgcattaataagatgaagaataaactgaacaagataagggccgagaaggggaaatag

SEQ ID NO: 21 - DNA, 651 bp, Escherichia coli ECONIH5
  source 1..651: mol_type = genomic DNA
atgagagagttagcccggctggagagaccggagattcttgaccagtatatagccggtcaaaatgactggatggagattgatcagtctgcggtatggccgaaattaactgaaatgcagggcggattttgtgcctattgcgagtgccggttgaacagatgtcatattgagcatttcaggccaaggggaaagtttcctgctctgacgtttatctggaataacctgtttggttcttgtggcgattcaagaaaaagtggcgggtggtcacgttgcggtatatataaggacaatggtgctggcgcctacaatgctgatgatcttataaaacctgatgaagaaaatcctgacgactacctgctatttctcactactggagaggttgtaccggctatcggactcacggggagagcgcttaaaaaagcgcaggaaactatccgtgtttttaacctgaacggtgacataaagttgtttggcagtcgcagaactgcagtgcaagcaatcatgcctaatgtcgaatatttgtatactctactcgaagagtttgacgaagatgactggaatgaaatgcttagagatgagctcgaaaagatagaatctgatgaatacaaaacggccctaaaacatgcatggactttcaaccaagagttcgcataa

SEQ ID NO: 22 - protein, 550 aa, Escherichia coli ECONIH5
MTKQYERKAKGGNLLSAFELYQRNSDKAPGLGEMLVGEWFEMCRDYIQDGHVDESGIFRPDNAFYLRRLTLKDFRRFSLLEIKLEEDLTVIIGNNGKGKTSILYAIAKTLSWFVANILKEGGSGQRLSEMTDIKNDAEDRYSDVSSTFFFGKGLKSVPIRLSRSALGTAERRDSEVKPAKDLADIWRVINEVNTINLPTFALYNVERSQPFNRNIKDNTGRREERFDAYSQTLGGAGRFDHFVEWYIYLHKRTVSDISSSIKELEQQVNDLQRTVDGGMVSVKSLLEQMKFKLSEAIERNDAAVSSRVLTESVQKSIVEKAICSVVPSISNIWVEMITGSDLVKVTNDGHDVTIDQLSDGQRVFLSLVADLARRMVMLNPLLENPLEGRGIVLIDEIELHLHPKWQQEVILNLRSAFPNIQFIITTHSPIVLSTIEKRCIREFEPNDDGDQSFLDSPDMQTKGSENAQILEQVMNVHSTPPGIAESHWLGNFELLLLDNSGELDNHSQVLYDQIKAHFGIDSIELKKADSLIRINKMKNKLNKIRAEKGK

SEQ ID NO: 23 - protein, 216 aa, Escherichia coli ECONIH5
MRELARLERPEILDQYIAGQNDWMEIDQSAVWPKLTEMQGGFCAYCECRLNRCHIEHFRPRGKFPALTFIWNNLFGSCGDSRKSGGWSRCGIYKDNGAGAYNADDLIKPDEENPDDYLLFLTTGEVVPAIGLTGRALKKAQETIRVFNLNGDIKLFGSRRTAVQAIMPNVEYLYTLLEEFDEDDWNEMLRDELEKIESDEYKTALKHAWTFNQEFA

SEQ ID NO: 24 - DNA, 47 bp, Artificial
  source 1..47: mol_type = other DNA
ccaggagaaaggatccatgagcaaaacagttactgtaacaatgaagg

SEQ ID NO: 25 - DNA, 45 bp, Artificial
  source 1..45: mol_type = other DNA
gaggatcgaattcttatgtaaatagggtaactggctcaggttctt

SEQ ID NO: 26 - DNA, 54 bp, Artificial
  source 1..54: mol_type = other DNA
gagaaaggatccatgactatctggttttatttaatcattcaaaaaattaaagag

SEQ ID NO: 27 - DNA, 46 bp, Artificial
  source 1..46: mol_type = other DNA
agaggatcgaattcaatgattccttatagttaattggaggaaggta

SEQ ID NO: 28 - DNA, 47 bp, Artificial
  source 1..47: mol_type = other DNA
gagaaaggatcctaaaatttcagtgcagaacacggggctagcaattc

SEQ ID NO: 29 - DNA, 46 bp, Artificial
  source 1..46: mol_type = other DNA
gaggatcgaattcatctgacttcctcgtaatttggtagatcgcctg

SEQ ID NO: 30 - DNA, 47 bp, Artificial
  source 1..47: mol_type = other DNA
gagaaaggatcctaataactgaggaaacaagcatgtccaagaatgta

SEQ ID NO: 31 - DNA, 48 bp, Artificial
  source 1..48: mol_type = other DNA
gaggatcgaattcttagtttaaccgtaaagtattatctacttcaccat

SEQ ID NO: 32 - DNA, 44 bp, Artificial
  source 1..44: mol_type = other DNA
aggagaaaggatccatgaaaatggtatctgtggctgaattcgat

SEQ ID NO: 33 - DNA, 44 bp, Artificial
  source 1..44: mol_type = other DNA
agaggatcgaattcttaatccatgtcgaaagacaacgtaggttc

SEQ ID NO: 34 - DNA, 49 bp, Artificial
  source 1..49: mol_type = other DNA
ggagaaaggatccctaatatagcactgagcaagttctttaaaatttgac

SEQ ID NO: 35 - DNA, 49 bp, Artificial
  source 1..49: mol_type = other DNA
tagaggatcgaattccgggccgtgtaggattcgaacctacgttgtcttt

SEQ ID NO: 36 - DNA, 45 bp, Artificial
  source 1..45: mol_type = other DNA
aggagaaaggatccactacacgggggtgtaatcgaattggcatag

SEQ ID NO: 37 - DNA, 48 bp, Artificial
  source 1..48: mol_type = other DNA
agaggatcgaattcttagtcgaacttaggagtgacagttaaggagaac

SEQ ID NO: 38 - DNA, 54 bp, Artificial
  source 1..54: mol_type = other DNA
ggagaaaggatccatgctaaattctctgtataatatatctataaatttgaaaga

SEQ ID NO: 39 - DNA, 47 bp, Artificial
  source 1..47: mol_type = other DNA
ctagaggatcgaattcttagtcaattacttttgaggcttcaaggtag

SEQ ID NO: 40 - DNA, 46 bp, Artificial
  source 1..46: mol_type = other DNA
caggagaaaggatccatgacagaagaagtagctaagagtcctgaga

SEQ ID NO: 41 - DNA, 47 bp, Artificial
  source 1..47: mol_type = other DNA
tagaggatcgaattcttaggagttattaccaccattttgagcttttg

SEQ ID NO: 42 - DNA, 47 bp, Artificial
  source 1..47: mol_type = other DNA
ccctatttacataagaattcgatcctctagagtcgacctgcaggcat

SEQ ID NO: 43 - DNA, 46 bp, Artificial
  source 1..46: mol_type = other DNA
aactgttttgctcatggatcctttctcctggtaccgagctcgaatt

SEQ ID NO: 44 - DNA, 47 bp, Artificial
  source 1..47: mol_type = other DNA
tataaggaatcattgaattcgatcctctagagtcgacctgcaggcat

SEQ ID NO: 45 - DNA, 49 bp, Artificial
  source 1..49: mol_type = other DNA
accagatagtcatggatcctttctcctggtaccgagctcgaattcgcta

SEQ ID NO: 46 - DNA, 49 bp, Artificial
  source 1..49: mol_type = other DNA
tacgaggaagtcagatgaattcgatcctctagagtcgacctgcaggcat

SEQ ID NO: 47 - DNA, 47 bp, Artificial
  source 1..47: mol_type = other DNA
ctgaaattttaggatcctttctcctggtaccgagctcgaattcgcta

SEQ ID NO: 48 - DNA, 47 bp, Artificial
  source 1..47: mol_type = other DNA
tacggttaaactaagaattcgatcctctagagtcgacctgcaggcat

SEQ ID NO: 49 - DNA, 46 bp, Artificial
  source 1..46: mol_type = other DNA
tttcctcagttattaggatcctttctcctggtaccgagctcgaatt

SEQ ID NO: 50 - DNA, 48 bp, Artificial
  source 1..48: mol_type = other DNA
ttcgacatggattaagaattcgatcctctagagtcgacctgcaggcat

SEQ ID NO: 51 - DNA, 45 bp, Artificial
  source 1..45: mol_type = other DNA
gataccattttcatggatcctttctcctggtaccgagctcgaatt

SEQ ID NO: 52 - DNA, 49 bp, Artificial
  source 1..49: mol_type = other DNA
aatcctacacggcccggaattcgatcctctagagtcgacctgcaggcat

SEQ ID NO: 53 - DNA, 45 bp, Artificial
  source 1..45: mol_type = other DNA
cagtgctatattagggatcctttctcctggtaccgagctcgaatt

SEQ ID NO: 54 - DNA, 45 bp, Artificial
  source 1..45: mol_type = other DNA
aagttcgactaagaattcgatcctctagagtcgacctgcaggcat

SEQ ID NO: 55 - DNA, 48 bp, Artificial
  source 1..48: mol_type = other DNA
ttacacccccgtgtagtggatcctttctcctggtaccgagctcgaatt

SEQ ID NO: 56 - DNA, 45 bp, Artificial
  source 1..45: mol_type = other DNA
gtaattgactaagaattcgatcctctagagtcgacctgcaggcat

SEQ ID NO: 57 - DNA, 46 bp, Artificial
  source 1..46: mol_type = other DNA
cagagaatttagcatggatcctttctcctggtaccgagctcgaatt

SEQ ID NO: 58 - DNA, 46 bp, Artificial
  source 1..46: mol_type = other DNA
taataactcctaagaattcgatcctctagagtcgacctgcaggcat

SEQ ID NO: 59 - DNA, 46 bp, Artificial
  source 1..46: mol_type = other DNA
tacttcttctgtcatggatcctttctcctggtaccgagctcgaatt

SEQ ID NO: 60 - DNA, 54 bp, Artificial; identical to SEQ ID NO: 38
  source 1..54: mol_type = other DNA

SEQ ID NO: 61 - DNA, 49 bp, Artificial
  source 1..49: mol_type = other DNA
tagaggatcgaattcttagaaatttagcttcatagcaagaaaatttttc

SEQ ID NO: 62 - DNA, 49 bp, Artificial
  source 1..49: mol_type = other DNA
gaagctaaatttctaagaattcgatcctctagagtcgacctgcaggcat

SEQ ID NO: 63 - DNA, 49 bp, Artificial
  source 1..49: mol_type = other DNA
atacagagaatttagcatggatcctttctcctggtaccgagctcgaatt

SEQ ID NO: 64 - DNA, 49 bp, Artificial
  source 1..49: mol_type = other DNA
ttagaatctgctgagtgattttgacacctcctagtatatagaaaatgtg

SEQ ID NO: 65 - DNA, 60 bp, Artificial
  source 1..60: mol_type = other DNA
gcgaccttgagtctagaatttataagatatattatattagaaatttagcttcatagcaag

SEQ ID NO: 66 - DNA, 49 bp, Artificial
  source 1..49: mol_type = other DNA
aaaatctgagtgactatctcacagtgtacggacctaaagttcccccata

SEQ ID NO: 67 - DNA, 49 bp, Artificial
  source 1..49: mol_type = other DNA
atactaggaggtgtcaaaatcactcagcagattctaaagctattgcctt

SEQ ID NO: 68 - DNA, 49 bp, Artificial
  source 1..49: mol_type = other DNA
tatcttataaattctagactcaaggtcgctcctagcgagtggcctttat

SEQ ID NO: 69 - DNA, 40 bp, Artificial
  source 1..40: mol_type = other DNA
gtttcttaccacgagctacagcaggtggattagcttcgta

SEQ ID NO: 70 - DNA, 40 bp, Artificial
  source 1..40: mol_type = other DNA
tacgaagctaatccacctgctgtagctcgtggtaagaaac

SEQ ID NO: 71 - DNA, 42 bp, Artificial
  source 1..42: mol_type = other DNA
attcgtttcagaaagcgagtaccggaagcagtgatttcccaa

SEQ ID NO: 72 - DNA, 42 bp, Artificial
  source 1..42: mol_type = other DNA
ttgggaaatcactgcttccggtactcgctttctgaaacgaat

SEQ ID NO: 73 - DNA, 42 bp, Artificial
  source 1..42: mol_type = other DNA
tacaattagttccctaccatactgaccaccacgaacgttaat

SEQ ID NO: 74 - DNA, 42 bp, Artificial
  source 1..42: mol_type = other DNA
attaacgttcgtggtggtcagtatggtagggaactaattgta

SEQ ID NO: 75 - DNA, 41 bp, Artificial
  source 1..41: mol_type = other DNA
acgcatggagttccttgagttccttagctgaaactggttta

SEQ ID NO: 76 - DNA, 41 bp, Artificial
  source 1..41: mol_type = other DNA
taaaccagtttcagctaaggaactcaaggaactccatgcgt

SEQ ID NO: 77 - DNA, 49 bp, Artificial
  source 1..49: mol_type = other DNA
ccgtacactgtgagatagtcactcagatttttatggtatattttaaagg

SEQ ID NO: 78 - RNA, 140 nt, SP15 phage
  source 1..140: mol_type = tRNA
ctaatatagcactgagcaagttctttaaaatttgacttgctcagtgccttaaaacttggtataatagttacctaatttgaaaacatatttaaaagtgtttaaatgagaatttttgaatacttctaaatatgttggattag

SEQ ID NO: 79 - RNA, 159 nt, Ec phage
  source 1..159: mol_type = tRNA
tcgccagcaaaaataactggttacctttaatccgttacggatgaaaattacgcaaccagttcatttttctcaacgtaacactttacagcggcgcgtcatttgatatgatgcgccccgcttcccgataagggagcaggccagtaaaaagcattaccccgt

SEQ ID NO: 80 - DNA, 32767 bp, T5_8e1 phage; identical to SEQ ID NO: 1
  source 1..32767: mol_type = genomic DNA

SEQ ID NO: 81 - DNA, 32767 bp, T5_8e2 phage; identical to SEQ ID NO: 1
  source 1..32767: mol_type = genomic DNA

SEQ ID NO: 82 - DNA, 32767 bp, SP15m_8e1 phage
  source 1..32767: mol_type = genomic DNA
ggtgcagtgggtcgggcgaaaatacttagtctgctaaccgccacccccgttacaattaccatgctaattgtttcaccctgcaaccattttaattgcagggtgaaacaatttcaactttaattattacgcaacttttaatttctcaatatattgttgcgggctgcaactatattctgcgcgttcttcttcggtcatactttcccaacataattgcaggcggtcggctaggaattgataatcattatcatcgtcgagcgattcatcaataaaggtttcacctatcaatgtaacaccgattgatagaatatcgttaatagcttgcgcgtccagcgttttaaatccgtatgatgccgccgctgatagcacgcctttatgatcatcaatcatcgtaaaatcagcgttcggatataactgtttaaataactcaaaataataagatttataaactgcgtctttgctgtggtatatttcgctaactttatcagcttcaaaatatttgtgcagcgtgtcacgggagaacacgcggatattgctgttcccacgccctcgcaatccttgcttgcgtaggaagtaataatctgacttgctcattagtcgagcggtgcaaataatgtttaaagtatttgcgtcattcatgcactggcgcatatatgtaacaaggggcaataaggaatcttgcattattaaatcatgtttgcaggcttcatttttatacttatttaaatctaaattgccctcgctatcaaagcaaggcgctacacgatgaaacgaattaatgatagtgccgtctaaatcccaaatcataacgcgggaaatatgcgggaaattacgggtaatattcattttaacttgattcattttgttacgttctccatttaagggattagattaattcaatctagcccactaattatattttgttagtgggctatgtttaattaactattagaatgctagaccgaaagcgagagcgtcggcaataaagctaacatcttcacctgatacataggaacgaatccccgcacaagtatatacttttgcgctgatcaattgatcatcgaggcaagcggggcaaggcgcgacaactgcaaaggctaggccggattttacagcgtcgatgataatcgtttcttgtttcaccgtatcaatataaacgcctgcggccttaatgtaactacttgcgcagccttgcgtataggcaaaggtagtaacctgcaaggcgtcgttaaattcgattaaatcatcgacaacgtgccccgcctcgacgtgataacgctcaccattagaataaaccagaacaattgaggattgagcgcgatcgaatggaatattttgctttttcatatttatataactccaattagtttaataaggggtttaatttatttgataataatctgcatttgatacggcgttaattcaccgtttacgggtaaattattatcgcttagccactcataaaaagcaccatcatcatcaaaagggacaatatcgttatcacgggaatcgacggaaataataccatccgtattagttttggcggctaggataggcccgaagctgtaaactttatcagattccatttcatccggtgaaatgaatactttttcgtccaatgttttgggtaatgtaactttcattctaatttagctcctgtaatagcggctatatttcaagccgctagggtaataatttaattatgcaaagaatttaccgttcttaaagtcgatcaaagtacgctgaccgtttgcataggtaattaaatgcgtttgtgtccagcttgacgcgccaacgttgtaacccatatccagactaccagctacgccagcggtatataccccgccgtaaatgctggcggtatgagtgtgccccgtgttcagtttacccaatttcttaaactgtttcggattgccacggctgccgtttatgccattgtgaccgtgtacgccgcattcaatgcctgcaattttaaatgattggtcagtcgttaggaaaatggcgttaaactcgcaacctgcaaccttacgcagcgcataatctagcacgttgaaagtatcgtctttttctgcaatagctccataaatcgcggcattaaggcggtgatatagttccgcgtttgctgggtcgtctttaatgttagcattacgatcatcaagccaacgggataacgccagatcatggttagattcaacaatgattgtttgcgagaaatcgcgctccattgattccagtacgcgccccgtatcgatgagatcatccagaactttatcacgtccggaggcatactgttttgctaggaatacacccgaagcgcggttgtgatggttgcgtgatgtaaagtcgtgaacgtcatggataaactgatattttggtttaagaatatcaagcaagctattttcgccagcccatgacgcagcggcgcattcttcatctaatttttcagcgtggatgtcgccatattgtaaacctaaaacgtgccccgttgtttcatagcatccggcaggagtagcgcaaacattcagatcataaaacacgccgctttcgtccattgtttcaagctggcgaacaaaaaattccccgtcctcatcgaactcaacaatcagcgcaccgaaattatgcagcgcctcggccttttgtcctgctttctgctgaatgtaatttttgagcgttgccgttccggttgaatacatgcggcgcacaatttcaccttttaaagctggcacgctttcggcggtgattttagccgctccaattgccagaccttccagattaagcgcggttgcagtttcagcgaatccagaaagcggataatctgcggttggcaaaacattaatttcagccatgaaagcaaaacggcggttatttaaaaacacgtttttattgcagatatatttatcaaaagcggaatcatatttgattccgtctgcgccctcgccattttgaaaaccgtttttgttatagatatattttgaaacgagcaaatcagcgccgatatatttagcaaattgctccagtgaggctaaaaagtttttatgcgggaaagtattattctgaatcgatgtaataataaagcgtttgccttgttttacttcccagctttccaccgtgctagaaacaatccccgccgcttctgggcgctcatcgtttttaatggcttttgctactttcgccgctttcggtttagctggtttatttgcttccaaccagtcgcagatagcggtcgagtgttttgttgtatcgtagaccgcttttgatatatcgtcgcagacctccagtttagtagcgcgcagacgtttaccatagaaattaaagtcagcggccattttcaggataacggtttgtttttctgcggaaataatcatagtataaaactccattaaagggactaggttaataacggcaatattgccaaatataacgccgcaaatgagtggcgttataatttgcaacattaatttaaaggtataaggctagaactaacaccacaagcaacggcggcaataaaacaaatcagacctaaacgctttgccaatttagacttacgtttaaaataatatgaatctaaatcattttgaaaataagcgaatagtaacgaggccgccataataaataagcctagaatgagggattcagtagggtaaaagatcattttaataactccagtcaaagggaaattatagtggggaatattccccactaattaaatttattcgcctgcggcttgtttcacttcatcggcaacgcctaacagttgcgccacggcgtccagcgtttccagttttgcgctttccagtgatgccagatcgtcggcgtctttgataatgccggaatcgatggcgtgttttgcaattacgcgcacataatgcgctttgcggattgagctaccgccgccaactttgcgcggcttatcgcttttctgatacgctttcgcgctggtcaattttgagcgaacggacacgggagaagccgcgcccactgctttcgcgatctctttcaggccgtcgctatttgcgaaatctaaaccgttttcattaattaactgctggtacatggtaacagctttttgggtgttttcttcattccatgcaaattttgcggatttttcggttttaacgttagccatgattgtagctcctattagtttaatttaagggataagattaacataatgttaatcgttatataccccgaactactggggtatataaagttaacactaaattataaaacagcttcccatttttcgttacgctggacaacctttacaacgtcgccggatttaacgcgaacgctaaaaacggttttgccgttgttactacgttccgtttcagcgtataccgcgtcgattgtatcaaatggcataagcgccgcgcctttaatgcgttcggcctttccggttaattcatccgttttagtaacgaaaggaataaaaacggattgaccaattttaggcgtggtaataatgttttgcatagtataaactccaagttatttaggggattgttccgcattacctgctagaaagtagcaggtaataagcaacaatccgctcgccaatataatcaatttaaagaactccacgcaggccgctatatcccagttagggggcggggcacattatggtaagtgccgaccgtcaaattttatcaaattatcgctcttatcgaactgggtacatcttaaagcctatcggctagggtgtcaaactattttttgcagttttttatggttttccttcaggtcgatcataatattacgccagatcatttccagaccttgctggcggcctttcttgtactgcgtgaatcggtattttaccgatctttgcgctactgtcaacaaattttttgttttgctatctagtgccttgctaggcttgccagtgatcaataaagtttgtttcatatcgtcgattccttataatgtataagtttaccgccgataggctttaagatgtacccaatttttaaagagcgcggcggtaacttcccgccgtgtagttcgtcattgccgtcctacgtgataaataataggggattcccgaaaatggcgcaaccttatttttgtaaagaaacgtaaagacacgattcaccgcacgccgtccggcggcatgggcgcggcgcactaaaattaaaagaaacgggcgcgcgagtaccacaaaacagagcaaataggcaagtaattttttcatttatatttgctttgccctacttgacaaaacttaaaaagctcgtggtagcgataaacgagggtaggcaatgcaatggcacggctaaaactttcatcgcgttctagggcgttttaggcgcattctagccttgttgataacttatccccaaaagcaaaaatgaaattttcctagttatccacttgacttttattttccagtggataactacttattttatgaaataaattaattgacttttatttgttagtatgcatcggaagaatagcagactaataattactagaataataatcatgctggtggattgtaacggcctaaactatcagcagactattaatcacgaaaaatctcgttagctaactaactatttcatgatgtataatatacatataaattaatgagaaataataattataataaataataactacagtaaataataactataagaaactatcggcctaagtgagaaccactatcatttaagttatccacaacgttatccacagcacaaaataatttgacacgataggcggcgatataagggcttatccacagacttatccacaggttatcctactgtataaatatacagggtagaaaggtagtgttaacaactgcaatcaattttaagcggcctaaaacgctttctaacgagctaaatgcggtggggtaatattaaagtaaagccttcacccgtcgccctggtggcttcgccgtgttttgctctttattgcaccgctgcgcggttagcataaaactaggcgctaggcaaggaaaataaaaaggtaaaataatatttgcctatgttagaaaattacctttatcattcactcaccgattaacgagggaggccgaacaaatgaggctatataaaccagataacgcaaccgtcttaaaaggtgcgctgcgtaacctgctggacggtagcagaacaaccagcatcaaacattttgttttcaatattgaaactattcatcaaaacttttttggtgattatgatgcttataatatggatagttttctaccgttatataaacaaggggcaacgcttgttttatataatcaggaatctcacttgcttactagtcgagggccagatactgattttattttagtaaaaggcaacacagtaaaagcctatgatgcgggggcgggcttagaagttttcacaatagaaaactatgaggctaatgataatgatctttatgatgtagaaaattttctcgattcattttggcgttatttatcagttggatggaatcgatcagattatgacgggtatcgttttgcggctgtaatggcttttgatgataacggtaattttttattaccatcggaattatacccgtatgtgcataatgagctagtacaagaagcgggttttattttctggaaagatgaagatcagattattgacagcgtagaaaaccatgctgtaaattctaacactcaaagcgttaaaactcaaactactgaaaacaaaggaaaaaacaccatgaccaagatcgctaatattgttgccgctaataaatccgctgttgtaaacgctgcaaaactggaagcgggtaaaattgcactgactcaaattacgaaagtagcggctaaaaaagcaccgtttatgattaaaggttatattgatacacctatcggtcgagtagtgattgccaacctgctgagcgtagcggttgaccagtacgccccaagtaaccaaaaggcgaaagcggtggcaggtgcagctatggaagcggctatgttagaaatggtgcaaagttttaacatcgctgagatgattgatgaaatggtaaaaggtattgatatttctacttttaccactagcaccgaaagcgagtaataatattaagcggggattgttaccccgctttactattcccttgttaactaataggaggctaataaatggcggatgaaaaatatggcttctcactgggagaagtgagcacggcaaaacatgatatgatcattttggtcgattgtcatactggctattgcggggaagggaacaccgaggaatattttgttcctactggtacggatctggacgctttcgctcaggaaatggctattgataatgcctctcgttttggtagcgatggttacgaagacgaagaaactggcgaatggtatgataatgaaaacgtatatgcaagcctttatcattatcaattaagtaaatccggcacatatgtaaacggcggcgatcctattaattccgtcatgagattaattattaaatatggcggcgtcgagataattgacaacaaagcggtaatatatgcaaaccgattaaaacagcttgtttatattcctgatagtacccgatgggatgaatatgctgttttgcatgacgaattgaaacgatgtttcaatattgaatccttacaagtagtctaatgtaaagttttgtaaaggtcgccttttatggtggccttttttgttataatgcctttacaccgtttgaggacggttgaaaattttcccaaaaattggaggcttaaaatggttgcttactcttctgctagtcatctgttcaccgctcaaggctgggtatctaaccgcgttattattcacgaaatggtgcaagaatatggcattgctaaaacttacactaccattcaggcgctttatgataatgatcaaatcgatcagcaaacggctggctttttgctggataccctgaaagcagaacattgcaccaaaaaacaagcggctaaaattgttttaatgtaattaataacgggggatattatatcccccgctaactaggaggatgaaaatggttatttttcgagctattctggcgggtatcttgggcgctattttatctttatttgcaatagctttcgacgttcacgcggttattatcggcgcgggtatcgctgtattttcttatctgctgggctgcatgactagtaaaggagaataaaaatgatccgcaacgtttcccttgcacgttcgaaaggctttaagctggtggacgttaacacgttcgagcgtgaagattgtaaaatcgaatatgtagcacgtaataagaatgcctttcgtgttaccgagaaaaaattcgataagcgcggcaacgtgatcgctgaaacggttaaacactttgccaccttttacgctgcgtttcggggagtgttataaaatggtaatttatgaaggtaatcgttttgttgctaattgccgtccggcattattagcaaactatttaaaccagctttcaccagcttataagggcgttattaatatttatgagggcacggcgcattataaaatcaatgcggtcgttgcccgtgaactagcgtttcaatttttgacctttgcatcttgtgacgttcaggttatgggtgaagcgttaattgcagaaaatgaagatgattttattaatattttccgcaagatatgcaccgagcgcctgataatgaaaggcgcgtatattcaatccactgcggatagtattgaaacagcgtttcgaaaggtggcgcaatgagattatatattttcgcgggtaatgttgaggctgcaaatgattccgctggtggcgataacgttcgtcactactggcaaaaatatatttactaggggttattatgagcaataaaattattgtgaccaaaactaccacaacggttgacgttttttatgtgcctgatacgccggaaaaccggcaagcggtcgagcggggcgaatatgatagcgttatttatgatcacgatggttactaccaacatttggtggattcctacggggaggaggaaaaaatcacgcatcaattaccggactgacaacaagcggggatctgctccccgtttttcacgcctccagttaaatacctctttgttttagtatccccaccaaaattaaacgcgtcagaatgcgatctaggacgttttagcggtatattagaattattcactacataggaatactgtatatttatacagtaggataagctgtggataagtctgttaataacgcttcaaaatggctaggattctgtcaagtcaaatcgtgctgttaataagtctgtggataacttaaataacagtgtttctcacttccattcttaaatgagaatcattatcattcgcattccactgtctaaccgataatcatttcactttttgaatagttctcatttcacttcttaaatgagaatcattatcattcgcattccacttcttaaatgataatgattctcattcaaagtcgcagggcaattgccctgcgcttttgtgcaaatccgacatttgcccccatggattacgcgtgggcatgtatgtgcaaatccgacaatttttggtagtgtgcaaatccgacccgaaaaatttttatagtgtgcaaatccgacaatgaattttcccaaaaactccagcaatcacgaactgcgttcgaatcctgtggaattagctagaatatgtgcaaatccgacatgtgttgaggtgtgcgaatccgacaagatttttatgacttcgatgagaaggtgtgtgattgtataggtttgaggaaaagatgagagagcgagagaaattttggggctagaaggatgtgggcgcaggattggtgcggagcacctgatttgcaggtattttgggggagagttgagataatttgggaagatttgagataggtgcagaaaaagtaaaattttattagctaaatggggcaaaatagcttgacaagtgaaaattcttgtggctctaaaaactcaggcaatcacgggccttcggcccgaaataatgctgctattttcaggagagtaagagttcctaaaaacttaggcgtttgtgcaaatccgaccataaatttctagaaacacaatgtgcaaatccgacagtaaaatccagaaatgtgttttcaaaaaatgtctcctagaaataaccgccctccctataaccgccctatattaaccgcctattgctagagtttctaggaacaatgaaaaccgcctgagttgactagagttttcctagaaacttaggagtctagaagaaagtgttgtgccatcctagtagatgagcggcaacaggtgtatcatcttgaacacagatattgcctttaaaaatatttaaataatataaagaaaaagagacccccaatttcatgagaatctctcctgggggcgcgtgattaattacgtgagtactcatgccgtcataccgctgttgctaggccgcaagctatacgagacattcgtgtaataatcatcgcccctagagttaatcaactagagtagttgttaatctatgagattattataacatgtttgggtatgagaatgcaagaactttttgttaacttttattcctccttcttggatttgagtttgatgcctaaggatgcgaagtagatataagttgctaaataggaagcagtggatcctgtatcatcgtaatccatagttccacgagctgctctagtatattcaggagcatagtttaatatcgtgtaacttggcattcctagcgacttacatagttctttaaatgtatcttcgtatttatggcacatgaaatgcacagcattttctaatggcgttaactctagatctttatggagagctacagtcaaactcgctagcattgtgccaatcccacgataaacttcatctttaactagagttggtttctctttttctagtggaggaaggtgggcatatttcccatgtttgaaagggataagatcttcgctagctaatgcttctttaaatgatgcttccttaaatcttgggagatcttcatcgattaggatatgaatagcattagaggagaaaccttttgcttcaggatctaaagctttcaacgctttattcacttctacatatgagcctgaccaaactacttgttttgcatctcgatcatacttgatcttacctttatcccacctagcaggataatgatctcctaaaaacattactgcatatttttcttcctcagttagctgggaaagactcttttgtgtagcaccacgcgctaactgaatgagacgttttaatttttcagcttctttaatcatatatcagacgcttgctcccctgtttctttcttttctgtcttaggttttcttgcaacttctccaaaggttcctttggttctttctttagctggaagatctactttataccataggattcctaattgttgcgctaaatgggctatattctttggtgttatacttggaacatcttccctatcagaaactttagaaattatatcaagtaactctcctatttttggcttactagtagttattagaatatattctaatgtttctatttctacattttcatctttatagtaaagactaagagtaattaaatcgtcaccagcagaagttatttttgttttaccaaatatcattaactacctctcttatcttcattaagagcagctcccaacgcttcaaggatagtatcatttatactcccaggcctaagattattaaagtgagtaacatagatgggacttctaaaaccctcagcatccgcaggtgctacgcttcgcatatcagattcaaaagcttcttgagtatgttgcaactgtacagaagggccgtaatcttcaccaactcgatatgaggaattattttctataacgccaccacatggaacattgtgcaaatccgacgttattttaggattaaatgcgataccacttttggtccaggaacctccaacagtcacaggagtactagggcggttcacctcagtctttacgagtttataaccagcatctattaatgcgttaataaggttatcagctggaatccgagccttgccaaagatcttacgagcttcttttaatttatgctcaagatctttacaggctttaatatcagtgtgcgcaaaggttaatttcatagatttgaactgtacagtggcagttaagtctttaaaatcataatcccatgtatttaattcatggtctggtactacttgaacaggttgttgtgcatataaagtcattacttattctccaatttgtctagtagcttgtgcgctgctatgttatattgtttaagttcacgattaaggatttggttttcacactttagctctagattcttattattaagaatattgcagatcagtagaagtgctaatataactagcaaggaacctacgagcattaaaagaaaaagagtttccattatttaactcccatgtaacgtttgagatatatgatgaagtcttctgctgtatgctctacgctaccttgagctacaaatagtttgagggcttcacgttgtagtttaagagcagccaactcaccacgtaattttattagatcttctgctagttctttagctctgcgcataatagcaaatgatacaaatgttacaataaataacataactgctaaaataattactatgatctccatattaacatccagctcttatcatatatttgggcatgttctactaattcatttatcgatgtagaattatcgtagataccctctagtaaacgttttctgtcaaatttatcaaccaaatactctgtgccatttatcactaccctatacagctctggaactaaggggtgtttgtttggtattgggcgactacctaagtctatttcattatatccccacgttgttttaaatagtttgttgctaagtgctgctagtgggtttgaccatacaatatagctactcactacttatctccattcttagctttgaaaacttattataccaaattatatgattatcgtcaattacaaatttatggtaacatgctggtacggtataagttccataatccgtgacacgctgcacaaccttgtgtgcacacagtcgacaaccatgcccttctaaatgagatctagcagtttgccagtaataaccatcgtgatctggacaatagatctcgacttgctgttgcattgtcttataatttacacgctcatatccgaagaaagccccgtgagctgcaacggctttcttgataaatataaggtttagtgcttcttgctggaagtcgggatgtagctgcttaatcttagttctattaatagatccatccgatttaatgaacctatttattggaaagttgttagcttcctcgattaataattcatttactttctctctcatattaaatagtctcacagttaaggtagaaacattcgtaagcatctccagtaaactctttatcttgtagtaaacacttagcttggtcttccggtactccagcatctaataattgttgtttacttggcttttcagcgaatacttttacaaaatactcaccatcctgattatactcatttatatctctggtaaggacatatacttgcatttgaagttccttgaaaacataaaaggccagaacaattaagtcctggcctctagaattaatgaagttgtttaccacttcgtaacatagtggctgtttccataagacctagcgtagcatcacgcttattgatctgtttaccaagttcatcggtacgtttaccaatgtaagcgttaatagccatattcatagctgtagcgagatcttctttggttatctcttcatcgtctaaggctaatttagccaaagaatcaaatgtgctagagagtcctataagatctgaggtttctccagccagaataggattaatattatctactgttacttctagcatggagttaacaatatcttcaccatctattagaccagattcaatattactctcccactccttcatctgctccaataatggatttttcttttctgtcatggtagaggtttcctgtgtcagtcggtaagaaggatgattgagctttaggcggatgttgtttagcaatccagctaagaatcagtacacgactaggaacaatatcagtgttgtaccagaaatcatgaacccattgacgagcattctcaaacttaccaaatttatatgctttcttaaacaattcaaacccaaaacaatctggtgtaaagtctacttcacgatattgaactactttagaaccagttaggtcttggatcgctgcattaatttctgtatgcgagaattttgtttcgtgaaacttattaaagaatcggtagttgaagcgtccgttcgtttcgacaaacaactggatgaaaagatcgttaaattggttatcaaaccagtaattctgtagttgttgtagtgctgtcatttacgaactccgttaattgccacgatgatgccttcatacataaaaggaagtagttcagaagtgtagaagatattttccgttattcctagatgtcgaaaaagtatattaaataatgctgttagaaatacaatctggggcagtaatacaaaatactcagttacaatctttggtgcccgataaacaagacgttttatcattgtttttaagtctccttattactttggcctgctccacaataatgaaaactgcggggctaatagtgctattagccccgcagtaattggtactaaatcaatcatgggagacgccatacgtaattagctgtctgtagaaccttaggtgtgtcatcatgatacattactacagactttggtgaatagctatcagctagctctttacgaatcatcttacattcttcaccagtatcgatatttttaactatcactttcatattaagaggtgttaatacagaaagcggtttccagaagtcctcaatctcaattcctacctttttctcgattaccatgaggacttctagtgtatcatctggaatactaatattattattcacaaactgtaatatctcatgtaaggtatttaattcattaaaattaagcttcatctttaagaatatcctcaaccatatcacaggactgttgcaattcgtcagcaatgcgcttaatatcggtcttcgtcactctaccgattaacatcaccagtaacatagaaagtataataagtgggactggaataacaaataaagctaccttaacaacattctttggcgtccatgtgtggtacttggtaaccagtacaccaaccacaattagataaaacgctagaataaacatcatcattttttaatctccgtaattatctgtgcacgcattactttattaggtaattttgtattcccagctattgcttcaatattatttagtttttcttttagaatatctgagcgtctctgtgctagttcaatatcttgttcttgttctattaagcggcagtgaagtccactattagtagtaagcatactctctatattttttcgcatgcttacaataccaataatcccgccaatcgctactagtgtagtaagaactagtaacccaataagaatttcaatcaacattaattatatactcccttagtccttatttcttacctttcagttgcttaacttcacgctcaaaagatgctgcacgacgttcggcagtcgcttgatgctctttagcaaaacgagcttcctgttttgcaaggttgaacgccatagcattcttattcagagaatcatacatctttttcatcgccggaatagacatcttcatgagctgaccctcaaaaccctgcatgtcgaggagaattgccagaacgttagccatttcgtttttagtcatgttttccattagaatttcctctctcattaacttatgaacttattatacagaattttaaggcttaaagcaactgaattttttaattacttaccaatcgttaacaacgccggagaactcagaagcaaaaactttttcaaatttctctgcaatttcaggatgatctttgcagatcagctcaatacatgcttctggagtcattccttcatcttcaggatcaccatagtatttatcccaaagatcatcgggaatgatatgctccgccaaatcttggaaagagactaactgataacgttctgcctcctcagcgataagaatttcgcatagatctttatctatatcgctacgataatccgcaattaataaggcattgcaagcatgacactcccaaaccatcaagcgttcagaaataggattagacttatcctgtacgtaagactgaaacagggttcggaaagttgccttaacttgttcaaacttatctgctgctgcgaaaactagagctttatcaactttgttcattttgattccttctcatcaatttatacagtaattatacagaaacttaagcattttagcaaataaaacttttaattaaaatgcctaatcctgtgccaatagcaatacaaatgattataagtattgctatcgcctgtatgattcgtttaataataacctcagctatatacttagacatttatatcgccacgcaatacagcagctacgtcttctcctatttgtaatacctcgccggtagtacaattaaccactctatcgtaactagtaaacttaccagacacaatatcctctagtggaattggagttctactcatttcaaatgagacattaatataacgtgggtcacgtaaagaagtagtatgtacatgtccgtgaatatttagtttgccacgaagttcattgggatgcaaagggcagtgagatagccaaaactttttgccacctccagtctgtttgcctagagcttgaatatcgtcataaacttccgctaagtccctaatactcagtccttgacgctccgcatcatgattacccataatgagttgattagggacattgtggataaccgactttaatttggccagaccttcacgacctactgcaatatctcctagcaaaataagttttgttcgtttaccaatatgcttggacaaagtatctagaatatactcgtcgtgctctttcatgttcttaaaccacggacggaaacgtaacgctccagggtggtctagatgcaagtctgaccagaatttaactttcattactcttttccttattctgtattaaactatcaacccaagaggttaacactttggttttaaactcctcgggagtctctccttccttaaggtctacctcattaaggtaggtagtaagccttgtttctatatctatttcagtaggagaattaaaacaaaaattgactgctattccagaatatattactccggtatctcctttgacgaaagcattaactaatgccctccaacgaagggcatcaatacgcattgctcgtaattcttctcgtacttctttcattctatcattcattaaagagtcctctgtacaccgcagctattatttttgtctgtggtaaatgtggtgattttgccagtttcatcattaacttgcgcaaccgtcaactgcccgttgaagacaccgccagtatctaggtaaacacggtttttatagagaagcgggtaaggtactccagtatgcccatggaacacaaagtctactccactaactggaggtacttctaccatgtatttttctttaaatcctgcataacgctggaaatacgagtgttcctcgccatttttagacaaatggaagcctatttcttggattacatctcgatcccataagtatggttcaacatggtatccaggatggtcatgcgggtcttccttagctgcttctacttgtgcaataaggttatcccatactggggtttctacttcgttaccacattctttgtacgtaaaaggtacaccaccatgaacaacaccatacttcttaccacgatgtctaacagttaggaatactggcattttttcagccatgtcttcggcaatatttttaatggtatctgcatctagctcattcatagcccacataccaccgttatacatccaattagcccaatctcccacaatcataaactggtcgtggtttccacgaacgctacaaaaacgtggattatataagaatttagctaaaacttgtaggttctgcgtgcctcgatcaattaaatcccccacgcatataacgcaatctttcttgccgttatagccagctaattgtagggcatcttctagcaaatcattgcatccatgaatatcgccaacaaagaataagttaacatcatcaggtactactagtgttttatgcacattaaattcttttttcataattattcccaaataacatttaaaatagttgtgccatattcattagatagttggagagtataaccctctttattgagggcttttatagcttcataactaatttcgtcacggttaaactgcacataagaacctccaatctctacagaagatactatcctccgcttaacccatctatatgttttctttcggctcttaagggacgcggctctatttatcctagctaaacgttttgcttgctctgctaacatttaatcctcctatcaatctatacaaatattataccaaaatttttagcaaaaagcaagtaaaataaaagcctgatccgctaagatcaggcttggtttattaatcctctggattatcatccaggaaatttttaatagcttcgtgcatagtttctttacgaagctgacgtccaatcaaaatatgattagcttctattcgaccattaggtaagcgatctgccagaactactacaggtacttgacgtacaccaaatttctgcattaattctgtattatcagtctctttatggatttccaaattatagtcattgactactttatcaaatactggttcgaaaagtttacatgggttacaggtggaaccttttaatagatagactaatttagacatttttatttcctttgctggcaaactcaccgtggagttcttctagtttttcatctctccatgcaattgcttcttccaaagaactgcacgttttcatataattgattcctgctctagagatttttactctaaaagacttccctctttgagatatattttttaatcccaataggttatttttattagccgatttcctattaaaagcattttgagcttttgtagcttctcttaagttaccaatacgattgtttagcgtattggtatcatcatgatctactatatcaggtaaatagcctttgtgcataaagaagattgctctatgcgcaagtattcgttctccatcaatagagagcattagatagccatcagcattaatagacccagcaggcatattgttaaggctagtattccaacctcttgtaccttccggtctaggtttccaggttagagtaccatcttcgtggtactctaatacctctaataatctctccctagtaatcacaatttattaatggcctctaagaagtttttcatagtttttacggttgcggtgctcagatcaagatttacacccaaacactcggttaatgcttcctgataaggagcctttaatctgccttctgggacttctaccttcttatactctttatttttgacctttttaatcatagtctctagtacaagaagcggtaatttagcaccttcaatatcagtacccaaaagttcagttaaaattttattaagatcaagacgagttaactttttgcccttagacatagatgcacctacctttgtatcaatagatttttccgctttcttttcgagctttttgtactcaggagagtcatgatcacggagtgcaatgtttagctcgtaatgtggtatacgaaaatgttccgccatttgagtgtagaaacgatcagacataatatatacctctcttaactaatttatgtatatattatataataactagggctaaaagtcaactacttttttatcttaatctactgcatgtataaatcttttcctaactagatacatagttattgggtaaattgagtacataagtatcggggagaaaagggtgaaatacgctgtaactcccccagctaacatcaaaggtattaatgctagagtaagggccataagaatcataccgaatgaaacagccagagctatggatataggattctctagttccatccataaccaacaatatttcgtatctctatggcaattgcatttacaaacgccgaatgaacccataattatatactctagtccgtgaataacctttattaataagctatttcgggtagttaatgcaatgatagtaaagactatcattaaaacgaatactactagacttattttccagatacctagcagcatcatagtgaatagttctgcaaacatggctttctcctatcttcaaaaattattaaagccccctttgcctaaaaaggcgggaatattcccgcctaagttattaattaaactagttcgacatgaccgccatcataggtaccacgttttatttcatcgtgatagtctcccgaagcattccaatcagcaccaaaacgaagtttaatgcctagctctttaccagcttgttcaaaagcctttttaactgcccaaaatgcttctaagtcattccaatcaattttgccattaatatatggagcaaaatcaatagcatccccagtaatatgtttgcttttactaggatcttttagaaatgaagtaccattagcaatgttctgggcactttgtgctactgtacgaataccttgcacgattgtgaaatcatacggagatagttctaaagccctacgagctactttttgtagctcgggcttaacggtagctaattgtttttcactatttttaccaaatttaaaactcatattgatctacctaaagatctctgttgtggggaacagagctttgctaaatattccttgaactgttcagaatcagctgtatctaccggattatctttccaagcaataccaatgtacccagcatagatattttttagattgaagtatggacaagtgtatatgtaattaaaagtaacgtttttaaacgcaggtatatttaaccccatatatttatttactcttacacttaaatccgatgcgtagttaaagccctctaaatgacgtctgtataattcagacgttttatttaccgctttatcggccaagtcagccctatctaattgcgcattactttcccatgcaataatattggaataatcattgatagcatctggtttatacttgactacaaaaacagcatctgcacccgtttgagagaagagaaccatgctcttttccctcgccacattagggaagttatctatcctctgggtttgtaaatcttgtaaaactgcagacgtggaaaaagtctttaagaatgacatcacttcactagtattactaacaaataagaaaataatgacagcaactaagatagttagcagacgtttaagaagcgatgctggatctttcgcttcttggagcagtaccgttaataattgtaagaacttttccaattgtaacctcctctaaccagtaccattatactaattttggaggaaaattacaatgtgtttttaaagatcacttctggagcataaaattttgtcgttgtcaagaagaattttagataaaagaaaagccagggtcgttaaaccctggcttaaaattacttactcttcgttatgctcctcggattgaggtaactgggctttattatattgctcagatcgatattttgccaagatttcaatacgcttatggatttctttgctatctagatagatatttttgttgtcttttaccatctcgtcgatttcgtctatagagaagaacggatagtagacatctagcatcatatcttctacgaacttgttgtaagattcataggctttcttgatttcttgacccttctcacagaatccgccagagaacgtgtgtcccattagcgtagcatgtggatgtactacccatccatgacaggataggaaaattgtgcagtaagcagaagcactaggaccaatcaggtgtcctataactgttccacggcaattagcaattaagttagataactgtgcagcagtatcaacataaccaccagggccattaatcatcagattaatttcgtcgtcctcatttgcttgcataagtaccattgataaatcacggtattcatccggcgggcctaattcttcatcaaagaaaaaggtatactcattagactggcgaatggagtgaaacaggttagtcttttcttcttttttattagtcatagcgatccttgattatccaactagtggttctagctctaagtcacagaagttataaacttctagtttaaggttattgataccatcgaatttattaactaattcgtgagtaatatattttgcaggaataccactttcagatggatgatctgatttaatagtgaacttctgctcagcgggtactacatttactatcaaagaatccatatctaaatggtttgtttctctgagtaactctccttcattggggaatctaacatctgttattacggcgacatctgggtcgtctttagcgatggattgctccagaattatgagccaaatgcgttcatgtaccagctgccttcctagctctgttcctacgagctgtaacatttttctcggagaaataaataaactataaagtccgtcttctttattctctgagataagttgttgaggattaagatatttttcctcaaaaatcggccaaacgtacgagaagtcttcaaacttattgataccgtatttaaaccatacgtctctagctcgctccaattgagattgtgtgaccgtaaaccattggtcaatctctttccccctgcgctctcctagaaactctggagttacaccgaggattacggatgcaagttcataaacgggcttagcaaaactataacgacggggtaaacacgttggatacgtgtcattacaccaatcgataattaattttgcaacggtatcttttcccgaaccagcttcaccatgtaaaccgactaatactgacattaatctttcctattgttaattggtggataatatactaaacaacgtttttcttgcaaatcttggcggtagaagcaaaccatactagtcagtcgtgagatatatgaatattctgcctcacggcattttgccaacatattccaatctttgtatggtacaacaactactacgccatcttccccatttgtagctaatttcttttcaaacttaaagtcaaagctacaaggctgaagtcctttaggccaatccacatgggcttgctttaactcatgtgacggctctggtactaccgtttctgcacagcctgtgattgtgattgcggctgcgagcagtattccaagtttccagttaaacatgctaatctttcctcgaactccttactctgctttttagcaattaatgtaaccaatccaggctttgcagctataatatcttggcgactaagagctttgtctaactgcttaatctttttgtctagatctgcttgcgaaatattattcattgtgaaatactgattcattctagtctcacgaagttcgctttcagctttcaccttattgagggaagtctctagagaagaaatctttttagtagccaccgcaagatctcctgctaaagtctccactttatctactaagtgataagcaccgaacccgatgcctatcgctagacctgctcccaggatatacatcttgttattccaaactaagtctacaaaccatttccgcattagcctgtactcgcaaactcaccgtggagttctttgagtttggtatcccgccattttatagcctcttccaaactcttaagtgttttcgaaacttgcttaccatgtttggtaattcttacttggtaagtcccatttgtttttctatggatatttttaacgcctaaatggttatcgcttcttactttttggttacaagcattatcagatcttgtagcaggccttagattctcaaatctatcattagttgagtctttgtccttgtgatcaactatttcaggccattctccagtatgccatgcatagattaatctatgtgcccctatagctatggaaccattatatagttcaactactctatgccctgtactttgtctagatcctgctactgttccggcgaatatcttattaaaatgttcgtccccttccctgggtttccagataagattaccatcttcttggtaatcgaacattcttcttagctcttccttactgatcatcttttcatattcctaaaagaagtaacagtatcaaatccatgtgcagctaagcgatccttatcggaaatcgtaatagtatttggttcgccggttcctaacacgccccagatatattgctcgatcatctggtgcaaacggtataagttactttcaatttcctgccacggaatacctgactgatggaaacgaatgttagtctgaatcacgaagttacgaacatcatcgttatcgttcttcttgatacctttcacatatgcaatcggtacacgcagttcggacaagatacgttctgctttaggttttgcttcaacgagcaaatcacgcattgtttcacgaacatctccgcgactcttatccattaagtaagagcgagcatgcaatcccatctcttccattttatcgaacatagtgtcgaggttgaacgttttgaagctaaatgctggatgccagcagtacagctcgtgtaaccagtaaacttcacctgcaacaaatagtgggtttacaaaatattcgaaatcaccacggaaagatagcgaaccatcacgaaatacctgacgactatgcacgatgttcttttctgcatcatcagttactttaaccagtagctcttcagttttacgctcccaaacacgatctgcatcaaataaactgttctgcaaatcatatacatcggcgaatttagaaatgatcctcatatttaatcctcttgcctcaatctataaacatattatacaaaagttgggcatctaagcaactaaaattttattataaaaatagcccagtcgcaaaagtgcaggctgggctttgtcattatttgcttttgctagtaagctgacttagtgtcaatcttatgtaatattagtttctctagctttgcgtagtacccctgcatttctccacaatttgatgtcagcaactgtttctttataaggagctatggtaaaacctagtgggccagcactaaataatcctaagaaccctacaatacgcatgtagaacaagcattctttggctgtcatattatttactgcttttttctgcttttcatctttaaacttctgttcttgatcaccaatacgtagatatttaacaaaccattcagcagaatgttcgtccaaatgtctaataatagctatcgcatatccagcaccgattaaaaaccaagttgcaacaagaattagtaatatagtcatattatctccagttagggctagcagccacctcaccacttaccgcactaaggggcacgactcccttatccgtaacagttgcaggtgacgcaactcggtcctacgcgagttctttaagtattctgcatttcagctttaaattttttcatattacgagtttttctataaaagaaaaacacagatgttgggcctagaagaatatccacaataaatatcacagatctagcacatctgagtaatgttttatcatcaagaggtggcagatctaacggtcgagttttatgtataacgtataatattacatctttattcttagaaatataaagatcatcaaccaagctgtaaatagcaaccacagatccaatgacaaaccaaagagcaaatggagagataatcatttcagatccttttcattaattagaatattagtaaacagtggagtaactcctagactcatagtaggtccaaacgtattcatggctacccatagctgcatagtgatcatcccatctttaatctctggatctttatattcttcgatacgtttcttggtaaaagcaactatatctggattatttttattttcctgaatatagtcatgccaaaactgagtattctcactacgtaggaatgttaaaacatccttagttgctggaatctgcactgtgctgttgatgtttagtcttttcacgttcttctctccgacgtttgcgttcttttatcatatgagctgctacaacttcatggtagtagtcattaatgttatcttctggcaagaaatgcttaatagtctctagctgacaaataactcgatgaagatggttatttggtagacacaattttatacctgcaacaaatccagagaagcctggaacactgaacatgggttgggcttctactctaccttcagagttgatattaagctcaattgagatacccattttcacgctataaagctggcaatattctccgttaccagaccttgaccaaacagtgaagtcctcatcaatttgatcttgaatttctgtaatagcaaatttaattctaggatctaaattattcatcttcaccttcaaagtcgcaatcataacgacaagtaaaagaatcagaactattagtacgttgagtggttatttcaccgcgtttgctaatagtaacggctggagtagagaagtttttattagtatatatttctactttaccattacgttccttaacatcacgcactttaccatactcggtaataatgccgttctgttggactttaacattaccatttttcatagaaactttggtagatgccagagaaccgaaactaactgtggagatcatcagtgcaataataaacttattcatcttcatcctccccactacaatcacgacatacatcataatcgttgaaagaacgttcgtgagcttcacaccaccaagaacaagaatcgcagagaaacatttcggttttctctagtgcttgacctaaaagatcatcagcttcctcagcagtaatcttcaatccgcacacatctgccacacgttctttaattaaacgacctgcttcgtgataagacatacaggttcccacaacatcatgttcaagaacatgaacagcacagtctagacgagttttcatttcaaacctctctcatcaatttataaatatattatagcaagaaaagagaggtttagcaaatgaattatttcagaatttagtcatagcaccaccataatccacgcttacgcatgtcatgatcgcgattataatcataattttctggatctttcatcacgcggtggagttcttgacgattcccttgacgaaccattttattagaatgccacttaacattcttactaatagaattccagttataaccatcctttttctcattacgaatggttgcttccttcatttcctgttctacatcatcccaggatttagcataaataacacgaatccagtagccattttctttgatgaaagaatattcttgagagaattgttctttagacttccaccactgatcaccagattgtttacgataagtacggctcatattacctccattaagtcttttaaattaacctaatgtggatgaattttgttatacatatattatgtacctttatacagaaaaaccccagactacttattcaatagctggggtttgttattaattacagatcggggcgttcatcttcgaaacagcctgagctaattccttctccgaatcctacaaagccatcaaattcatcatttgagatgcccataatcattgcttccattttcctaatctccgaaattttcatgcctgctttactattcttataatatttgcgagggttcccgcacatccaacaagaacagatgcaaggagtagtagtgataatacctaaccgcttagggctttcttcatgtgggaagactgtccaatacttcttgcggttgttcttcacacgttgccggtgatggcgtcttaatgctcgatccacacatttctcctaaaacttgggagataaacggagtttgctcgactaccttgcgtagctgggagaaatcatatccaaaccccattacatcgcctgagtaaatgtacgactaataacgtcgttctgttgttcacgagtcagtgcattaaatcgaacagcgtagccagagacacggatggtcaactgaggatatttttcaggatgtttctgcgcatccaaaagctgatcacggcttaacacattgacatttaggtgctgaccaccttcgatttgaggggcgacttccaccttaacttcacggaaggcttcgggatcgaattgtggtgtgataccttctagatcttcaactagaactttctgtttaagttcaccattgtcggagtatagctgaataatctgattttcatgaacaaggttaattacgccagacttaagattttgatatgctttcattagatctccctgatgttagaatttggctcagctctttattgtctatagtttaccacgatatacagaaactgtcttaccagtttggttcataacgtatgctacttcatcttcttttaagaagattgcttgatctattccagaaatagctatgcttttatttctgggattaaaccctacgcttttaccaacatgaatctgctcaccaccatcagtggacattattttaactgttaacataattgctcctatatttagctatctctagctcttttaatggtagttagtagtggatttgaaccactgtagtcgctccgtatgaaggaggtgcataaccactctgccaactaactgttatgttttactagactaagtaagtattctttatactctttagaccaattagcttttttaaactttcctggacgcatagtcttaattcctagatttggtactccgggagggatttaaacccccgatctctcggttatcagccgagtgctttagatcgctaagctaccgaagtattagaatatttacatcatacactgtctaagtaagaagtataatggaatttagcttctccagtcttatctacttctacctcagttcgtggtacttgacgaaccacaccatgaatcatcttatagcgaatgcctttagctggttcatgatcttttgggaatacttgtttaaccgttactactttatatccttcacgcggtgttaacactactacttgatcaccttctttgattttccaagaagatggaaattcataggtatatctttgaccaccagtttggaatactacagaaagataacgtttcatttggtttccctctcattaatttatatagatattataacaagaaataagagagaaggcaaatgaatttttaaatttggtgctcccaccaggaatcgaacccggttcagatgcttacaaggcaactgcatcgccagcaatgctttaggagcgatgatcccgttatttcaacgggatttctttttcaataacaggagacttatcagtcataactgtcattgccatttgttgtagaaattcaaaggtgaaggctacacgttcttcaccaatctctacttctacacgtttcttttgtttatcaatctttacttttaggttgtcagccatcttcgggttctcgttgctgtactacttctagccagtctggtagaagaaactttgtacgaaattcttcgtaagtttctttgggataaaagctaaaacctcctttctcatcattcaggataacagaaccgtcagtttgttcatatgctcgatatgtttctccaataatgataactcgcttatcagtacttttattatgaaactcaaaaacgtgcataatgtttccttaaagttggagcggctagagggaatcgaaccctactcagcgaggcttggaaggcctgcgacacaacccgtgtgcttaaccgcttattatttggctggagaaggaggaatcgaacctaccattaacggagtcaaaggccgttgtgctaaccgttacactactctccaagtatttggctgggatgccacggattgaacgtggaaccttcggagtcagaggccgacgatctgccaattgatctacatcccaataattctttactttatgtaaatagggtaactgtgctaacggtcaggtaattaatcaaatcgctgtaagtcttggtgctatcactcagactctggctggtctgcaggctaaactgccggcttaatattaaggggaggagcccattatgagtaaatatggttttgtaaataacggacttaatcaaagtatgggctcccagcagcccattccgggtctggataacccctacttacaacaattgcaacagcgtttagcagaagcgcaacagatgcaacaacaactccagcaaaaccctggaagtgtgagtcctatgcaaatgatgcagcaaatgagcgggcagtcgcaaatgcctcaacaaatgcagcaacagatgccgcagcagcaagttcagcagcaaacccaacaaccgcaggtttctgcggaaggacaggcagtactagcccttttcgaagacttcacaaagacagaggatgggaagcagcttgtatcacttatgggtaagtttaatagcttctgccaaagccaagttgcaaaagctcaaaatggtggtaataactcctaaggagaaattatgtgttgcagaaaacctgtttcgtgctgcccaatgcctgtagcacgttgttgctctccagcaatgtttacacaaataccggcgttcaatccctttgcctttaagcctactcttatcctgccccctagagtagattttcagtcaagattggcctcccgtatgggtggttgctgtacaccgagagtgtggttctgaagaaccaaacaataaagcccctagtcgaaagacttaggggcttttctgtatttaagataaaagaaaagccctgcgctctccagggaacgcagggcttacttcagatgttacatgcggatattatttattacgcatatccatgatcatttgaccatcgtagccagtacctaccacagtctgtggtacaccaccttgatatttctgagcacgaatcatttcgacttccagttgtttccaacgaatcatctcaggagtaatggtacgttgcagtgcggcgttagcttcagcttctttcttagctgcgtacagtttagcatctgcgtcacgttcattagcgatagcttggttgttgcgagcttcacgatctgcttctgcttgtttaactttttgctgtgcttcctgttcaacacgagctaattcagctttagcagcattaacctgttcttcacgaactttggtattctgtacctgttccatgattaccggtggcaaagtaatatcctgaaggaatacctgcttaactgtgtaaccatatgggcgtgcatactcttcaacttcctgttgaattgcagtttgcaattgagcctgaattttagcatcaaacaaatcttgtgctttaggtacagacttaccaaactcacgaatagtagacagtaatttttcagttacatatttgtctaacgcttgatcctgagtacctgcgttaatacggttaattggtgccttagaaccatcaaactgcaacataacagtcaggtcaacagtggatttaaacttatcctggctaggaacctgaagtttatctaattttacagcaatatcttttgtactaaaagtgtcgaaagatgcaaatgggtttacaagatggaaacctggtaatactgggttaggatctactttacccagaaatgtttgggttttaaccgtaccatcagaaacaatagtatatgaattaaaggctagaatcaagcctgctaaaccaactacagcaccaataccccaacgtttaatagtacgaattactttctgctcagaagtcagttctttcatatttttagtattaaacatatatttcctttgttttagttacagttaataaaattggccgaggtgacaggattcgaacctgcataaaggaatttagaagactcctgcctctcccttagactacaccccgtttaaatatttttaagaactctcgtaaaaactcttaaaaatacagacgataccgggagagtcataagtctcactcattaagtatttcaagacaaaatacagtaacgtctattattttccagtttaagtcagggtgacttagtggttaggtcctgcggtatattgaggactcggttaggcttggggtcatgacttcccgccttttgctgctactcaacaggagttatcgcgaattacctgtgctattgtgcaccattagtgacatctctcatgtcagcatttcccactttgtggatagcttgaaaaactactccgatatggagaaaaaacttcactatcctagaataccttctaaagttcttctttagcctggacatagttaaatcgtaataaaactattcagcagactggttggttagcctggaaccaactaccgcgtggtttaggcagtgcgcaactaacctcggaagcttttacgttaaaagcatcagttatccagttcttaccgaccgtaggattcgaacctatatcttccaccagttacggcttgataataccaattatactaggacggcagtgttactacataagtgatttccacaccccactatttataaattagagaagagtttaggggagaggtttcagacgcctcattttacacgttctagccactaaccgggattgccgccccctgtgtactagttttacaactaacctaccgactctattcaacgaatcttagtgctcgacgcatcttacattaagacaagttcagcgtaatcggctcgctgttctctaatttatgaatatattatacagaatttataagcatttagcaaataaatttttaattaaattcaccagcaatctgagcagcagtaccaccatcataacgcccaggaaattcttccttaatcgctttcatcagcataccttttgtaattccag

SEQ ID NO: 83 - DNA, 32767 bp, SP15m_8e2 phage; identical to SEQ ID NO: 3
  source 1..32767: mol_type = genomic DNA

SEQ ID NO: 84 - DNA, 32767 bp, T2_6e1 phage
  source 1..32767: mol_type = genomic DNA
atagtatcacaactaaaaccctatgtaaacaactttgtgaaattattttaaatcttctaatcgtttcttcatcttagaaccgttcttagcgatttcgcctgcatcagagcataatgctaaaagcgctttaactttagtttggtctcctttaaaagatgaaggatcaacagcagcaagttctttaatacgagagaaaagacgctcagcttcagctaaagccattccaagttttacttccataccatgggaagattcagtaatagtagtttttgtagcaaactctttgaaagttttcattttattttcctaattaattttgatgagataatagtatcactacctcatcagtatgtaaacaactttgtgaaattattttaaatcatctgcccaatcgagtttaagaggctctttgtattcacgatctaatacgaccggaatttgtacatcaccgctaaatgataggggcccaacattataagacaatgttatatgcggtgtgtaatcatcaaaatcatgtgtagcacctaatgcccgcgcatacatgtgtcgacagcgcagatattcagaatctagcacaagtacaagagtcgatccatcttgtgttttccatacttctaaatgtccagaagaagctacttcaaaacttccactcgatggaacatatggaacatttactcttgaataacatatagtcgaatgaattttttctctaggaactggattaggaacacgtaaagagcgctggagttcttccagcgcatcaagtgttaattctgaaaacttagctgctacataaagacccgttgaaaagtctttaaattccattattcttcatcttttgcttcatctgcagattcagcagtaagattcttgacagcttcaacgatttcttcaactttgatggtatcgccagtgatacctactgcacgagcaatttcagccaaagttccttgcagaattttggattcttccatcagacgagccgcttggtcctgtgtatcaagaatgcgagatttcagagttacgatttcagcagacagtttttgttcaatagtttgttcagacattatagtacctttagtgtatttttaattttagaaaaaagttcttcaatagaaccatcgtttgtaattactaaatcgccatcacgaattggcaatccagcttctgtaatatgtgtatcattggatttttgaccaggacgaactacatgaattactgtagcacccatcgccctagccgcatccatttcatgatcttgacgggtatcaggaacgatataataatcataacctgagttaaatttatcaagataatctaaagcaaataattttacccagtacatgcggtcgaagttattaacaatcaaatccgtacctagggcttgcatcagacgacggactgaccattgatcttcaatattatttataacgtcagtaatcttgttaaatgctacgaaattaactgattcttttccttcgtcatcaaaaacaaacacacctttaattgggcttttaccattaagatagcaaaatgcttgttccataatcgtgattacttctaatttagtcagatttaaattagtctcacgatcatagtcaattccttcaaactctttacgagttaagcaaggatagtcagtgtttgctgcaaatactccccatgcataagccaatgcatccttaataggaccagcaagttggtatttaactgcagaataattgctcatgataaaatcagcagtagtatcttttccactacgctttacaccacttaaaaagattagtttcatgtgtttctcctcaaatttaattaagattataacacacaaaactgaagcattaaacttctgctataatttttccatctttttctacttgaaaataggtgtaaggaatcgtagctgtacatactaaagccgggtctgaatcttctgtgtagctaaattctacttcagataggtcagaaacccaaggcttataaaaatttattgacatcacgatttcagttttgctattatctaagatgtaaagcgtaatgtactcaggacctgttttttgggcagtattttcacctgtaagatagttgctagttcctagcatccattcatacattcctatccatgacttaagttcttcatcaactataaatctcacaatgagtggatcgtactcaaatgtagcacctggacgttgtgctcggcccagtccaaacggcccagtcacggtatcagtaacaggtattctaattcctggaataggaactgactgagcatttaaagtaaaagcagatgtagtattactatgtggtattgatactacaaagttagttgtatttgcttggttaaaaatttgttgcagagcttgcgacatatattcctcataatgctttataactgttggtggtataatgggtctaagtcccttccattcaattccatttagaacaaacaacagaaaagaatggaagataatagaattagatatttgaccagactttgtttgcagagaaacgttttccttttgaaacgaactgctgaagtggcatcaacacaacgttcgcccagtctttcggggcgatttcaacaaggctacccataatattaccaggtatatacgccttaatcatttgatctgcacctctaaatcctttcacttgactccaatcaatttttaatttcgttttattagtaatagtaggtgtatttgcatattgctttaaaagctcttctagaaattgctgacgagctttaggtggaatatagtgcaagttcaatccgtacattaaattatgcttacctaaaccaaggtaaattatcaaaggaaatttatcccaataaggaagagtttccttgtgtttagcatcataagcaaaagcatatattcgtcccggctgcgggcgaacaactttatgtccttttacttgcttaatagtttcggcaaaccactttctggttttattattaattgctgcaccttcattacgaattttatcacgcaatgtttgtctgaatgaatttatcataagcagttgtctttcttgcttattgagtttattcattggttttgattcaagtttttgaatcttttcagccgttttaattcctgaagcatattttgacattgctgaagtaaacgtagagtatttgattcctctttcttcagcaaattgctttcctgtcattccttttgctttggcctttttgtattcaagacctatctgaatccatttcttttcgtttaatgattgcttaacctttggaacttggggagtgctttcattaattatttgaaaaatagccattatgcccccttaaagccaagagctcgtaatccatcttctgttagaattctaaattttattccacgcttttcagctaaagattgtgctgctttccatttgtcggtattaacagaatatgtataaatttcattcataaatcttttcttcgctgcggttgttagatgtgctggtttaaccggtggttgtgtttcttttttaggttttatttcaataaaaaattcttgcccagaagaatctttcatccaaatatccatgaagtatctacgttttttcccttctgcattacaaaaataaggaattactgctgtttcactaccccatgcaataatttctggatttttatctaaccattcaaaaaagaatttttcccaatttgatctatacgtaatttttttagggtcacctctatactttgatatatttttaggaacccattttccagaatatgccattggattctccttataaatagataatatatttataaacaggagggcccatgctctttacattttttgatccgattgaatatgcggccaaaacggtgaataaaaacgcgccgactattcctatgacagatatttttagaaactataaagactattttaaacgcgctcttgcgggataccgcttacgtacttattatattaaaggttcaccacgcccggaagaattagcaaatactatatatggaaatacgcagttgtattgggttttattgatgtgtaatgataattatgatccgtattatggatggattacttcgcaagaagctgcttatcaagcatctatacaaaaatacaaaaatgtgggtggagaccaaatagtatatcatgtgaatgagaacggtgaaaaattttataatttaatatcatacgatgataatccatatgtttggtatgacaaaggcgataaagctagaaaatatcctcaatatgaaggagcacttgctgcggtcgatacgtatgaagcgtctgttcttgaaaatgaaaaacttcgtcaaataaaaataatagcaaaatcagacatcaattcatttatgaacgaccttatacgtataatggagaaatcttatggaaatgataagtaataaccttaattggtttgttggtgttgttgaagatagaatggacccattaaaattaggtcgtgttcgtgttcgtgtggttggtttgcatccacctcaaagagcacaaggtgatgtaatgggtattccaactgaaaaattaccatggatgtcagttattcaacctataacttctgcagcaatgtctggaattgggggctccgttactggtccggtagaaggaactagagtttatggtcattttttggacaaatggaaaactaatggaattgtccttggcacgtatggtggaatagttcgcgaaaaaccgaatagacttgaaggattttctgacccaactggacagtatcctagacgtctaggaaatgatactaacgtactaaaccaaggcggagaagtaggatatgattcctcttctaacgttattcaagatagtaacttagacactgcaataaatcccgatgatagaccactatcagagattccaaccgatgataatccaaatatgtcaatggctgaaatgcttcgccgtgatgaaggattaagattaaaagtttattgggataccgaaggatatccgacaattggtattggtcatcttatcatgaaacagccagttcgtgatatggctcaaattaataaagttttatcaaaacaagttggtcgtgaaattactggaaacccaggttctattacgatggaagaggcgacgactttatttgagcgtgatttggctgatatgcaacgtgacattaaatcgcattctaaagtaggaccagtctggcaagctgtcaaccgttctcgtcaaatggcgttagaaaatatggcatttcagatgggtgttggtggtgtagctaaatttaacacaatgttaactgctatgttagcaggagattgggaaaaagcatataaagccggtcgtgattcattgtggtatcaacaaacaaaaggccgtgcatcccgtgttactatgattattcttacgggaaatttggaatcatatggtgttgaagtgaaaaccccagctaggtctctatcagcaatggctgctactgtagctaaatcttctgaccctgctgacactcctattccaaatgactcgagaattttattcaaagaaccagtttcttcatataaaggtgaatatccttatgtgcatacaatggaaactgaaagcggacatattcaggaatttgatgatacccctgggcaagaacgatacagattagttcatccaactggaacttatgaagaagtatcaccgtcaggaagaagaacaagaaaaactgttgataatttgtatgatataaccaacgctgatggtaattttttggtagccggtgataaaaagactaacgtcggtggatcagaaatttattacaacatggataatcgtcttcaccagatagatggaagcaatacaatatttgtgcgtggcgatgaaactaagacagttgaaggtaatggaactatcctagttaaaggtaatgttactattgtagttgaaggtaatgctgacattacagttaaaggagatgctaccactttagttgaaggtaatcaaactaatacagtaaatggaaatctttcttggaaagttgctgggacagttgattgggacgttggtggtgattggacagaaaaaatggcatctatgagttctatttcatctggtcaatacacaattgatggatcgaggattgacattggctaatatacttccaatgagcgctgatttaggagaatccatggaaggttcttctatcgacgtcacctttaccgctcaattagaaacaggtgaaacgttagtatctataaatataactagttacgaagaaactcctggagttttagtagaagaaaatcgcttatatggaacatatgaatctgtatttggtttcggaaatgacgcgttgaaatatcgtttaggcgatgaatttaaaactgctgcttcatgggaagaacttcctactgattctatactcagttgtatttgtggaaagctcctcaaaacctccagaagacattcacttacgaagtaacattaatatatgactaccaagaacaaagtgaatctggaggttctggcagtaattctaggtcatcttctgatactactgaaccgacagatcctcctgctccagtaagaaaaactctagttaaaaattatactaaaactatagttggaaattggagtcgttgggctaataaattgagaagctatgtgtatgagaggccataaatgtcaggattaagttatgataagtgtgttactgctggccatgaagcgtggcctccaacagttgtgaatgctacacaaagtaaagtattcactggaggaattgctgttctcgtagcaggcgatccaattacagaacatacagaaattaaaaagccatatgaaacacatggcggagtgacacaacccagaacttctaaggtatatgtcactggaaagaaagctgttcaaatggctgatccaatatcatgcggtgatactgtggctcaggcatcatctaaagtattcattaaataggatttaaaatggcaaatacccctgtaaattatcaattaacaagaacagcaaatgctattcccgagatattcgtcgggggtacgtttgctgaaataaaacaaaacctcattgaatggcttaatggccaaaatgaatttttggattatgattttgaaggctcaagattaaacgttctgtgtgaccttttggcttataatacgctgtacattcaacagtttggtaatgctgctgtgtatgaaagctttatgcgtactgctaacttacgaagttcagttgttcaagctgcgcaagataacggatatttacctacttcaaaatccgctgcgcagacagaaattatgttaacatgcactgacgcattgaataggaattacattacgattcctcgcggaactcgctttttagcatatgcaaaagatacttctgttaatccatataacttcgtttctaccgaagacgttattgctattcgtgataaaaataaccaatattttccgcgtttaaaattggctcagggacgtatagtaagaactgaaatcatttatgataaattaacacctattatcatttatgataaaaatattgatagaaaccaggttaaattatatgttgatggagcggaatggattaactggacgagaaagtcaatggttcatgctggttcaacatcaacgatttactatatgcgtgaaactattgatggaaacactgaattctattttggcgaaggtgaaatttctgttaatgcttctgaaggagctttgactgctaattatattggaggtcttaaacctactcagaactctacgattgttattgagtacatcagtactaatggtgctgacgcgaacggagcagtaggattttcatacgcagatacattaacaaatataactgtcatcaatattaatgaaaatccaaacgatgacccagattttgttggggcagatggaggcggtgatccagaagatattgagcgtattcgcgaattgggtactattaaacgcgaaacccaacaacgatgcgtaactgcgactgactacgatacattcgtttcagagagatttggttctattattcaagcagttcaaactttcactgattctactaaacctgggtatgcatttattgctgctaaacctaaatcaggattgtatttaactactgtacaacgtgaagatattaaaaattatctcaaagactataatttagctcctattacgccatcaattatttctcctaattatctttttattaagactaatttaaaagtcacatatgctttaaataagctgcaagaatccgaacagtggcttgaaggtcaaataattgataaaattgatcgctattataccgaagatgtagaaatttttaactcatctttcgctaaatctaagatgttgacatacgtagatgatgcagatcattctgtcattggttcatcagcgactattcaaatggttcgtgaagtacaaaacttctataaaacgcctgaagcgggtattaaatacaataatcaaataaaagatcgttctatggaatctaatacgttttcatttaattctggacgaaaggttgtaaatcctgatactggtttagaagaagatgtattatatgacgttcgtatagtatcaacagaccgagattctaaaggaattggtaaagttattattggtccatttgcttctggcgatgttacagaaaatgaaaacattcagccgtatacaggcaacgattttaacaaattagcaaattctgatggacgtgacaaatactatgttatcggtgaaataaattatccagctgatgtgatttattggaatatcgctaaaattaatttaacatctgaaaaatttgaagttcagactattgaattatattctgacccaaccgatgatgttatctttactcgcgatggttcactgattgtatttgaaaatgacttacgtccacaatacttaactatcgatttggagcctatatcacaatgacagtaaaagcaccttcagtcactagtctcagaatttccaagttatccgcaaatcaggtgcaagtacgctgggatgacgttggtgctaatttctactattttgtagaaatcgctgagacaaaaacaaactcgggggaaaaactcccgagtgatcaatatcgttggattaatttaggatatacagcaaataatagtttcttttttgatgatgctgatccattaacaacatacattattagagtagccacagctgcgcaagattttgagcagtctgactggatttatacagaagagtttgaaacttttgctacaaatgcttatacatttcaaaacatgattgaaatgcaattagccaataaattcattcaggaaaaatttactcttaataattctgattatgttaattttaataatgacactataatggctgcattgatgaatgaatcgttccaattcagcccatcatatgttgatgtttcatcaatcagtaattttattattggtgaaaatgagtatcatgaaatacaaggttctattcaacaagtatgtaaggatattaaccgagtttatttgatggaatcagaagggattctatatctttttgagcgttatcaacctgtagttaaagtatctaatgataaaggacaaacctggaaagatgtaaagctcttcaatgaccgtgtaggatatcctttatctaagactgtatattaccaatctgcaaacacaacatacgttctaggatacgacaagattttctacggccgtaaatctactgatgttagatggtccgctgatgatgttagatttagttcacaggatataacattcgctaaacttggtgttcaattgcatctaggatttgatgtagaaatttttgtcacttatgcgactttacctgcgaatgtatatcgaattgcagaagctattacctgcacggatgattatatctatgttgttgccagagataaagttagatacataaaaacgagtaatgcacctatagattctgatccattatctccaacatattcggaaagactttttgaacctgataccatgactataactggaaatcctaaagcagtatgttataaaatggattctattggtgataaagtttttgctcttattattggtgaagttgaaacattaaatgccaatccgaggacttcaaaaataattgattccgctgataaaggaatatatgttttaaatcatgacacaaaaacatggaaaagagttttcggtaatactgaagaagaaagaagacgcattcaacccggatatgcgaatatgtcaactgacggtaaattagtttctctgtcttcgagtaattttaaatttttaagtgataatgttgttaatgaccctgaaactgcagcaaaatatcagttaattggcgctgttaaatatgaatttcctcgtgaatggttagctgataagcattatcatatgatggcatttatagctgatgaaaaatctgattgggagacttttactcctcaaccaatgaaatactacgcagaaccgttctttaactggtctaaaaaatctaacacacgttgttggataaacaactctgatagagttgtagtagtttatgctgatttaaaatacaccaaagttatagaaaatattccggaaacatcgccagatagattagttcatgaatactgggatgatggtgattgcactatagtaatgccaaatgttaaattcactggatttaaaaaatacgcatcaggaatgcttttctataaagcctctggtgaaataatttcttactatgattttaactatcgtgtgagagatacagtagaaattatttggaagccaactggagtatttttaaaagcatttttacaaaaccaagagcatgagactccttggtcaccagaagaagagcgtggattagctgacccagatttaagaccattaattggcacaatgatgcctgattcttatttgctacaggattcgaattttgaagcattttgcgaagcatatattcaatatctttctgatggatacggaactcaatacaataatttacggaatcttattcgtaatcagtatccacgagaagagcatgcatgggaatatttgtggtcagagatatataaaagaaacatttatttaaatgctgataaacgcgatgctgttgcgagattctttgaatcacgtagctacgatttttattctactaaaggaattgaagcatcatacaagtttctttttaaagttctttataatgaagaagttgaaattgaaattgaatctggggctggtgctgaatatgacataatcgttcaatctgattctttgactgaagatttagtaggacaaacgatttatacggcaacaggaagatgtaatgttacttatatagaaagaagctattctaatggtaaattgcaatggaccgtaactattcataatcttttgggaagattaattgctggtcaagaagttaaagcagaaagactccctagttttgaaggcgaaattattcgtggcgttaaaggaaaggatttgcttcaaaacaatatagactatattaatagaagtagatcatactatgtaatgaaaattaaatccaatttaccttcttcccgctggaaatctgacgttattcgttttgttcatccagtaggatttggatttatagcaattacccttttaacaatgtttattaatgttggtttaactcttaaacatacagagactataattaataaatacaaaaactataaatgggattctggattgcctactgaatacgctgatagagtagctaaattgactccaactggcgaaattgagcatgattcagtaacaggcgaagcaatttatgagcctggcccaatggctggtgtaaaatatcctcttcctgatgactataatgctgaaaataataattcaatatttcaaggtcaattgccgtctgaacgacgtaaattaatgagtcctttatttgatgcatctggaacaacatttgcacaatttagagatttagttaataaacgtctaaaagacaatataggaaatccaagagaccctgaaaatccaacacaggttaaaatagatgaatgattcaagtgttatctatcgtgcgatagttacttcaaaatttagaacagaaaaaatgttgaatttttataattcaattggaagtggtccggataaaaacactatctttatcacatttggaagatcagaaccgtggtcatcaaatgaaaatgaggtgggctttgccccaccttatcctaccgattctgtattaggtgtaactgacatgtggactcatatgatgggaacagtaaaagttcttccatcaatgcttgatgcagttattcctcgtcgagattggggagatactagatatccggatccatacacatttagaattaacgatattgtagtgtgtaactcagctccttacaacgctactgaatcaggcgcgggttggttagtgtatcgttgtttagatgttcctgataccggaatgtgttcaatagcatctttaactgataaagatgaatgccttaaattaggaggaaaatggactccttctgctaggtcaatgactccgcctgaaggccgaggagatgctgaaggaacaattgaacccggagacgggtatgtgtgggaatatctttttgagattccgcctgatgtatctataaatagatgcacgaatgaatatatcgtggttccttggactgaggaattaaaagaggacccgactagatggggatatgaagataatctcacttggcaacaagatgattttggattaatttaccgtgttaaggcaaatactattcgttttaaagcatatttaaactcagtttattttcctgaagctgcattgccaggaaataaaggatttagacaaatatcaataatcacgaatcctcttgaagctaaagttcatccaaatgacccaaacgttaaagctgaaaaggattattatgacccagaagatttaatgaggcattcgggcgaaatgatttatatggaaaataggccacctattattatggcaatggatcaaacagaagaaatcaatattctgtttacattttaaattaagggagcccatgggctccctttttctttataaatactataaactcataaggaaaccgctatgttcattcaagaaccaaagaaattgattgataccggcgaaattggtaacgcttctactggtgatatcttattcgacggtggtaataaaattaatagtgattttaacgcaatttataatgcgtttggcgatcagcgtaaaatggcagtagcaaatggcactggagcagatggtcaaattatccatgctactggatattatcaaaaacactctattacagagtacgcaactccagtaaaagttggcactaggcatgatattgatacctctactgtaggtgttaaagttatcattgaaagaggcgaacttggcgactgcgttgaatttattaactctaatggatcaatatcagttactaatcctctaacaattcaagctattgattcaattaaaggtgtttcaggtaatttagtagtaactagcccatatagtaaagttactttacgctgtatttcatctgataattctacatcggtttggaattattctattgaaagtatgtttggacaaaaggaatcaccagctgaaggtacatggaatgtttctacatccggatcagttgatattccactatttcaacgcactgaatacaatatggctaaattgctagttacgtgccaatcagtagatggaagaaaaattaaaacagcagaaataaatattcttgtggatactgttaattcagaggtaatttcttctgaatatgctgtcatgcgagttgggaatgaaaccgaagaagatgaaatcgctaatattgcatttagtattaaagaaaactatgtaacggcgactataagttcttcaactgtcggtatgagagcagcagttaaagttatcgctacgcagaaaatcggggtggctcaataatgaaacaaaatattaatatcggtaatgttgtagatgatggtaccggtgactacctgcgtaaaggtggtataaaaataaatgaaaactttgatgagctttattatgaactcggtgatggtgatgttccatattcagccggtgcctggaaaacttataatgcttcatcaggacaaacattaacagcagaatggggaaaatcatacgctattaatacatcttctggaagagtgactataaatcttccaaagggtacagttaatgattacaacaaggtaattagagctagagacgtatttgctacatggaacgtcaacccagttacactagtagctgcttccggcgatacgattaaagggtctgcagtaccagttgaaattaatgttcaattcagcgatttagaactagtgtattgtgccccaggacgttgggaatatgtcaaaaataaacaaattgacaaaattaccagttcagacattagtaatgtagctcgtaaagaatttttagtcgaagtccaagggcaaacagactttttagatgttttcagtggaactagttataatgtaaataacatcagagtaaaacatcgtggtaacgaattatattatggcgatgtgtttagcgaaaacagcgattttggctctccaggcgaaaatgaaggagaactggttcctcttgatggatttaatattcgattaagacagccttgtaatattggtgacactgttcaaattgaaacatttatggatggtgtatcgcagtggagaagttcatatacaagacgtcaaattagattgttagattcaaaattaacgtcaaaaacttctctagaaggaagtatttacgttactgatttatcaacaatgaaatcaattccattttctgcttttggattaattccaggagaacctattaatcctaattctcttgaagttagttttaatggaattttacaagaattggctggaacagttggaatgccattatttcattgtgttggtgccgattcagacgatgaagtagaatgctctgttttaggtggaacttgggaacaatctcataccgattattcagttgaaactgatgaaaacggcataccagaaattttacatttcgatagagtatttgagcatggtgacattatcaatatcacctggtttaataatgatttgggtacattattaacaaaagatgagattattgatgaaactgataatctctatgtatcgcaaggaccgggagtagatatttccggtgatgtaaatttaacagactttgataaaattggttggccaaatgtagaagcagttcaatcttatcaacgcgaatttactgctgtttcaaatatctttgatacgatttatcctattggaactatatatgaaaacgctgttaatccaaataaccctgttacatatatgggattcggctcatggaaattatttgggcaaggaaaagttttagttggatggaatgaagatatttcggaccctaactttgctctaaataacaacgatttagattctggtggaaatccttcgcatactgcaggcggaacaggtggttctacttctgttacattggaaaatgctaatcttcctgcaaccgagacagatgaagaagttctaatagttgatgaaaatggatcagtcattgttggtggatgtcaatacgatccagatgaatccggtccaatttatactaaataccgtgaagctaaagcatctactaactctactcacactccgccaacatcaataactaacattcaaccatatattacagtttatcgttggataaggattgcataatgagtttacttaataacaaagcgggagttatttcccgcttagccgattttcttggttttagacctaaaactggcgacattgatgtaatgaatcgtcaatcagtcgggtcagtgacaatatctcaattagcgaaaggattttatgaaccaaacatagaatcagctattaatgacgttcataatttttctataaaagacgttggtacaattattactaataaaactggtgtttctcctgagggtgtttctcaaactgattattgggcattttctggaactgtaacagacgattctcttcctccgggttctcctgttacggtattagtatttggtcttccagtttcagcaacaactggaatgacggcaattgagtttgttgcaaaagttcgtgttgcccttcaagaagctattgcatcatttactgctatcaactcatataaagaccatccaacagatggtagtaaattagaagttacttatttagataatcaaaaacatgtattaagcacatattctacatatggaataactatttcgcaggaaattatttctgagtctaaacctggctatggtacatggaatttattaggcgcacaaactgtaactttagataatcagcagactcctacagtattttatcattttgagagaacagcatgagtaataatacatatcaacacgtttctaatgaatctcgttatgtaaaatttgatcctaccgatacgaattttccaccagagattactgatgttcaggctgctatagcagccatttctcctgctggcgtaaatggagttcctgatgcatcgtcaacaacaaagggaattttatttcttgccactgaacaggaagttatcgatggaactaataataccaaagcagttacaccagcaacgttggcaacaagattatcatatccaaacgcaactgaagctgtttacggattaacaagatattcaaccgatgatgaagccattgccggagttaataatgaatcttctataactccagctaaatttactgttgctcttaataatgtctttgaaactcgtgtttcaactgaatcatcaaatggggttattaaaatttcatctttaccgcaagcattggcaggtgcagatgatactactgcaatgactccattaaaaacacaacaattagctgttaaattgattgcgcaaattgctccttctaaaaatgctgctacagaatctgagcaaggtgtaattcagttagctacagtagcacaggctcgtcagggaactttaagagaaggatacgcaatttctccttatacgtttatgaattctactgctactgaagaatataaaggcgtaattaaattaggaacgcaatcagaagttaactcgaataatgcttctgttgcggttactggagcaactcttaatggtcgtggttctacgacgtcaatgagaggcgtagttaaattaactacaaccgccggttcacagagtggaggcgatgcttcatcagccttagcttggaatgctgacgttatccaccaaagaggcggtcaaactattaatggaacacttcgcattaataatacgcttacaatagcttcaggtggggcaaatattaccggaacagttaacatgactggcggttatattcaaggtaaacgcgtcgtaacacaaaatgaaattgatagaactattcctgtcggagctattatgatgtgggccgctgatagtcttcctagtgatgcttggcgtttttgccacggtggaactgtttcagcgtcagattgtccattatatgcttctagaattggaacaagatatggcggaagctcatcaaatcctggattgcctgacatgcgcggtctttttgttcgtggctctggccgtggctctcatttaacaaatccaaatgttaatggtaatgaccaatttggtaaacctagattaggtgtaggttgtactggtggatatgttggtgaagtacagaaacaacagatgtcttatcataaacatgctggtggatttggtgagtatgatgattctggggcattcggtaatactcgtagatcaaattttgttggtacacgtaaaggacttgactgggataaccgttcatacttcactaatgacgggtatgaaattgacccagcatcacaacgaaattccagatatacattaaatcgtcctgaattaattggaaatgaaacacgtccatggaacatttctttaaactacataattaaggtaaaagaatgacagatattgtactgaatgacttaccattcgttgacggccctcctgcagagggccagagccgcatttcctggattaaaaacggcgaagaaatattaggagctgacacgcagtatggaagcgaaggttcaatgaatagacctacagtttctgtactaagaaatgtcgaagttctcgataaaaacattggaatacttaaaacatctttagaaaccgcaaatagtgatattaaaacaattcagggcatcttagatgtatctggtgatattgaagctttggcccaaataggtatcaataaaaaggatatttctgacctcaaaacgctaaccagtgaacatacagaaatattaaatggacctaatagtacagttgacaacattcttgctgatattggtccatttaactctgaggccaactctgtatacagaacaatcagaaatgatttactgtggataaagcgtgaacttggacaatacgcaggtcaagatattaatggtcttcctgttgtaggaaatcctagtagtggaatgaagcatcgcattattaataatactgatgccattacttcacagggaatacgtttaagcgaattagaaacaaaatttattgaatctgatgtaggttctttgactattgaagttggtaatcttcgtgaagagcttggaccgaaaccaccatcattttcacaaaacgtttatagtcgtttaaatgaaattgacactaaacagacaacatttgaatctgacattagtgctattaagacctcaataggatatccaggaaataattcgattattactagtgttaatacaaacactgataatattgcatctattaatttagagctaaatcaaagtggaggtattaaacagcgtttaaccgttattgaaacttctattggttcagatgatattccttcgagtattaaaggccaaatcaaagataatacaactttaatcgaatctctaaatggaatcgtcggtgaaaacacttcatctggtttaagagcgaatgtttcatggttaaacaaaattgttggaactgattctagcggtggacaaccttctccttctgggtctcttttaaaccgagtttctacaattgaaacttctgtttcaggattgaataacgatgttcaaaacctacaagtagagattggtaataatagcgcaggaattaaagggcaagttgtagcgttaaatactttagtaaatggaactaatccaaacggttcaacagtcgaagaacgcggattaaccaattcaataaaagctaacgaaaccaacattgcatcagttacacaagaagtgaatacagctaaaggtaatatatcttctttacaaagcggtgttcaagctctccaagaagccggttatattcctgaagcgccaagagatgggcaagcttacgttcgtaaagacggcgaatgggtattgctttctacctttttatcaccagcataacatggggccgcaaggccccaaaggattttaaatgtcaggatataattctcagaatccaaaggaactcaaagatgtcattctaagacgtttaggggctccaattattaatgttgagttaacacccgatcaaatttacgattgtatccagcgtgccctagaattatacggtgaataccattttgatggactcaataaagggtttcatgtgttttacgtaggggatgacgaagaaaagtacaagaccggagtcttcgatttaagaggttctaacgtatttgcagtaactcgcattttacgcacaaatattgggtcaataacatctatggatggaaacgctacatatccgtggtttactgactttcttttgggaatggctggtattaatggcggaatgggaacgtcttgtaatagattttatggaccaaatgcctttggtgccgatttggggtattttactcaacttaccagttatatgggaatgatgcaggatatgctctctcctattccagacttttggtttaattcagcaaatgaacagctcaaagtcatgggaaacttccaaaaatatgatttaattatcgtagaaagctggactaaatcatacattgatacaaacaaaatggttggaaatacagtaggatatggaacagtcgttccacaagataactggtcattatctgaacgatataataacccagacaacaatttagtaggtcgtgttgttggtcaagacccaaatgttaagcaaggtgcttacaataatcgttgggtgaaagactatgcaacagctttagctaaagaattaaatggtcaaattttagcacgccaccagggaatgatgcttcctggcggtgttacaattgatggacaacgcttaatagaagaagctcgattagaaaaagaagcactgcgcgaagaattatacttacttgaccctccatttggaattttggtaggttaatatggctacttacgataaaaatctttttgctaaattggaaaaccgcacaggttattctcagaccaatgaaactgaaatactaaatccttatgtaaatttcaatcattataaaaacagccaaatattagctgatgtattagtagctgaaagcattcaaatgcgaggtgtagaatgctattatgttccaagagagtatgtttcccctgatttgatattcggcgaagacttgaaaaataaatttactaaagcttggaaatttgctgcatatttaaattcatttgaaggatatgaaggagctaaatcgttctttagtaattttggtatgcaagtacaggatgaagttactttgtccattaatccaaacttgtttaaacaccaagtaaatggaaaagaaccgaaagaaggcgatttgatatattttcctatggataacagcttatttgaaattaactgggttgaaccatatgatccattttatcaattaggccaaaacgctattcgtaaaattacggcaggtaaattcatttattctggagaagaaattaatccagttctacagaaaaatgaaggaattaacattccagaatttagtgaattagaattaaatcctgttcgcaatcttaacggtattcatgacattaatattgatcagtatgctgaagtagatcaaattaattctgaagctaaagaatatgttgaaccctatgttgttgtcaataacagaggcaaatctttcgaatctagcccatttgataatgatttcatggattaataaatattataaactaattaaagcccagattaggagaagtcatgtttggttatttttataattcgtcttttagacgatatgctaccttgatgggcgatttgttttcaaatatccaaatcaaacgtcagttagaatctggtgataagtttatacgtgttcctattacatatgcatcaaaggaacactttatgatgaaattgaataaatggacatcaataaattcacaagaagatgtagctaaagttgaaaccattctacctcgtataaatttacatttagttgattttagctataatgctccatttaaaacaaacattttaaatcagaatttactgcaaaaaggtgcaacttctgtagtatcgcagtataatccatctcctattaaaatgatttatgaattgagtatctttactcgctacgaagatgatatgtttcaaatagttgaacagattcttccatattttcaacctcattttaatacaactatgtacgagcagtttggaaatgatattccatttaaaagggatatcaaaattgtactgatgtctgctgctatagacgaagctatagatggggataatttatctcgtcgtagaattgaatggtcattaacatttgaagtaaatggatggatgtatcctccagtagatgatgcagaaggattaattcgtactacttatacagattttcacgccaatacaagagatttgcctgatggcgaaggtgtttttgaatctgtcgatagcgaagttgttcctcgagatattaacccagaagactgggatggaacagtaaaacaaactttcactagtaatgtaaatagaccaacaccgccagaacctcctggcccaagaacatagaggttattatggaaggtcttgatataaacaaacttttagatatttctgacctccccggaattgacggggaggaaatcaaagtatatgaacctctgcaattagtagaagttaaaagcaatccacaaaaccgtactcctgacttagaagatgattatggagtagttcgtcgaaatatgcattttcaacaacaaatgctaatggacgcggccaagatttttcttgagacggcaaagaatgctgattctcctcgtcacatggaagtatttgcaactcttatggggcaaatgactacgacgaacagagaaatactgaagcttcataaagatatgaaagatattacatctgagcaggttggcaccaaaggcgctgttcctacaggtcaaatgaatattcagaatgcgacagtattcatgggttcaccaacagaattaatggacgaaattggtgatgcttacgaggctcaagaagctcgtgagaaggtgataaatggaacaaccaattaatgcattaaatgatttccatccgttaaatgaagctggaaaaattttaataaaacacccaagcttagcggaaagaaaagatgaagatggaattcattggataaaatctcagtgggatggaaaatggtatcctgaaaaattcagtgattaccttcgtctacacaaaatagtaaaaattccaaacaactctgataagcctgaattatttcaaacttataaagataagaataataaaagatctcggtatatgggtcttcctaacttgaaacgagctaatattaaaacacaatggactcgtgaaatggttgaggaatggaaaaaatgccgagacgatattgtttattttgcagaaacatactgtgctattactcatattgactatggtgtcataaaggttcaattacgtgactatcagcgtgatatgctcaaaataatgtcatctaaacgtatgactgtttgtaatctatcgcgtcagctcggtaaaacaacggtagtagctattttccttgcacactttgtatgttttaacaaggataaagctgtaggtattcttgcgcacaaaggctcaatgtctgcggaagttttagaccgtactaagcaagcaattgaactgcttcctgactttttacagccaggtatagttgaatggaataagggttcaattgaactagataatggttcttcaattggcgcttatgcttcctctcctgacgcagttcgtggtaactcgttcgcaatgatttacattgacgaatgtgcgtttattccaaacttccatgattcctggcttgctattcaaccagtaatttcatctggtcgtcgttcgaaaattattattactacgactcctaatggattaaatcatttttatgatatttggactgctgctgttgaaggtaaatctggatttgaaccatatactgctatttggaattcagttaaagaacgtctttataacgatgaagatatttttgacgatggatggcaatggagcatacaaaccattaatggttctactttagctcaatttcgtcaagaacacaccgcagcgtttgaagggacttctggtacattaatttcgggaatgaaattagctattatggatttcattgaagtaactccagatgatcatggttttcatcgatttaaaagccctgaaccagatagaaaatatattgcaactctagactgctcagaaggtcgtgggcaagattaccacgctttgcatattattgatgttaccgatgatgtgtgggaacaggttggtgttttgcactcaaacactatttctcatttaattctacctgacatcgttatgcgttatttagtagaatacaatgaatgcccagtttatattgaattaaatagtactggtgtgtcagttgcaaaatcgctttatatggatttagaatacgaaggtgttatctgtgattcatatactgatttaggaatgaaacaaactaaacgcacgaaagcagtaggatgttccacgctaaaagaccttattgaaaaagataagcttattattcatcaccgagcgactattcaagaatttagaacgtttagtgaaaaaggcgtgtcttgggcggctgaagaaggttatcacgacgatttagtaatgtctttagtaatttttggatggttatcaacacaatcaaaatttattgattatgcggataaagatgacacgcgattagcatctgaagtattttcaaaagagcttcaagatatgagcgacgactacgcgccagttatatttgtggattcggttcattctgctgagtatgttccagtatctcatggtatgtcaatggtataaatatattaaagcatattaaagaggattaaaaatgactttattatctccgggcattgagctcaaagaaactacggttcaaagcaccgtggttaataactctactggtacagcagctttggccggtaaattccagtggggtcctgcttttcagattaaacaggttacaaatgaagtagatttagttaatacttttggtcaaccaaccgctgaaactgctgactattttatgtctgcgatgaatttcttgcagtacggaaatgacttacgagtagttcgtgctgttgatagagataccgctaaaaactcatcaccaatcgctggtaatattgaatacacaatttctaccccaggtagtaactatgcggttggagataaaatcacagtcaaatatgtttcagatgatattgaaactgaaggtaaaattactgaagtagacgcagatggaaaaattaagaaaattaatattcctactgcaaaaattatcgctaaagcgaaagaagtcggtgaatatccaacactaggttctaactggactgcggaaatttcttcatcttcctctggtttagctgcagtaataactcttggaaaaattattactgattctggtattttattagctgaaattgaaaatgctgaagctgctatgacagcggttgactttcaagcaaatcttaaaaaatatggaattccaggagtagtagcgctttatccaggcgaattaggcgataaaattgaaattgaaatcgtatctaaagctgactatgcaaaaggagcttctgcattactcccaatttatccaggtggtggtactcgtgcatctactgccaaagcagtgtttggatatggaccgcaaactgattcacaatacgctattatagttcgtcgcaatgatgctattgttcaaagcgttgttctttcaactaagcgtggtgaaaaagatatttacgatagtaacatctatatcgatgactttttcgcaaaaggcggctcagaatatatttttgcaactgcacaaaactggccagaaggcttctctggaattttaactctgtctggtggattatcatcaaatgctgaagtaacagcaggagatttgatggaagcttgggacttctttgctgaccgtgaatccgttgatgttcaactgtttattgcgggttcttgtgccggtgaatctttagaaacagcatctactgtccaaaaacacgtcgtttcaattggggatgctcgccaagattgcttagtattgtgctctcctccgcgtgaaactgtagttggaattcctgtaactcgtgcagtagataatttagttaactggagaactgcggcaggttcatacactgataataactttaatatcagttcaacctacgcagcaattgatggtaactataagtatcagtatgacaaatataatgatgtgaatcgttgggttccattagcagctgatattgctggtttatgcgcaagaactgataacgtatctcagacttggatgtctccagctggttataatcgtggccagattcttaacgttattaaacttgctattgaaactcgccaggctcagcgcgaccgtttataccaagaagctatcaacccagtaactggtacaggtggcgatggttacgtattgtatggtgataaaacagctacttctgttccttctccatttgatcgtattaacgttcgtcgtctgtttaatatgttgaaaacgaatatcggacgtagttcaaaatatcgtttgttcgaattaaacaacgcgtttactcgttcatcattccgcacagaaactgcccagtacttgcagggaattaaagctctcggtggaatttatgaatatcgtgtagtttgcgatacaacaaataacactccgtcagtaattgatagaaatgagtttgttgcaacattctacatccaacctgcgcgcagtataaattatattactttgaatttcgtcgcaacggctactggtgcagatttcgatgagttaactggtcttgcaggttaatacggtgcattctaaaggcctgtttcggcaggccatataaatacactatatccttaattctttaattctatatgccctaggttaaacatagggatataaatactacagaggctaatatgtttgtagatgatgtaacacgcgcgtttgaatcaggtgattttgcgcgacctaacttattccaagtagaaatttcttatcttggacaaaattttacgtttcaatgtaaagccactgctttaccagctggtattgtagaaaaaattccagtcggatttatgaaccgtaaaattaacgtagcaggcgatcgtacattcgatgactggactgttacagtaatgaacgatgaagctcatgatgctcgccagaagttcgttgattggcaaagcattgctgcggggcaaggaaacgaaattactggtggaaaacctgcagagtataaaaagagcgctatcgttcgtcaatatgctcgtgacgctaaaacagtaacaaaagaaattgaaattaaaggtctgtggcctactaacgtgggtgaacttcaattagattgggattcaaacaatgaaatccaaacatttgaagtaactcttgctctcgattattgggaataaaatgaatggggagaaatccccatcctgcttaaagcagagaagtccattataaatataactataattcccatttggagaatacaatgaaatttaatgtattaagtttgtttgctccatgggctaaaatggacgaacgaaattttaaagaccaagaaaaagaagatcttgtttccattacagccccaaagcttgatgatggagcgagagaatttgaagtaagctcgaatgaagctgcttctccttataatgctgcattccaaacaatttttggttcatatgaaccaggaatgaaaactactcgtgagcttattgatacatatcgtaatctcatgaataactatgaagtggacaatgcagtttcagaaatcgtttcagacgctatcgtctatgaagatgatactgaagttgtagcgttaaatttggataaatctaaatttagtccaaaaattaaaaatatgatgttagatgaatttagtgatatattaaatcatctatcgtttcaacgaaaaggttctaatcattttagacgttggtatgttgattcaagaattttctttcataaaatcattgatccaaaacgtccaaaagaaggcataaaagaattacgtagattagaccctcgccgagttcagtatgttcgtgaaattataacagaaactgaagctggcacaaaaatagttaaaggttacaaagaatattttatatatgatactgcccatgagtcatatgcatgtgatggtagaatgtatgaagctggcacaaaaataaaaattcctaaagctgccgtcgtttatgcccattctggattagttgattgttgcggtaaaaatatcatcgggtatttgcatcgtgctgttaaacctgctaaccaattaaaattattagaagatgctgtagtcatttatcgcattactcgtgctcctgaccgtcgtgtttggtatgtagacacaggtaatatgcctgctcgtaaagctgctgagcacatgcaacatgttatgaacacgatgaaaaaccgtgtagtatatgatgcatcaacaggtaaaataaaaaatcaacagcataatatgtctatgaccgaagactattggttgcagcgccgtgatggtaaagctgtgacagaagttgatactcttcctggtgctgataatactggcaatatggaagatattcgttggtttagacaagctctttatatggcattacgtgttcctctttcacgcattccgcaagaccaacaaggcggtgtgatgtttgattctggaactagcattacacgtgatgaattaacgtttgctaaatttattcgtgagttgcagcacaagtttgaagaagttttcctagatccgcttaaaacaaatcttttgcttaaaggtataattacagaagatgagtggaatgatgaaataaataatattaagatagaatttcatcgggatagctactttgctgagctcaaagaagcagaaattttggaacgaagaattaatatgctaaccatggcagaaccatttattggtaaatatatttctcacagaactgctatgaaagatattttgcagatgactgatgaagaaatagaacaagaagccaagcaaattgaagaagagtctaaagaggctcgtttccaagaccccgaccaagaacaagaggatttttaatggaaggtttaattgaagctattaaatcaaacgacctcgtagccgctcgtaaattatttgctgaagccatggctgcaagaacgattgatttaattaaagaagaaaaaatcgctatcgctcgtaatttcttaatcgaaggtgaagaacctgaagacgaggatgaagatgaagatgatgacgaagatagcgatgataaagacgaagactctgacgaagacgaggatgatgaataatgcttctgatccctgaaactcatgaattagttctcgaaagtgtcgaagcacttattactgaagcacagggtcgctttgacgaattgtcttctgctttaaataaagacgatataaatacaattgtcgagaatatgcttgatgatgaaactgatttagcggttgcattagcttctattaatgaaaatatgccgttaaatgaatttatcgttaaacatgtttccgcccgtggtgaaattactcgcactaaagatcgcaaaacccgcgaacgaaatgcatttcaaaccactgggctgtctaaagcaaaacgtagacaaattgctcgtaaagctaccaaaacgaagattgccaatccagcaggtcaatctcgtgctcagcgtaagcgtaaaaaagctcttaaacgccgtaaagcattaggattaagctaatgaatgaaccccaattactaattgaaacttggggtcaacctggcgaaattattgatggcgtgccaatgcttgaatctcatgatggaaaagacttaggtttaaaaccgggtttatacatcgaaggaatattcatgcaagcggaagtcgtcaatagaaataaacgtctttatccaaaacgtatattagaaaaagcggtaaaagactatattaatgagcaagttttaactaaacaagctctcggagaattaaatcatcctccacgcgctaatgttgacccgatgcaagccgctatcattatagaagatatgtggtggaaaggaaatgacgtatacggacgagctcgtgttattgaaggtgaccatggtcctggagataaattagcagctaatattcgtgccggatggattccaggagtttcttctcgtggattaggttcattgactgacacaaataaaggttatcgtatcgtaaacgaaggattcaaattaactgtaggtgttgatgcagtatggggtccaagtgctccagatgcatgggtaactcctaaggaaattaccgaatcacagacggcggaagccgatacaagtgccgatgacgcctatatggctctcgcagaggccatgaaaaaagcgttataaatattattatctaaacaacaggactacaaaatgcttaaagaacaactgattgccgaagcgcagaaaattgatgcttccgttgctcttgatagtattttcgaatcagttaatatttctccggaagcaaaagaaactttcggcactgtattcgaagctaccgtcaagcagcacgccgttaaattagctgaatctcatatcgctaaaattgctgaaaaagcagaagaagaagtagaaaaaaataaagaagaagccgaagaaaaagctgagaagaaaatcgctgagcaagcttctaaattcattgaccatcttgcaaaagaatggctcgctgaaaataaattagcagttgataaaggcatcaaagccgaactgtttgaatccatgcttggtggattaaaagagctctttgttgaacacaacgttgttgttccagaagaatcagttgatattgtagctgaaatggaagaagagctgcaagaacataaagaagaatcagctcgtctgttcgaagaactcaatatgcgcgacgcatatatcaattatgtgcagcgtgaagtggcattgagcgaaagtactaaagatctgactgagtctcaaaaagaaaaagtctctgctctggtcgaaggtatggattattcagatgcattctcaagtaaattgagtgccatcgtagaaatggtgaagaagtctaataaagatgaaagcactattactgatggtataaatactcctgatactgaagcagccggactgaatttcgtcactgaagctgtagaagataaagctgcacatggtgcagaagatattgtaagtgtatatgcgaaagtcgcatctcgtttctaattttaaaggttaacacaaatgactatcaaaactaaagctgaacttttgaacaaatggaagccattactggaaggtgaaggtttaccggaaattgctaatagcaaacaagcgattatcgctaaaatctttgaaaaccaggaaaaagatttccagacagctccggaatataaagacgaaaaaattgctcaggcattcggttctttcttaacagaagctgaaatcggtggtgaccacggttacaatgctaccaacatcgctgcaggtcagacttctggcgcagtaactcagattggcccagctgttatgggtatggtacgtcgtgctattcctaacctgattgctttcgatatttgtggtgttcagccgatgaacagcccgactggccaggtattcgcactgcgcgcagtatacggtaaagacccggtcgcttctggtgctaaagaagcattccacccaatgtatggtccagatgcaatgttctctggtcagggtgctgctaagaaattcgctgctttgaaagcaagtgatactcttgaagtcggaactatttacactcacttcttccaggaaactggtactgtatatctgcaagctacagaagttaaacaaatcgatgtcggtgctagtgatgcagctaaattagatgctgaaattaagaaacaaatggaagctggtgtactggtagaaatcgctgaaggtatggctacttctatcgctgaacttcaggaaggtttcaatggttctaccgataacccatggaatgaaatgggcttccgtatcgataagcaagttatcgaagctaaatctcgccagctgaaagctgcttactctattgaattagcacaagacctccgcgctgttcacggtatggatgctgatgctgaactgtctggtattctggctacagaaattatgctggaaatcaaccgtgaagttgttgattggattaactactcagctcaggttggtaaatctggtatgaccctgactccaggttctaaagctggtgtatttgacttccaggacccaatcgatattcgtggtgctcgctgggcgggtgaatcctttaaagctctgttgttccagattgacaaagaagcagttgaaattgctcgtcagaccggtcgtggtgaaggtaacttcattatcgcttcccgtaacgtagttaacgttctggcttcagttgataccggcatttcttatgctgcacagggtctggctaccggcttcaacactgatactaccaagtcagtatttgctggtgttctgggtggtaaataccgcgtatatatcgaccagtatgctaaacaggattatttcactgtaggttataaaggtccgaacgaaatggatgctggtatttactatgctccatatgtagctctgactccgctgcgtggttccgatccgaagaacttccaaccggtaatgggattcaaaactcgttacggtatcggtatcaacccatttgcagaatccgctgctcaggctccggcttctcgcatccagagcggtatgccttctattctgaatagccttggtaaaaacgcttactttagacgtgtatatgttaaaggtatctaatctttgacgatttaagggaccttcgggtccctttagttgtttttatggtataaataaatcatataaaccaaaaggaaagcgcaatggctaaaatcaacgaacttctgcgcgaatcaaccacaacgaatagcaactcaatcggtcgcccaaatctcgttgctttgactcgcgctaccactaaattaatatattctgacattgtagcaacgcaaagaactaatcaacctgttgctgctttttatggtatcaaataccttaacccagacaacgaatttacatttaaaactggtgctacttatgctggcgaagctggatatgtagaccgagaacaaatcacagaattaacagaagagtctaaattaactctcaataaaggcgatttattcaaatataataatatcgtttataaagt

SEQ ID NO: 85 - DNA, 32767 bp, T2_6e2 phage; identical to SEQ ID NO: 84
  source 1..32767: mol_type = genomic DNA

SEQ ID NO: 86 - DNA, 32767 bp, SP15m_6e1 phage
  source 1..32767: mol_type = genomic DNA
ggtgcagtgggtcgggcgaaaatacttagtctgctaaccgccacccccgttacaattaccatgctaattgtttcaccctgcaaccattttaattgcagggtgaaacaatttcaactttaattattacgcaacttttaatttctcaatatattgttgcgggctgcaactatattctgcgcgttcttcttcggtcatactttcccaacataattgcaggcggtcggctaggaattgataatcattatcatcgtcgagcgattcatcaataaaggtttcacctatcaatgtaacaccgattgatagaatatcgttaatagcttgcgcgtccagcgttttaaatccgtatgatgccgccgctgatagcacgcctttatgatcatcaatcatcgtaaaatcagcgttcggatataactgtttaaataactcaaaataataagatttataaactgcgtctttgctgtggtatatttcgctaactttatcagcttcaaaatatttgtgcagcgtgtcacgggagaacacgcggatattgctgttcccacgccctcgcaatccttgcttgcgtaggaagtaataatctgacttgctcattagtcgagcggtgcaaataatgtttaaagtatttgcgtcattcatgcactggcgcatatatgtaacaaggggcaataaggaatcttgcattattaaatcatgtttgcaggcttcatttttatacttatttaaatctaaattgccctcgctatcaaagcaaggcgctacacgatgaaacgaattaatgatagtgccgtctaaatcccaaatcataacgcgggaaatatgcgggaaattacgggtaatattcattttaacttgattcattttgttacgttctccatttaagggattagattaattcaatctagcccactaattatattttgttagtgggctatgtttaattaactattagaatgctagaccgaaagcgagagcgtcggcaataaagctaacatcttcacctgatacataggaacgaatccccgcacaagtatatacttttgcgctgatcaattgatcatcgaggcaagcggggcaaggcgcgacaactgcaaaggctaggccggattttacagcgtcgatgataatcgtttcttgtttcaccgtatcaatataaacgcctgcggccttaatgtaactacttgcgcagccttgcgtataggcaaaggtagtaacctgcaaggcgtcgttaaattcgattaaatcatcgacaacgtgccccgcctcgacgtgataacgctcaccattagaataaaccagaacaattgaggattgagcgcgatcgaatggaatattttgctttttcatatttatataactccaattagtttaataaggggtttaatttatttgataataatctgcatttgatacggcgttaattcaccgtttacgggtaaattattatcgcttagccactcataaaaagcaccatcatcatcaaaagggacaatatcgttatcacgggaatcgacggaaataataccatccgtattagttttggcggctaggataggcccgaagctgtaaactttatcagattccatttcatccggtgaaatgaatactttttcgtccaatgttttgggtaatgtaactttcattctaatttagctcctgtaatagcggctatatttcaagccgctagggtaataatttaattatgcaaagaatttaccgttcttaaagtcgatcaaagtacgctgaccgtttgcataggtaattaaatgcgtttgtgtccagcttgacgcgccaacgttgtaacccatatccagactaccagctacgccagcggtatataccccgccgtaaatgctggcggtatgagtgtgccccgtgttcagtttacccaatttcttaaactgtttcggattgccacggctgccgtttatgccattgtgaccgtgtacgccgcattcaatgcctgcaattttaaatgattggtcagtcgttaggaaaatggcgttaaactcgcaacctgcaaccttacgcagcgcataatctagcacgttgaaagtatcgtctttttctgcaatagctccataaatcgcggcattaaggcggtgatatagttccgcgtttgctgggtcgtctttaatgttagcattacgatcatcaagccaacgggataacgccagatcatggttagattcaacaatgattgtttgcgagaaatcgcgctccattgattccagtacgcgccccgtatcgatgagatcatccagaactttatcacgtccggaggcatactgttttgctaggaatacacccgaagcgcggttgtgatggttgcgtgatgtaaagtcgtgaacgtcatggataaactgatattttggtttaagaatatcaagcaagctattttcgccagcccatgacgcagcggcgcattcttcatctaatttttcagcgtggatgtcgccatattgtaaacctaaaacgtgccccgttgtttcatagcatccggcaggagtagcgcaaacattcagatcataaaacacgccgctttcgtccattgtttcaagctggcgaacaaaaaaattccccgtcctcatcgaactcaacaatcagcgcaccgaaattatgcagcgcctcggccttttgtcctgctttctgctgaatgtaatttttgagcgttgccgttccggttgaatacatgcggcgcacaatttcaccttttaaagctggcacgctttcggcggtgattttagccgctccaattgccagaccttccagattaagcgcggttgcagtttcagcgaatccagaaagcggataatctgcggttggcaaaacattaatttcagccatgaaagcaaaacggcggttatttaaaaacacgtttttattgcagatatatttatcaaaagcggaatcatatttgattccgtctgcgccctcgccattttgaaaaccgtttttgttatagatatattttgaaacgagcaaatcagcgccgatatatttagcaaattgctccagtgaggctaaaaagtttttatgcgggaaagtattattctgaatcgatgtaataataaagcgtttgccttgttttacttcccagctttccaccgtgctagaaacaatccccgccgcttctgggcgctcatcgtttttaatggcttttgctactttcgccgctttcggtttagctggtttatttgcttccaaccagtcgcagatagcggtcgagtgttttgttgtatcgtagaccgcttttgatatatcgtcgcagacctccagtttagtagcgcgcagacgtttaccatagaaattaaagtcagcggccattttcaggataacggtttgtttttctgcggaaataatcatagtataaaactccattaaagggactaggttaataacggcaatattgccaaatataacgccgcaaatgagtggcgttataatttgcaacattaatttaaaggtataaggctagaactaacaccacaagcaacggcggcaataaaacaaatcagacctaaacgctttgccaatttagacttacgtttaaaataatatgaatctaaatcattttgaaaataagcgaatagtaacgaggccgccataataaataagcctagaatgagggattcagtagggtaaaagatcattttaataactccagtcaaagggaaattatagtggggaatattccccactaattaaatttattcgcctgcggcttgtttcacttcatcggcaacgcctaacagttgcgccacggcgtccagcgtttccagttttgcgctttccagtgatgccagatcgtcggcgtctttgataatgccggaatcgatggcgtgttttgcaattacgcgcacataatgcgctttgcggattgagctaccgccgccaactttgcgcggcttatcgcttttctgatacgctttcgcgctggtcaattttgagcgaacggacacgggagaagccgcgcccactgctttcgcgatctctttcaggccgtcgctatttgcgaaatctaaaccgttttcattaattaactgctggtacatggtaacagctttttgggtgttttcttcattccatgcaaattttgcggatttttcggttttaacgttagccatgattgtagctcctattagtttaatttaagggataagattaacataatgttaatcgttatataccccgaactactggggtatataaagttaacactaaattataaaacagcttcccatttttcgttacgctggacaacctttacaacgtcgccggatttaacgcgaacgctaaaaacggttttgccgttgttactacgttccgtttcagcgtataccgcgtcgattgtatcaaatggcataagcgccgcgcctttaatgcgttcggcctttccggttaattcatccgttttagtaacgaaaggaataaaaacggattgaccaattttaggcgtggtaataatgttttgcatagtataaactccaagttatttaggggattgttccgcattacctgctagaaagtagcaggtaataagcaacaatccgctcgccaatataatcaatttaaagaactccacgcaggccgctatatcccagttagggggcggggcacattatggtaagtgccgaccgtcaaattttatcaaattatcgctcttatcgaactgggtacatcttaaagcctatcggctagggtgtcaaactattttttgcagttttttatggttttccttcaggtcgatcataatattacgccagatcatttccagaccttgctggcggcctttcttgtactgcgtgaatcggtattttaccgatctttgcgctactgtcaacaaattttttgttttgctatctagtgccttgctaggcttgccagtgatcaataaagtttgtttcatatcgtcgattccttataatgtataagtttaccgccgataggctttaagatgtacccaatttttaaagagcgcggcggtaacttcccgccgtgtagttcgtcattgccgtcctacgtgataaataataggggattcccgaaaatggcgcaaccttatttttgtaaagaaacgtaaagacacgattcaccgcacgccgtccggcggcatgggcgcggcgcactaaaattaaaagaaacgggcgcgcgagtaccacaaaacagagcaaataggcaagtaattttttcatttatatttgctttgccctacttgacaaaacttaaaaagctcgtggtagcgataaacgagggtaggcaatgcaatggcacggctaaaactttcatcgcgttctagggcgttttaggcgcattctagccttgttgataacttatccccaaaagcaaaaatgaaattttcctagttatccacttgacttttattttccagtggataactacttattttatgaaataaattaattgacttttatttgttagtatgcatcggaagaatagcagactaataattactagaataataatcatgctggtggattgtaacggcctaaactatcagcagactattaatcacgaaaaatctcgttagctaactaactatttcatgatgtataatatacatataaattaatgagaaataataattataataaataataactacagtaaataataactataagaaactatcggcctaagtgagaaccactatcatttaagttatccacaacgttatccacagcacaaaataatttgacacgataggcggcgatataagggcttatccacagacttatccacaggttatcctactgtataaatatacagggtagaaaggtagtgttaacaactgcaatcaattttaagcggcctaaaacgctttctaacgagctaaatgcggtggggtaatattaaagtaaagccttcacccgtcgccctggtggcttcgccgtgttttgctctttattgcaccgctgcgcggttagcataaaactaggcgctaggcaaggaaaataaaaaggtaaaataatatttgcctatgttagaaaattacctttatcattcactcaccgattaacgagggaggccgaacaaatgaggctatataaaccagataacgcaaccgtcttaaaaggtgcgctgcgtaacctgctggacggtagcagaacaaccagcatcaaacattttgttttcaatattgaaactattcatcaaaacttttttggtgattatgatgcttataatatggatagttttctaccgttatataaacaaggggcaacgcttgttttatataatcaggaatctcacttgcttactagtcgagggccagatactgattttattttagtaaaaggcaacacagtaaaagcctatgatgcgggggcgggcttagaagttttcacaatagaaaactatgaggctaatgataatgatctttatgatgtagaaaattttctcgattcattttggcgttatttatcagttggatggaatcgatcagattatgacgggtatcgttttgcggctgtaatggcttttgatgataacggtaattttttattaccatcggaattatacccgtatgtgcataatgagctagtacaagaagcgggttttattttctggaaagatgaagatcagattattgacagcgtagaaaaccatgctgtaaattctaacactcaaagcgttaaaactcaaactactgaaaacaaaggaaaaaacaccatgaccaagatcgctaatattgttgccgctaataaatccgctgttgtaaacgctgcaaaactggaagcgggtaaaattgcactgactcaaattacgaaagtagcggctaaaaaagcaccgtttatgattaaaggttatattgatacacctatcggtcgagtagtgattgccaacctgctgagcgtagcggttgaccagtacgccccaagtaaccaaaaggcgaaagcggtggcaggtgcagctatggaagcggctatgttagaaatggtgcaaagttttaacatcgctgagatgattgatgaaatggtaaaaggtattgatatttctacttttaccactagcaccgaaagcgagtaataatattaagcggggattgttaccccgctttactattcccttgttaactaataggaggctaataaatggcggatgaaaaatatggcttctcactgggagaagtgagcacggcaaaacatgatatgatcattttggtcgattgtcatactggctattgcggggaagggaacaccgaggaatattttgttcctactggtacggatctggacgctttcgctcaggaaatggctattgataatgcctctcgttttggtagcgatggttacgaagacgaagaaactggcgaatggtatgataatgaaaacgtatatgcaagcctttatcattatcaattaagtaaatccggcacatatgtaaacggcggcgatcctattaattccgtcatgagattaattattaaatatggcggcgtcgagataattgacaacaaagcggtaatatatgcaaaccgattaaaacagcttgtttatattcctgatagtacccgatgggatgaatatgctgttttgcatgacgaattgaaacgatgtttcaatattgaatccttacaagtagtctaatgtaaagttttgtaaaggtcgccttttatggtggccttttttgttataatgcctttacaccgtttgaggacggttgaaaattttcccaaaaattggaggcttaaaatggttgcttactcttctgctagtcatctgttcaccgctcaaggctgggtatctaaccgcgttattattcacgaaatggtgcaagaatatggcattgctaaaacttacactaccattcaggcgctttatgataatgatcaaatcgatcagcaaacggctggctttttgctggataccctgaaagcagaacattgcaccaaaaaacaagcggctaaaattgttttaatgtaattaataacgggggatattatatcccccgctaactaggaggatgaaaatggttatttttcgagctattctggcgggtatcttgggcgctattttatctttatttgcaatagctttcgacgttcacgcggttattatcggcgcgggtatcgctgtattttcttatctgctgggctgcatgactagtaaaggagaataaaaatgatccgcaacgtttcccttgcacgttcgaaaggctttaagctggtggacgttaacacgttcgagcgtgaagattgtaaaatcgaatatgtagcacgtaataagaatgcctttcgtgttaccgagaaaaaattcgataagcgcggcaacgtgatcgctgaaacggttaaacactttgccaccttttacgctgcgtttcggggagtgttataaaatggtaatttatgaaggtaatcgttttgttgctaattgccgtccggcattattagcaaactatttaaaccagctttcaccagcttataagggcgttattaatatttatgagggcacggcgcattataaaatcaatgcggtcgttgcccgtgaactagcgtttcaatttttgacctttgcatcttgtgacgttcaggttatgggtgaagcgttaattgcagaaaatgaagatgattttattaatattttccgcaagatatgcaccgagcgcctgataatgaaaggcgcgtatattcaatccactgcggatagtattgaaacagcgtttcgaaaggtggcgcaatgagattatatattttcgcgggtaatgttgaggctgcaaatgattccgctggtggcgataacgttcgtcactactggcaaaaatatatttactaggggttattatgagcaataaaattattgtgaccaaaactaccacaacggttgacgttttttatgtgcctgatacgccggaaaaccggcaagcggtcgagcggggcgaatatgatagcgttatttatgatcacgatggttactaccaacatttggtggattcctacggggaggaggaaaaaatcacgcatcaattaccggactgacaacaagcggggatctgctccccgtttttcacgcctccagttaaatacctctttgttttagtatccccaccaaaattaaacgcgtcagaatgcgatctaggacgttttagcggtatattagaattattcactacataggaatactgtatatttatacagtaggataagctgtggataagtctgttaataacgcttcaaaatggctaggattctgtcaagtcaaatcgtgctgttaataagtctgtggataacttaaataacagtgtttctcacttccattcttaaatgagaatcattatcattcgcattccactgtctaaccgataatcatttcactttttgaatagttctcatttcacttcttaaatgagaatcattatcattcgcattccacttcttaaatgataatgattctcattcaaagtcgcagggcaattgccctgcgcttttgtgcaaatccgacatttgcccccatggattacgcgtgggcatgtatgtgcaaatccgacaatttttggtagtgtgcaaatccgacccgaaaaatttttatagtgtgcaaatccgacaatgaattttcccaaaaactccagcaatcacgaactgcgttcgaatcctgtggaattagctagaatatgtgcaaatccgacatgtgttgaggtgtgcgaatccgacaagatttttatgacttcgatgagaaggtgtgtgattgtataggtttgaggaaaagatgagagagcgagagaaattttggggctagaaggatgtgggcgcaggattggtgcggagcacctgatttgcaggtattttgggggagagttgagataatttgggaagatttgagataggtgcagaaaaagtaaaattttattagctaaatggggcaaaatagcttgacaagtgaaaattcttgtggctctaaaaactcaggcaatcacgggccttcggcccgaaataatgctgctattttcaggagagtaagagttcctaaaaacttaggcgtttgtgcaaatccgaccataaatttctagaaacacaatgtgcaaatccgacagtaaaatccagaaatgtgttttcaaaaaatgtctcctagaaataaccgccctccctataaccgccctatattaaccgcctattgctagagtttctaggaacaatgaaaaccgcctgagttgactagagttttcctagaaacttaggagtctagaagaaagtgttgtgccatcctagtagatgagcggcaacaggtgtatcatcttgaacacagatattgcctttaaaaatatttaaataatataaagaaaaagagacccccaatttcatgagaatctctcctgggggcgcgtgattaattacgtgagtactcatgccgtcataccgctgttgctaggccgcaagctatacgagacattcgtgtaataatcatcgcccctagagttaatcaactagagtagttgttaatctatgagattattataacatgtttgggtatgagaatgcaagaactttttgttaacttttattcctccttcttggatttgagtttgatgcctaaggatgcgaagtagatataagttgctaaataggaagcagtggatcctgtatcatcgtaatccatagttccacgagctgctctagtatattcaggagcatagtttaatatcgtgtaacttggcattcctagcgacttacatagttctttaaatgtatcttcgtatttatggcacatgaaatgcacagcattttctaatggcgttaactctagatctttatggagagctacagtcaaactcgctagcattgtgccaatcccacgataaacttcatctttaactagagttggtttctctttttctagtggaggaaggtgggcatatttcccatgtttgaaagggataagatcttcgctagctaatgcttctttaaatgatgcttccttaaatcttgggagatcttcatcgattaggatatgaatagcattagaggagaaaccttttgcttcaggatctaaagctttcaacgctttattcacttctacatatgagcctgaccaaactacttgttttgcatctcgatcatacttgatcttacctttatcccacctagcaggataatgatctcctaaaaacattactgcatatttttcttcctcagttagctgggaaagactcttttgtgtagcaccacgcgctaactgaatgagacgttttaatttttcagcttctttaatcatatatcagacgcttgctcccctgtttctttcttttctgtcttaggttttcttgcaacttctccaaaggttcctttggttctttctttagctggaagatctactttataccataggattcctaattgttgcgctaaatgggctatattctttggtgttatacttggaacatcttccctatcagaaactttagaaattatatcaagtaactctcctatttttggcttactagtagttattagaatatattctaatgtttctatttctacattttcatctttatagtaaagactaagagtaattaaatcgtcaccagcagaagttatttttgttttaccaaatatcattaactacctctcttatcttcattaagagcagctcccaacgcttcaaggatagtatcatttatactcccaggcctaagattattaaagtgagtaacatagatgggacttctaaaaccctcagcatccgcaggtgctacgcttcgcatatcagattcaaaagcttcttgagtatgttgcaactgtacagaagggccgtaatcttcaccaactcgatatgaggaattattttctataacgccaccacatggaacattgtgcaaatccgacgttattttaggattaaatgcgataccacttttggtccaggaacctccaacagtcacaggagtactagggcggttcacctcagtctttacgagtttataaccagcatctattaatgcgttaataaggttatcagctggaatccgagccttgccaaagatcttacgagcttcttttaatttatgctcaagatctttacaggctttaatatcagtgtgcgcaaaggttaatttcatagatttgaactgtacagtggcagttaagtctttaaaatcataatcccatgtatttaattcatggtctggtactacttgaacaggttgttgtgcatataaagtcattacttattctccaatttgtctagtagcttgtgcgctgctatgttatattgtttaagttcacgattaaggatttggttttcacactttagctctagattcttattattaagaatattgcagatcagtagaagtgctaatataactagcaaggaacctacgagcattaaaagaaaaagagtttccattatttaactcccatgtaacgtttgagatatatgatgaagtcttctgctgtatgctctacgctaccttgagctacaaatagtttgagggcttcacgttgtagtttaagagcagccaactcaccacgtaattttattagatcttctgctagttctttagctctgcgcataatagcaaatgatacaaatgttacaataaataacataactgctaaaataattactatgatctccatattaacatccagctcttatcatatatttgggcatgttctactaattcatttatcgatgtagaattatcgtagataccctctagtaaacgttttctgtcaaatttatcaaccaaatactctgtgccatttatcactaccctatacagctctggaactaaggggtgtttgtttggtattgggcgactacctaagtctatttcattatatccccacgttgttttaaatagtttgttgctaagtgctgctagtgggtttgaccatacaatatagctactcactacttatctccattcttagctttgaaaacttattataccaaattatatgattatcgtcaattacaaatttatggtaacatgctggtacggtataagttccataatccgtgacacgctgcacaaccttgtgtgcacacagtcgacaaccatgcccttctaaatgagatctagcagtttgccagtaataaccatcgtgatctggacaatagatctcgacttgctgttgcattgtcttataatttacacgctcatatccgaagaaagccccgtgagctgcaacggctttcttgataaatataaggtttagtgcttcttgctggaagtcgggatgtagctgcttaatcttagttctattaatagatccatccgatttaatgaacctatttattggaaagttgttagcttcctcgattaataattcatttactttctctctcatattaaatagtctcacagttaaggtagaaacattcgtaagcatctccagtaaactctttatcttgtagtaaacacttagcttggtcttccggtactccagcatctaataattgttgtttacttggcttttcagcgaatacttttacaaaatactcaccatcctgattatactcatttatatctctggtaaggacatatacttgcatttgaagttccttgaaaacataaaaggccagaacaattaagtcctggcctctagaattaatgaagttgtttaccacttcgtaacatagtggctgtttccataagacctagcgtagcatcacgcttattgatctgtttaccaagttcatcggtacgtttaccaatgtaagcgttaatagccatattcatagctgtagcgagatcttctttggttatctcttcatcgtctaaggctaatttagccaaagaatcaaatgtgctagagagtcctataagatctgaggtttctccagccagaataggattaatattatctactgttacttctagcatggagttaacaatatcttcaccatctattagaccagattcaatattactctcccactccttcatctgctccaataatggatttttcttttctgtcatggtagaggtttcctgtgtcagtcggtaagaaggatgattgagctttaggcggatgttgtttagcaatccagctaagaatcagtacacgactaggaacaatatcagtgttgtaccagaaatcatgaacccattgacgagcattctcaaacttaccaaatttatatgctttcttaaacaattcaaacccaaaacaatctggtgtaaagtctacttcacgatattgaactactttagaaccagttaggtcttggatcgctgcattaatttctgtatgcgagaattttgtttcgtgaaacttattaaagaatcggtagttgaagcgtccgttcgtttcgacaaacaactggatgaaaagatcgttaaattggttatcaaaccagtaattctgtagttgttgtagtgctgtcatttacgaactccgttaattgccacgatgatgccttcatacataaaaggaagtagttcagaagtgtagaagatattttccgttattcctagatgtcgaaaaagtatattaaataatgctgttagaaatacaatctggggcagtaatacaaaatactcagttacaatctttggtgcccgataaacaagacgttttatcattgtttttaagtctccttattactttggcctgctccacaataatgaaaactgcgagcactaatagtgctattagccccgcagtaattggtactaaatcaatcatgggagacgccatacgtaattagctgtctgtagaaccttaggtgtgtcatcatgatacattactacagactttggtgaatagctatcagctagctctttacgaatcatcttacattcttcaccagtatcgatatttttaactatcactttcatattaagaggtgttaatacagaaagcggtttccagaagtcctcaatctcaattcctacctttttctcgattaccatgaggacttctagtgtatcatctggaatactaatattattattcacaaactgtaatatctcatgtaaggtatttaattcattaaaattaagcttcatctttaagaatatcctcaaccatatcacaggactgttgcaattcgtcagcaatgcgcttaatatcggtcttcgtcactctaccgattaacatcaccagtaacatagaaagtataataagtgggactggaataacaaataaagctaccttaacaacattctttggcgtccatgtgtggtacttggtaaccagtacaccaaccacaattagataaaacgctagaataaacatcatcattttttaatctccgtaattatctgtgcacgcattactttattaggtaattttgtattcccagctattgcttcaatattatttagtttttcttttagaatatctgagcgtctctgtgctagttcaatatcttgttcttgttctattaagcggcagtgaagtccactattagtagtaagcatactctctatattttttcgcatgcttacaataccaataatcccgccaatcgctactagtgtagtaagaactagtaacccaataagaatttcaatcaacattaattatatactcccttagtccttatttcttacctttcagttgcttaacttcacgctcaaaagatgctgcacgacgttcggcagtcgcttgatgctctttagcaaaacgagcttcctgttttgcaaggttgaacgccatagcattcttattcagagaatcatacatctttttcatcgccggaatagacatcttcatgagctgaccctcaaaaccctgcatgtcgaggagaattgccagaacgttagccatttcgtttttagtcatgttttccattagaatttcctctctcattaacttatgaacttattatacagaattttaaggcttaaagcaactgaattttttaattacttaccaatcgttaacaacgccggagaactcagaagcaaaaactttttcaaatttctctgcaatttcaggatgatctttgcagatcagctcaatacatgcttctggagtcattccttcatcttcaggatcaccatagtatttatcccaaagatcatcgggaatgatatgctccgccaaatcttggaaagagactaactgataacgttctgcctcctcagcgataagaatttcgcatagatctttatctatatcgctacgataatccgcaattaataaggcattgcaagcatgacactcccaaaccatcaagcgttcagaaataggattagacttatcctgtacgtaagactgaaacagggttcggaaagttgccttaacttgttcaaacttatctgctgctgcgaaaactagagctttatcaactttgttcattttgattccttctcatcaatttatacagtaattatacagaaacttaagcattttagcaaataaaacttttaattaaaatgcctaatcctgtgccaatagcaatacaaatgattataagtattgctatcgcctgtatgattcgtttaataataacctcagctatatacttagacatttatatcgccacgcaatacagcagctacgtcttctcctatttgtaatacctcgccggtagtacaattaaccactctatcgtaactagtaaacttaccagacacaatatcctctagtggaattggagttctactcatttcaaatgagacattaatataacgtgggtcacgtaaagaagtagtatgtacatgtccgtgaatatttagtttgccacgaagttcattgggatgcaaagggcagtgagatagccaaaactttttgccacctccagtctgtttgcctagagcttgaatatcgtcataaacttccgctaagtccctaatactcagtccttgacgctccgcatcatgattacccataatgagttgattagggacattgtggataaccgactttaatttggccagaccttcacgacctactgcaatatctcctagcaaaataagttttgttcgtttaccaatatgcttggacaaagtatctagaatatactcgtcgtgctctttcatgttcttaaaccacggacggaaacgtaacgctccagggtggtctagatgcaagtctgaccagaatttaactttcattactcttttccttattctgtattaaactatcaacccaagaggttaacactttggttttaaactcctcgggagtctctccttccttaaggtctacctcattaaggtaggtagtaagccttgtttctatatctatttcagtaggagaattaaaacaaaaattgactgctattccagaatatattactccggtatctcctttgacgaaagcattaactaatgccctccaacgaagggcatcaatacgcattgctcgtaattcttctcgtacttctttcattctatcattcattaaagagtcctctgtacaccgcagctattatttttgtctgtggtaaatgtggtgattttgccagtttcatcattaacttgcgcaaccgtcaactgcccgttgaagacaccgccagtatctaggtaaacacggtttttatagagaagcgggtaaggtactccagtatgcccatggaacacaaagtctactccactaactggaggtacttctaccatgtatttttctttaaatcctgcataacgctggaaatacgagtgttcctcgccatttttagacaaatggaagcctatttcttggattacatctcgatcccataagtatggttcaacatggtatccaggatggtcatgcgggtcttccttagctgcttctacttgtgcaataaggttatcccatactggggtttctacttcgttaccacattctttgtacgtaaaaggtacaccaccatgaacaacaccatacttcttaccacgatgtctaacagttaggaatactggcattttttcagccatgtcttcggcaatatttttaatggtatctgcatctagctcattcatagcccacataccaccgttatacatccaattagcccaatctcccacaatcataaactggtcgtggtttccacgaacgctacaaaaacgtggattatataagaatttagctaaaacttgtaggttctgcgtgcctcgatcaattaaatcccccacgcatataacgcaatctttcttgccgttatagccagctaattgtagggcatcttctagcaaatcattgcatccatgaatatcgccaacaaagaataagttaacatcatcaggtactactagtgttttatgcacattaaattcttttttcataattattcccaaataacatttaaaatagttgtgccatattcattagatagttggagagtataaccctctttattgagggcttttatagcttcataactaatttcgtcacggttaaactgcacataagaacctccaatctctacagaagatactatcctccgcttaacccatctatatgttttctttcggctcttaagggacgcggctctatttatcctagctaaacgttttgcttgctctgctaacatttaatcctcctatcaatctatacaaatattataccaaaatttttagcaaaaagcaagtaaaataaaagcctgatccgctaagatcaggcttggtttattaatcctctggattatcatccaggaaatttttaatagcttcgtgcatagtttctttacgaagctgacgtccaatcaaaatatgattagcttctattcgaccattaggtaagcgatctgccagaactactacaggtacttgacgtacaccaaatttctgcattaattctgtattatcagtctctttatggatttccaaattatagtcattgactactttatcaaatactggttcgaaaagtttacatgggttacaggtggaaccttttaatagatagactaatttagacatttttatttcctttgctggcaaactcaccgtggagttcttctagtttttcatctctccatgcaattgcttcttccaaagaactgcacgttttcatataattgattcctgctctagagatttttactctaaaagacttccctctttgagatatattttttaatcccaataggttatttttattagccgatttcctattaaaagcattttgagcttttgtagcttctcttaagttaccaatacgattgtttagcgtattggtatcatcatgatctactatatcaggtaaatagcctttgtgcataaagaagattgctctatgcgcaagtattcgttctccatcaatagagagcattagatagccatcagcattaatagacccagcaggcatattgttaaggctagtattccaacctcttgtaccttccggtctaggtttccaggttagagtaccatcttcgtggtactctaatacctctaataatctctccctagtaatcacaatttattaatggcctctaagaagtttttcatagtttttacggttgcggtgctcagatcaagatttacacccaaacactcggttaatgcttcctgataaggagcctttaatctgccttctgggacttctaccttcttatactctttatttttgacctttttaatcatagtctctagtacaagaagcggtaatttagcaccttcaatatcagtacccaaaagttcagttaaaattttattaagatcaagacgagttaactttttgcccttagacatagatgcacctacctttgtatcaatagatttttccgctttcttttcgagctttttgtactcaggagagtcatgatcacggagtgcaatgtttagctcgtaatgtggtatacgaaaatgttccgccatttgagtgtagaaacgatcagacataatatatacctctcttaactaatttatgtatatattatataataactagggctaaaagtcaactacttttttatcttaatctactgcatgtataaatcttttcctaactagatacatagttattgggtaaattgagtacataagtatcggggagaaaagggtgaaatacgctgtaactcccccagctaacatcaaaggtattaatgctagagtaagggccataagaatcataccgaatgaaacagccagagctatggatataggattctctagttccatccataaccaacaatatttcgtatctctatggcaattgcatttacaaacgccgaatgaacccataattatatactctagtccgtgaataacctttattaataagctatttcgggtagttaatgcaatgatagtaaagactatcattaaaacgaatactactagacttattttccagatacctagcagcatcatagtgaatagttctgcaaacatggctttctcctatcttcaaaaattattaaagccccctttgcctaaaaaggcgggaatattcccgcctaagttattaattaaactagttcgacatgaccgccatcataggtaccacgttttatttcatcgtgatagtctcccgaagcattccaatcagcaccaaaacgaagtttaatgcctagctctttaccagcttgttcaaaagcctttttaactgcccaaaatgcttctaagtcattccaatcaattttgccattaatatatggagcaaaatcaatagcatccccagtaatatgtttgcttttactaggatcttttagaaatgaagtaccattagcaatgttctgggcactttgtgctactgtacgaataccttgcacgattgtgaaatcatacggagatagttctaaagccctacgagctactttttgtagctcgggcttaacggtagctaattgtttttcactatttttaccaaatttaaaactcatattgatctacctaaagatctctgttgtggggaacagagctttgctaaatattccttgaactgttcagaatcagctgtatctaccggattatctttccaagcaataccaatgtacccagcatagatattttttagattgaagtatggacaagtgtatatgtaattaaaagtaacgtttttaaacgcaggtatatttaaccccatatatttatttactcttacacttaaatccgatgcgtagttaaagccctctaaatgacgtctgtataattcagacgttttatttaccgctttatcggccaagtcagccctatctaattgcgcattactttcccatgcaataatattggaataatcattgatagcatctggtttatacttgactacaaaaacagcatctgcacccgtttgagagaagagaaccatgctcttttccctcgccacattagggaagttatctatcctctgggtttgtaaatcttgtaaaactgcagacgtggaaaaagtctttaagaatgacatcacttcactagtattactaacaaataagaaaataatgacagcaactaagatagttagcagacgtttaagaagcgatgctggatctttcgcttcttggagcagtaccgttaataattgtaagaacttttccaattgtaacctcctctaaccagtaccattatactaattttggaggaaaattacaatgtgtttttaaagatcacttctggagcataaaattttgtcgttgtcaagaagaattttagataaaagaaaagccagggtcgttaaaccctggcttaaaattacttactcttcgttatgctcctcggattgaggtaactgggctttattatattgctcagatcgatattttgccaagatttcaatacgcttatggatttctttgctatctagatagatatttttgttgtcttttaccatctcgtcgatttcgtctatagagaagaacggatagtagacatctagcatcatatcttctacgaacttgttgtaagattcataggctttcttgatttcttgacccttctcacagaatccgccagagaacgtgtgtcccattagcgtagcatgtggatgtactacccatccatgacaggataggaaaattgtgcagtaagcagaagcactaggaccaatcaggtgtcctataactgttccacggcaattagcaattaagttagataactgtgcagcagtatcaacataaccaccagggccattaatcatcagattaatttcgtcgtcctcatttgcttgcataagtaccattgataaatcacggtattcatccggcgggcctaattcttcatcaaagaaaaaggtatactcattagactggcgaatggagtgaaacaggttagtcttttcttcttttttattagtcatagcgatccttgattatccaactagtggttctagctctaagtcacagaagttataaacttctagtttaaggttattgataccatcgaatttattaactaattcgtgagtaatatattttgcaggaataccactttcagatggatgatctgatttaatagtgaacttctgctcagcgggtactacatttactatcaaagaatccatatctaaatggtttgtttctctgagtaactctccttcattggggaatctaacatctgttattacggcgacatctgggtcgtctttagcgatggattgctccagaattatgagccaaatgcgttcatgtaccagctgccttcctagctctgttcctacgagctgtaacatttttctcggagaaataaataaactataaagtccgtcttctttattctctgagataagttgttgaggattaagatatttttcctcaaaaatcggccaaacgtacgagaagtcttcaaacttattgataccgtatttaaaccatacgtctctagctcgctccaattgagattgtgtgaccgtaaaccattggtcaatctctttccccctgcgctctcctagaaactctggagttacaccgaggattacggatgcaagttcataaacgggcttagcaaaactataacgacggggtaaacacgttggatacgtgtcattacaccaatcgataattaattttgcaacggtatcttttcccgaaccagcttcaccatgtaaaccgactaatactgacattaatctttcctattgttaattggtggataatatactaaacaacgtttttcttgcaaatcttggcggtagaagcaaaccatactagtcagtcgtgagatatatgaatattctgcctcacggcattttgccaacatattccaatctttgtatggtacaacaactactacgccatcttccccatttgtagctaatttcttttcaaacttaaagtcaaagctacaaggctgaagtcctttaggccaatccacatgggcttgctttaactcatgtgacggctctggtactaccgtttctgcacagcctgtgattgtgattgcggctgcgagcagtattccaagtttccagttaaacatgctaatctttcctcgaactccttactctgctttttagcaattaatgtaaccaatccaggctttgcagctataatatcttggcgactaagagctttgtctaactgcttaatctttttgtctagatctgcttgcgaaatattattcattgtgaaatactgattcattctagtctcacgaagttcgctttcagctttcaccttattgagggaagtctctagagaagaaatctttttagtagccaccgcaagatctcctgctaaagtctccactttatctactaagtgataagcaccgaacccgatgcctatcgctagacctgctcccaggatatacatcttgttattccaaactaagtctacaaaccatttccgcattagcctgtactcgcaaactcaccgtggagttctttgagtttggtatcccgccattttatagcctcttccaaactcttaagtgttttcgaaacttgcttaccatgtttggtaattcttacttggtaagtcccatttgtttttctatggatatttttaacgcctaaatggttatcgcttcttactttttggttacaagcattatcagatcttgtagcaggccttagattctcaaatctatcattagttgagtctttgtccttgtgatcaactatttcaggccattctccagtatgccatgcatagattaatctatgtgcccctatagctatggaaccattatatagttcaactactctatgccctgtactttgtctagatcctgctactgttccggcgaatatcttattaaaatgttcgtccccttccctgggtttccagataagattaccatcttcttggtaatcgaacattcttcttagctcttccttactgatcatcttttcatattcctaaaagaagtaacagtatcaaatccatgtgcagctaagcgatccttatcggaaatcgtaatagtatttggttcgccggttcctaacacgccccagatatattgctcgatcatctggtgcaaacggtataagttactttcaatttcctgccacggaatacctgactgatggaaacgaatgttagtctgaatcacgaagttacgaacatcatcgttatcgttcttcttgatacctttcacatatgcaatcggtacacgcagttcggacaagatacgttctgctttaggttttgcttcaacgagcaaatcacgcattgtttcacgaacatctccgcgactcttatccattaagtaagagcgagcatgcaatcccatctcttccattttatcgaacatagtgtcgaggttgaacgttttgaagctaaatgctggatgccagcagtacagctcgtgtaaccagtaaacttcacctgcaacaaatagtgggtttacaaaatattcgaaatcaccacggaaagatagcgaaccatcacgaaatacctgacgactatgcacgatgttcttttctgcatcatcagttactttaaccagtagctcttcagttttacgctcccaaacacgatctgcatcaaataaactgttctgcaaatcatatacatcggcgaatttagaaatgatcctcatatttaatcctcttgcctcaatctataaacatattatacaaaagttgggcatctaagcaactaaaattttattataaaaatagcccagtcgcaaaagtgcaggctgggctttgtcattatttgcttttgctagtaagctgacttagtgtcaatcttatgtaatattagtttctctagctttgcgtagtacccctgcatttctccacaatttgatgtcagcaactgtttctttataaggagctatggtaaaacctagtgggccagcactaaataatcctaagaaccctacaatacgcatgtagaacaagcattctttggctgtcatattatttactgcttttttctgcttttcatctttaaacttctgttcttgatcaccaatacgtagatatttaacaaaccattcagcagaatgttcgtccaaatgtctaataatagctatcgcatatccagcaccgattaaaaaccaagttgcaacaagaattagtaatatagtcatattatctccagttagggctagcagccacctcaccacttaccgcactaaggggcacgactcccttatccgtaacagttgcaggtgacgcaactcggtcctacgcgagttctttaagtattctgcatttcagctttaaattttttcatattacgagtttttctataaaagaaaaacacagatgttgggcctagaagaatatccacaataaatatcacagatctagcacatctgagtaatgttttatcatcaagaggtggcagatctaacggtcgagttttatgtataacgtataatattacatctttattcttagaaatataaagatcatcaaccaagctgtaaatagcaaccacagatccaatgacaaaccaaagagcaaatggagagataatcatttcagatccttttcattaattagaatattagtaaacagtggagtaactcctagactcatagtaggtccaaacgtattcatggctacccatagctgcatagtgatcatcccatctttaatctctggatctttatattcttcgatacgtttcttggtaaaagcaactatatctggattatttttattttcctgaatatagtcatgccaaaactgagtattctcactacgtaggaatgttaaaacatccttagttgctggaatctgcactgtgctgttgatgtttagtcttttcacgttcttctctccgacgtttgcgttcttttatcatatgagctgctacaacttcatggtagtagtcattaatgttatcttctggcaagaaatgcttaatagtctctagctgacaaataactcgatgaagatggttatttggtagacacaattttatacctgcaacaaatccagagaagcctggaacactgaacatgggttgggcttctactctaccttcagagttgatattaagctcaattgagatacccattttcacgctataaagctggcaatattctccgttaccagaccttgaccaaacagtgaagtcctcatcaatttgatcttgaatttctgtaatagcaaatttaattctaggatctaaattattcatcttcaccttcaaagtcgcaatcataacgacaagtaaaagaatcagaactattagtacgttgagtggttatttcaccgcgtttgctaatagtaacggctggagtagagaagtttttattagtatatatttctactttaccattacgttccttaacatcacgcactttaccatactcggtaataatgccgttctgttggactttaacattaccatttttcatagaaactttggtagatgccagagaaccgaaactaactgtggagatcatcagtgcaataataaacttattcatcttcatcctccccactacaatcacgacatacatcataatcgttgaaagaacgttcgtgagcttcacaccaccaagaacaagaatcgcagagaaacatttcggttttctctagtgcttgacctaaaagatcatcagcttcctcagcagtaatcttcaatccgcacacatctgccacacgttctttaattaaacgacctgcttcgtgataagacatacaggttcccacaacatcatgttcaagaacatgaacagcacagtctagacgagttttcatttcaaacctctctcatcaatttataaatatattatagcaagaaaagagaggtttagcaaatgaattatttcagaatttagtcatagcaccaccataatccacgcttacgcatgtcatgatcgcgattataatcataattttctggatctttcatcacgcggtggagttcttgacgattcccttgacgaaccattttattagaatgccacttaacattcttactaatagaattccagttataaccatcctttttctcattacgaatggttgcttccttcatttcctgttctacatcatcccaggatttagcataaataacacgaatccagtagccattttctttgatgaaagaatattcttgagagaattgttctttagacttccaccactgatcaccagattgtttacgataagtacggctcatattacctccattaagtcttttaaattaacctaatgtggatgaattttgttatacatatattatgtacctttatacagaaaaaccccagactacttattcaatagctggggtttgttattaattacagatcggggcgttcatcttcgaaacagcctgagctaattccttctccgaatcctacaaagccatcaaattcatcatttgagatgcccataatcattgcttccattttcctaatctccgaaattttcatgcctgctttactattcttataatatttgcgagggttcccgcacatccaacaagaacagatgcaaggagtagtagtgataatacctaaccgcttagggctttcttcatgtgggaagactgtccaatacttcttgcggttgttcttcacacgttgccggtgatggcgtcttaatgctcgatccacacatttctcctaaaacttgggagataaacggagtttgctcgactaccttgcgtagctgggagaaatcatatccaaaccccattacatcgcctgagtaaatgtacgactaataacgtcgttctgttgttcacgagtcagtgcattaaatcgaacagcgtagccagagacacggatggtcaactgaggatatttttcaggatgtttctgcgcatccaaaagctgatcacggcttaacacattgacatttaggtgctgaccaccttcgatttgaggggcgacttccaccttaacttcacggaaggcttcgggatcgaattgtggtgtgataccttctagatcttcaactagaactttctgtttaagttcaccattgtcggagtatagctgaataatctgattttcatgaacaaggttaattacgccagacttaagattttgatatgctttcattagatctccctgatgttagaatttggctcagctctttattgtctatagtttaccacgatatacagaaactgtcttaccagtttggttcataacgtatgctacttcatcttcttttaagaagattgcttgatctattccagaaatagctatgcttttatttctgggattaaaccctacgcttttaccaacatgaatctgctcaccaccatcagtggacattattttaactgttaacataattgctcctatatttagctatctctagctcttttaatggtagttagtagtggatttgaaccactgtagtcgctccgtatgaaggaggtgcataaccactctgccaactaactgttatgttttactagactaagtaagtattctttatactctttagaccaattagcttttttaaactttcctggacgcatagtcttaattcctagatttggtactccgggagggatttaaacccccgatctctcggttatcagccgagtgctttagatcgctaagctaccgaagtattagaatatttacatcatacactgtctaagtaagaagtataatggaatttagcttctccagtcttatctacttctacctcagttcgtggtacttgacgaaccacaccatgaatcatcttatagcgaatgcctttagctggttcatgatcttttgggaatacttgtttaaccgttactactttatatccttcacgcggtgttaacactactacttgatcaccttctttgattttccaagaagatggaaattcataggtatatctttgaccaccagtttggaatactacagaaagataacgtttcatttggtttccctctcattaatttatatagatattataacaagaaataagagagaaggcaaatgaatttttaaatttggtgctcccaccaggaatcgaacccggttcagatgcttacaaggcaactgcatcgccagcaatgctttaggagcgatgatcccgttatttcaacgggatttctttttcaataacaggagacttatcagtcataactgtcattgccatttgttgtagaaattcaaaggtgaaggctacacgttcttcaccaatctctacttctacacgtttcttttgtttatcaatctttacttttaggttgtcagccatcttcgggttctcgttgctgtactacttctagccagtctggtagaagaaactttgtacgaaattcttcgtaagtttctttgggataaaagctaaaacctcctttctcatcattcaggataacagaaccgtcagtttgttcatatgctcgatatgtttctccaataatgataactcgcttatcagtacttttattatgaaactcaaaaacgtgcataatgtttccttaaagttggagcggctagagggaatcgaaccctactcagcgaggcttggaaggcctgcgacacaacccgtgtgcttaaccgcttattatttggctggagaaggaggaatcgaacctaccattaacggagtcaaaggccgttgtgctaaccgttacactactctccaagtatttggctgggatgccacggattgaacgtggaaccttcggagtcagaggccgacgatctgccaattgatctacatcccaataattctttactttatgtaaatagggtaactgtgctaacggtcaggtaattaatcaaatcgctgtaagtcttggtgctatcactcagactctggctggtctgcaggctaaactgccggcttaatattaaggggaggagcccattatgagtaaatatggttttgtaaataacggacttaatcaaagtatgggctcccagcagcccattccgggtctggataacccctacttacaacaattgcaacagcgtttagcagaagcgcaacagatgcaacaacaactccagcaaaaccctggaagtgtgagtcctatgcaaatgatgcagcaaatgagcgggcagtcgcaaatgcctcaacaaatgcagcaacagatgccgcagcagcaagttcagcagcaaacccaacaaccgcaggtttctgcggaaggacaggcagtactagcccttttcgaagacttcacaaagacagaggatgggaagcagcttgtatcacttatgggtaagtttaatagcttctgccaaagccaagttgcaaaagctcaaaatggtggtaataactcctaaggagaaattatgtgttgcagaaaacctgtttcgtgctgcccaatgcctgtagcacgttgttgctctccagcaatgtttacacaaataccggcgttcaatccctttgcctttaagcctactcttatcctgccccctagagtagattttcagtcaagattggcctcccgtatgggtggttgctgtacaccgagagtgtggttctgaagaaccaaacaataaagcccctagtcgaaagacttaggggcttttctgtatttaagataaaagaaaagccctgcgctctccagggaacgcagggcttacttcagatgttacatgcggatattatttattacgcatatccatgatcatttgaccatcgtagccagtacctaccacagtctgtggtacaccaccttgatatttctgagcacgaatcatttcgacttccagttgtttccaacgaatcatctcaggagtaatggtacgttgcagtgcggcgttagcttcagcttctttcttagctgcgtacagtttagcatctgcgtcacgttcattagcgatagcttggttgttgcgagcttcacgatctgcttctgcttgtttaactttttgctgtgcttcctgttcaacacgagctaattcagctttagcagcattaacctgttcttcacgaactttggtattctgtacctgttccatgattaccggtggcaaagtaatatcctgaaggaatacctgcttaactgtgtaaccatatgggcgtgcatactcttcaacttcctgttgaattgcagtttgcaattgagcctgaattttagcatcaaacaaatcttgtgctttaggtacagacttaccaaactcacgaatagtagacagtaatttttcagttacatatttgtctaacgcttgatcctgagtacctgcgttaatacggttaattggtgccttagaaccatcaaactgcaacataacagtcaggtcaacagtggatttaaacttatcctggctaggaacctgaagtttatctaattttacagcaatatcttttgtactaaaagtgtcgaaagatgcaaatgggtttacaagatggaaacctggtaatactgggttaggatctactttacccagaaatgtttgggttttaaccgtaccatcagaaacaatagtatatgaattaaaggctagaatcaagcctgctaaaccaactacagcaccaataccccaacgtttaatagtacgaattactttctgctcagaagtcagttctttcatatttttagtattaaacatatatttcctttgttttagttacagttaataaaattggccgaggtgacaggattcgaacctgcataaaggaatttagaagactcctgcctctcccttagactacaccccgtttaaatatttttaagaactctcgtaaaaactcttaaaaatacagacgataccgggagagtcataagtctcactcattaagtatttcaagacaaaatacagtaacgtctattattttccagtttaagtcagggtgacttagtggttaggtcctgcggtatattgaggactcggttaggcttggggtcatgacttcccgccttttgctgctactcaacaggagttatcgcgaattacctgtgctattgtgcaccattagtgacatctctcatgtcagcatttcccactttgtggatagcttgaaaaactactccgatatggagaaaaaacttcactatcctagaataccttctaaagttcttctttagcctggacatagttaaatcgtaataaaactattcagcagactggttggttagcctggaaccaactaccgcgtggtttaggcagtgcgcaactaacctcggaagcttttacgttaaaagcatcagttatccagttcttaccgaccgtaggattcgaacctatatcttccaccagttacggcttgataataccaattatactaggacggcagtgttactacataagtgatttccacaccccactatttataaattagagaagagtttaggggagaggtttcagacgcctcattttacacgttctagccactaaccgggattgccgccccctgtgtactagttttacaactaacctaccgactctattcaacgaatcttagtgctcgacgcatcttacattaagacaagttcagcgtaatcggctcgctgttctctaatttatgaatatattatacagaatttataagcatttagcaaataaatttttaattaaattcaccagcaatctgagcagcagtaccaccatcataacgcccaggaaattcttccttaatcgctttcatcagcataccttttgtaattcc

SEQ ID NO: 87 - DNA, 32767 bp, SP15m_6e2 phage
  source 1..32767: mol_type = genomic DNA
ggtgcagtgggtcgggcgaaaatacttagtctgctaaccgccacccccgttacaattaccatgctaattgtttcaccctgcaaccattttaattgcagggtgaaacaatttcaactttaattattacgcaacttttaatttctcaatatattgttgcgggctgcaactatattctgcgcgttcttcttcggtcatactttcccaacataattgcaggcggtcggctaggaattgataatcattatcatcgtcgagcgattcatcaataaaggtttcacctatcaatgtaacaccgattgatagaatatcgttaatagcttgcgcgtccagcgttttaaatccgtatgatgccgccgctgatagcacgcctttatgatcatcaatcatcgtaaaatcagcgttcggatataactgtttaaataactcaaaataataagatttataaactgcgtctttgctgtggtatatttcgctaactttatcagcttcaaaatatttgtgcagcgtgtcacgggagaacacgcggatattgctgttcccacgccctcgcaatccttgcttgcgtaggaagtaataatctgacttgctcattagtcgagcggtgcaaataatgtttaaagtatttgcgtcattcatgcactggcgcatatatgtaacaaggggcaataaggaatcttgcattattaaatcatgtttgcaggcttcatttttatacttatttaaatctaaattgccctcgctatcaaagcaaggcgctacacgatgaaacgaattaatgatagtgccgtctaaatcccaaatcataacgcgggaaatatgcgggaaattacgggtaatattcattttaacttgattcattttgttacgttctccatttaagggattagattaattcaatctagcccactaattatattttgttagtgggctatgtttaattaactattagaatgctagaccgaaagcgagagcgtcggcaataaagctaacatcttcacctgatacataggaacgaatccccgcacaagtatatacttttgcgctgatcaattgatcatcgaggcaagcggggcaaggcgcgacaactgcaaaggctaggccggattttacagcgtcgatgataatcgtttcttgtttcaccgtatcaatataaacgcctgcggccttaatgtaactacttgcgcagccttgcgtataggcaaaggtagtaacctgcaaggcgtcgttaaattcgattaaatcatcgacaacgtgccccgcctcgacgtgataacgctcaccattagaataaaccagaacaattgaggattgagcgcgatcgaatggaatattttgctttttcatatttatataactccaattagtttaataaggggtttaatttatttgataataatctgcatttgatacggcgttaattcaccgtttacgggtaaattattatcgcttagccactcataaaaagcaccatcatcatcaaaagggacaatatcgttatcacgggaatcgacggaaataataccatccgtattagttttggcggctaggataggcccgaagctgtaaactttatcagattccatttcatccggtgaaatgaatactttttcgtccaatgttttgggtaatgtaactttcattctaatttagctcctgtaatagcggctatatttcaagccgctagggtaataatttaattatgcaaagaatttaccgttcttaaagtcgatcaaagtacgctgaccgtttgcataggtaattaaatgcgtttgtgtccagcttgacgcgccaacgttgtaacccatatccagactatcagctacgccagcggtatataccccgccgtaaatgctggcggtatgagtgtgccccgtgttcagtttacccaatttcttaaactgtttcggattgccacggctgccgtttatgccattgtgaccgtgtacgccgcattcaatgcctgcaattttaaatgattggtcagtcgttaggaaaatggcgttaaactcgcaacctgcaaccttacgcagcgcataatctagcacgttgaaagtatcgtctttttctgcaatagctccataaatcgcggcattaaggcggtgatatagttccgcgtttgctgggtcgtctttaatgttagcattacgatcatcaagccaacgggataacgccagatcatggttagattcaacaatgattgtttgcgagaaatcgcgctccattgattccagtacgcgccccgtatcgatgagatcatccagaactttatcacgtccggaggcatactgttttgctaggaatacacccgaagcgcggttgtgatggttgcgtgatgtaaagtcgtgaacgtcatggataaactgatattttggtttaagaatatcaagcaagctattttcgccagcccatgacgcagcggcgcattcttcatctaatttttcagcgtggatgtcgccatattgtaaacctaaaacgtgccccgttgtttcatagcatccggcaggagtagcgcaaacattcagatcataaaacacgccgctttcgtccattgtttcaagctggcgaacaaaaaattccccgtcctcatcgaactcaacaatcagcgcaccgaaattatgcagcgcctcggccttttgtcctgctttctgctgaatgtaatttttgagcgttgccgttccggttgaatacatgcggcgcacaatttcaccttttaaagctggcacgctttcggcggtgattttagccgctccaattgccagaccttccagattaagcgcggttgcagtttcagcgaatccagaaagcggataatctgcggttggcaaaacattaatttcagccatgaaagcaaaacggcggttatttaaaaacacgtttttattgcagatatatttatcaaaagcggaatcatatttgattccgtctgcgccctcgccattttgaaaaccgtttttgttatagatatattttgaaacgagcaaatcagcgccgatatatttagcaaattgctccagtgaggctaaaaagtttttatgcgggaaagtattattctgaatcgatgtaataataaagcgtttgccttgttttacttcccagctttccaccgtgctagaaacaatccccgccgcttctgggcgctcatcgtttttaatggcttttgctactttcgccgctttcggtttagctggtttatttgcttccaaccagtcgcagatagcggtcgagtgttttgttgtatcgtagaccgcttttgatatatcgtcgcagacctccagtttagtagcgcgcagacgtttaccatagaaattaaagtcagcggccattttcaggataacggtttgtttttctgcggaaataatcatagtataaaactccattaaagggactaggttaataacggcaatattgccaaatataacgccgcaaatgagtggcgttataatttgcaacattaatttaaaggtataaggctagaactaacaccacaagcaacggcggcaataaaacaaatcagacctaaacgctttgccaatttagacttacgtttaaaataatatgaatctaaatcattttgaaaataagcgaatagtaacgaggccgccataataaataagcctagaatgagggattcagtagggtaaaagatcattttaataactccagtcaaagggaaattatagtggggaatattccccactaattaaatttattcgcctgcggcttgtttcacttcatcggcaacgcctaacagttgcgccacggcgtccagcgtttccagttttgcgctttccagtgatgccagatcgtcggcgtctttgataatgccggaatcgatggcgtgttttgcaattacgcgcacataatgcgctttgcggattgagctaccgccgccaactttgcgcggcttatcgcttttctgatacgctttcgcgctggtcaattttgagcgaacggacacgggagaagccgcgcccactgctttcgcgatctctttcaggccgtcgctatttgcgaaatctaaaccgttttcattaattaactgctggtacatggtaacagctttttgggtgttttcttcattccatgcaaattttgcggatttttcggttttaacgttagccatgattgtagctcctattagtttaatttaagggataagattaacataatgttaatcgttatataccccgaactactggggtatataaagttaacactaaattataaaacagcttcccatttttcgttacgctggacaacctttacaacgtcgccggatttaacgcgaacgctaaaaacggttttgccgttgttactacgttccgtttcagcgtataccgcgtcgattgtatcaaatggcataagcgccgcgcctttaatgcgttcggcctttccggttaattcatccgttttagtaacgaaaggaataaaaacggattgaccaattttaggcgtggtaataatgttttgcatagtataaactccaagttatttaggggattgttccgcattacctgctagaaagtagcaggtaataagcaacaatccgctcgccaatataatcaatttaaagaactccacgcaggccgctatatcccagttagggggcggggcacattatggtaagtgccgaccgtcaaattttatcaaattatcgctcttatcgaactgggtacatcttaaagcctatcggctagggtgtcaaactattttttgcagttttttatggttttccttcaggtcgatcataatattacgccagatcatttccagaccttgctggcggcctttcttgtactgcgtgaatcggtattttaccgatctttgcgctactgtcaacaaattttttgttttgctatctagtgccttgctaggcttgccagtgatcaataaagtttgtttcatatcgtcgattccttataatgtataagtttaccgccgataggctttaagatgtacccaatttttaaagagcgcggcggtaacttcccgccgtgtagttcgtcattgccgtcctacgtgataaataataggggattcccgaaaatggcgcaaccttatttttgtaaagaaacgtaaagacacgattcaccgcacgccgtccggcggcatgggcgcggcgcactaaaattaaaagaaacgggcgcgcgagtaccacaaaacagagcaaataggcaagtaattttttcatttatatttgctttgccctacttgacaaaacttaaaaagctcgtggtagcgataaacgagggtaggcaatgcaatggcacggctaaaactttcatcgcgttctagggcgttttaggcgcattctagccttgttgataacttatccccaaaagcaaaaatgaaattttcctagttatccacttgacttttattttccagtggataactacttattttatgaaataaattaattgacttttatttgttagtatgcatcggaagaatagcagactaataattactagaataataatcatgctggtggattgtaacggcctaaactatcagcagactattaatcacgaaaaatctcgttagctaactaactatttcatgatgtataatatacatataaattaatgagaaataataattataataaataataactacagtaaataataactataagaaactatcggcctaagtgagaaccactatcatttaagttatccacaacgttatccacagcacaaaataatttgacacgataggcggcgatataagggcttatccacagacttatccacaggttatcctactgtataaatatacagggtagaaaggtagtgttaacaactgcaatcaattttaagcggcctaaaacgctttctaacgagctaaatgcggtggggtaatattaaagtaaagccttcacccgtcgccctggtggcttcgccgtgttttgctctttattgcaccgctgcgcggttagcataaaactaggcgctaggcaaggaaaataaaaaggtaaaataatatttgcctatgttagaaaattacctttatcattcactcaccgattaacgagggaggccgaacaaatgaggctatataaaccagataacgcaaccgtcttaaaaggtgcgctgcgtaacctgctggacggtagcagaacaaccagcatcaaacattttgttttcaatattgaaactattcatcaaaacttttttggtgattatgatgcttataatatggatagttttctaccgttatataaacaaggggcaacgcttgttttatataatcaggaatctcacttgcttactagtcgagggccagatactgattttattttagtaaaaggcaacacagtaaaagcctatgatgcgggggcgggcttagaagttttcacaatagaaaactatgaggctaatgataatgatctttatgatgtagaaaattttctcgattcattttggcgttatttatcagttggatggaatcgatcagattatgacgggtatcgttttgcggctgtaatggcttttgatgataacggtaattttttattaccatcggaattatacccgtatgtgcataatgagctagtacaagaagcgggttttattttctggaaagatgaagatcagattattgacagcgtagaaaaccatgctgtaaattctaacactcaaagcgttaaaactcaaactactgaaaacaaaggaaaaaacaccatgaccaagatcgctaatattgttgccgctaataaatccgctgttgtaaacgctgcaaaactggaagcgggtaaaattgcactgactcaaattacgaaagtagcggctaaaaaagcaccgtttatgattaaaggttatattgatacacctatcggtcgagtagtgattgccaacctgctgagcgtagcggttgaccagtacgccccaagtaaccaaaaggcgaaagcggtggcaggtgcagctatggaagcggctatgttagaaatggtgcaaagttttaacatcgctgagatgattgatgaaatggtaaaaggtattgatatttctacttttaccactagcaccgaaagcgagtaataatattaagcggggattgttaccccgctttactattcccttgttaactaataggaggctaataaatggcggatgaaaaatatggcttctcactgggagaagtgagcacggcaaaacatgatatgatcattttggtcgattgtcatactggctattgcggggaagggaacaccgaggaatattttgttcctactggtacggatctggacgctttcgctcaggaaatggctattgataatgcctctcgttttggtagcgatggttacgaagacgaagaaactggcgaatggtatgataatgaaaacgtatatgcaagcctttatcattatcaattaagtaaatccggcacatatgtaaacggcggcgatcctattaattccgtcatgagattaattattaaatatggcggcgtcgagataattgacaacaaagcggtaatatatgcaaaccgattaaaacagcttgtttatattcctgatagtacccgatgggatgaatatgctgttttgcatgacgaattgaaacgatgtttcaatattgaatccttacaagtagtctaatgtaaagttttgtaaaggtcgccttttatggtggccttttttgttataatgcctttacaccgtttgaggacggttgaaaattttcccaaaaattggaggcttaaaatggttgcttactcttctgctagtcatctgttcaccgctcaaggctgggtatctaaccgcgttattattcacgaaatggtgcaagaatatggcattgctaaaacttacactaccattcaggcgctttatgataatgatcaaatcgatcagcaaacggctggctttttgctggataccctgaaagcagaacattgcaccaaaaaacaagcggctaaaattgttttaatgtaattaataacgggggatattatatcccccgctaactaggaggatgaaaatggttatttttcgagctattctggcgggtatcttgggcgctattttatctttatttgcaatagctttcgacgttcacgcggttattatcggcgcgggtatcgctgtattttcttatctgctgggctgcatgactagtaaaggagaataaaaatgatccgcaacgtttcccttgcacgttcgaaaggctttaagctggtggacgttaacacgttcgagcgtgaagattgtaaaatcgaatatgtagcacgtaataagaatgcctttcgtgttaccgagaaaaaattcgataagcgcggcaacgtgatcgctgaaacggttaaacactttgccaccttttacgctgcgtttcggggagtgttataaaatggtaatttatgaaggtaatcgttttgttgctaattgccgtccggcattattagcaaactatttaaaccagctttcaccagcttataagggcgttattaatatttatgagggcacggcgcattataaaatcaatgcggtcgttgcccgtgaactagcgtttcaatttttgacctttgcatcttgtgacgttcaggttatgggtgaagcgttaattgcagaaaatgaagatgattttattaatattttccgcaagatatgcaccgagcgcctgataatgaaaggcgcgtatattcaatccactgcggatagtattgaaacagcgtttcgaaaggtggcgcaatgagattatatattttcgcgggtaatgttgaggctgcaaatgattccgctggtggcgataacgttcgtcactactggcaaaaatatatttactaggggttattatgagcaataaaattattgtgaccaaaactaccacaacggttgacgttttttatgtgcctgatacgccggaaaaccggcaagcggtcgagcggggcgaatatgatagcgttatttatgatcacgatggttactaccaacatttggtggattcctacggggaggaggaaaaaatcacgcatcaattaccggactgacaacaagcggggatctgctccccgtttttcacgcctccagttaaatacctctttgttttagtatccccaccaaaattaaacgcgtcagaatgcgatctaggacgttttagcggtatattagaattattcactacataggaatactgtatatttatacagtaggataagctgtggataagtctgttaataacgcttcaaaatggctaggattctgtcaagtcaaatcgtgctgttaataagtctgtggataacttaaataacagtgtttctcacttccattcttaaatgagaatcattatcattcgcattccactgtctaaccgataatcatttcactttttgaatagttctcatttcacttcttaaatgagaatcattatcattcgcattccacttcttaaatgataatgattctcattcaaagtcgcagggcaattgccctgcgcttttgtgcaaatccgacatttgcccccatggattacgcgtgggcatgtatgtgcaaatccgacaatttttggtagtgtgcaaatccgacccgaaaaatttttatagtgtgcaaatccgacaatgaattttcccaaaaactccagcaatcacgaactgcgttcgaatcctgtggaattagctagaatatgtgcaaatccgacatgtgttgaggtgtgcgaatccgacaagatttttatgacttcgatgagaaggtgtgtgattgtataggtttgaggaaaagatgagagagcgagagaaattttggggctagaaggatgtgggcgcaggattggtgcggagcacctgatttgcaggtattttgggggagagttgagataatttgggaagatttgagataggtgcagaaaaagtaaaattttattagctaaatggggcaaaatagcttgacaagtgaaaattcttgtggctctaaaaactcaggcaatcacgggccttcggcccgaaataatgctgctattttcaggagagtaagagttcctaaaaacttaggcgtttgtgcaaatccgaccataaatttctagaaacacaatgtgcaaatccgacagtaaaatccagaaatgtgttttcaaaaaatgtctcctagaaataaccgccctccctataaccgccctatattaaccgcctattgctagagtttctaggaacaatgaaaaccgcctgagttgactagagttttcctagaaacttaggagtctagaagaaagtgttgtgccatcctagtagatgagcggcaacaggtgtatcatcttgaacacagatattgcctttaaaaatatttaaataatataaagaaaaagagacccccaatttcatgagaatctctcctgggggcgcgtgattaattacgtgagtactcatgccgtcataccgctgttgctaggccgcaagctatacgagacattcgtgtaataatcatcgcccctagagttaatcaactagagtagttgttaatctatgagattattataacatgtttgggtatgagaatgcaagaactttttgttaacttttattcctccttcttggatttgagtttgatgcctaaggatgcgaagtagatataagttgctaaataggaagcagtggatcctgtatcatcgtaatccatagttccacgagctgctctagtatattcaggagcatagtttaatatcgtgtaacttggcattcctagcgacttacatagttctttaaatgtatcttcgtatttatggcacatgaaatgcacagcattttctaatggcgttaactctagatctttatggagagctacagtcaaactcgctagcattgtgccaatcccacgataaacttcatctttaactagagttggtttctctttttctagtggaggaaggtgggcatatttcccatgtttgaaagggataagatcttcgctagctaatgcttctttaaatgatgcttccttaaatcttgggagatcttcatcgattaggatatgaatagcattagaggagaaaccttttgcttcaggatctaaagctttcaacgctttattcacttctacatatgagcctgaccaaactacttgttttgcatctcgatcatacttgatcttacctttatcccacctagcaggataatgatctcctaaaaacattactgcatatttttcttcctcagttagctgggaaagactcttttgtgtagcaccacgcgctaactgaatgagacgttttaatttttcagcttctttaatcatatatcagacgcttgctcccctgtttctttcttttctgtcttaggttttcttgcaacttctccaaaggttcctttggttctttctttagctggaagatctactttataccataggattcctaattgttgcgctaaatgggctatattctttggtgttatacttggaacatcttccctatcagaaactttagaaattatatcaagtaactctcctatttttggcttactagtagttattagaatatattctaatgtttctatttctacattttcatctttatagtaaagactaagagtaattaaatcgtcaccagcagaagttatttttgttttaccaaatatcattaactacctctcttatcttcattaagagcagctcccaacgcttcaaggatagtatcatttatactcccaggcctaagattattaaagtgagtaacatagatgggacttctaaaaccctcagcatccgcaggtgctacgcttcgcatatcagattcaaaagcttcttgagtatgttgcaactgtacagaagggccgtaatcttcaccaactcgatatgaggaattattttctataacgccaccacatggaacattgtgcaaatccgacgttattttaggattaaatgcgataccacttttggtccaggaacctccaacagtcacaggagtactagggcggttcacctcagtctttacgagtttataaccagcatctattaatgcgttaataaggttatcagctggaatccgagccttgccaaagatcttacgagcttcttttaatttatgctcaagatctttacaggctttaatatcagtgtgcgcaaaggttaatttcatagatttgaactgtacagtggcagttaagtctttaaaatcataatcccatgtatttaattcatggtctggtactacttgaacaggttgttgtgcatataaagtcattacttattctccaatttgtctagtagcttgtgcgctgctatgttatattgtttaagttcacgattaaggatttggttttcacactttagctctagattcttattattaagaatattgcagatcagtagaagtgctaatataactagcaaggaacctacgagcattaaaagaaaaagagtttccattatttaactcccatgtaacgtttgagatatatgatgaagtcttctgctgtatgctctacgctaccttgagctacaaatagtttgagggcttcacgttgtagtttaagagcagccaactcaccacgtaattttattagatcttctgctagttctttagctctgcgcataatagcaaatgatacaaatgttacaataaataacataactgctaaaataattactatgatctccatattaacatccagctcttatcatatatttgggcatgttctactaattcatttatcgatgtagaattatcgtagataccctctagtaaacgttttctgtcaaatttatcaaccaaatactctgtgccatttatcactaccctatacagctctggaactaaggggtgtttgtttggtattgggcgactacctaagtctatttcattatatccccacgttgttttaaatagtttgttgctaagtgctgctagtgggtttgaccatacaatatagctactcactacttatctccattcttagctttgaaaacttattataccaaattatatgattatcgtcaattacaaatttatggtaacatgctggtacggtataagttccataatccgtgacacgctgcacaaccttgtgtgcacacagtcgacaaccatgcccttctaaatgagatctagcagtttgccagtaataaccatcgtgatctggacaatagatctcgacttgctgttgcattgtcttataatttacacgctcatatccgaagaaagccccgtgagctgcaacggctttcttgataaatataaggtttagtgcttcttgctggaagtcgggatgtagctgcttaatcttagttctattaatagatccatccgatttaatgaacctatttattggaaagttgttagcttcctcgattaataattcatttactttctctctcatattaaatagtctcacagttaaggtagaaacattcgtaagcatctccagtaaactctttatcttgtagtaaacacttagcttggtcttccggtactccagcatctaataattgttgtttacttggcttttcagcgaatacttttacaaaatactcaccatcctgattatactcatttatatctctggtaaggacatatacttgcatttgaagttccttgaaaacataaaaggccagaacaattaagtcctggcctctagaattaatgaagttgtttaccacttcgtaacatagtggctgtttccataagacctagcgtagcatcacgcttattgatctgtttaccaagttcatcggtacgtttaccaatgtaagcgttaatagccatattcatagctgtagcgagatcttctttggttatctcttcatcgtctaaggctaatttagccaaagaatcaaatgtgctagagagtcctataagatctgaggtttctccagccagaataggattaatattatctactgttacttctagcatggagttaacaatatcttcaccatctattagaccagattcaatattactctcccactccttcatctgctccaataatggatttttcttttctgtcatggtagaggtttcctgtgtcagtcggtaagaaggatgattgagctttaggcggatgttgtttagcaatccagctaagaatcagtacacgactaggaacaatatcagtgttgtaccagaaatcatgaacccattgacgagcattctcaaacttaccaaatttatatgctttcttaaacaattcaaacccaaaacaatctggtgtaaagtctacttcacgatattgaactactttagaaccagttaggtcttggatcgctgcattaatttctgtatgcgagaattttgtttcgtgaaacttattaaagaatcggtagttgaagcgtccgttcgtttcgacaaacaactggatgaaaagatcgttaaattggttatcaaaccagtaattctgtagttgttgtagtgctgtcatttacgaactccgttaattgccacgatgatgccttcatacataaaaggaagtagttcagaagtgtagaagatattttccgttattcctagatgtcgaaaaagtatattaaataatgctgttagaaatacaatctggggcagtaatacaaaatactcagttacaatctttggtgcccgataaacaagacgttttatcattgtttttaagtctccttattactttggcctgctccacaataatgaaaactgcgagcactaatagtgctattagccccgcagtaattggtactaaatcaatcatgggagacgccatacgtaattagctgtctgtagaaccttaggtgtgtcatcatgatacattactacagactttggtgaatagctatcagctagctctttacgaatcatcttacattcttcaccagtatcgatatttttaactatcactttcatattaagaggtgttaatacagaaagcggtttccagaagtcctcaatctcaattcctacctttttctcgattaccatgaggacttctagtgtatcatctggaatactaatattattattcacaaactgtaatatctcatgtaaggtatttaattcattaaaattaagcttcatctttaagaatatcctcaaccatatcacaggactgttgcaattcgtcagcaatgcgcttaatatcggtcttcgtcactctaccgattaacatcaccagtaacatagaaagtataataagtgggactggaataacaaataaagctaccttaacaacattctttggcgtccatgtgtggtacttggtaaccagtacaccaaccacaattagataaaacgctagaataaacatcatcattttttaatctccgtaattatctgtgcacgcattactttattaggtaattttgtattcccagctattgcttcaatattatttagtttttcttttagaatatctgagcgtctctgtgctagttcaatatcttgttcttgttctattaagcggcagtgaagtccactattagtagtaagcatactctctatattttttcgcatgcttacaataccaataatcccgccaatcgctactagtgtagtaagaactagtaacccaataagaatttcaatcaacattaattatatactcccttagtccttatttcttacctttcagttgcttaacttcacgctcaaaagatgctgcacgacgttcggcagtcgcttgatgctctttagcaaaacgagcttcctgttttgcaaggttgaacgccatagcattcttattcagagaatcatacatctttttcatcgccggaatagacatcttcatgagctgaccctcaaaaccctgcatgtcgaggagaattgccagaacgttagccatttcgtttttagtcatgttttccattagaatttcctctctcattaacttatgaacttattatacagaattttaaggcttaaagcaactgaattttttaattacttaccaatcgttaacaacgccggagaactcagaagcaaaaactttttcaaatttctctgcaatttcaggatgatctttgcagatcagctcaatacatgcttctggagtcattccttcatcttcaggatcaccatagtatttatcccaaagatcatcgggaatgatatgctccgccaaatcttggaaagagactaactgataacgttctgcctcctcagcgataagaatttcgcatagatctttatctatatcgctacgataatccgcaattaataaggcattgcaagcatgacactcccaaaccatcaagcgttcagaaataggattagacttatcctgtacgtaagactgaaacagggttcggaaagttgccttaacttgttcaaacttatctgctgctgcgaaaactagagctttatcaactttgttcattttgattccttctcatcaatttatacagtaattatacagaaacttaagcattttagcaaataaaacttttaattaaaatgcctaatcctgtgccaatagcaatacaaatgattataagtattgctatcgcctgtatgattcgtttaataataacctcagctatatacttagacatttatatcgccacgcaatacagcagctacgtcttctcctatttgtaatacctcgccggtagtacaattaaccactctatcgtaactagtaaacttaccagacacaatatcctctagtggaattggagttctactcatttcaaatgagacattaatataacgtgggtcacgtaaagaagtagtatgtacatgtccgtgaatatttagtttgccacgaagttcattgggatgcaaagggcagtgagatagccaaaactttttgccacctccagtctgtttgcctagagcttgaatatcgtcataaacttccgctaagtccctaatactcagtccttgacgctccgcatcatgattacccataatgagttgattagggacattgtggataaccgactttaatttggccagaccttcacgacctactgcaatatctcctagcaaaataagttttgttcgtttaccaatatgcttggacaaagtatctagaatatactcgtcgtgctctttcatgttcttaaaccacggacggaaacgtaacgctccagggtggtctagatgcaagtctgaccagaatttaactttcattactcttttccttattctgtattaaactatcaacccaagaggttaacactttggttttaaactcctcgggagtctctccttccttaaggtctacctcattaaggtaggtagtaagccttgtttctatatctatttcagtaggagaattaaaacaaaaattgactgctattccagaatatattactccggtatctcctttgacgaaagcattaactaatgccctccaacgaagggcatcaatacgcattgctcgtaattcttctcgtacttctttcattctatcattcattaaagagtcctctgtacaccgcagctattatttttgtctgtggtaaatgtggtgattttgccagtttcatcattaacttgcgcaaccgtcaactgcccgttgaagacaccgccagtatctaggtaaacacggtttttatagagaagcgggtaaggtactccagtatgcccatggaacacaaagtctactccactaactggaggtacttctaccatgtatttttctttaaatcctgcataacgctggaaatacgagtgttcctcgccatttttagacaaatggaagcctatttcttggattacatctcgatcccataagtatggttcaacatggtatccaggatggtcatgcgggtcttccttagctgcttctacttgtgcaataaggttatcccatactggggtttctacttcgttaccacattctttgtacgtaaaaggtacaccaccatgaacaacaccatacttcttaccacgatgtctaacagttaggaatactggcattttttcagccatgtcttcggcaatatttttaatggtatctgcatctagctcattcatagcccacataccaccgttatacatccaattagcccaatctcccacaatcataaactggtcgtggtttccacgaacgctacaaaaacgtggattatataagaatttagctaaaacttgtaggttctgcgtgcctcgatcaattaaatcccccacgcatataacgcaatctttcttgccgttatagccagctaattgtagggcatcttctagcaaatcattgcatccatgaatatcgccaacaaagaataagttaacatcatcaggtactactagtgttttatgcacattaaattcttttttcataattattcccaaataacatttaaaatagttgtgccatattcattagatagttggagagtataaccctctttattgagggcttttatagcttcataactaatttcgtcacggttaaactgcacataagaacctccaatctctacagaagatactatcctccgcttaacccatctatatgttttctttcggctcttaagggacgcggctctatttatcctagctaaacgttttgcttgctctgctaacatttaatcctcctatcaatctatacaaatattataccaaaatttttagcaaaaagcaagtaaaataaaagcctgatccgctaagatcaggcttggtttattaatcctctggattatcatccaggaaatttttaatagcttcgtgcatagtttctttacgaagctgacgtccaatcaaaatatgattagcttctattcgaccattaggtaagcgatctgccagaactactacaggtacttgacgtacaccaaatttctgcattaattctgtattatcagtctctttatggatttccaaattatagtcattgactactttatcaaatactggttcgaaaagtttacatgggttacaggtggaaccttttaatagatagactaatttagacatttttatttcctttgctggcaaactcaccgtggagttcttctagtttttcatctctccatgcaattgcttcttccaaagaactgcacgttttcatataattgattcctgctctagagatttttactctaaaagacttccctctttgagatatattttttaatcccaataggttatttttattagccgatttcctattaaaagcattttgagcttttgtagcttctcttaagttaccaatacgattgtttagcgtattggtatcatcatgatctactatatcaggtaaatagcctttgtgcataaagaagattgctctatgcgcaagtattcgttctccatcaatagagagcattagatagccatcagcattaatagacccagcaggcatattgttaaggctagtattccaacctcttgtaccttccggtctaggtttccaggttagagtaccatcttcgtggtactctaatacctctaataatctctccctagtaatcacaatttattaatggcctctaagaagtttttcatagtttttacggttgcggtgctcagatcaagatttacacccaaacactcggttaatgcttcctgataaggagcctttaatctgccttctgggacttctaccttcttatactctttatttttgacctttttaatcatagtctctagtacaagaagcggtaatttagcaccttcaatatcagtacccaaaagttcagttaaaattttattaagatcaagacgagttaactttttgcccttagacatagatgcacctacctttgtatcaatagatttttccgctttcttttcgagctttttgtactcaggagagtcatgatcacggagtgcaatgtttagctcgtaatgtggtatacgaaaatgttccgccatttgagtgtagaaacgatcagacataatatatacctctcttaactaatttatgtatatattatataataactagggctaaaagtcaactacttttttatcttaatctactgcatgtataaatcttttcctaactagatacatagttattgggtaaattgagtacataagtatcggggagaaaagggtgaaatacgctgtaactcccccagctaacatcaaaggtattaatgctagagtaagggccataagaatcataccgaatgaaacagccagagctatggatataggattctctagttccatccataaccaacaatatttcgtatctctatggcaattgcatttacaaacgccgaatgaacccataattatatactctagtccgtgaataacctttattaataagctatttcgggtagttaatgcaatgatagtaaagactatcattaaaacgaatactactagacttattttccagatacctagcagcatcatagtgaatagttctgcaaacatggctttctcctatcttcaaaaattattaaagccccctttgcctaaaaaggcgggaatattcccgcctaagttattaattaaactagttcgacatgaccgccatcataggtaccacgttttatttcatcgtgatagtctcccgaagcattccaatcagcaccaaaacgaagtttaatgcctagctctttaccagcttgttcaaaagcctttttaactgcccaaaatgcttctaagtcattccaatcaattttgccattaatatatggagcaaaatcaatagcatccccagtaatatgtttgcttttactaggatcttttagaaatgaagtaccattagcaatgttctgggcactttgtgctactgtacgaataccttgcacgattgtgaaatcatacggagatagttctaaagccctacgagctactttttgtagctcgggcttaacggtagctaattgtttttcactatttttaccaaatttaaaactcatattgatctacctaaagatctctgttgtggggaacagagctttgctaaatattccttgaactgttcagaatcagctgtatctaccggattatctttccaagcaataccaatgtacccagcatagatattttttagattgaagtatggacaagtgtatatgtaattaaaagtaacgtttttaaacgcaggtatatttaaccccatatatttatttactcttacacttaaatccgatgcgtagttaaagccctctaaatgacgtctgtataattcagacgttttatttaccgctttatcggccaagtcagccctatctaattgcgcattactttcccatgcaataatattggaataatcattgatagcatctggtttatacttgactacaaaaacagcatctgcacccgtttgagagaagagaaccatgctcttttccctcgccacattagggaagttatctatcctctgggtttgtaaatcttgtaaaactgcagacgtggaaaaagtctttaagaatgacatcacttcactagtattactaacaaataagaaaataatgacagcaactaagatagttagcagacgtttaagaagcgatgctggatctttcgcttcttggagcagtaccgttaataattgtaagaacttttccaattgtaacctcctctaaccagtaccattatactaattttggaggaaaattacaatgtgtttttaaagatcacttctggagcataaaattttgtcgttgtcaagaagaattttagataaaagaaaagccagggtcgttaaaccctggcttaaaattacttactcttcgttatgctcctcggattgaggtaactgggctttattatattgctcagatcgatattttgccaagatttcaatacgcttatggatttctttgctatctagatagatatttttgttgtcttttaccatctcgtcgatttcgtctatagagaagaacggatagtagacatctagcatcatatcttctacgaacttgttgtaagattcataggctttcttgatttcttgacccttctcacagaatccgccagagaacgtgtgtcccattagcgtagcatgtggatgtactacccatccatgacaggataggaaaattgtgcagtaagcagaagcactaggaccaatcaggtgtcctataactgttccacggcaattagcaattaagttagataactgtgcagcagtatcaacataaccaccagggccattaatcatcagattaatttcgtcgtcctcatttgcttgcataagtaccattgataaatcacggtattcatccggcgggcctaattcttcatcaaagaaaaaggtatactcattagactggcgaatggagtgaaacaggttagtcttttcttcttttttattagtcatagcgatccttgattatccaactagtggttctagctctaagtcacagaagttataaacttctagtttaaggttattgataccatcgaatttattaactaattcgtgagtaatatattttgcaggaataccactttcagatggatgatctgatttaatagtgaacttctgctcagcgggtactacatttactatcaaagaatccatatctaaatggtttgtttctctgagtaactctccttcattggggaatctaacatctgttattacggcgacatctgggtcgtctttagcgatggattgctccagaattatgagccaaatgcgttcatgtaccagctgccttcctagctctgttcctacgagctgtaacatttttctcggagaaataaataaactataaagtccgtcttctttattctctgagataagttgttgaggattaagatatttttcctcaaaaatcggccaaacgtacgagaagtcttcaaacttattgataccgtatttaaaccatacgtctctagctcgctccaattgagattgtgtgaccgtaaaccattggtcaatctctttccccctgcgctctcctagaaactctggagttacaccgaggattacggatgcaagttcataaacgggcttagcaaaactataacgacggggtaaacacgttggatacgtgtcattacaccaatcgataattaattttgcaacggtatcttttcccgaaccagcttcaccatgtaaaccgactaatactgacattaatctttcctattgttaattggtggataatatactaaacaacgtttttcttgcaaatcttggcggtagaagcaaaccatactagtcagtcgtgagatatatgaatattctgcctcacggcattttgccaacatattccaatctttgtatggtacaacaactactacgccatcttccccatttgtagctaatttcttttcaaacttaaagtcaaagctacaaggctgaagtcctttaggccaatccacatgggcttgctttaactcatgtgacggctctggtactaccgtttctgcacagcctgtgattgtgattgcggctgcgagcagtattccaagtttccagttaaacatgctaatctttcctcgaactccttactctgctttttagcaattaatgtaaccaatccaggctttgcagctataatatcttggcgactaagagctttgtctaactgcttaatctttttgtctagatctgcttgcgaaatattattcattgtgaaatactgattcattctagtctcacgaagttcgctttcagctttcaccttattgagggaagtctctagagaagaaatctttttagtagccaccgcaagatctcctgctaaagtctccactttatctactaagtgataagcaccgaacccgatgcctatcgctagacctgctcccaggatatacatcttgttattccaaactaagtctacaaaccatttccgcattagcctgtactcgcaaactcaccgtggagttctttgagtttggtatcccgccattttatagcctcttccaaactcttaagtgttttcgaaacttgcttaccatgtttggtaattcttacttggtaagtcccatttgtttttctatggatatttttaacgcctaaatggttatcgcttcttactttttggttacaagcattatcagatcttgtagcaggccttagattctcaaatctatcattagttgagtctttgtccttgtgatcaactatttcaggccattctccagtatgccatgcatagattaatctatgtgcccctatagctatggaaccattatatagttcaactactctatgccctgtactttgtctagatcctgctactgttccggcgaatatcttattaaaatgttcgtccccttccctgggtttccagataagattaccatcttcttggtaatcgaacattcttcttagctcttccttactgatcatcttttcatattcctaaaagaagtaacagtatcaaatccatgtgcagctaagcgatccttatcggaaatcgtaatagtatttggttcgccggttcctaacacgccccagatatattgctcgatcatctggtgcaaacggtataagttactttcaatttcctgccacggaatacctgactgatggaaacgaatgttagtctgaatcacgaagttacgaacatcatcgttatcgttcttcttgatacctttcacatatgcaatcggtacacgcagttcggacaagatacgttctgctttaggttttgcttcaacgagcaaatcacgcattgtttcacgaacatctccgcgactcttatccattaagtaagagcgagcatgcaatcccatctcttccattttatcgaacatagtgtcgaggttgaacgttttgaagctaaatgctggatgccagcagtacagctcgtgtaaccagtaaacttcacctgcaacaaatagtgggtttacaaaatattcgaaatcaccacggaaagatagcgaaccatcacgaaatacctgacgactatgcacgatgttcttttctgcatcatcagttactttaaccagtagctcttcagttttacgctcccaaacacgatctgcatcaaataaactgttctgcaaatcatatacatcggcgaatttagaaatgatcctcatatttaatcctcttgcctcaatctataaacatattatacaaaagttgggcatctaagcaactaaaattttattataaaaatagcccagtcgcaaaagtgcaggctgggctttgtcattatttgcttttgctagtaagctgacttagtgtcaatcttatgtaatattagtttctctagctttgcgtagtacccctgcatttctccacaatttgatgtcagcaactgtttctttataaggagctatggtaaaacctagtgggccagcactaaataatcctaagaaccctacaatacgcatgtagaacaagcattctttggctgtcatattatttactgcttttttctgcttttcatctttaaacttctgttcttgatcaccaatacgtagatatttaacaaaccattcagcagaatgttcgtccaaatgtctaataatagctatcgcatatccagcaccgattaaaaaccaagttgcaacaagaattagtaatatagtcatattatctccagttagggctagcagccacctcaccacttaccgcactaaggggcacgactcccttatccgtaacagttgcaggtgacgcaactcggtcctacgcgagttctttaagtattctgcatttcagctttaaattttttcatattacgagtttttctataaaagaaaaacacagatgttgggcctagaagaatatccacaataaatatcacagatctagcacatctgagtaatgttttatcatcaagaggtggcagatctaacggtcgagttttatgtataacgtataatattacatctttattcttagaaatataaagatcatcaaccaagctgtaaatagcaaccacagatccaatgacaaaccaaagagcaaatggagagataatcatttcagatccttttcattaattagaatattagtaaacagtggagtaactcctagactcatagtaggtccaaacgtattcatggctacccatagctgcatagtgatcatcccatctttaatctctggatctttatattcttcgatacgtttcttggtaaaagcaactatatctggattatttttattttcctgaatatagtcatgccaaaactgagtattctcactacgtaggaatgttaaaacatccttagttgctggaatctgcactgtgctgttgatgtttagtcttttcacgttcttctctccgacgtttgcgttcttttatcatatgagctgctacaacttcatggtagtagtcattaatgttatcttctggcaagaaatgcttaatagtctctagctgacaaataactcgatgaagatggttatttggtagacacaattttatacctgcaacaaatccagagaagcctggaacactgaacatgggttgggcttctactctaccttcagagttgatattaagctcaattgagatacccattttcacgctataaagctggcaatattctccgttaccagaccttgaccaaacagtgaagtcctcatcaatttgatcttgaatttctgtaatagcaaatttaattctaggatctaaattattcatcttcaccttcaaagtcgcaatcataacgacaagtaaaagaatcagaactattagtacgttgagtggttatttcaccgcgtttgctaatagtaacggctggagtagagaagtttttattagtatatatttctactttaccattacgttccttaacatcacgcactttaccatactcggtaataatgccgttctgttggactttaacattaccatttttcatagaaactttggtagatgccagagaaccgaaactaactgtggagatcatcagtgcaataataaacttattcatcttcatcctccccactacaatcacgacatacatcataatcgttgaaagaacgttcgtgagcttcacaccaccaagaacaagaatcgcagagaaacatttcggttttctctagtgcttgacctaaaagatcatcagcttcctcagcagtaatcttcaatccgcacacatctgccacacgttctttaattaaacgacctgcttcgtgataagacatacaggttcccacaacatcatgttcaagaacatgaacagcacagtctagacgagttttcatttcaaacctctctcatcaatttataaatatattatagcaagaaaagagaggtttagcaaatgaattatttcagaatttagtcatagcaccaccataatccacgcttacgcatgtcatgatcgcgattataatcataattttctggatctttcatcacgcggtggagttcttgacgattcccttgacgaaccattttattagaatgccacttaacattcttactaatagaattccagttataaccatcctttttctcattacgaatggttgcttccttcatttcctgttctacatcatcccaggatttagcataaataacacgaatccagtagccattttctttgatgaaagaatattcttgagagaattgttctttagacttccaccactgatcaccagattgtttacgataagtacggctcatattacctccattaagtcttttaaattaacctaatgtggatgaattttgttatacatatattatgtacctttatacagaaaaaccccagactacttattcaatagctggggtttgttattaattacagatcggggcgttcatcttcgaaacagcctgagctaattccttctccgaatcctacaaagccatcaaattcatcatttgagatgcccataatcattgcttccattttcctaatctccgaaattttcatgcctgctttactattcttataatatttgcgagggttcccgcacatccaacaagaacagatgcaaggagtagtagtgataatacctaaccgcttagggctttcttcatgtgggaagactgtccaatacttcttgcggttgttcttcacacgttgccggtgatggcgtcttaatgctcgatccacacatttctcctaaaacttgggagataaacggagtttgctcgactaccttgcgtagctgggagaaatcatatccaaaccccattacatcgcctgagtaaatgtacgactaataacgtcgttctgttgttcacgagtcagtgcattaaatcgaacagcgtagccagagacacggatggtcaactgaggatatttttcaggatgtttctgcgcatccaaaagctgatcacggcttaacacattgacatttaggtgctgaccaccttcgatttgaggggcgacttccaccttaacttcacggaaggcttcgggatcgaattgtggtgtgataccttctagatcttcaactagaactttctgtttaagttcaccattgtcggagtatagctgaataatctgattttcatgaacaaggttaattacgccagacttaagattttgatatgctttcattagatctccctgatgttagaatttggctcagctctttattgtctatagtttaccacgatatacagaaactgtcttaccagtttggttcataacgtatgctacttcatcttcttttaagaagattgcttgatctattccagaaatagctatgcttttatttctgggattaaaccctacgcttttaccaacatgaatctgctcaccaccatcagtggacattattttaactgttaacataattgctcctatatttagctatctctagctcttttaatggtagttagtagtggatttgaaccactgtagtcgctccgtatgaaggaggtgcataaccactctgccaactaactgttatgttttactagactaagtaagtattctttatactctttagaccaattagcttttttaaactttcctggacgcatagtcttaattcctagatttggtactccgggagggatttaaacccccgatctctcggttatcagccgagtgctttagatcgctaagctaccgaagtattagaatatttacatcatacactgtctaagtaagaagtataatggaatttagcttctccagtcttatctacttctacctcagttcgtggtacttgacgaaccacaccatgaatcatcttatagcgaatgcctttagctggttcatgatcttttgggaatacttgtttaaccgttactactttatatccttcacgcggtgttaacactactacttgatcaccttctttgattttccaagaagatggaaattcataggtatatctttgaccaccagtttggaatactacagaaagataacgtttcatttggtttccctctcattaatttatatagatattataacaagaaataagagagaaggcaaatgaatttttaaatttggtgctcccaccaggaatcgaacccggttcagatgcttacaaggcaactgcatcgccagcaatgctttaggagcgatgatcccgttatttcaacgggatttctttttcaataacaggagacttatcagtcataactgtcattgccatttgttgtagaaattcaaaggtgaaggctacacgttcttcaccaatctctacttctacacgtttcttttgtttatcaatctttacttttaggttgtcagccatcttcgggttctcgttgctgtactacttctagccagtctggtagaagaaactttgtacgaaattcttcgtaagtttctttgggataaaagctaaaacctcctttctcatcattcaggataacagaaccgtcagtttgttcatatgctcgatatgtttctccaataatgataactcgcttatcagtacttttattatgaaactcaaaaacgtgcataatgtttccttaaagttggagcggctagagggaatcgaaccctactcagcgaggcttggaaggcctgcgacacaacccgtgtgcttaaccgcttattatttggctggagaaggaggaatcgaacctaccattaacggagtcaaaggccgttgtgctaaccgttacactactctccaagtatttggctgggatgccacggattgaacgtggaaccttcggagtcagaggccgacgatctgccaattgatctacatcccaataattctttactttatgtaaatagggtaactgtgctaacggtcaggtaattaatcaaatcgctgtaagtcttggtgctatcactcagactctggctggtctgcaggctaaactgccggcttaatattaaggggaggagcccattatgagtaaatatggttttgtaaataacggacttaatcaaagtatgggctcccagcagcccattccgggtctggataacccctacttacaacaattgcaacagcgtttagcagaagcgcaacagatgcaacaacaactccagcaaaaccctggaagtgtgagtcctatgcaaatgatgcagcaaatgagcgggcagtcgcaaatgcctcaacaaatgcagcaacagatgccgcagcagcaagttcagcagcaaacccaacaaccgcaggtttctgcggaaggacaggcagtactagcccttttcgaagacttcacaaagacagaggatgggaagcagcttgtatcacttatgggtaagtttaatagcttctgccaaagccaagttgcaaaagctcaaaatggtggtaataactcctaaggagaaattatgtgttgcagaaaacctgtttcgtgctgcccaatgcctgtagcacgttgttgctctccagcaatgtttacacaaataccggcgttcaatccctttgcctttaagcctactcttatcctgccccctagagtagattttcagtcaagattggcctcccgtatgggtggttgctgtacaccgagagtgtggttctgaagaaccaaacaataaagcccctagtcgaaagacttaggggcttttctgtatttaagataaaagaaaagccctgcgctctccagggaacgcagggcttacttcagatgttacatgcggatattatttattacgcatatccatgatcatttgaccatcgtagccagtacctaccacagtctgtggtacaccaccttgatatttctgagcacgaatcatttcgacttccagttgtttccaacgaatcatctcaggagtaatggtacgttgcagtgcggcgttagcttcagcttctttcttagctgcgtacagtttagcatctgcgtcacgttcattagcgatagcttggttgttgcgagcttcacgatctgcttctgcttgtttaactttttgctgtgcttcctgttcaacacgagctaattcagctttagcagcattaacctgttcttcacgaactttggtattctgtacctgttccatgattaccggtggcaaagtaatatcctgaaggaatacctgcttaactgtgtaaccatatgggcgtgcatactcttcaacttcctgttgaattgcagtttgcaattgagcctgaattttagcatcaaacaaatcttgtgctttaggtacagacttaccaaactcacgaatagtagacagtaatttttcagttacatatttgtctaacgcttgatcctgagtacctgcgttaatacggttaattggtgccttagaaccatcaaactgcaacataacagtcaggtcaacagtggatttaaacttatcctggctaggaacctgaagtttatctaattttacagcaatatcttttgtactaaaagtgtcgaaagatgcaaatgggtttacaagatggaaacctggtaatactgggttaggatctactttacccagaaatgtttgggttttaaccgtaccatcagaaacaatagtatatgaattaaaggctagaatcaagcctgctaaaccaactacagcaccaataccccaacgtttaatagtacgaattactttctgctcagaagtcagttctttcatatttttagtattaaacatatatttcctttgttttagttacagttaataaaattggccgaggtgacaggattcgaacctgcataaaggaatttagaagactcctgcctctcccttagactacaccccgtttaaatatttttaagaactctcgtaaaaactcttaaaaatacagacgataccgggagagtcataagtctcactcattaagtatttcaagacaaaatacagtaacgtctattattttccagtttaagtcagggtgacttagtggttaggtcctgcggtatattgaggactcggttaggcttggggtcatgacttcccgccttttgctgctactcaacaggagttatcgcgaattacctgtgctattgtgcaccattagtgacatctctcatgtcagcatttcccactttgtggatagcttgaaaaactactccgatatggagaaaaaacttcactatcctagaataccttctaaagttcttctttagcctggacatagttaaatcgtaataaaactattcagcagactggttggttagcctggaaccaactaccgcgtggtttaggcagtgcgcaactaacctcggaagcttttacgttaaaagcatcagttatccagttcttaccgaccgtaggattcgaacctatatcttccaccagttacggcttgataataccaattatactaggacggcagtgttactacataagtgatttccacaccccactatttataaattagagaagagtttaggggagaggtttcagacgcctcattttacacgttctagccactaaccgggattgccgccccctgtgtactagttttacaactaacctaccgactctattcaacgaatcttagtgctcgacgcatcttacattaagacaagttcagcgtaatcggctcgctgttctctaatttatgaatatattatacagaatttataagcatttagcaaataaatttttaattaaattcaccagcaatctgagcagcagtaccaccatcataacgcccaggaaattcttccttaatcgctttcatcagcataccttttgtaattcca

SEQ ID NO: 88 - DNA, 32767 bp, T2_6e1 phage; identical to SEQ ID NO: 84
  source 1..32767: mol_type = genomic DNA

SEQ ID NO: 89 - DNA, 32767 bp, T2_6e2 phage; identical to SEQ ID NO: 84
  source 1..32767: mol_type = genomic DNA

SEQ ID NO: 90 - DNA, 876 bp, T5j phage
  source 1..876: mol_type = genomic DNA
atgagtaaatcctggggaaaatttattgaagaagaggaagctgaaatggcttcccgtcgtaatctaatgattgtcgatggaactaacttaggctttcgcttcaaacataacaatagtaaaaaaccatttgcctcaagttatgtttcaactattcaatctctggcaaaatcctactctgccagaactacgattgttctaggtgataagggaaaatctgtatttcgtctagaacatctaccagagtataaaggtaatcgtgatgaaaagtacgcacaacgtacggaagaggagaaagcgctagatgagcagttctttgagtatttgaaggatgctttcgagttgtgtaaaactacattcccaacttttaccattcgtggtgtagaagcagacgatatggcagcttatattgttaagctcatcgggcatctttatgatcacgtttggctaatatctacagatggtgactgggatactttattaacggataaagtttctcgtttttctttcacaacacgtcgtgagtatcatcttcgtgatatgtatgaacatcataatgttgatgatgttgagcagtttatctccctgaaagcaattatgggagatctaggagataatattcgtggtgttgaaggaataggagcaaaacgcggatataatattattcgtgagtttggtaacgtactggatattattgatcagcttccactgcctggaaagcagaaatatatacagaacctgaatgcatcggaagaactgcttttccgaaacttgattctggttgatttacctacctactgtgtggatgctattgctgctgtaggtcaagatgtgttagataagtttacaaaagatattttggagattgcagaacaatga

SEQ ID NO: 91 - protein, 291 aa, T5j phage
MSKSWGKFIEEEEAEMASRRNLMIVDGTNLGFRFKHNNSKKPFASSYVSTIQSLAKSYSARTTIVLGDKGKSVFRLEHLPEYKGNRDEKYAQRTEEEKALDEQFFEYLKDAFELCKTTFPTFTIRGVEADDMAAYIVKLIGHLYDHVWLISTDGDWDTLLTDKVSRFSFTTRREYHLRDMYEHHNVDDVEQFISLKAIMGDLGDNIRGVEGIGAKRGYNIIREFGNVLDIIDQLPLPGKQKYIQNLNASEELLFRNLILVDLPTYCVDAIAAVGQDVLDKFTKDILEIAEQ

SEQ ID NO: 92 - DNA, 558 bp, T2
  source 1..558: mol_type = genomic DNA
atgcagaaaacgaatccgggtttacagagactatttcagattccgacatttaccctatcgaacagtgacttgactagtgaaatgaaggtcaaaattgctgatacagcaagatactctttaaaacaaaacccgaaccaggataaagcagaagttattgaaagatgtcgtatcgctgtgtacgcagaattttttgtagcagattggctaagcgggtatgttaacaaaggccaagaggatgttaatgacccatatacatatgcatgggatgtattggcgcatccaaaatactgtgggcttcgtgtagaagtcaaaacacatcaaactgactcacgatggatttcggtaacaaccggatgcagcggagagtatccatatggttctggaataaatctagggcccattctaaatcatcaagtcgctgactgtataattatattcaacactaaagaaattcatccaggtgtcatccagtacactccgaaattcatcggtgatagagaagaccttcgtaaggttgtaagaaaaagcaactacaacggatggtatctttccatttaa

SEQ ID NO: 93 - protein, 185 aa, T2
MQKTNPGLQRLFQIPTFTLSNSDLTSEMKVKIADTARYSLKQNPNQDKAEVIERCRIAVYAEFFVADWLSGYVNKGQEDVNDPYTYAWDVLAHPKYCGLRVEVKTHQTDSRWISVTTGCSGEYPYGSGINLGPILNHQVADCIIIFNTKEIHPGVIQYTPKFIGDREDLRKVVRKSNYNGWYLSI

SEQ ID NO: 94 - DNA, 60 bp, Artificial
  source 1..60: mol_type = other DNA
attctttactttatgtaaatagggtaactgttaaatttggtgttggatgatggagtcgaa

SEQ ID NO: 95 - DNA, 60 bp, Artificial
  source 1..60: mol_type = other DNA
gcgatttgattaattacctgaccgttagcactaatatagcactgagcaagttctttaaaa

SEQ ID NO: 96 - DNA, 75 bp, Artificial
  source 1..75: mol_type = other DNA
attctttactttatgtaaatagggtaactggaatttataagatatattatattagaaatttagcttcatagcaag

SEQ ID NO: 97 - DNA, 63 bp, Artificial
  source 1..63: mol_type = other DNA
gcgatttgattaattacctgaccgttagcattttgacacctcctagtatatagaaaatgtgtg

SEQ ID NO: 98 - DNA, 25 bp, Artificial
  source 1..25: mol_type = other DNA
cgtgcataatgtttccttaaagttg

SEQ ID NO: 99 - DNA, 25 bp, Artificial
  source 1..25: mol_type = other DNA
agcccatactttgattaagtccgtt

SEQ ID NO: 100 - RNA, 76 nt, Escherichia coli DH10B
  source 1..76: mol_type = tRNA
gggtcgttagctcagttggtagagcagttgacttttaatcaattggtcgcaggttcgaatcctgcacgacccacca

SEQ ID NO: 101 - RNA, 73 nt, Escherichia coli DH10B
  source 1..73: mol_type = tRNA
gctcctctgactggactcgaaccagtgacatacggattaacagtccgccgttctaccgactgaactacagagg

SEQ ID NO: 102 - RNA, 76 nt, phage SP15
  source 1..76: mol_type = tRNA
aggtcgctagctcaataggtttagtagcatccgacttttaatcggaaggttctgggttcgagtcccaggcgatcta

SEQ ID NO: 103 - RNA, 80 nt, phage SP16
  source 1..80: mol_type = tRNA
gggtcgttagccaagcggtttggcggtggactgttaatccatgtcgaaagacaacgtaggttcgaatcctacacggcccg

SEQ ID NO: 104 - DNA, 40 bp, Artificial
  source 1..40: mol_type = other DNA
taattgcgttgcgcaaaaatcagtttaaacagggccaacc

SEQ ID NO: 105 - DNA, 36 bp, Artificial
  source 1..36: mol_type = other DNA
ccaagctgcgatttcctgaatttcgcaaagcaggat

SEQ ID NO: 106 - DNA, 36 bp, Artificial
  source 1..36: mol_type = other DNA
atcctgctttgcgaaattcaggaaatcgcagcttgg

SEQ ID NO: 107 - DNA, 40 bp, Artificial
  source 1..40: mol_type = other DNA
gctagttattgcgtatgcaaaaattaatcaggggaactgt

SEQ ID NO: 108 - DNA, 40 bp, Artificial
  source 1..40: mol_type = other DNA
attaatttttgcatacgcaataactagcataaccccttgg

SEQ ID NO: 109 - DNA, 40 bp, Artificial
  source 1..40: mol_type = other DNA
gtttaaactgatttttgcgcaacgcaattaatgtaagtta

SEQ ID NO: 110 - DNA, 40 bp, Artificial
  source 1..40: mol_type = other DNA
aggagaaaggatccatggcaaataagctggcgacatttca

SEQ ID NO: 111 - DNA, 40 bp, Artificial
  source 1..40: mol_type = other DNA
gaggatcgaattctcaggaaaaaattccctgattaaaact

SEQ ID NO: 112 - DNA, 40 bp, Artificial
  source 1..40: mol_type = other DNA
gaattttttcctgagaattcgatcctctagagtcgacctg

SEQ ID NO: 113 - DNA, 40 bp, Artificial
  source 1..40: mol_type = other DNA
atttgccatggatcctttctcctggtaccgagctcgaatt

SEQ ID NO: 114 - DNA, 7647 bp, JBEAAAI-19-0008
  source 1..7647: mol_type = genomic DNA
aaaatcagtttaaacagggccaaccccgagcatagatatgatacgttgccatctcgcccgcctaatgggggagcggaaaatgaagatctccgacgttttacgagaaacagggcttagccgcaatacagtgaccctgatgtacagggaaacagctcaaaagatagacgtcgaggcgttggataagctctgccagctttttgcttgtgaagtggcggatattcttgaattcacggatgaatagcgtgacaactatagagacatcctgtgcccgcgacgtgtcaaaatcattaggcgtaacccatgactaaagaacaacaaattgagcaaggtttaatcgccaggctacaagacctcaaatacacctaccgcagcgacattcacgacaaggctagcttggagcagaacttccgtaagaagtttgaagctttgaaccgagtcaacctatccgatgcagaattcaaccgcctccgtgaagagatcatcacagcggatgtctttttggctgcccaggcgctgcgtgaaaaggggaaatttacccgtgaagatggcactccgttggaatacatgctggttaatcttaaagactggtgtaaaaacgactttgaagtaattagccagcttcgtatcaacacagataacagtcaccatcgctatgacgtgattctattgctcaatggcttaccactggtacagattgagctgaagtcactacagctcagtcctcgcagagcgatggagcaaatcgttgagtataaaaacgatactggcaacggctataccaatactctgctgtgcttcatgcagttgtttatcgtcagtaatggtaacgatacgcgttatttcgccaataaccgcaaagagcacttcagcttcaatgccgatgagcgcttcctgcccatttatcagcatgctgacaagagcaataagaagattgctcatttgcacgactttgctgatgacttcctagccaagtgcaccttgggtcagctgatcagccgctatatggtgttggtacaaagcgagcaaaaaatgctcatcatgcgcccgtatcaaatctatgccgttaaagctattgtggatgctattcaccagaaccgtggtaatggctatatctggcataccacaggctctggtaaaacactcacgtcattcaaagcctctacgctattgaaagataatcccgatattgaaaaatgtttatttgtggtcgatcgcaaagatctcgatcgccaaacgcgagaggaattcaacaaattccaggaaggatgtgtagagcaaaacaccaacaccgaaacgctcgtacgccgcatgttatcggaagactatgccgataaagtgattgtcactaccattcaaaagcttggtctggccttggatgagaatagcaaacgcaacaaggctcagcagaaaaatggcaaacagacctataaagagcgtttggagccgctgcgtgataagcgcgtggtatttatcttcgacgaatgtcaccgctctcaatttggtgagaaccataaagccattaaagaatttttccccaaagctcagttatttggttttaccggcacacctatttttgacgaaaattcaagctatcagcaagtagatggcaacctagcctctttcaaaaccacggaagatattttcgaaaaagagctacacgcctatactatcacccacgccattgaggacaaaaacgtactgagtttccacattgactattatgggaaagacgatggtaaaggtggtcaaaccaagcctaagaaaaaagaactgccaccacctgaagcggtaataaaagctattctcgacaaacacgatagcgccacaaatcagcgccgctttaatgccgtattggcaacagcatcgatcaatcacgccatcgagtactttgagctatttaaaacgcttcaagcacaaaagcagtctgaagacgaaaatttcgagccattgaatatcgcctgtgtattctcccccccggcccagatcgctaaagagaacgatggtaatggcagtgtaaacggcaacaagaatgcggcagacattaagcagcttcaggaagatctgccccaagaaagtgtcgacaaccaggtagaacccgaaaagaaaaagtcagccctgatggcgattgttgccaactacaacgagcaatacggcaccaatcacaccattaacgaattcgatctttactatcaggatgtgcagcagcgcatcaaagaccaaaagtacagcaatgttgattaccctcgtaaaaacaaaatcgacatcaccattgtggtggacatgctattaaccggttttgactcaaaatacctcaatactctgtatgtggataaaaacctgaagcatcacggccttatccaggcattctcgcgtaccaatcgtgtgctcaacgacacaaaaccgtggggcaacattctggacttccgttatcaggaaaacgaagtcaacgcagcaattgagttgttttctggtgggccgaaagataaagcccgagaaatctggctggtcgatccagcgcacaaagtggttgaggcattccagaaaagggtggacgaattgcaaacctttatggagtccaaaggcttaagctgtgagccatctgaggtgcataacctgaaaggcgatacggccaaggccgagtttatcaaccactttaaagaagtgcagaagctgaaaacccagctagatcaatacacggatctggacgaagaaagtaaagccgccatcgaacaaaaactgccaacagatactttgcggggcttcaaagccatttacctcgatacagctatggagttaaagcgtaaacaaggtaaaagtgatgacaacgaagaatcggtggagcagcttgagtttgatctagtgctttttgcctccagtattatcgactatgactacatcatggggctgattgccaaatccacgcaaaaaactggcaagcagaagatgacgcgccaggagctgatcgacctgatcagcgccaatgctaacttgatggaagagcgtgaagatattattgcctacatcaatagcctcaaggcgggtgaagcacttaatgaaaagcaaatccgcgaaggctatcaaacttataaagcgcagaaagccgcgcaggtattaacgcaaattgctgagaaacatggcttgcaaactcaatctcttcaggcgtttgtggacagcattttagatcgcatgatttttgatggcgaacaattaacagacttacttgctcccttagaactcggttggaaagcgcgtcgcgtggcagagctggccttgatggaagatttagtaccttacctacaaaaacaggccgatgggcgcgaaatttcgggattagatgcatatgagtgatcaaaaaagagagtttattccagagttacgtttttctgaatttctagcttccaaagggtggaagattcgaagtgttagtgaaacatgtgataagccttttagcggggggacaccatcatctacgaaaaaagaatattatggtggagatattccctttattcgctcaggtgaaatagataaggaaaagacagagctcttccttactcaagatggcctttcgaactcttctgcaaagctggtaaaaaagggagatatattagtagctttatatggcgctaatagcggcgaagtggcattgagtaaaattgaaggcgcgattaatcaggcaattttatgtctgcgttcaaaaacgaataatgcctttcttttccagtacctcgtatacagaaaaaactatataaccaagaaatacttgcagggagggcaagggaacctttcgggagacatcattaagtcaattgagcttcttttcccagagagagatgagcaacaaaaaatcgctgactgtctggcttccatcgatgggctaattacacagcacacccagaagctcgaagccctcaaattccataaaaaaggattgatgcaacaactctttccagcccaaggtgaaaccgtacccaagctgcgatttcctgaatttcgcaaagcaggatgttggaagcttaagcccattgggaaggtcttggctgaaaaacaaaggccgatagatatggaggacgatgaggagtattccttggtgacagtcaagcgccgatatggaggattggtttcaagagggatatacaagggaaggacaatcaaagttaaatcgcaatttgaagttcatgaaaatgatttcctgatttctaagcgtcagattgttcattgtgcttgtggtgtcgttccaaaagaactgcatggttcgattgtttctaatgagtattctgttctagtgccgaagaaagacaatgatgttcacttttttgactactttgcgcagcaacctgaagtaagcctatcttttttgcagtgtagcattgggattgttattgaaaagatgatattcaaactaaaggattggctgaaagaagagtttctatttccagagattgaggagcaacagaaaattgcgcaatttctcggcgattttgacgagattatagataaacagtatcaaaaaattgaatcgctaaaagagcataaaaaaggcctaatgcaaaaactctttcctgttatggatgaggtggtttgatggcaaataagctggcgacatttcaggaactgggcgagattgcagctcatctacgtgaaaaacttgaagataaaaaatatgtactcctgttcgcatataatggcacaggaaagactcggttatcaatggagtttaaggagctaggtaagaatggtgatgacagggatacgctttacttcaacgcatttaccgaagacctgtttaattgggataacgatctggaacacgattctaaacgggtattgcgattaaatcgtgagtctcgcttttttgacggtttagaggagttggagatggaaaacagaatagctccaatactcgcccgttacgccgactttaatttctatattgattacaccgattgggaaatcatatttttccgtgagacagacagtgaaggcgacccaattcctattaaggtatctcgtggtgaggaaaatatatttatctggtgtttttttcttgtggttgcgcggttggcattagatagcgaggaaggcgctgtctattcgtgggttaaattcatatatatagatgatcctatatcttcgttagatgataacaacgctgtagctgtagcacatcacttggctcaattatttaaaacatcgagaaacgacataaaagtgactttatcttcgcatcacacgttattttttaatgtaatgtgtaatgaatggggaaatgcagttaagtatttcctgggtaaaaacgaaggtggtaatggatacaccttgaaaccgatgtatggagatacggctaggttctatcacgtggcaatgttgagggatctaaaaaaagctgctgactcaggagagctatatacttaccacttcaatattctacgtaaccttatggaaaaaactgctacttttcatggctatactgactttagtcactttataagcgtggaaaatgatgatgacgagaaaacattattaacaaggttggttcaggtgttgaatcatggtggttattcgttacttgaacccattgaaatgattcccgaaaacaagtcacatttccgaaaaatcctgaatgattttctgaaaacatatagttttaatcagggaattttttcctgatctctttaaagtgaagaataaacgatgaccaaagaacaactcaatcagcttggtaaaacactctgggatatcgcggatcaattacgcggcgccatgaatgccgatgacttccgcgattacatgctgtcttttctattcctgcgttatctgtctgataactatgagcaggccgccaaaaaggaattgggccgtgattaccccgaaccgggcaatgatgatcgtcgcgcaccattagcaatctggtatcagaacaaccaagctgatattgccgattttgaaaaacaaatgcgtcttaaaacccattatgttattgagcctgcgtttctgtggagcagtgtggccgaaatggcgcgtacccagcatgcggatttgctggatacactatggaaggggttcaaatatattgaagagaagtccttcaacagcacgtttcagggcttgttctcggaaatcaacctgcactctgaaaagctaggcaaaaagcctgccgatcgtaatgccaagctttgtgccattatccaaaagattgccgaaggtatttctggttttagcaatgccagggacgatctgggtgatgcctatgaatacttgattggccagtttgcagcaggttctggaaaaaaagctggtgagttttatacacctcaacaagtttctaccatcttgtcagaaattgtcacattagatagccaagacccgacgacaggcccaaagaaaaaaattaaacaagtgatggatttcgcctgtggttcaggctcgttgctattgaatgtacgaaacaggttaggtgatgaaggcggttctataggtaaaatatttggccaagagaaaaatatcactacctataaccttgcgcgcatgaacatgcttttgcatggggtaaaagatactgagtttgaaattcatcacggcgatacgttagagaatgactgggatattcttaatgagatgaatcctgcgaagaaaatgcagttcgacgccatcgtcgctaacccacctttcagtttgcgttgggagccgaccgaggcattaggtgaagatttccgcttcaagaactatggtcttgcgcctaaatcagcggcagatttcgcctttcttctgcacggctttcacttcctcagcgatgacggggttatggcgattattctgccgcacggtgttttatttcgtggcggtgcagaagagcggatacgtaccaagttgttaaaagatgggcatatcgataccgtcattggccttcctgccaatctgttcttctcaacgggcatacctgtttgcattctggtgctcaaacgctgtaagaagtcagacgatgtcttgtttatcaacgccgcagaacacttcgagaaaggaaaacgtcagaattaccttcgaagaactgacgaaatgcctaatggagagttgggcgatatagaaaaaattatcgacacctaccaattccgaaaggaagaagagcgatattctcgtcgtgtgtctatggaagagattgagaaaaacggcttcaatctgaatatctcacgttatgtcagtacagcacaggctgaaaaaagaatagatctaaaagatgtccacagtgagttggtatcattggaagaaagaattaagagagcaacgctcactcataacgcgttcctcgaagaactaggactaccaccacttcccttagccgaaaaagactaatctggagtgatgtaacttataggtgaaatatagagcccaaatcatcagtatccgggctctatatttatcaatttagccttcagtaaggcaatgttattagtcagcacaagaaaggcgctgccaagattatgtaaagaatgagcgtccgcttcacgctcacagcggactgtcagattttacttgtttcaacctataaagctgttaggttaaatttgtgttaatacaaaattgtcgcacccagaagttcccccacgtcagcccaaccgtttatccacagttcccctgattaatttttgcata

SEQ ID NO: 115 - DNA, 1086 bp, JBEAAAI-19-0008
  source 1..1086: mol_type = genomic DNA
atggcaaataagctggcgacatttcaggaactgggcgagattgcagctcatctacgtgaaaaacttgaagataaaaaatatgtactcctgttcgcatataatggcacaggaaagactcggttatcaatggagtttaaggagctaggtaagaatggtgatgacagggatacgctttacttcaacgcatttaccgaagacctgtttaattgggataacgatctggaacacgattctaaacgggtattgcgattaaatcgtgagtctcgcttttttgacggtttagaggagttggagatggaaaacagaatagctccaatactcgcccgttacgccgactttaatttctatattgattacaccgattgggaaatcatatttttccgtgagacagacagtgaaggcgacccaattcctattaaggtatctcgtggtgaggaaaatatatttatctggtgtttttttcttgtggttgcgcggttggcattagatagcgaggaaggcgctgtctattcgtgggttaaattcatatatatagatgatcctatatcttcgttagatgataacaacgctgtagctgtagcacatcacttggctcaattatttaaaacatcgagaaacgacataaaagtgactttatcttcgcatcacacgttattttttaatgtaatgtgtaatgaatggggaaatgcagttaagtatttcctgggtaaaaacgaaggtggtaatggatacaccttgaaaccgatgtatggagatacggctaggttctatcacgtggcaatgttgagggatctaaaaaaagctgctgactcaggagagctatatacttaccacttcaatattctacgtaaccttatggaaaaaactgctacttttcatggctatactgactttagtcactttataagcgtggaaaatgatgatgacgagaaaacattattaacaaggttggttcaggtgttgaatcatggtggttattcgttacttgaacccattgaaatgattcccgaaaacaagtcacatttccgaaaaatcctgaatgattttctgaaaacatatagttttaatcagggaattttttcctga

SEQ ID NO: 116 - DNA, 3048 bp, JBEAAAI-19-0008
  source 1..3048: mol_type = genomic DNA
atgactaaagaacaacaaattgagcaaggtttaatcgccaggctacaagacctcaaatacacctaccgcagcgacattcacgacaaggctagcttggagcagaacttccgtaagaagtttgaagctttgaaccgagtcaacctatccgatgcagaattcaaccgcctccgtgaagagatcatcacagcggatgtctttttggctgcccaggcgctgcgtgaaaaggggaaatttacccgtgaagatggcactccgttggaatacatgctggttaatcttaaagactggtgtaaaaacgactttgaagtaattagccagcttcgtatcaacacagataacagtcaccatcgctatgacgtgattctattgctcaatggcttaccactggtacagattgagctgaagtcactacagctcagtcctcgcagagcgatggagcaaatcgttgagtataaaaacgatactggcaacggctataccaatactctgctgtgcttcatgcagttgtttatcgtcagtaatggtaacgatacgcgttatttcgccaataaccgcaaagagcacttcagcttcaatgccgatgagcgcttcctgcccatttatcagcatgctgacaagagcaataagaagattgctcatttgcacgactttgctgatgacttcctagccaagtgcaccttgggtcagctgatcagccgctatatggtgttggtacaaagcgagcaaaaaatgctcatcatgcgcccgtatcaaatctatgccgttaaagctattgtggatgctattcaccagaaccgtggtaatggctatatctggcataccacaggctctggtaaaacactcacgtcattcaaagcctctacgctattgaaagataatcccgatattgaaaaatgtttatttgtggtcgatcgcaaagatctcgatcgccaaacgcgagaggaattcaacaaattccaggaaggatgtgtagagcaaaacaccaacaccgaaacgctcgtacgccgcatgttatcggaagactatgccgataaagtgattgtcactaccattcaaaagcttggtctggccttggatgagaatagcaaacgcaacaaggctcagcagaaaaatggcaaacagacctataaagagcgtttggagccgctgcgtgataagcgcgtggtatttatcttcgacgaatgtcaccgctctcaatttggtgagaaccataaagccattaaagaatttttccccaaagctcagttatttggttttaccggcacacctatttttgacgaaaattcaagctatcagcaagtagatggcaacctagcctctttcaaaaccacggaagatattttcgaaaaagagctacacgcctatactatcacccacgccattgaggacaaaaacgtactgagtttccacattgactattatgggaaagacgatggtaaaggtggtcaaaccaagcctaagaaaaaagaactgccaccacctgaagcggtaataaaagctattctcgacaaacacgatagcgccacaaatcagcgccgctttaatgccgtattggcaacagcatcgatcaatcacgccatcgagtactttgagctatttaaaacgcttcaagcacaaaagcagtctgaagacgaaaatttcgagccattgaatatcgcctgtgtattctcccccccggcccagatcgctaaagagaacgatggtaatggcagtgtaaacggcaacaagaatgcggcagacattaagcagcttcaggaagatctgccccaagaaagtgtcgacaaccaggtagaacccgaaaagaaaaagtcagccctgatggcgattgttgccaactacaacgagcaatacggcaccaatcacaccattaacgaattcgatctttactatcaggatgtgcagcagcgcatcaaagaccaaaagtacagcaatgttgattaccctcgtaaaaacaaaatcgacatcaccattgtggtggacatgctattaaccggttttgactcaaaatacctcaatactctgtatgtggataaaaacctgaagcatcacggccttatccaggcattctcgcgtaccaatcgtgtgctcaacgacacaaaaccgtggggcaacattctggacttccgttatcaggaaaacgaagtcaacgcagcaattgagttgttttctggtgggccgaaagataaagcccgagaaatctggctggtcgatccagcgcacaaagtggttgaggcattccagaaaagggtggacgaattgcaaacctttatggagtccaaaggcttaagctgtgagccatctgaggtgcataacctgaaaggcgatacggccaaggccgagtttatcaaccactttaaagaagtgcagaagctgaaaacccagctagatcaatacacggatctggacgaagaaagtaaagccgccatcgaacaaaaactgccaacagatactttgcggggcttcaaagccatttacctcgatacagctatggagttaaagcgtaaacaaggtaaaagtgatgacaacgaagaatcggtggagcagcttgagtttgatctagtgctttttgcctccagtattatcgactatgactacatcatggggctgattgccaaatccacgcaaaaaactggcaagcagaagatgacgcgccaggagctgatcgacctgatcagcgccaatgctaacttgatggaagagcgtgaagatattattgcctacatcaatagcctcaaggcgggtgaagcacttaatgaaaagcaaatccgcgaaggctatcaaacttataaagcgcagaaagccgcgcaggtattaacgcaaattgctgagaaacatggcttgcaaactcaatctcttcaggcgtttgtggacagcattttagatcgcatgatttttgatggcgaacaattaacagacttacttgctcccttagaactcggttggaaagcgcgtcgcgtggcagagctggccttgatggaagatttagtaccttacctacaaaaacaggccgatgggcgcgaaatttcgggattagatgcatatgagtga

SEQ ID NO: 117 - DNA, 1248 bp, JBEAAAI-19-0008
  source 1..1248: mol_type = genomic DNA
atgcatatgagtgatcaaaaaagagagtttattccagagttacgtttttctgaatttctagcttccaaagggtggaagattcgaagtgttagtgaaacatgtgataagccttttagcggggggacaccatcatctacgaaaaaagaatattatggtggagatattccctttattcgctcaggtgaaatagataaggaaaagacagagctcttccttactcaagatggcctttcgaactcttctgcaaagctggtaaaaaagggagatatattagtagctttatatggcgctaatagcggcgaagtggcattgagtaaaattgaaggcgcgattaatcaggcaattttatgtctgcgttcaaaaacgaataatgcctttcttttccagtacctcgtatacagaaaaaactatataaccaagaaatacttgcagggagggcaagggaacctttcgggagacatcattaagtcaattgagcttcttttcccagagagagatgagcaacaaaaaatcgctgactgtctggcttccatcgatgggctaattacacagcacacccagaagctcgaagccctcaaattccataaaaaaggattgatgcaacaactctttccagcccaaggtgaaaccgtacccaagctgcgatttcctgaatttcgcaaagcaggatgttggaagcttaagcccattgggaaggtcttggctgaaaaacaaaggccgatagatatggaggacgatgaggagtattccttggtgacagtcaagcgccgatatggaggattggtttcaagagggatatacaagggaaggacaatcaaagttaaatcgcaatttgaagttcatgaaaatgatttcctgatttctaagcgtcagattgttcattgtgcttgtggtgtcgttccaaaagaactgcatggttcgattgtttctaatgagtattctgttctagtgccgaagaaagacaatgatgttcacttttttgactactttgcgcagcaacctgaagtaagcctatcttttttgcagtgtagcattgggattgttattgaaaagatgatattcaaactaaaggattggctgaaagaagagtttctatttccagagattgaggagcaacagaaaattgcgcaatttctcggcgattttgacgagattatagataaacagtatcaaaaaattgaatcgctaaaagagcataaaaaaggcctaatgcaaaaactctttcctgttatggatgaggtggtttga

SEQ ID NO: 118 - DNA, 1656 bp, JBEAAAI-19-0008
  source 1..1656: mol_type = genomic DNA
atgaccaaagaacaactcaatcagcttggtaaaacactctgggatatcgcggatcaattacgcggcgccatgaatgccgatgacttccgcgattacatgctgtcttttctattcctgcgttatctgtctgataactatgagcaggccgccaaaaaggaattgggccgtgattaccccgaaccgggcaatgatgatcgtcgcgcaccattagcaatctggtatcagaacaaccaagctgatattgccgattttgaaaaacaaatgcgtcttaaaacccattatgttattgagcctgcgtttctgtggagcagtgtggccgaaatggcgcgtacccagcatgcggatttgctggatacactatggaaggggttcaaatatattgaagagaagtccttcaacagcacgtttcagggcttgttctcggaaatcaacctgcactctgaaaagctaggcaaaaagcctgccgatcgtaatgccaagctttgtgccattatccaaaagattgccgaaggtatttctggttttagcaatgccagggacgatctgggtgatgcctatgaatacttgattggccagtttgcagcaggttctggaaaaaaagctggtgagttttatacacctcaacaagtttctaccatcttgtcagaaattgtcacattagatagccaagacccgacgacaggcccaaagaaaaaaattaaacaagtgatggatttcgcctgtggttcaggctcgttgctattgaatgtacgaaacaggttaggtgatgaaggcggttctataggtaaaatatttggccaagagaaaaatatcactacctataaccttgcgcgcatgaacatgcttttgcatggggtaaaagatactgagtttgaaattcatcacggcgatacgttagagaatgactgggatattcttaatgagatgaatcctgcgaagaaaatgcagttcgacgccatcgtcgctaacccacctttcagtttgcgttgggagccgaccgaggcattaggtgaagatttccgcttcaagaactatggtcttgcgcctaaatcagcggcagatttcgcctttcttctgcacggctttcacttcctcagcgatgacggggttatggcgattattctgccgcacggtgttttatttcgtggcggtgcagaagagcggatacgtaccaagttgttaaaagatgggcatatcgataccgtcattggccttcctgccaatctgttcttctcaacgggcatacctgtttgcattctggtgctcaaacgctgtaagaagtcagacgatgtcttgtttatcaacgccgcagaacacttcgagaaaggaaaacgtcagaattaccttcgaagaactgacgaaatgcctaatggagagttgggcgatatagaaaaaattatcgacacctaccaattccgaaaggaagaagagcgatattctcgtcgtgtgtctatggaagagattgagaaaaacggcttcaatctgaatatctcacgttatgtcagtacagcacaggctgaaaaaagaatagatctaaaagatgtccacagtgagttggtatcattggaagaaagaattaagagagcaacgctcactcataacgcgttcctcgaagaactaggactaccaccacttcccttagccgaaaaagactaa